European Patent Specification EP 3 609 535 B1, published June 25, 2025. Title: HBV Vaccine. Applicant: Oxford University Innovation Limited. The sequence listing filed with the application follows.

SEQUENCE LISTING (61 sequences)

SEQ ID NO: 1 - DNA, 3215 bp, Hepatitis B virus
ctccacaacattccaccaagctctgctagatcccagagtgaggggcctatactttcctgctggtggctccagttccggaacagtaaaccctgttccgactactgcctcacccatatcgtcaatcttctcgaggactggggaccctgcaccgaacatggagaacacaacatcaggattcctaggacccctgctcgtgttacaggcggggtttttcttgttgacaagaatcctcacaataccacagagtctagactcgtggtggacttctctcaattttctagggggagcacccacgtgtcctggccaaaattcgcagtccccaacctccaatcactcaccaacctcttgtcctccaatttgtcctggctatcgctggatgtgtctgcggcgttttatcatattcctcttcatcctgctgctatgcctcatcttcttgttggttcttctggactaccaaggtatgttgcccgtttgtcctctacttccaggaacatcaactaccagcacgggaccatgcaagacctgcacgattcctgctcaaggaacctctatgtttccctcttgttgctgtacaaaaccttcggacggaaactgcacttgtattcccatcccatcatcctgggctttcgcaagattcctatgggagtgggcctcagtccgtttctcctggctcagtttactagtgccatttgttcagtggttcgtagggctttcccccactgtttggctttcagttatatggatgatgtggtattgggggccaagtctgtacaacatcttgagtccctttttacctctattaccaattttcttttgtctttgggtatacatttgaaccctaataaaaccaaacgttggggctactcccttaacttcatgggatatgtaattggaagttggggtactttaccacaggaacatattgtactaaaaatcaagcaatgttttcgaaaactgcctgtaaatagacctattgattggaaagtatgtcaaagaattgtgggtcttttgggctttgctgccccttttacacaatgtggctatcctgccttaatgcctttatatgcatgtatacaatctaagcaggctttcactttctcgccaacttacaaggcctttctgtgtaaacaatatctgaacctttaccccgttgcccggcaacggtcaggtctctgccaagtgtttgctgacgcaacccccactggatggggcttggccataggccatcggcgcatgcgtggaacctttgtggctcctctgccgatccatactgcggaactcctagcagcttgttttgctcgcagccggtctggagcgaaacttatcggaaccgacaactctgttgtcctctctcggaaatacacctcctttccatggctgctagggtgtgctgccaactggatcctgcgcgggacgtcctttgtctacgtcccgtcggcgctgaatcccgcggacgacccgtctcggggccgtttgggactctaccgtccccttcttcatctgccgttccggccgaccacggggcgcacctctctttacgcggtctccccgtctgtgccttctcatctgccggaccgtgtgcacttcgcttcacctctgcacgtcgcatggagaccaccgtgaacgcccaccaggtcttgcccaaggtcttacataagaggactcttggactctcagcaatgtcaacgaccgaccttgaggcatacttcaaagactgtttgtttaaagactgggaggagttgggggaggagattaggttaatgatctttgtactaggaggctgtaggcataaattggtctgttcaccagcaccatgcaactttttcacctctgcctaatcatctcatgttcatgtcctactgttcaagcctccaagctgtgccttgggtggctttggggcatggacattgacccgtataaagaatttggagcttctgtggagttactctcttttttgccttctgacttctttccttctattcgagatctcctcgacaccgcctctgctctgtatcgggaggccttagagtctccggaacattgttcacctcaccatacagcactcaggcaagctattctgtgttggggtgagttgatgaatctggccacctgggtgggaagtaatttggaagacccagcatccagggaattagtagtcagctatgtcaatgttaatatgggcctaaaaatcagacaactattgtggtttcacatttcctgtcttacttttggaagagaaactgttcttgagtatttggtgtcttttggagtgtggattcgcactcctcccgcttacagaccaccaaatgcccctatcttatcaacacttccggaaactactgttgttagacgacgaggcaggtcccctagaagaagaactccctcgcctcgcagacgaaggtctcaatcgccgcgtcgcagaagatctcaatctcgggaatctcaatgttagtatcccttggactcataaggtgggaaactttactgggctttattcttctactgtacctgtctttaatcctgagtggcaaactccctcctttcctcacattcatttacaggaggacattattaatagatgtcaacaatatgtgggccctcttacagttaatgaaaaaaggagattaaaattaattatgcctgctaggttctatcctaaccttaccaaatatttgcccttggacaaaggcattaaaccttattatcctgaacatgcagttaatcattacttcaaaactaggcattatttacatactctgtggaaggctggcattctatataagagagaaactacacgcagcgcctcattttgtgggtcaccatattcttgggaacaagagctacagcatgggaggttggtcttccaaacctcgacaaggcatggggacgaatctttctgttcccaatcctctgggattctttcccgatcaccagttggaccctgcgttcggagccaactcaaacaatccagattgggacttcaaccccaacaaggatcactggccagaggcaaatcaggtaggagcgggagcattcgggccagggttcaccccaccacacggcggtcttttggggtggagccctcaggctcagggcatattgacaacagtgccagcagcacctcctcctgcctccaccaatcggcagtcaggaagacagcctactcccatctctccacctctaagagacagtcatcctcaggccatgcagtggaa

SEQ ID NO: 2 - DNA, 3215 bp, Artificial Sequence
  HBV consensus sequence
ctccacaacattccaccaagctctgctagatcccagagtgaggggcctatattttcctgctggtggctccagttccggaacagtaaaccctgttccgactactgcctcacccatatcgtcaatcttctcgaggactggggaccctgcaccgaacatggagaacacaacatcaggattcctaggacccctgctcgtgttacaggcggggtttttcttgttgacaagaatcctcacaataccacagagtctagactcgtggtggacttctctcaattttctagggggagcacccacgtgtcctggccaaaattcgcagtccccaacctccaatcactcaccaacctcttgtcctccaatttgtcctggctatcgctggatgtgtctgcggcgttttatcatattcctcttcatcctgctgctatgcctcatcttcttgttggttcttctggactaccaaggtatgttgcccgtttgtcctctacttccaggaacatcaactaccagcacgggaccatgcaagacctgcacgattcctgctcaaggaacctctatgtttccctcttgttgctgtacaaaaccttcggacggaaactgcacttgtattcccatcccatcatcctgggctttcgcaagattcctatgggagtgggcctcagtccgtttctcctggctcagtttactagtgccatttgttcagtggttcgtagggctttcccccactgtttggctttcagttatatggatgatgtggtattgggggccaagtctgtacaacatcttgagtccctttttacctctattaccaattttcttttgtctttgggtatacatttgaaccctaataaaaccaaacgttggggctactcccttaacttcatgggatatgtaattggaagttggggtactttaccacaggaacatattgtactaaaaatcaagcaatgttttcgaaaactgcctgtaaatagacctattgattggaaagtatgtcaaagaattgtgggtcttttgggctttgctgccccttttacacaatgtggctatcctgccttgatgcctttatatgcatgtatacaatctaagcaggctttcactttctcgccaacttacaaggcctttctgtgtaaacaatatctgaacctttaccccgttgcccggcaacggtcaggtctctgccaagtgtttgctgacgcaacccccactggatggggcttggccataggccatcggcgcatgcgtggaacctttgtggctcctctgccgatccatactgcggaactcctagcagcttgttttgctcgcagccggtctggagcgaaacttatcggaaccgacaactctgttgtcctctctcggaaatacacctcctttccatggctgctagggtgtgctgccaactggatcctgcgcgggacgtcctttgtctacgtcccgtcggcgctgaatcccgcggacgacccgtctcggggccgtttgggactctaccgtccccttcttcatctgccgttccggccgaccacggggcgcacctctctttacgcggtctccccgtctgtgccttctcatctgccggaccgtgtgcacttcgcttcacctctgcacgtcgcatggagaccaccgtgaacgcccaccaggtcttgcccaaggtcttacataagaggactcttggactctcagcaatgtcaacgaccgaccttgaggcatacttcaaagactgtttgtttaaagactgggaggagttgggggaggagattaggttaatgatctttgtactaggaggctgtaggcataaattggtctgttcaccagcaccatgcaactttttcacctctgcctaatcatctcatgttcatgtcctactgttcaagcctccaagctgtgccttgggtggctttggggcatggacattgacccgtataaagaatttggagcttctgtggagttactctcttttttgccttctgacttctttccttctattcgagatctcctcgacaccgcctctgctctgtatcgggaggccttagagtctccggaacattgttcacctcaccatacagcactcaggcaagctattctgtgttggggtgagttgatgaatctggccacctgggtgggaagtaatttggaagacccagcatccagggaattagtagtcagctatgtcaatgttaatatgggcctaaaaatcagacaactattgtggtttcacatttcctgtcttacttttggaagagaaactgttcttgagtatttggtgtcttttggagtgtggattcgcactcctcccgcttacagaccaccaaatgcccctatcttatcaacacttccggaaactactgttgttagacgacgaggcaggtcccctagaagaagaactccctcgcctcgcagacgaaggtctcaatcgccgcgtcgcagaagatctcaatctcgggaatctcaatgttagtatcccttggactcataaggtgggaaactttactgggctttattcttctactgtacctgtctttaatcctgagtggcaaactccctcctttcctcacattcatttacaggaggacattattaatagatgtcaacaatatgtgggccctcttacagttaatgaaaaaaggagattaaaattaattatgcctgctaggttctatcctaaccttaccaaatatttgcccttggacaaaggcattaaaccgtattatcctgaacatgcagttaatcattacttcaaaactaggcattatttacatactctgtggaaggctggcattctatataagagagaaactacacgcagcgcctcattttgtgggtcaccatattcttgggaacaagagctacagcatgggaggttggtcttccaaacctcgacaaggcatggggacgaatctttctgttcccaatcctctgggattctttcccgatcaccagttggaccctgcgttcggagccaactcaaacaatccagattgggacttcaaccccaacaaggatcactggccagaggcaaatcaggtaggagcgggagcattcgggccagggttcaccccaccacacggcggtcttttggggtggagccctcaggctcagggcatattgacaacagtgccagcagcacctcctcctgcctccaccaatcggcagtcaggaagacagcctactcccatctctccacctctaagagacagtcatcctcaggccatgcagtggaa

SEQ ID NO: 3 - protein, 1525 aa, Artificial Sequence
  Vaccine construct
MSLLWGGVTVLAAMLIAGQVASVVFLVKGGGPGGGMQLFHLCLIISCSCPTVQASKLCLGWLWGMDIDPYKEFGASVELLSFLPSDFFPSIRDLLDTASALYREALESPEHCSPHHTALRQAILCWGELMNLATWVGSNLEDPASRELVVSYVNVNMGLKIRQLLWFHISCLTFGRETVLEYLVSFGVWIRTPPAYRPPNAPILSTLPETTVVRRRGRSPRRRTPSPRRRRSQSPRRRRSQSRESQCGGGSGGGMPLSYQHFRKLLLLDDEAGPLEEELPRLADEGLNRRVAEDLNLGNLNVSIPWTHKVGNFTGLASSTVPVFNPEWQTPSFPHIHLQEDIINRCQQYVGPLTVNEKRRLKLIMPARFYPNLTKYLPLDKGIKPYYPEHAVNHYFKTRHYLHTLWKAGILYKRETTRSASFCGSPYSWEQELQHGRLVFQTSTRHGDESFCSQSSGILSRSPVGPCVRSQLKQSRLGLQPQQGSLARGKSGRSGSIRARVHPTTRRSFGVEPSGSGHIDNSASSTSSCLHQSAVRKTAYSHLSTSKRQSSSGHAVELHNIPPSSARSQSEGPIFSAWWLQFRNSKPASDYALTHIVNLLEDWGPATEHGEHNIRIPRTPARVTGGVFLVDKNPHNTTESRLVVDFSQFSRGSTHVSWPKFAVPNLQSLTNLLSSNLSWLSLDVSAAFYHIPLHPAAMPHLLVGSSGLPRYVARLSSTSRNINYQHGTMQDLHDSCSRNLYVSLLLLYKTFGRKLHLYSHPIILGFRKIPMGVGLSPFLLAQFTSAICSVVRRAFPHCLAFSYMDDVVLGAKSVQHLESLFTSITNFLLSLGIHLNPNKTKRWGYSLNFMGYVIGSWGTLPQEHIVLKIKQCFRKLPVNRPIDWKVCQRIVGLLGFAAPFTQCGYPALMPLYACIQSKQAFTFSPTYKAFLCKQYLNLYPVARQRSGLCQVFADATPTGWGLAIGHRAMRGTFVAPLPIHTAELLAACFARSRSGAKLIGTDNSVVLSRKYTSFPWLLGCAANWILRGTSFVYVPSALNPAADPSAGRLGLYRPLLHLPFRPTTGRTSLYAVSPSVPSHLPDRVHFASPLHVAWRPPRKRRAPVKQTLNFDLLKLAGDVESNPGPMGGWSSKPRQGMGTNLSVPNPLGFFPDHQLDPAFGANSNNPDWDFNPNKDHWPEANQVGAGAFGPGFTPPHGGLLGWSPQAQGILTTVPAAPPPASTNRQSGRQPTPISPPLRDSHPQAMQWNSTTFHQALLDPRVRGLYFPAGGSSSGTVNPVPTTASPISSIFSRTGDPAPNMENTTSGFLGPLLVLQAGFFLLTRILTIPQSLDSWWTSLNFLGGAPTCPGQNSQSPTSNHSPTSCPPICPGYRWMCLRRFIIFLFILLLCLIFLLVLLDYQGMLPVCPLLPGTSTTSTGPCKTCTIPAQGTSMFPSCCCTKPSDGNCTCIPIPSSWAFARFLWEWASVRFSWLSLLVPFVQWFVGLSPTVWLSVIWMMWYWGPSLYNILSPFLPLLPIFFCLWVYI

SEQ ID NO: 4 - protein, 26 aa, Unknown
  Shark Invariant Chain
SLLWGGVTVLAAMLIAGQVASVVFLV

SEQ ID NO: 5 - protein, 8 aa, Artificial Sequence
  Linker peptide
KGGGPGGG

SEQ ID NO: 6 - protein, 183 aa, Hepatitis B virus
MDIDPYKEFGASVELLSFLPSDFFPSIRDLLDTASALYREALESPEHCSPHHTALRQAILCWGELMNLATWVGSNLEDPASRELVVSYVNVNMGLKIRQLLWFHISCLTFGRETVLEYLVSFGVWIRTPPAYRPPNAPILSTLPETTVVRRRGRSPRRRTPSPRRRRSQSPRRRRSQSRESQC

SEQ ID NO: 7 - protein, 7 aa, Artificial Sequence
  Linker peptide
GGGSGGG

SEQ ID NO: 8 - protein, 772 aa, Hepatitis B virus
MPLSYQHFRKLLLLDDEAGPLEEELPRLADEGLNRRVAEDLNLGNLNVSIPWTHKVGNFTGLASSTVPVFNPEWQTPSFPHIHLQEDIINRCQQYVGPLTVNEKRRLKLIMPARFYPNLTKYLPLDKGIKPYYPEHAVNHYFKTRHYLHTLWKAGILYKRETTRSASFCGSPYSWEQELQHGRLVFQTSTRHGDESFCSQSSGILSRSPVGPCVRSQLKQSRLGLQPQQGSLARGKSGRSGSIRARVHPTTRRSFGVEPSGSGHIDNSASSTSSCLHQSAVRKTAYSHLSTSKRQSSSGHAVELHNIPPSSARSQSEGPIFSAWWLQFRNSKPASDYALTHIVNLLEDWGPATEHGEHNIRIPRTPARVTGGVFLVDKNPHNTTESRLVVDFSQFSRGSTHVSWPKFAVPNLQSLTNLLSSNLSTFGRKLHLYSHPIILGFRKIPMGVGLSPFLLAQFTSAICSVVRRAFPHCLAFSYMDDVVLGAKSVQHLESLFTSITNFLLSLGIHLNPNKTKRWGYSLNFMGYVIGSWGTLPQEHIVLKIKQCFRKLPVNRPIDWKVCQRIVGLLGFAAPFTQCGYPALMPLYACIQSKQAFTFSPTYKAFLCKQYLNLYPVARQRSGLCQVFADATPTGWGLAIGHRAMRGTFVAPLPIHTAELLAACFARSRSGAKLIGTDNSVVLSRKYTSFPWLLGCAANWILRGTSFVYVPSALNPAADPSAGRLGLYRPLLHLPFRPTTGRTSLYAVSPSVPSHLPDRVHFASPLHVAWRPP

SEQ ID NO: 9 - protein, 28 aa, Unknown
  Furin 2A
RKRRAPVKQTLNFDLLKLAGDVESNPGP

SEQ ID NO: 10 - protein, 226 aa, Hepatitis B virus
MENTTSGFLGPLLVLQAGFFLLTRILTIPQSLDSWWTSLNFLGGAPTCPGQNSQSPTSNHSPTSCPPICPGYRWMCLRRFIIFLFILLLCLIFLLVLLDYQGMLPVCPLLPGTSTTSTGPCKTCTIPAQGTSMFPSCCCTKPSDGNCTCIPIPSSWAFARFLWEWASVRFSWLSLLVPFVQWFVGLSPTVWLSVIWMMWYWGPSLYNILSPFLPLLPIFFCLWVYI

SEQ ID NO: 11 - protein, 1521 aa, Artificial Sequence
  Vaccine construct
MSLLWGGVTVLAAMLIAGQVASVVFLVKGGSMGGWSSKPRQGMGTNLSVPNPLGFFPDHQLDPAFGANSNNPDWDFNPNKDHWPEANQVGAGAFGPGFTPPHGGLLGWSPQAQGILTTVPAAPPPASTNRQSGRQPTPISPPLRDSHPQAMQWNSTTFHQALLDPRVRGLYFPAGGSSSGTVNPVPTTASPISSIFSRTGDPAPNMENTTSGFLGPLLVLQAGFFLLTRILTIPQSLDSWWTSLNFLGGAPTCPGQNSQSPTSNHSPTSCPPICPGYRWMCLRRFIIFLFILLLCLIFLLVLLDYQGMLPVCPLLPGTSTTSTGPCKTCTIPAQGTSMFPSCCCTKPSDGNCTCIPIPSSWAFARFLWEWASVRFSWLSLLVPFVQWFVGLSPTVWLSVIWMMWYWGPSLYNILSPFLPLLPIFFCLWVYIRKRRAPVKQTLNFDLLKLAGDVESNPGPMQLFHLCLIISCSCPTVQASKLCLGWLWGMDIDPYKEFGASVELLSFLPSDFFPSIRDLLDTASALYREALESPEHCSPHHTALRQAILCWGELMNLATWVGSNLEDPASRELVVSYVNVNMGLKIRQLLWFHISCLTFGRETVLEYLVSFGVWIRTPPAYRPPNAPILSTLPETTVVRRRGRSPRRRTPSPRRRRSQSPRRRRSQSRESQCGGGSGGGMPLSYQHFRKLLLLDDEAGPLEEELPRLADEGLNRRVAEDLNLGNLNVSIPWTHKVGNFTGLASSTVPVFNPEWQTPSFPHIHLQEDIINRCQQYVGPLTVNEKRRLKLIMPARFYPNLTKYLPLDKGIKPYYPEHAVNHYFKTRHYLHTLWKAGILYKRETTRSASFCGSPYSWEQELQHGRLVFQTSTRHGDESFCSQSSGILSRSPVGPCVRSQLKQSRLGLQPQQGSLARGKSGRSGSIRARVHPTTRRSFGVEPSGSGHIDNSASSTSSCLHQSAVRKTAYSHLSTSKRQSSSGHAVELHNIPPSSARSQSEGPIFSAWWLQFRNSKPASDYALTHIVNLLEDWGPATEHGEHNIRIPRTPARVTGGVFLVDKNPHNTTESRLVVDFSQFSRGSTHVSWPKFAVPNLQSLTNLLSSNLSWLSLDVSAAFYHIPLHPAAMPHLLVGSSGLPRYVARLSSTSRNINYQHGTMQDLHDSCSRNLYVSLLLLYKTFGRKLHLYSHPIILGFRKIPMGVGLSPFLLAQFTSAICSVVRRAFPHCLAFSYMDDVVLGAKSVQHLESLFTSITNFLLSLGIHLNPNKTKRWGYSLNFMGYVIGSWGTLPQEHIVLKIKQCFRKLPVNRPIDWKVCQRIVGLLGFAAPFTQCGYPALMPLYACIQSKQAFTFSPTYKAFLCKQYLNLYPVARQRSGLCQVFADATPTGWGLAIGHRAMRGTFVAPLPIHTAELLAACFARSRSGAKLIGTDNSVVLSRKYTSFPWLLGCAANWILRGTSFVYVPSALNPAADPSAGRLGLYRPLLHLPFRPTTGRTSLYAVSPSVPSHLPDRVHFASPLHVAWRPP

SEQ ID NO: 12 - protein, 1490 aa, Artificial Sequence
  Vaccine construct
MQLFHLCLIISCSCPTVQASKLCLGWLWGMDIDPYKEFGASVELLSFLPSDFFPSIRDLLDTASALYREALESPEHCSPHHTALRQAILCWGELMNLATWVGSNLEDPASRELVVSYVNVNMGLKIRQLLWFHISCLTFGRETVLEYLVSFGVWIRTPPAYRPPNAPILSTLPETTVVRRRGRSPRRRTPSPRRRRSQSPRRRRSQSRESQCGGGSGGGMPLSYQHFRKLLLLDDEAGPLEEELPRLADEGLNRRVAEDLNLGNLNVSIPWTHKVGNFTGLASSTVPVFNPEWQTPSFPHIHLQEDIINRCQQYVGPLTVNEKRRLKLIMPARFYPNLTKYLPLDKGIKPYYPEHAVNHYFKTRHYLHTLWKAGILYKRETTRSASFCGSPYSWEQELQHGRLVFQTSTRHGDESFCSQSSGILSRSPVGPCVRSQLKQSRLGLQPQQGSLARGKSGRSGSIRARVHPTTRRSFGVEPSGSGHIDNSASSTSSCLHQSAVRKTAYSHLSTSKRQSSSGHAVELHNIPPSSARSQSEGPIFSAWWLQFRNSKPASDYALTHIVNLLEDWGPATEHGEHNIRIPRTPARVTGGVFLVDKNPHNTTESRLVVDFSQFSRGSTHVSWPKFAVPNLQSLTNLLSSNLSWLSLDVSAAFYHIPLHPAAMPHLLVGSSGLPRYVARLSSTSRNINYQHGTMQDLHDSCSRNLYVSLLLLYKTFGRKLHLYSHPIILGFRKIPMGVGLSPFLLAQFTSAICSVVRRAFPHCLAFSYMDDVVLGAKSVQHLESLFTSITNFLLSLGIHLNPNKTKRWGYSLNFMGYVIGSWGTLPQEHIVLKIKQCFRKLPVNRPIDWKVCQRIVGLLGFAAPFTQCGYPALMPLYACIQSKQAFTFSPTYKAFLCKQYLNLYPVARQRSGLCQVFADATPTGWGLAIGHRAMRGTFVAPLPIHTAELLAACFARSRSGAKLIGTDNSVVLSRKYTSFPWLLGCAANWILRGTSFVYVPSALNPAADPSAGRLGLYRPLLHLPFRPTTGRTSLYAVSPSVPSHLPDRVHFASPLHVAWRPPRKRRAPVKQTLNFDLLKLAGDVESNPGPMGGWSSKPRQGMGTNLSVPNPLGFFPDHQLDPAFGANSNNPDWDFNPNKDHWPEANQVGAGAFGPGFTPPHGGLLGWSPQAQGILTTVPAAPPPASTNRQSGRQPTPISPPLRDSHPQAMQWNSTTFHQALLDPRVRGLYFPAGGSSSGTVNPVPTTASPISSIFSRTGDPAPNMENTTSGFLGPLLVLQAGFFLLTRILTIPQSLDSWWTSLNFLGGAPTCPGQNSQSPTSNHSPTSCPPICPGYRWMCLRRFIIFLFILLLCLIFLLVLLDYQGMLPVCPLLPGTSTTSTGPCKTCTIPAQGTSMFPSCCCTKPSDGNCTCIPIPSSWAFARFLWEWASVRFSWLSLLVPFVQWFVGLSPTVWLSVIWMMWYWGPSLYNILSPFLPLLPIFFCLWVYI

SEQ ID NO: 13 - protein, 1492 aa, Artificial Sequence
  Vaccine construct
MSLLWGGVTVLAAMLIAGQVASVVFLVKGGGPGGGMQLFHLCLIISCSCPTVQASKLCLGWLWGMDIDPYKEFGASVELLSFLPSDFFPSIRDLLDTASALYREALESPEHCSPHHTALRQAILCWGELMNLATWVGSNLEDPASRELVVSYVNVNMGLKIRQLLWFHISCLTFGRETVLEYLVSFGVWIRTPPAYRPPNAPILSTLPETTVVRRRGRSPRRRTPSPRRRRSQSPRRRRSQSRESQCGGGSGGGMPLSYQHFRKLLLLDDEAGPLEEELPRLADEGLNRRVAEDLNLGNLNVSIPWTHKVGNFTGLASSTVPVFNPEWQTPSFPHIHLQEDIINRCQQYVGPLTVNEKRRLKLIMPARFYPNLTKYLPLDKGIKPYYPEHAVNHYFKTRHYLHTLWKAGILYKRETTRSASFCGSPYSWEQELQHGRLVFQTSTRHGDESFCSQSSGILSRSPVGPCVRSQLKQSRLGLQPQQGSLARGKSGRSGSIRARVHPTTRRSFGVEPSGSGHIDNSASSTSSCLHQSAVRKTAYSHLSTSKRQSSSGHAVELHNIPPSSARSQSEGPIFSAWWLQFRNSKPASDYALTHIVNLLEDWGPATEHGEHNIRIPRTPARVTGGVFLVDKNPHNTTESRLVVDFSQFSRGSTHVSWPKFAVPNLQSLTNLLSSNLSTFGRKLHLYSHPIILGFRKIPMGVGLSPFLLAQFTSAICSVVRRAFPHCLAFSYMDDVVLGAKSVQHLESLFTSITNFLLSLGIHLNPNKTKRWGYSLNFMGYVIGSWGTLPQEHIVLKIKQCFRKLPVNRPIDWKVCQRIVGLLGFAAPFTQCGYPALMPLYACIQSKQAFTFSPTYKAFLCKQYLNLYPVARQRSGLCQVFADATPTGWGLAIGHRAMRGTFVAPLPIHTAELLAACFARSRSGAKLIGTDNSVVLSRKYTSFPWLLGCAANWILRGTSFVYVPSALNPAADPSAGRLGLYRPLLHLPFRPTTGRTSLYAVSPSVPSHLPDRVHFASPLHVAWRPPKSPNSNNPDWDFNPNKDHWPEANQVGAGAFGPGFTPPHGGLLGWSPQAQGILTTVPAAPPPASTNRQSGRQPTPISPPLRDSHPQAMQWNSTTFHQALLDPRVRGLYFPAGGSSSGTVNPVPTTASPISSIFSRTGDPAPNGSKGKRKRRAPVKQTLNFDLLKLAGDVESNPGPMGGWSSKPRQGMGTNLSVPNPLGFFPDHQLDPAFGANSNNPDWDFNPNKDHWPEANQVGLEGGSGGMENTTSGFLGPLLVLQAGFFLLTRILTIPQSLDSWWTSLNFLGGAPTCPGQNSQSPTSNHSPTSCPPICPGYRWMCLRRFIIFLFILLLCLIFLLVLLDYQGMLPVCPLLPGTSTTSTGPCKTCTIPAQGTSMFPSCCCTKPSDGNCTCIPIPSSWAFARFLWEWASVRFSWLSLLVPFVQWFVGLSPTVWLSVIWMMWYWGPSLYNILSPFLPLLPIFFCLWVYI

SEQ ID NO: 14 - protein, 4 aa, Artificial Sequence
  Linker peptide
KGGS

SEQ ID NO: 15 - protein, 138 aa, Hepatitis B virus
NSNNPDWDFNPNKDHWPEANQVGAGAFGPGFTPPHGGLLGWSPQAQGILTTVPAAPPPASTNRQSGRQPTPISPPLRDSHPQAMQWNSTTFHQALLDPRVRGLYFPAGGSSSGTVNPVPTTASPISSIFSRTGDPAPN

SEQ ID NO: 16 - protein, 29 aa, Hepatitis B virus
MQLFHLCLIISCSCPTVQASKLCLGWLWG

SEQ ID NO: 17 - protein, 159 aa, Hepatitis B virus
SKLCLGWLWGMDIDPYKEFGASVELLSFLPSDFFPSIRDLLDTASALYREALESPEHCSPHHTALRQAILCWGELMNLATWVGSNLEDPASRELVVSYVNVNMGLKIRQLLWFHISCLTFGRETVLEYLVSFGVWIRTPPAYRPPNAPILSTLPETTVV

SEQ ID NO: 18 - protein, 226 aa, Hepatitis B virus; identical to SEQ ID NO: 10

SEQ ID NO: 19 - protein, 843 aa, Hepatitis B virus
MPLSYQHFRKLLLLDDEAGPLEEELPRLADEGLNRRVAEDLNLGNLNVSIPWTHKVGNFTGLYSSTVPVFNPEWQTPSFPHIHLQEDIINRCQQYVGPLTVNEKRRLKLIMPARFYPNLTKYLPLDKGIKPYYPEHAVNHYFKTRHYLHTLWKAGILYKRETTRSASFCGSPYSWEQELQHGRLVFQTSTRHGDESFCSQSSGILSRSPVGPCVRSQLKQSRLGLQPQQGSLARGKSGRSGSIRARVHPTTRRSFGVEPSGSGHIDNSASSTSSCLHQSAVRKTAYSHLSTSKRQSSSGHAVELHNIPPSSARSQSEGPIFSCWWLQFRNSKPCSDYCLTHIVNLLEDWGPCTEHGEHNIRIPRTPARVTGGVFLVDKNPHNTTESRLVVDFSQFSRGSTHVSWPKFAVPNLQSLTNLLSSNLSWLSLDVSAAFYHIPLHPAAMPHLLVGSSGLPRYVARLSSTSRNINYQHGTMQDLHDSCSRNLYVSLLLLYKTFGRKLHLYSHPIILGFRKIPMGVGLSPFLLAQFTSAICSVVRRAFPHCLAFSYMDDVVLGAKSVQHLESLFTSITNFLLSLGIHLNPNKTKRWGYSLNFMGYVIGSWGTLPQEHIVLKIKQCFRKLPVNRPIDWKVCQRIVGLLGFAAPFTQCGYPALMPLYACIQSKQAFTFSPTYKAFLCKQYLNLYPVARQRSGLCQVFADATPTGWGLAIGHRRMRGTFVAPLPIHTAELLAACFARSRSGAKLIGTDNSVVLSRKYTSFPWLLGCAANWILRGTSFVYVPSALNPADDPSRGRLGLYRPLLHLPFRPTTGRTSLYAVSPSVPSHLPDRVHFASPLHVAWRPP

SEQ ID NO: 20 - protein, 5 aa, Artificial Sequence
  Linker peptide
GSKGK

SEQ ID NO: 21 - protein, 59 aa, Hepatitis B virus
MGGWSSKPRQGMGTNLSVPNPLGFFPDHQLDPAFGANSNNPDWDFNPNKDHWPEANQVG

SEQ ID NO: 22 - protein, 7 aa, Artificial Sequence
  Linker peptide
LEGGSGG

SEQ ID NO: 23 - protein, 1539 aa, Hepatitis B virus
MSLLWGGVTVLAAMLIAGQVASVVFLVSKSGPPSGKSNSNNPDWDFNPNKDHWPEANQVGAGAFGPGFTPPHGGLLGWSPQAQGILTTVPAAPPPASTNRQSGRQPTPISPPLRDSHPQAMQWNSTTFHQALLDPRVRGLYFPAGGSSSGTVNPVPTTASPISSIFSRTGDPAPNGSKSGSKMPLSYQHFRKLLLLDDEAGPLEEELPRLADEGLNRRVAEDLNLGNLNVSIPWTHKVGNFTGLASSTVPVFNPEWQTPSFPHIHLQEDIINRCQQYVGPLTVNEKRRLKLIMPARFYPNLTKYLPLDKGIKPYYPEHAVNHYFKTRHYLHTLWKAGILYKRETTRSASFCGSPYSWEQELQHGRLVFQTSTRHGDESFCSQSSGILSRSPVGPCVRSQLKQSRLGLQPQQGSLARGKSGRSGSIRARVHPTTRRSFGVEPSGSGHIDNSASSTSSCLHQSAVRKTAYSHLSTSKRQSSSGHAVELHNIPPSSARSQSEGPIFSAWWLQFRNSKPASDYALTHIVNLLEDWGPATEHGEHNIRIPRTPARVTGGVFLVDKNPHNTTESRLVVDFSQFSRGSTHVSWPKFAVPNLQSLTNLLSSNLSWLSLDVSAAFYHIPLHPAAMPHLLVGSSGLPRYVARLSSTSRNINYQHGTMQDLHDSCSRNLYVSLLLLYKTFGRKLHLYSHPIILGFRKIPMGVGLSPFLLAQFTSAICSVVRRAFPHCLAFSYMDDVVLGAKSVQHLESLFTSITNFLLSLGIHLNPNKTKRWGYSLNFMGYVIGSWGTLPQEHIVLKIKQCFRKLPVNRPIDWKVCQRIVGLLGFAAPFTQCGYPALMPLYACIQSKQAFTFSPTYKAFLCKQYLNLYPVARQRSGLCQVFADATPTGWGLAIGHRAMRGTFVAPLPIHTAELLAACFARSRSGAKLIGTDNSVVLSRKYTSFPWLLGCAANWILRGTSFVYVPSALNPAADPSAGRLGLYRPLLHLPFRPTTGRTSLYAVSPSVPSHLPDRVHFASPLHVAWRPPSKSPGSGPPMQLFHLCLIISCSCPTVQASKLCLGWLWGMDIDPYKEFGASVELLSFLPSDFFPSIRDLLDTASALYREALESPEHCSPHHTALRQAILCWGELMNLATWVGSNLEDPASRELVVSYVNVNMGLKIRQLLWFHISCLTFGRETVLEYLVSFGVWIRTPPAYRPPNAPILSTLPETTVVRRRGRSPRRRTPSPRRRRSQSPRRRRSQSRESQCMGGWSSKPRQGMGTNLSVPNPLGFFPDHQLDPAFGANSNNPDWDFNPNKDHWPEANQVGASKGGKSGMENTTSGFLGPLLVLQAGFFLLTRILTIPQSLDSWWTSLNFLGGAPTCPGQNSQSPTSNHSPTSCPPICPGYRWMCLRRFIIFLFILLLCLIFLLVLLDYQGMLPVCPLLPGTSTTSTGPCKTCTIPAQGTSMFPSCCCTKPSDGNCTCIPIPSSWAFARFLWEWASVRFSWLSLLVPFVQWFVGLSPTVWLSVIWMMWYWGPSLYNILSPFLPLLPIFFCLWVYI

SEQ ID NO: 24 - DNA, 7143 bp, Artificial Sequence
  Vaccine construct
gtaatctattcgatataccgttgctaacagtatactggcccaataactgtggatggaaaatctataataatacattaatatcatccgatggtgctagggttatttggatggatgcgtataaattttcttgcggtttatctttacaagactattgttatcattggggtagcaaaccagagagccgaccattcgatttaataaaaaaatcagatgctaaacgcaattctaaatcgttggtcaaagaatctatggcatccttgaaatccttgtacgaggcattcgagacacaatcaggagcgttagaagttttaatgagtccatgtaggatgttttcgttttctagaatagaagacatgttcttaactagtgtcattaatagagtatccgagaatactggaatggggatgtattatcctaccaacgatataccttctctatttatcgaatcatctatctgtctagattatattatagtaaataatcaggaatccaacaaatatcgtatcaaatctgttctcgatatcatttcttcaaaacaataccctgcaggacgtcccaactacgttaaaaatggtacaaaaggaaagttatatatcgcgttgtgtaaagttaccgtacctactaacgaccatattccagtagtttatcacgatgatgacaatactaccacctttattacagtattgacgtccgtcgatattgaaactgctatcagagcaggatattcgatagtcgaattaggggctttacaatgggataataatattccagaacttaaaaacggtttactggatagtatcaagatgatttatgacttgaacgcagttacaacaaataatttattggaacagctcatagaaaatattaactttaacaactctagtataatttcgttgttttatacatttgccattagttattgccgagcattcatttactcaattatggaaaccatagatccggtgtatatatctcagttcagttataaagaattatacgttagtagctcttataaagatattaatgaatccatgagtcagatggtaaaattataaaaagtgaaaaacaatattatttttatcgttggttgttacactatgtctctgctgtggggcggagtgacagtgctggccgctatgctgattgctggacaggtggccagcgtggtgttcctggtgtctaagtctggacctcctagcggcaagagcaacagcaacaaccccgactgggacttcaaccccaacaaggaccattggccagaggccaatcaagtcggagccggcgcttttggccctggctttacacctcctcatggcggactgcttggatggtcacctcaggctcagggcatcctgacaacagtgcctgctgctccacctcctgccagcaccaatagacagtctggcagacagcccacacctatcagccctccactgagagacagccatcctcaggccatgcagtggaacagcaccacctttcatcaggccctgctggaccctagagtgcggggcctttattttcctgccggcggatctagcagcggcaccgtgaatcctgtgcctacaaccgcctctcctatcagcagcatcttcagcagaaccggcgatcccgctcctaacggcagcaagtctggctccaagatgcccctgagctaccagcacttcagaaaactgctgctgctggacgacgaggccggacctctggaagaagaactgcctagactggccgacgagggcctgaatagaagagtggccgaggacctgaacctgggcaacctgaatgtgtctatcccctggacacacaaagtgggcaacttcacaggcctggccagctctaccgtgcctgtgttcaatcccgagtggcagacccctagcttccctcacatccatctgcaagaggacatcatcaaccggtgccagcagtacgtgggccctctgaccgtgaacgagaagcggagactgaagctgatcatgcccgccagattctaccccaacctgaccaagtacctgcctctggacaagggcatcaagccttactaccctgagcacgccgtgaaccactacttcaagacccggcactacctgcacaccctgtggaaggccggcatcctgtataagagagagacaaccagaagcgccagcttctgcggcagcccttactcttgggagcaagagctgcagcacggcagactggtgttccagacctctacaagacacggcgacgagtctttctgcagccagagcagcggaatcctgagcagatctcctgtgggaccttgtgtgcggagccagctgaaacagagtagactgggcctgcagcctcagcagggatctctggctagaggaaagagcggcagaagcggcagcatcagagccagagtgcaccctaccaccagaagaagctttggcgtcgagcctagcggctccggccacatcgataatagcgccagcagcaccagcagctgcctgcatcagtccgccgttagaaagaccgcctacagccacctgagcacctccaagagacagagcagctctggacacgccgtggaactgcacaacatccctccaagcagcgccagatctcagagcgagggccctatcttttctgcctggtggctgcagttcagaaacagcaagcccgccagcgactacgccctgacacacatcgtgaacctgctggaagattggggccctgccacagaacacggcgagcacaatatcagaatccccagaacacccgccagagtgacaggcggagtgtttctggtggacaagaaccctcacaacaccaccgagagcaggctggtggtggacttcagccagtttagcagaggcagcacccacgtgtcctggcctaaattcgccgtgcctaacctgcagagcctgaccaatctgctgagcagcaacctgagctggctgagcctggatgtgtccgccgccttctatcacatcccactgcatcctgccgccatgcctcatctgcttgtgggaagttctggcctgcctagatacgtggccaggctgtcctctaccagccggaacatcaattaccagcacgggaccatgcaggacctgcacgacagctgtagccggaacctgtacgttagcctgctcctgctgtacaagaccttcggcagaaagctgcacctgtactctcaccccatcatcctgggcttcagaaagatccccatgggcgtgggcctgtctccatttctgctggcccagtttaccagcgccatctgctctgttgtgcggagagcctttcctcactgcctggccttcagctacatggacgatgtggtgctgggcgccaagtctgtgcagcacctggaaagcctgtttacctccatcaccaactttctgctgtccctgggaatccatctgaaccctaacaagaccaagagatggggctacagcctgaacttcatgggctacgtgatcggcagctggggcacactgcctcaagagcacatcgtgctgaaaatcaagcagtgctttcggaagctgcccgtgaacagacccatcgactggaaagtgtgccagcggatcgttggcctgctgggatttgccgctcctttcacacagtgcggctaccccgctctcatgcctctgtatgcctgtatccagagcaagcaggccttcacattcagccctacctacaaggccttcctgtgcaagcagtacctgaatctgtaccccgtggccagacagagaagcggcctgtgtcaagtgttcgccgatgccacacctacaggatggggactcgccattggacacagggccatgagaggaacctttgtggcccctctgcctatccacacagccgaattgctggctgcctgcttcgccagaagtagatccggcgccaagctgatcggcaccgacaattctgtggtcctgagccggaagtacaccagctttccatggctgctgggctgtgccgccaactggattctgagaggcaccagcttcgtgtacgtgcccagcgctcttaaccctgccgctgatccttctgctgggagactcggcctgtacagacctctgctgcatctgcccttcagacccaccacaggcagaaccagcctgtatgccgtgtctcctagcgtgccaagccatctgcctgatcgggtgcactttgcctctccacttcatgtggcttggcggccacctagcaagagccctggatctggaccacctatgcagctgtttcacctgtgcctgatcatctcttgcagctgccctacagtgcaggccagcaagctgtgtctcggatggctctggggcatggacatcgacccctacaaagaattcggcgccagcgtcgagctgctgagcttcctgcctagcgacttcttcccctccatccgggatctgctggatactgctagcgccctgtatcgcgaggccctggaatctcctgagcactgttctccacaccacactgccctgagacaggctatcctgtgttggggcgagctgatgaacctggccacatgggtcggaagcaacctggaagatcccgccagcagagaactggtggtgtcctacgtgaacgtgaacatgggcctgaagatcagacagctgctgtggttccacatctcctgcctgacctttggccgggaaaccgtgctggaatacctggtgtcctttggcgtgtggatcagaacccctccagcctaccgacctcctaacgctcctatcctgtctaccctgcctgagacaacagtcgtgcggcggagaggaagaagccctagaagaaggaccccatctcctcggcggagaagatcacagtcccctcggagaagaagatcccagagccgggaatcccagtgctgatttttgttcgacattaaaaattgaaaataaatacaaaggttcttgagggttgtgttaaattgaaagcgagaaataatcataaatatgattcaggtgacggatccatgggaggctggtccagcaaacccagacaaggcatgggcaccaatctgagcgtgcccaatcctctgggattcttcccagaccaccagctggatcctgccttcggcgccaacagcaacaaccccgactgggacttcaaccccaacaaggaccattggccagaggccaatcaagtgggcgctagcaaaggcggcaagagcggcatggagaataccacctctggctttctgggccctctgctggttctgcaggccggcttctttctgctgacccggatcctgacaatccctcagagcctggatagctggtggacaagcctgaacttccttggcggcgctcctacatgccctggccagaattctcagagccccaccagcaatcacagccccacaagctgccctccaatctgccctggctacagatggatgtgcctgcggcggttcatcatctttctgttcatcctgctgctgtgcctgatcttcctgctggtgctgctggactatcagggcatgctgcctgtgtgtcctctgctgcctggcaccagcacaacatctacaggcccttgcaagacctgcacaatcccagctcagggcacctccatgtttcccagctgctgttgcaccaagcctagcgacggcaactgcacatgcatccccattccttccagctgggccttcgccagatttctgtgggaatgggccagcgtgcggttcagctggctgtctctgcttgtgcctttcgtgcagtggttcgtgggcctgtctcctacagtgtggctgagcgtgatctggatgatgtggtactggggccctagcctgtacaatattctgagccccttcctgcctctgctcccaatcttcttctgcctgtgggtgtacatctgattaaccgagtttctgcattattgtaattcgtatgctggcaccatcaaagaatcacttctaaaagatatcaatatcacacatacaaatattactaccctattgaatgagacagccaaggttatcaagttagtaaaatctctggtagataaagaagatactgatattgtgaataatttcattaccaaagaaattaaaaacagagacaaaatagttaatagtttgtctctatcaaacctggactttcgtttgtaaattggggctttttgtacaataaatgggtgttgccaatgattcatcccctgaatatcaatggatgtctccccatagattatcagatactgttatattaggagactgtttgtattttaacaatataatgtcccaattagatttacaccaaaattgggctccatcagttagattgttaaattattttaagaattttaataaggaaacactactaaagatagaagagaatgattacattaattcatcctttttccaacaaaaggataaacgattttatcctataaacgacgatttttatcacatatctacaggaggatatggtatagtctttaagatagataactatgtagtaaaatttgtattcgaggccacaaaattatatagtcccatggaaactacggcggagttcacagtacccaaatttctatacaacaatctaaagggagatgaaaaaaaattaatcgtgtgtgcgtgggccatgggattaaactataaattaacatttttacatactctgtataaacgtgttcttcatatgttgctattattgatacaaactatggatggtcaggaactatcattgagatattcttctaaagtttttttaaaggcgtttaacgagagaaaggacagtatcaaattcgtgaaattactatcccacttttatccggcagttattaacagtaatattaatgttataaactattttaaccgcatgtttcactttttcgaacatgaaaagagaactaactacgaatacgaaagaggaaatattataatttttcccctagcactgtattcggcagataaagtagataccgagctagctatcaaattaggatttaaatctttggtacaatacataaagtttatctttttacagatggctctgttatacattaaaatttacgaactaccatgctgcgacaactttttacacgcagatcttaaacccgataatatcttactttttgattccaatgaaccaataataattcatctaaaggataaaaagtttgtttttaatgaacgtattaaatcggcattaaacgactttgacttttcccaag

SEQ ID NO: 25 - protein, 1524 aa, Artificial Sequence
  Vaccine construct
MSLLWGGVTVLAAMLIAGQVASVVFLVKGGGPGGGMQLFHLCLIISCSCPTVQASKLCLGWLWGMDIDPYKEFGASVELLSFLPSDFFPSIRDLLDTASALYREALESPEHCSPHHTALRQAILCWGELMNLATWVGSNLEDPASRELVVSYVNVNMGLKIRQLLWFHISCLTFGRETVLEYLVSFGVWIRTPPAYRPPNAPILSTLPETTVVRRRGRSPRRRTPSPRRRRSQSPRRRRSQSRESQCGGGSGGGMPLSYQHFRKLLLLDDEAGPLEEELPRLADEGLNRRVAEDLNLGNLNVSIPWTHKVGNFTGLASSTVPVFNPEWQTPSFPHIHLQEDIINRCQQYVGPLTVNEKRRLKLIMPARFYPNLTKYLPLDKGIKPYYPEHAVNHYFKTRHYLHTLWKAGILYKRETTRSASFCGSPYSWEQELQHGRLVFQTSTRHGDESFCSQSSGILSRSPVGPCVRSQLKQSRLGLQPQQGSLARGKSGRSGSIRARVHPTTRRSFGVEPSGSGHIDNSASSTSSCLHQSAVRKTAYSHLSTSKRQSSSGHAVELHNIPPSSARSQSEGPIFSAWWLQFRNSKPASDYALTHIVNLLEDWGPATEHGEHNIRIPRTPARVTGGVFLVDKNPHNTTESRLVVDFSQFSRGSTHVSWPKFAVPNLQSLTNLLSSNLSTFGRKLHLYSHPIILGFRKIPMGVGLSPFLLAQFTSAICSVVRRAFPHCLAFSYMDDVVLGAKSVQHLESLFTSITNFLLSLGIHLNPNKTKRWGYSLNFMGYVIGSWGTLPQEHIVLKIKQCFRKLPVNRPIDWKVCQRIVGLLGFAAPFTQCGYPALMPLYACIQSKQAFTFSPTYKAFLCKQYLNLYPVARQRSGLCQVFADATPTGWGLAIGHRAMRGTFVAPLPIHTAELLAACFARSRSGAKLIGTDNSVVLSRKYTSFPWLLGCAANWILRGTSFVYVPSALNPAADPSAGRLGLYRPLLHLPFRPTTGRTSLYAVSPSVPSHLPDRVHFASPLHVAWRPPKSPNSNNPDWDFNPNKDHWPEANQVGAGAFGPGFTPPHGGLLGWSPQAQGILTTVPAAPPPASTNRQSGRQPTPISPPLRDSHPQAMQWNSTTFHQALLDPRVRGLYFPAGGSSSGTVNPVPTTASPISSIFSRTGDPAPNGSKGKRKRRAPVKQTLNFDLLKLAGDVESNPGPMDAMKRGLCCVLLLCGAVFVSPSQEIHARFRRMGGWSSKPRQGMGTNLSVPNPLGFFPDHQLDPAFGANSNNPDWDFNPNKDHWPEANQVGLEGGSGGMENTTSGFLGPLLVLQAGFFLLTRILTIPQSLDSWWTSLNFLGGAPTCPGQNSQSPTSNHSPTSCPPICPGYRWMCLRRFIIFLFILLLCLIFLLVLLDYQGMLPVCPLLPGTSTTSTGPCKTCTIPAQGTSMFPSCCCTKPSDGNCTCIPIPSSWAFARFLWEWASVRFSWLSLLVPFVQWFVGLSPTVWLSVIWMMWYWGPSLYNILSPFLPLLPIFFCLWVYI

SEQ ID NO: 26 - protein, 1571 aa, Artificial Sequence
  Vaccine construct
MSLLWGGVTVLAAMLIAGQVASVVFLVSKSGPPSGKSNSNNPDWDFNPNKDHWPEANQVGAGAFGPGFTPPHGGLLGWSPQAQGILTTVPAAPPPASTNRQSGRQPTPISPPLRDSHPQAMQWNSTTFHQALLDPRVRGLYFPAGGSSSGTVNPVPTTASPISSIFSRTGDPAPNGSKSGSKMPLSYQHFRKLLLLDDEAGPLEEELPRLADEGLNRRVAEDLNLGNLNVSIPWTHKVGNFTGLASSTVPVFNPEWQTPSFPHIHLQEDIINRCQQYVGPLTVNEKRRLKLIMPARFYPNLTKYLPLDKGIKPYYPEHAVNHYFKTRHYLHTLWKAGILYKRETTRSASFCGSPYSWEQELQHGRLVFQTSTRHGDESFCSQSSGILSRSPVGPCVRSQLKQSRLGLQPQQGSLARGKSGRSGSIRARVHPTTRRSFGVEPSGSGHIDNSASSTSSCLHQSAVRKTAYSHLSTSKRQSSSGHAVELHNIPPSSARSQSEGPIFSAWWLQFRNSKPASDYALTHIVNLLEDWGPATEHGEHNIRIPRTPARVTGGVFLVDKNPHNTTESRLVVDFSQFSRGSTHVSWPKFAVPNLQSLTNLLSSNLSWLSLDVSAAFYHIPLHPAAMPHLLVGSSGLPRYVARLSSTSRNINYQHGTMQDLHDSCSRNLYVSLLLLYKTFGRKLHLYSHPIILGFRKIPMGVGLSPFLLAQFTSAICSVVRRAFPHCLAFSYMDDVVLGAKSVQHLESLFTSITNFLLSLGIHLNPNKTKRWGYSLNFMGYVIGSWGTLPQEHIVLKIKQCFRKLPVNRPIDWKVCQRIVGLLGFAAPFTQCGYPALMPLYACIQSKQAFTFSPTYKAFLCKQYLNLYPVARQRSGLCQVFADATPTGWGLAIGHRAMRGTFVAPLPIHTAELLAACFARSRSGAKLIGTDNSVVLSRKYTSFPWLLGCAANWILRGTSFVYVPSALNPAADPSAGRLGLYRPLLHLPFRPTTGRTSLYAVSPSVPSHLPDRVHFASPLHVAWRPPSKSPGSGPPMQLFHLCLIISCSCPTVQASKLCLGWLWGMDIDPYKEFGASVELLSFLPSDFFPSIRDLLDTASALYREALESPEHCSPHHTALRQAILCWGELMNLATWVGSNLEDPASRELVVSYVNVNMGLKIRQLLWFHISCLTFGRETVLEYLVSFGVWIRTPPAYRPPNAPILSTLPETTVVRRRGRSPRRRTPSPRRRRSQSPRRRRSQSRESQCMDAMKRGLCCVLLLCGAVFVSPSQEIHARFRRMGGWSSKPRQGMGTNLSVPNPLGFFPDHQLDPAFGANSNNPDWDFNPNKDHWPEANQVGASKGGKSGMENTTSGFLGPLLVLQAGFFLLTRILTIPQSLDSWWTSLNFLGGAPTCPGQNSQSPTSNHSPTSCPPICPGYRWMCLRRFIIFLFILLLCLIFLLVLLDYQGMLPVCPLLPGTSTTSTGPCKTCTIPAQGTSMFPSCCCTKPSDGNCTCIPIPSSWAFARFLWEWASVRFSWLSLLVPFVQWFVGLSPTVWLSVIWMMWYWGPSLYNILSPFLPLLPIFFCLWVYI

SEQ ID NO: 27 - DNA, 7239 bp, Artificial Sequence
  Vaccine construct
gtaatctattcgatataccgttgctaacagtatactggcccaataactgtggatggaaaatctataataatacattaatatcatccgatggtgctagggttatttggatggatgcgtataaattttcttgcggtttatctttacaagactattgttatcattggggtagcaaaccagagagccgaccattcgatttaataaaaaaatcagatgctaaacgcaattctaaatcgttggtcaaagaatctatggcatccttgaaatccttgtacgaggcattcgagacacaatcaggagcgttagaagttttaatgagtccatgtaggatgttttcgttttctagaatagaagacatgttcttaactagtgtcattaatagagtatccgagaatactggaatggggatgtattatcctaccaacgatataccttctctatttatcgaatcatctatctgtctagattatattatagtaaataatcaggaatccaacaaatatcgtatcaaatctgttctcgatatcatttcttcaaaacaataccctgcaggacgtcccaactacgttaaaaatggtacaaaaggaaagttatatatcgcgttgtgtaaagttaccgtacctactaacgaccatattccagtagtttatcacgatgatgacaatactaccacctttattacagtattgacgtccgtcgatattgaaactgctatcagagcaggatattcgatagtcgaattaggggctttacaatgggataataatattccagaacttaaaaacggtttactggatagtatcaagatgatttatgacttgaacgcagttacaacaaataatttattggaacagctcatagaaaatattaactttaacaactctagtataatttcgttgttttatacatttgccattagttattgccgagcattcatttactcaattatggaaaccatagatccggtgtatatatctcagttcagttataaagaattatacgttagtagctcttataaagatattaatgaatccatgagtcagatggtaaaattataaaaagtgaaaaacaatattatttttatcgttggttgttacactatgtctctgctgtggggcggagtgacagtgctggccgctatgctgattgctggacaggtggccagcgtggtgttcctggtgtctaagtctggacctcctagcggcaagagcaacagcaacaaccccgactgggacttcaaccccaacaaggaccattggccagaggccaatcaagtcggagccggcgcttttggccctggctttacacctcctcatggcggactgcttggatggtcacctcaggctcagggcatcctgacaacagtgcctgctgctccacctcctgccagcaccaatagacagtctggcagacagcccacacctatcagccctccactgagagacagccatcctcaggccatgcagtggaacagcaccacctttcatcaggccctgctggaccctagagtgcggggcctttattttcctgccggcggatctagcagcggcaccgtgaatcctgtgcctacaaccgcctctcctatcagcagcatcttcagcagaaccggcgatcccgctcctaacggcagcaagtctggctccaagatgcccctgagctaccagcacttcagaaaactgctgctgctggacgacgaggccggacctctggaagaagaactgcctagactggccgacgagggcctgaatagaagagtggccgaggacctgaacctgggcaacctgaatgtgtctatcccctggacacacaaagtgggcaacttcacaggcctggccagctctaccgtgcctgtgttcaatcccgagtggcagacccctagcttccctcacatccatctgcaagaggacatcatcaaccggtgccagcagtacgtgggccctctgaccgtgaacgagaagcggagactgaagctgatcatgcccgccagattctaccccaacctgaccaagtacctgcctctggacaagggcatcaagccttactaccctgagcacgccgtgaaccactacttcaagacccggcactacctgcacaccctgtggaaggccggcatcctgtataagagagagacaaccagaagcgccagcttctgcggcagcccttactcttgggagcaagagctgcagcacggcagactggtgttccagacctctacaagacacggcgacgagtctttctgcagccagagcagcggaatcctgagcagatctcctgtgggaccttgtgtgcggagccagctgaaacagagtagactgggcctgcagcctcagcagggatctctggctagaggaaagagcggcagaagcggcagcatcagagccagagtgcaccctaccaccagaagaagctttggcgtcgagcctagcggctccggccacatcgataatagcgccagcagcaccagcagctgcctgcatcagtccgccgttagaaagaccgcctacagccacctgagcacctccaagagacagagcagctctggacacgccgtggaactgcacaacatccctccaagcagcgccagatctcagagcgagggccctatcttttctgcctggtggctgcagttcagaaacagcaagcccgccagcgactacgccctgacacacatcgtgaacctgctggaagattggggccctgccacagaacacggcgagcacaatatcagaatccccagaacacccgccagagtgacaggcggagtgtttctggtggacaagaaccctcacaacaccaccgagagcaggctggtggtggacttcagccagtttagcagaggcagcacccacgtgtcctggcctaaattcgccgtgcctaacctgcagagcctgaccaatctgctgagcagcaacctgagctggctgagcctggatgtgtccgccgccttctatcacatcccactgcatcctgccgccatgcctcatctgcttgtgggaagttctggcctgcctagatacgtggccaggctgtcctctaccagccggaacatcaattaccagcacgggaccatgcaggacctgcacgacagctgtagccggaacctgtacgttagcctgctcctgctgtacaagaccttcggcagaaagctgcacctgtactctcaccccatcatcctgggcttcagaaagatccccatgggcgtgggcctgtctccatttctgctggcccagtttaccagcgccatctgctctgttgtgcggagagcctttcctcactgcctggccttcagctacatggacgatgtggtgctgggcgccaagtctgtgcagcacctggaaagcctgtttacctccatcaccaactttctgctgtccctgggaatccatctgaaccctaacaagaccaagagatggggctacagcctgaacttcatgggctacgtgatcggcagctggggcacactgcctcaagagcacatcgtgctgaaaatcaagcagtgctttcggaagctgcccgtgaacagacccatcgactggaaagtgtgccagcggatcgttggcctgctgggatttgccgctcctttcacacagtgcggctaccccgctctcatgcctctgtatgcctgtatccagagcaagcaggccttcacattcagccctacctacaaggccttcctgtgcaagcagtacctgaatctgtaccccgtggccagacagagaagcggcctgtgtcaagtgttcgccgatgccacacctacaggatggggactcgccattggacacagggccatgagaggaacctttgtggcccctctgcctatccacacagccgaattgctggctgcctgcttcgccagaagtagatccggcgccaagctgatcggcaccgacaattctgtggtcctgagccggaagtacaccagctttccatggctgctgggctgtgccgccaactggattctgagaggcaccagcttcgtgtacgtgcccagcgctcttaaccctgccgctgatccttctgctgggagactcggcctgtacagacctctgctgcatctgcccttcagacccaccacaggcagaaccagcctgtatgccgtgtctcctagcgtgccaagccatctgcctgatcgggtgcactttgcctctccacttcatgtggcttggcggccacctagcaagagccctggatctggaccacctatgcagctgtttcacctgtgcctgatcatctcttgcagctgccctacagtgcaggccagcaagctgtgtctcggatggctctggggcatggacatcgacccctacaaagaattcggcgccagcgtcgagctgctgagcttcctgcctagcgacttcttcccctccatccgggatctgctggatactgctagcgccctgtatcgcgaggccctggaatctcctgagcactgttctccacaccacactgccctgagacaggctatcctgtgttggggcgagctgatgaacctggccacatgggtcggaagcaacctggaagatcccgccagcagagaactggtggtgtcctacgtgaacgtgaacatgggcctgaagatcagacagctgctgtggttccacatctcctgcctgacctttggccgggaaaccgtgctggaatacctggtgtcctttggcgtgtggatcagaacccctccagcctaccgacctcctaacgctcctatcctgtctaccctgcctgagacaacagtcgtgcggcggagaggaagaagccctagaagaaggaccccatctcctcggcggagaagatcacagtcccctcggagaagaagatcccagagccgggaatcccagtgctgatttttgttcgacattaaaaattgaaaataaatacaaaggttcttgagggttgtgttaaattgaaagcgagaaataatcataaatatgattcaggtgacggatccatggacgctatgaagaggggcctgtgctgtgtgctgctgctgtgcggagctgtgtttgtgtcccctagccaagagatccacgccagattcagaagaatgggcggctggtccagcaagcccagacaaggcatgggcaccaatctgagcgtgcccaatcctctgggattcttcccagaccaccagctggatcctgccttcggcgccaacagcaacaaccccgactgggacttcaaccccaacaaggaccattggccagaggccaatcaagtgggcgctagcaaaggcggcaagagcggcatggagaataccacctctggctttctgggccctctgctggttctgcaggccggcttctttctgctgacccggatcctgacaatccctcagagcctggatagctggtggacaagcctgaacttccttggcggcgctcctacatgccctggccagaattctcagagccccaccagcaatcacagccccacaagctgccctccaatctgccctggctacagatggatgtgcctgcggcggttcatcatctttctgttcatcctgctgctctgcctgatcttcctgctggtgctcctggactatcagggcatgctgcctgtgtgtcctctgctgcctggcaccagcacaacatctacaggcccttgcaagacctgcacaatcccagctcagggcacctccatgtttcccagctgctgttgcaccaagcctagcgacggcaactgcacatgcatccccattccttccagctgggccttcgccagatttctgtgggaatgggccagcgtgcggttcagctggctgtctctgcttgtgcctttcgtgcagtggttcgtgggcctgtctcctacagtgtggctgagcgtgatctggatgatgtggtactggggccctagcctgtacaatattctgagccccttcctgcctctgctcccaatcttcttctgcctgtgggtgtacatctgattaaccgagtttctgcattattgtaattcgtatgctggcaccatcaaagaatcacttctaaaagatatcaatatcacacatacaaatattactaccctattgaatgagacagccaaggttatcaagttagtaaaatctctggtagataaagaagatactgatattgtgaataatttcattaccaaagaaattaaaaacagagacaaaatagttaatagtttgtctctatcaaacctggactttcgtttgtaaattggggctttttgtacaataaatgggtgttgccaatgattcatcccctgaatatcaatggatgtctccccatagattatcagatactgttatattaggagactgtttgtattttaacaatataatgtcccaattagatttacaccaaaattgggctccatcagttagattgttaaattattttaagaattttaataaggaaacactactaaagatagaagagaatgattacattaattcatcctttttccaacaaaaggataaacgattttatcctataaacgacgatttttatcacatatctacaggaggatatggtatagtctttaagatagataactatgtagtaaaatttgtattcgaggccacaaaattatatagtcccatggaaactacggcggagttcacagtacccaaatttctatacaacaatctaaagggagatgaaaaaaaattaatcgtgtgtgcgtgggccatgggattaaactataaattaacatttttacatactctgtataaacgtgttcttcatatgttgctattattgatacaaactatggatggtcaggaactatcattgagatattcttctaaagtttttttaaaggcgtttaacgagagaaaggacagtatcaaattcgtgaaattactatcccacttttatccggcagttattaacagtaatattaatgttataaactattttaaccgcatgtttcactttttcgaacatgaaaagagaactaactacgaatacgaaagaggaaatattataatttttcccctagcactgtattcggcagataaagtagataccgagctagctatcaaattaggatttaaatctttggtacaatacataaagtttatctttttacagatggctctgttatacattaaaatttacgaactaccatgctgcgacaactttttacacgcagatcttaaacccgataatatcttactttttgattccaatgaaccaataataattcatctaaaggataaaaagtttgtttttaatgaacgtattaaatcggcattaaacgactttgacttttcccaag

SEQ ID NO: 28 - DNA, 97 bp, Artificial Sequence
  Promoter
tcgacattaaaaattgaaaataaatacaaaggttcttgagggttgtgttaaattgaaagcgagaaataatcataaatatgattcaggtgacggatcc

SEQ ID NO: 29 - DNA, 96 bp, Artificial Sequence
  TPA sequence
atggacgctatgaagaggggcctgtgctgtgtgctgctgctgtgcggagctgtgtttgtgtcccctagccaagagatccacgccagattcagaaga

SEQ ID NO: 30 - protein, 32 aa, Artificial Sequence
  TPA peptide
MDAMKRGLCCVLLLCGAVFVSPSQEIHARFRR

SEQ ID NO: 31 - protein, 10 aa, Artificial Sequence
  Linker peptide
SKSGPPSGKS

SEQ ID NO: 32 - protein, 7 aa, Artificial Sequence
  Linker peptide
GSKSGSK

SEQ ID NO: 33 - protein, 9 aa, Artificial Sequence
  Linker peptide
SKSPGSGPP

SEQ ID NO: 34 - protein, 8 aa, Artificial Sequence
  Linker peptide
ASKGGKSG

SEQ ID NO: 35 - DNA, 1097 bp, Artificial Sequence
  F11 left flank
gtaatctattcgatataccgttgctaacagtatactggcccaataactgtggatggaaaatctataataatacattaatatcatccgatggtgctagggttatttggatggatgcgtataaattttcttgcggtttatctttacaagactattgttatcattggggtagcaaaccagagagccgaccattcgatttaataaaaaaatcagatgctaaacgcaattctaaatcgttggtcaaagaatctatggcatccttgaaatccttgtacgaggcattcgagacacaatcaggagcgttagaagttttaatgagtccatgtaggatgttttcgttttctagaatagaagacatgttcttaactagtgtcattaatagagtatccgagaatactggaatggggatgtattatcctaccaacgatataccttctctatttatcgaatcatctatctgtctagattatattatagtaaataatcaggaatccaacaaatatcgtatcaaatctgttctcgatatcatttcttcaaaacaataccctgcaggacgtcccaactacgttaaaaatggtacaaaaggaaagttatatatcgcgttgtgtaaagttaccgtacctactaacgaccatattccagtagtttatcacgatgatgacaatactaccacctttattacagtattgacgtccgtcgatattgaaactgctatcagagcaggatattcgatagtcgaattaggggctttacaatgggataataatattccagaacttaaaaacggtttactggatagtatcaagatgatttatgacttgaacgcagttacaacaaataatttattggaacagctcatagaaaatattaactttaacaactctagtataatttcgttgttttatacatttgccattagttattgccgagcattcatttactcaattatggaaaccatagatccggtgtatatatctcagttcagttataaagaattatacgttagtagctcttataaagatattaatgaatccatgagtcagatggtaaaattataaaaagtgaaaaacaatattatttttatcgttggttgttacact

SEQ ID NO: 36 - DNA, 1319 bp, Artificial Sequence
  F11 right flank
ttaaccgagtttctgcattattgtaattcgtatgctggcaccatcaaagaatcacttctaaaagatatcaatatcacacatacaaatattactaccctattgaatgagacagccaaggttatcaagttagtaaaatctctggtagataaagaagatactgatattgtgaataatttcattaccaaagaaattaaaaacagagacaaaatagttaatagtttgtctctatcaaacctggactttcgtttgtaaattggggctttttgtacaataaatgggtgttgccaatgattcatcccctgaatatcaatggatgtctccccatagattatcagatactgttatattaggagactgtttgtattttaacaatataatgtcccaattagatttacaccaaaattgggctccatcagttagattgttaaattattttaagaattttaataaggaaacactactaaagatagaagagaatgattacattaattcatcctttttccaacaaaaggataaacgattttatcctataaacgacgatttttatcacatatctacaggaggatatggtatagtctttaagatagataactatgtagtaaaatttgtattcgaggccacaaaattatatagtcccatggaaactacggcggagttcacagtacccaaatttctatacaacaatctaaagggagatgaaaaaaaattaatcgtgtgtgcgtgggccatgggattaaactataaattaacatttttacatactctgtataaacgtgttcttcatatgttgctattattgatacaaactatggatggtcaggaactatcattgagatattcttctaaagtttttttaaaggcgtttaacgagagaaaggacagtatcaaattcgtgaaattactatcccacttttatccggcagttattaacagtaatattaatgttataaactattttaaccgcatgtttcactttttcgaacatgaaaagagaactaactacgaatacgaaagaggaaatattataatttttcccctagcactgtattcggcagataaagtagataccgagctagctatcaaattaggatttaaatctttggtacaatacataaagtttatctttttacagatggctctgttatacattaaaatttacgaactaccatgctgcgacaactttttacacgcagatcttaaacccgataatatcttactttttgattccaatgaaccaataataattcatctaaaggataaaaagtttgtttttaatgaacgtattaaatcggcattaaacgactttgacttttcccaag

SEQ ID NO: 37 - DNA, 3741 bp, Artificial Sequence
  Vaccine construct
atgtctctgctgtggggcggagtgacagtgctggccgctatgctgattgctggacaggtggccagcgtggtgttcctggtgtctaagtctggacctcctagcggcaagagcaacagcaacaaccccgactgggacttcaaccccaacaaggaccattggccagaggccaatcaagtcggagccggcgcttttggccctggctttacacctcctcatggcggactgcttggatggtcacctcaggctcagggcatcctgacaacagtgcctgctgctccacctcctgccagcaccaatagacagtctggcagacagcccacacctatcagccctccactgagagacagccatcctcaggccatgcagtggaacagcaccacctttcatcaggccctgctggaccctagagtgcggggcctttattttcctgccggcggatctagcagcggcaccgtgaatcctgtgcctacaaccgcctctcctatcagcagcatcttcagcagaaccggcgatcccgctcctaacggcagcaagtctggctccaagatgcccctgagctaccagcacttcagaaaactgctgctgctggacgacgaggccggacctctggaagaagaactgcctagactggccgacgagggcctgaatagaagagtggccgaggacctgaacctgggcaacctgaatgtgtctatcccctggacacacaaagtgggcaacttcacaggcctggccagctctaccgtgcctgtgttcaatcccgagtggcagacccctagcttccctcacatccatctgcaagaggacatcatcaaccggtgccagcagtacgtgggccctctgaccgtgaacgagaagcggagactgaagctgatcatgcccgccagattctaccccaacctgaccaagtacctgcctctggacaagggcatcaagccttactaccctgagcacgccgtgaaccactacttcaagacccggcactacctgcacaccctgtggaaggccggcatcctgtataagagagagacaaccagaagcgccagcttctgcggcagcccttactcttgggagcaagagctgcagcacggcagactggtgttccagacctctacaagacacggcgacgagtctttctgcagccagagcagcggaatcctgagcagatctcctgtgggaccttgtgtgcggagccagctgaaacagagtagactgggcctgcagcctcagcagggatctctggctagaggaaagagcggcagaagcggcagcatcagagccagagtgcaccctaccaccagaagaagctttggcgtcgagcctagcggctccggccacatcgataatagcgccagcagcaccagcagctgcctgcatcagtccgccgttagaaagaccgcctacagccacctgagcacctccaagagacagagcagctctggacacgccgtggaactgcacaacatccctccaagcagcgccagatctcagagcgagggccctatcttttctgcctggtggctgcagttcagaaacagcaagcccgccagcgactacgccctgacacacatcgtgaacctgctggaagattggggccctgccacagaacacggcgagcacaatatcagaatccccagaacacccgccagagtgacaggcggagtgtttctggtggacaagaaccctcacaacaccaccgagagcaggctggtggtggacttcagccagtttagcagaggcagcacccacgtgtcctggcctaaattcgccgtgcctaacctgcagagcctgaccaatctgctgagcagcaacctgagctggctgagcctggatgtgtccgccgccttctatcacatcccactgcatcctgccgccatgcctcatctgcttgtgggaagttctggcctgcctagatacgtggccaggctgtcctctaccagccggaacatcaattaccagcacgggaccatgcaggacctgcacgacagctgtagccggaacctgtacgttagcctgctcctgctgtacaagaccttcggcagaaagctgcacctgtactctcaccccatcatcctgggcttcagaaagatccccatgggcgtgggcctgtctccatttctgctggcccagtttaccagcgccatctgctctgttgtgcggagagcctttcctcactgcctggccttcagctacatggacgatgtggtgctgggcgccaagtctgtgcagcacctggaaagcctgtttacctccatcaccaactttctgctgtccctgggaatccatctgaaccctaacaagaccaagagatggggctacagcctgaacttcatgggctacgtgatcggcagctggggcacactgcctcaagagcacatcgtgctgaaaatcaagcagtgctttcggaagctgcccgtgaacagacccatcgactggaaagtgtgccagcggatcgttggcctgctgggatttgccgctcctttcacacagtgcggctaccccgctctcatgcctctgtatgcctgtatccagagcaagcaggccttcacattcagccctacctacaaggccttcctgtgcaagcagtacctgaatctgtaccccgtggccagacagagaagcggcctgtgtcaagtgttcgccgatgccacacctacaggatggggactcgccattggacacagggccatgagaggaacctttgtggcccctctgcctatccacacagccgaattgctggctgcctgcttcgccagaagtagatccggcgccaagctgatcggcaccgacaattctgtggtcctgagccggaagtacaccagctttccatggctgctgggctgtgccgccaactggattctgagaggcaccagcttcgtgtacgtgcccagcgctcttaaccctgccgctgatccttctgctgggagactcggcctgtacagacctctgctgcatctgcccttcagacccaccacaggcagaaccagcctgtatgccgtgtctcctagcgtgccaagccatctgcctgatcgggtgcactttgcctctccacttcatgtggcttggcggccacctagcaagagccctggatctggaccacctatgcagctgtttcacctgtgcctgatcatctcttgcagctgccctacagtgcaggccagcaagctgtgtctcggatggctctggggcatggacatcgacccctacaaagaattcggcgccagcgtcgagctgctgagcttcctgcctagcgacttcttcccctccatccgggatctgctggatactgctagcgccctgtatcgcgaggccctggaatctcctgagcactgttctccacaccacactgccctgagacaggctatcctgtgttggggcgagctgatgaacctggccacatgggtcggaagcaacctggaagatcccgccagcagagaactggtggtgtcctacgtgaacgtgaacatgggcctgaagatcagacagctgctgtggttccacatctcctgcctgacctttggccgggaaaccgtgctggaatacctggtgtcctttggcgtgtggatcagaacccctccagcctaccgacctcctaacgctcctatcctgtctaccctgcctgagacaacagtcgtgcggcggagaggaagaagccctagaagaaggaccccatctcctcggcggagaagatcacagtcccctcggagaagaagatcccagagccgggaatcccagtgctga

SEQ ID NO: 38 - DNA, 882 bp, Hepatitis B virus
atgggaggctggtccagcaaacccagacaaggcatgggcaccaatctgagcgtgcccaatcctctgggattcttcccagaccaccagctggatcctgccttcggcgccaacagcaacaaccccgactgggacttcaaccccaacaaggaccattggccagaggccaatcaagtgggcgctagcaaaggcggcaagagcggcatggagaataccacctctggctttctgggccctctgctggttctgcaggccggcttctttctgctgacccggatcctgacaatccctcagagcctggatagctggtggacaagcctgaacttccttggcggcgctcctacatgccctggccagaattctcagagccccaccagcaatcacagccccacaagctgccctccaatctgccctggctacagatggatgtgcctgcggcggttcatcatctttctgttcatcctgctgctgtgcctgatcttcctgctggtgctgctggactatcagggcatgctgcctgtgtgtcctctgctgcctggcaccagcacaacatctacaggcccttgcaagacctgcacaatcccagctcagggcacctccatgtttcccagctgctgttgcaccaagcctagcgacggcaactgcacatgcatccccattccttccagctgggccttcgccagatttctgtgggaatgggccagcgtgcggttcagctggctgtctctgcttgtgcctttcgtgcagtggttcgtgggcctgtctcctacagtgtggctgagcgtgatctggatgatgtggtactggggccctagcctgtacaatattctgagccccttcctgcctctgctcccaatcttcttctgcctgtgggtgtacatctga

SEQ ID NO: 39 - DNA, 12012 bp, Artificial Sequence
  Vector
ccaccgcctcggacctggccgacctcatcttccccgagcgcctcaggctgacgctgcgcaacggcctgcccgactttatgagccaaagcatgttgcaaaaactttcggtaaaaaatgtaattactccctcctgcacaggcagcaaagcccccgctccctccagaaacacatacaaagcctcagcgtccatagcttaccgagcacggcaggcgcaagagtcagagaaaaggctgagctctaacctgactgcccgctcctgtgctcaatatataagccctaacctacactgacgtaaaagggcccaaaagtctaaaaaaataacccgcccaaaatgacacacacgcccagcacacgcccagaaaccggtgacacactcaaaaaaatacgtgcgcttcctcaaacgcccaaaccggcgtcatttccgggttcccacgctacgtcaccgctcagcgactttcaaattccgtcgaccgttaaaaacgtcactcgccccgcccctaacggtcgcccttctctcggccaatcaccttcctcccttcccaaattcaaacgcctcatttgcatattaacgcgcacaaaaagtttgaggtatatatttgaatgatggtttaaacgcggccgccaggcctacccactagtcaattcgggaggatcgaaacggcagatcgcaaaaaacagtacatacagaaggagacatgaacatgaacatcaaaaaaattgtaaaacaagccacagttctgacttttacgactgcacttctggcaggaggagcgactcaagccttcgcgaaagaaaataaccaaaaagcatacaaagaaacgtacggcgtctctcatattacacgccatgatatgctgcagatccctaaacagcagcaaaacgaaaaataccaagtgcctcaattcgatcaatcaacgattaaaaatattgagtctgcaaaaggacttgatgtgtgggacagctggccgctgcaaaacgctgacggaacagtagctgaatacaacggctatcacgttgtgtttgctcttgcgggaagcccgaaagacgctgatgacacatcaatctacatgttttatcaaaaggtcggcgacaactcaatcgacagctggaaaaacgcgggccgtgtctttaaagacagcgataagttcgacgccaacgatccgatcctgaaagatcagacgcaagaatggtccggttctgcaacctttacatctgacggaaaaatccgtttattctacactgactattccggtaaacattacggcaaacaaagcctgacaacagcgcaggtaaatgtgtcaaaatctgatgacacactcaaaatcaacggagtggaagatcacaaaacgatttttgacggagacggaaaaacatatcagaacgttcagcagtttatcgatgaaggcaattatacatccggcgacaaccatacgctgagagaccctcactacgttgaagacaaaggccataaataccttgtattcgaagccaacacgggaacagaaaacggataccaaggcgaagaatctttatttaacaaagcgtactacggcggcggcacgaacttcttccgtaaagaaagccagaagcttcagcagagcgctaaaaaacgcgatgctgagttagcgaacggcgccctcggtatcatagagttaaataatgattacacattgaaaaaagtaatgaagccgctgatcacttcaaacacggtaactgatgaaatcgagcgcgcgaatgttttcaaaatgaacggcaaatggtacttgttcactgattcacgcggttcaaaaatgacgatcgatggtattaactcaaacgatatttacatgcttggttatgtatcaaactctttaaccggcccttacaagccgctgaacaaaacagggcttgtgctgcaaatgggtcttgatccaaacgatgtgacattcacttactctcacttcgcagtgccgcaagccaaaggcaacaatgtggttatcacaagctacatgacaaacagaggcttcttcgaggataaaaaggcaacatttgcgccaagcttcttaatgaacatcaaaggcaataaaacatccgttgtcaaaaacagcatcctggagcaaggacagctgacagtcaactaataacagcaaaaagaaaatgccgatacttcattggcattttcttttatttctcaacaagatggtgaattgactagtgggtagatccacaggacgggtgtggtcgccatgatcgcgtagtcgatagtggctccaagtagcgaagcgagcaggactgggcggcggccaaagcggtcggacagtgctccgagaacgggtgcgcatagaaattgcatcaacgcatatagcgctagcagcacgccatagtgactggcgatgctgtcggaatggacgatatcccgcaagaggcccggcagtaccggcataaccaagcctatgcctacagcatccagggtgacggtgccgaggatgacgatgagcgcattgttagatttcatacacggtgcctgactgcgttagcaatttaactgtgataaactaccgcattaaagcttatcgatgataagctgtcaaacatgagaattgatccggaacccttaatataacttcgtataatgtatgctatacgaagttattaggtccctcgactatagggtcaccgtcgacagcgacacacttgcatcggatgcagcccggttaacgtgccggcacggcctgggtaaccaggtattttgtccacataaccgtgcgcaaaatgttgtggataagcaggacacagcagcaatccacagcaggcatacaaccgcacaccgaggttactccgttctacaggttacgacgacatgtcaatacttgcccttgacaggcattgatggaatcgtagtctcacgctgatagtctgatcgacaatacaagtgggaccgtggtcccagaccgataatcagaccgacrayacgagtgggaycgtggtcccagactaataatcagaccgacgatacgagtgggaccgtggtcccagactaataatcagaccgacgatacgagtgggaccgtggtyccagwctratwatcagaccgacgatacragtggracmgtggkcccagasakaatawtcagrccgagwtaygcwktckggcctgtaacaaaggacattaagtaaagacagatamrmgtgrgactaaaacgtggtcccagtctgattatcagaccgacgatacgagtgggaccgtggtcccagactaataatcagaccgacgatacgagtgggaccgtggtcccagactaataatcagaccgacgatacgagtgggaccgtggtcccagtctgattatcagaccgacgatacaagtggaacagtgggcccagagagaatattcaggccagttatgctttctggcctgtaacaaaggacattaagtaaagacagataaacgtagactaaaacgtggtcgcatcagggtgctggcttttcaagttccttaagaatggcctcaattttctctatacactcagttggaacacgagacctgtccaggttaagcaccattttatcgcccttatacaatactgtcgctccaggagcaaactgatgtcgtgagcttaaactagttcttgatgcagatgacgttttaagcacagaagttaaaagagtgataacttcttcagcttcaaatatcaccccagcttttttctgctcatgaaggttagatgcctgctgcttaagtaattcctctttatctgtaaaggctttttgaagtgcatcacctgaccgggcagatagttcaccggggtgagaaaaaagagcaacaactgatttaggcaatttggcggtgttgatacagcgggtaataatcttacgtgaaatattttccgcatcagccagcgcagaaatatttccagcaaattcattctgcaatcggcttgcataacgctgaccacgttcataagcacttgttgggcgataatcgttacccaatctggataatgcagccatctgctcatcatccagctcgccaaccagaacacgataatcactttcggtaagtgcagcagctttacgacggcgactcccatcggcaatttctatgacaccagatactcttcgaccgaacgccggtgtctgttgaccagtcagtagaaaagaagggatgagatcatccagtgcgtcctcagtaagcagctcctggtcacgttcattacctgaccatacccgagaggtcttctcaacactatcaccccggagcacttcaagagtaaacttcacatcccgaccacatacaggcaaagtaatggcattaccgcgagccattactcctacgcgcgcaattaacgaatccaccatcggggcagctggtgtcgataacgaagtatcttcaaccggttgagtattgagcgtatgttttggaataacaggcgcacgcttcattatctaatctcccagcgtggtttaatcagacgatcgaaaatttcattgcagacaggttcccaaatagaaagagcatttctccaggcaccagttgaagagcgttgatcaatggcctgttcaaaaacagttctcatccggatctgacctttaccaacttcatccgtttcacgtacaacattttttagaaccatgcttccccaggcatcccgaatttgctcctccatccacggggactgagagccattactattgctgtatttggtaagcaaaatacgtacatcaggctcgaaccctttaagatcaacgttcttgagcagatcacgaagcatatcgaaaaactgcagtgcggaggtgtagtcaaacaactcagcaggcgtgggaacaatcagcacatcagcagcacatacgacattaatcgtgccgatacccaggttaggcgcgctgtcaataactatgacatcatagtcatgagcaacagtttcaatggccagtcggagcatcaggtgtggatcggtgggcagtttaccttcatcaaatttgcccattaactcagtttcaatacggtgcagagccagacaggaaggaataatgtcaagccccggccagcaagtgggctttattgcataagtgacatcgtccttttccccaagatagaaaggcaggagagtgtcttctgcatgaatatgaagatctggtacccatccgtgatacattgaggctgttccctgggggtcgttaccttccacgagcaaaacacgtagccccttcagagccagatcctgagcaagatgaacagaaactgaggttttgtaaacgccacctttatgggcagcaaccccgatcaccggtggaaatacgtcttcagcacgtcgcaatcgcgtaccaaacacatcacgcatatgattaatttgttcaattgtataaccaacacgttgctcaacccgtcctcgaatttccatatccgggtgcggtagtcgccctgctttctcggcatctctgatagcctgagaagaaaccccaactaaatccgctgcttcacctattctccagcgccgggttattttcctcgcttccgggctgtcatcattaaactgtgcaatggcgatagccttcgtcatttcatgaccagcgtttatgcactggttaagtgtttccatgagtttcattctgaacatcctttaatcattgctttgcgtttttttattaaatcttgcaatttactgcaaagcaacaacaaaatcgcaaagtcatcaaaaaaccgcaaagttgtttaaaataagagcaacactacaaaaggagataagaagagcacatacctcagtcacttattatcactagcgctcgccgcagccgtgtaaccgagcatagcgagcgaactggcgaggaagcaaagaagaactgttctgtcagatagctcttacgctcagcgcaagaagaaatatccaccgtgggaaaaactccaggtagaggtacacacgcggatagccaattcagagtaataaactgtgataatcaaccctcatcaatgatgacgaactaacccccgatatcaggtcacatgacgaagggaaagagaaggaaatcaactgtgacaaactgccctcaaatttggcttccttaaaaattacagttcaaaaagtatgagaaaatccatgcaggctgaaggaaacagcaaaactgtgacaaattaccctcagtaggtcagaacaaatgtgacgaaccaccctcaaatctgtgacagataaccctcagactatcctgtcgtcatggaagtgatatcgcggaaggaaaatacgatatgagtcgtctggcggcctttctttttctcaatgtatgagaggcgcattggagttctgctgttgatctcattaacacagacctgcaggaagcggcggcggaagtcaggcatacgctggtaactttgaggcagctggtaacgctctatgatccagtcgattttcagagagacgatgcctgagccatccggcttacgatactgacacagggattcgtataaacgcatggcatacggattggtgatttcttttgtttcactaagccgaaactgcgtaaaccggttctgtaacccgataaagaagggaatgagatatgggttgatatgtacactgtaaagccctctggatggactgtgcgcacgtttgataaaccaaggaaaagattcatagcctttttcatcgccggcatcctcttcagggcgataaaaaaccacttccttccccgcgaaactcttcaatgcctgccgtatatccttactggcttccgcagaggtcaatccgaatatttcagcatatttagcaacatggatctcgcagataccgtcatgttcctgtagggtgccatcagattttctgatctggtcaacgaacagatacagcatacgtttttgatcccgggagagactatatgccgcctcagtgaggtcgtttgactggacgattcgcgggctatttttacgtttcttgtgattgataaccgctgtttccgccatgacagatccatgtgaagtgtgacaagtttttagattgtcacactaaataaaaaagagtcaataagcagggataactttgtgaaaaaacagcttcttctgagggcaatttgtcacagggttaagggcaatttgtcacagacaggactgtcatttgagggtgatttgtcacactgaaagggcaatttgtcacaacaccttctctagaaccagcatggataaaggcctacaaggcgctctaaaaaagaagatctaaaaactataaaaaaaataattataaaaatatccccgtggataagtggataaccccaagggaagttttttcaggcatcgtgtgtaagcagaatatataagtgctgttccctggtgcttcctcgctcactcgagggcttcgccctgtcgctcaactgcggcgagcactactggctgtaaaaggacagaccacatcatggttctgtgttcattaggttgttctgtccattgctgacataatccgctccacttcaacgtaacaccgcacgaagatttctattgttcctgaaggcatattcaaatcgttttcgttaccgcttgcaggcatcatgacagaacactacttcctataaacgctacacaggctcctgagattaataatgcggatctctacgataatgggagattttcccgactgtttcgttcgcttctcagtggataacagccagcttctctgtttaacagacaaaaacagcatatccactcagttccacatttccatataaaggccaaggcatttattctcaggataattgtttcagcatcgcaaccgcatcagactccggcatcgcaaactgcacccggtgccgggcagccacatccagcgcaaaaaccttcgtgtagacttccgttgaactgatggacttatgtcccatcaggctttgcagaactttcagcggtataccggcatacagcatgtgcatcgcataggaatggcggaacgtatgtggtgtgaccggaacagagaacgtcacaccgtcagcagcagcggcggcaaccgcctccccaatccaggtcctgaccgttctgtccgtcacttcccagatccgcgctttctctgtccttcctgtgcgacggttacgccgctccatgagcttatcgcgaataaatacctgtgacggaagatcacttcgcagaataaataaatcctggtgtccctgttgataccgggaagccctgggccaacttttggcgaaaatgagacgttgatcggcacgtaagaggttccaactttcaccataatgaaataagatcactaccgggcgtattttttgagttatcgagattttcaggagctaaggaagctaaaatggagaaaaaaatcactggatataccaccgttgatatatcccaatggcatcgtaaagaacattttgaggcatttcagtcagttgctcaatgtacctataaccagaccgttcagctggatattacggcctttttaaagaccgtaaagaaaaataagcacaagttttatccggcctttattcacattcttgcccgcctgatgaatgctcatccggagttccgtatggcaatgaaagacggtgagctggtgatatgggatagtgttcacccttgttacaccgttttccatgagcaaactgaaacgttttcatcgctctggagtgaataccacgacgatttccggcagtttctacacatatattcgcaagatgtggcgtgttacggtgaaaacctggcctatttccctaaagggtttattgagaatatgtttttcgtctcagccaatccctgggtgagtttcaccagttttgatttaaacgtggccaatatggacaacttcttcgcccccgttttcaccatgggcaaatattatacgcaaggcgacaaggtgctgatgccgctggcgattcaggttcatcatgccgtttgtgatggcttccatgtcggcagaatgcttaatgaattacaacagtactgcgatgagtggcagggcggggcgtaatttttttaaggcagttattggtgcccttaaacgcctggttgctacgcctgaataagtgataataagcggatgaatggcagaaattcgatgataagctgtcaaacatgagaattggtcgacggcgcgccaaagcttgcatgcctgcagccgcgtaacctggcaaaatcggttacggttgagtaataaatggatgccctgcgtaagcggggcacatttcattacctctttctccgcacccgacatagataataacttcgtatagtatacattatacgaagttatctagtagacttaatcgcgtttaaacccatcatcaataatatacctcaaactttttgtgcgcgttaatatgcaaatgaggcgtttgaatttgggaagggaggaaggtgattggccgagagaagggcgaccgttaggggcggggcgagtgacgttttgatgacgtgaccgcgaggaggagccagtttgcaagttctcgtgggaaaagtgacgtcaaacgaggtgtggtttgaacacggaaatactcaattttcccgcgctctctgacaggaaatgaggtgtttctaggcggatgcaagtgaaaacgggccattttcgcgcgaaaactgaatgaggaagtgaaaatctgagtaatttcgcgtttatgacagggaggagtatttgccgagggccgagtagactttgaccgattacgtgggggtttcgattaccgtgtttttcacctaaatttccgcgtacggtgtcaaagtccggtgtttttacgtaggtgtcagctgatcgccagggtatttaaacctgcgctctccagtcaagaggccactcttgagtgccagcgagaagagttttctcctccgcgcgcgagtcagatctacactttgaaaggcgatcgctagcgacatcgatcacaagtttgtacaaaaaagcaggctccaccatgggaacccgcgttttgagatttctgtcgccgactaaattcatgtcgcgcgatagtggtgtttatcgccgatagagatggcgatattggaaaaatcgatatttgaaaatatggcatattgaaaatgtcgccgatgtgagtttctgtgtaactgatatcgccatttttccaaaagtgatttttgggcatacgcgatatctggcgatagcgcttatatcgtttacgggggatggcgatagacgactttggtgacttgggcgattctgtgtgtcgcaaatatcgcagtttcgatataggtgacagacgatatgaggctatatcgccgatagaggcgacatcaagctggcacatggccaatgcatatcgatctatacattgaatcaatattggccattagccatattattcattggttatatagcataaatcaatattggctattggccattgcatacgttgtatccatatcataatatgtacatttatattggctcatgtccaacattaccgccatgttgacattgattattgactagttattaatagtaatcaattacggggtcattagttcatagcccatatatggagttccgcgttacataacttacggtaaatggcccgcctggctgaccgcccaacgacccccgcccattgacgtcaataatgacgtatgttcccatagtaacgccaatagggactttccattgacgtcaatgggtggagtatttacggtaaactgcccacttggcagtacatcaagtgtatcatatgccaagtacgccccctattgacgtcaatgacggtaaatggcccgcctggcattatgcccagtacatgaccttatgggactttcctacttggcagtacatctacgtattagtcatcgctattaccatggtgatgcggttttggcagtacatcaatgggcgtggatagcggtttgactcacggggatttccaagtctccaccccattgacgtcaatgggagtttgttttggcaccaaaatcaacgggactttccaaaatgtcgtaacaactccgccccattgacgcaaatgggcggtaggcgtgtacggtgggaggtctatataagcagagctctccctatcagtgatagagatctccctatcagtgatagagatcgtcgacgagctcgtttagtgaaccgtcagatcgcctggagacgccatccacgctgttttgacctccatagaagacaccgggaccgatccagcctccgcggccgggaacggtgcattggaacgcggattccccgtgccaagagtgacgtaagtaccgcctatagagtctataggcccacccccttggcttcttatgcatgctatactgtttttggcttggggtctatacacccccgcttcctcatgttataggtgatggtatagcttagcctataggtgtgggttattgaccattattgaccactcccctattggtgacgatactttccattactaatccataacatggctctttgccacaactctctttattggctatatgccaatacactgtccttcagagactgacacggactctgtatttttacaggatggggtctcatttattatttacaaattcacatatacaacaccaccgtccccagtgcccgcagtttttattaaacataacgtgggatctccacgcgaatctcgggtacgtgttccggacatgggctcttctccggtagcggcggagcttctacatccgagccctgctcccatgcctccagcgactcatggtcgctcggcagctccttgctcctaacagtggaggccagacttaggcacagcacgatgcccaccaccaccagtgtgccgcacaaggccgtggcggtagggtatgtgtctgaaaatgagctcggggagcgggcttgcaccgctgacgcatttggaagacttaaggcagcggcagaagaagatgcaggcagctgagttgttgtgttctgataagagtcagaggtaactcccgttgcggtgctgttaacggtggagggcagtgtagtctgagcagtactcgttgctgccgcgcgcgccaccagacataatagctgacagactaacagactgttcctttccatgggtcttttctgcagtcaccgtccttgacacgaagcttggtacc

SEQ ID NO: 40 - DNA, 29187 bp, Artificial Sequence
  Vector
gcggccgctcgagcatgcatctagagggccctattctatagtgtcacctaaatgctagagctcgctgatcagcctcgactgtgccttctagttgccagccatctgttgtttgcccctcccccgtgccttccttgaccctggaaggtgccactcccactgtcctttcctaataaaatgaggaaattgcatcgcattgtctgagtaggtgtcattctattctggggggtggggtggggcaggacagcaagggggaggattgggaagacaatagcaggcatgctggggatgcggtgggctctatggcttctgaggcggaaagaaccagctggggctcgaggggggatcgatcccgtcgagatatctagacccagctttcttgtacaaagtggtgatcgattcgacagatcgcgatcgcagtgagtagtgttctggggcgggggaggacctgcatgagggccagaatgactgaaatctgtgcttttctgtgtgttgcagcatcatgagcggaagcggctcctttgagggaggggtattcagcccttatctgacggggcgtctcccctcctgggcgggagtgcgtcagaatgtgatgggatccacggtggacggccggcccgtgcagcccgcgaactcttcaaccctgacctatgcaaccctgagctcttcgtcggtggacgcagctgccgccgcagctgctgcatccgccgccagcgccgtgcgcggaatggccatgggcgccggctactacggcactctggtggccaactcgagttccaccaataatcccgccagcctgaacgaggagaagctgctgctgctgatggcccagcttgaggccttgacccagcgcctgggcgagctgacccagcaggtggctcagctgcaggagcagacgcgggccgcggttgccacggtgaaatccaaataaaaaatgaatcaataaataaacggagacggttgttgattttaacacagagtctgaatctttatttgatttttcgcgcgcggtaggccctggaccaccggtctcgatcattgagcacccggtggatcttttccaggacccggtagaggtgggcttggatgttgaggtacatgggcatgagcccgtcccgggggtggaggtagctccattgcagggcctcgtgctcgggggtggtgttgtaaatcacccagtcatagcaggggcgcagggcgtggtgttgcacaatatctttgaggaggagactgatggccacgggcagccctttggtgtaggtgtttacaaatctgttgagctgggagggatgcatgcggggggagatgaggtgcatcttggcctggatcttgagattggcgatgttaccgcccagatcccgcctggggttcatgttgtgcaggaccaccagcacggtgtatccggtgcacttggggaatttatcatgcaacttggaagggaaggcgtgaaagaatttggcgacgcccttgtgtccgcccaggttttccatgcactcatccatgatgatggcaatgggcccgtgggcggcggcctgggcaaagacgtttcgggggtcggacacatcatagttgtggtcctgggtgaggtcatcataggccattttaatgaatttggggcggagggtgccggactgggggacaaaggtaccctcgatcccgggggcgtagttcccctcacagatctgcatctcccaggctttgagctcagagggggggatcatgtccacctgcggggcgataaagaacacggtttccggggcgggggagatgagctgggccgaaagcaagttccggagcagctgggacttgccgcagccggtggggccgtaaatgaccccgatgaccggctgcaggtggtagttgagggagagacagctgccgtcctcccggaggaggggggccacctcgttcatcatctcgcgcacgtgcatgttctcgcgcaccagttccgccaggaggcgctctccccccagagataggagctcctggagcgaggcgaagtttttcagcggcttgagtccgtcggccatgggcattttggagagggtctgttgcaagagttccaagcggtcccagagctcggtgatgtgctctacggcatctcgatccagcagacctcctcgtttcgcgggttgggacgactgcgggagtagggcaccagacgatgggcgtccagcgcagccagggtccggtccttccagggccgcagcgtccgcgtcagggtggtctccgtcacggtgaaggggtgcgcgccgggctgggcgcttgcgagggtgcgcttcaggctcatccggctggtcgaaaaccgctcccgatcggcgccctgcgcgtcggccaggtagcaattgaccatgagttcgtagttgagcgcctcggccgcgtggcctttggcgcggagcttacctttggaagtctgcccgcaggcgggacagaggagggacttgagggcgtagagcttgggggcgaggaagacggaatcgggggcgtaggcgtccgcgccgcagtgggcgcagacggtctcgcactccacgagccaggtgaggtcgggctggtcggggtcaaaaaccagtttcccgccgttctttttgatgcgtttcttacctttggtctccatgagctcgtgtccccgctgggtgacaaagaggctgtccgtgtccccgtagaccgactttatgggccggtcctcgagcggtgtgccgcggtcctcctcgtagaggaaccccgcccactccgagacgaaagcccgggtccaggccagcacgaaggaggccacgtgggacgggtagcggtcgttgtccaccagcgggtccactttttccagggtatgcaaacacatgtccccctcgtccacatccaggaaggtgattggcttgtaagtgtaggccacgtgaccgggggtcccggccgggggggtataaaagggggcgggcccctgctcgtcctcactgtcttccggatcgctgtccaggagcgccagctgttggggtaggtattccctctcgaaggcgggcatgacctcggcactcaggttgtcagtttctagaaacgaggaggatttgatattgacggtgccagcggagatgcctttcaagagcccctcgtccatctggtcagaaaagacgatttttttgttgtcgagcttggtggcgaaggagccgtagagggcgttggaaaggagcttggcgatggagcgcatggtctggtttttttccttgtcggcgcgctccttggccgcgatgttgagctgcacgtactcgcgcgccacgcacttccattcggggaagacggtggtcatctcgtcgggcacgattctgacctgccaacctcgattatgcagggtgatgaggtccacactggtggccacctcgccgcgcaggggctcgttggtccagcagaggcggccgcccttgcgcgagcagaaggggggcagagggtccagcatgacctcgtcgggggggtcggcatcgatggtgaagatgccgggcaggagatcggggtcgaagtagctgatggaagtggccagatcgtccagggaagcttgccattcgcgcacggccagcgcgcgctcgtagggactgaggggcgtgccccagggcatggggtgggtgagcgcggaggcgtacatgccgcagatgtcgtagacgtagaggggctcctcgaggatgccgatgtaggtggggtagcagcgccccccgcggatgctggcgcgcacgtagtcatacagctcgtgcgagggcgcgaggagccccgggcccaggttggtgcgactgggcttttcggcgcggtagacgatctggcgaaagatggcatgcgagttggaggagatggtgggcctttggaagatgttgaagtgggcgtgggggaggccgaccgagtcgcggatgaagtgggcgtaggagtcttgcagtttggcgacgagctcggcggtgacgaggacgtccagagcgcagtagtcgagggtctcctggatgatgtcatacttgagctggcccttttgtttccacagctcgcggttgagaaggaactcttcgcggtccttccagtactcttcgagggggaacccgtcctgatctgcacggtaagagcctagcatgtagaactggttgacggccttgtaggcgcagcagcccttctccacggggagggcgtaggcctgggcggccttgcgcagggaggtgtgcgtgagggcgaaggtgtccctgaccatgaccttgaggaactggtgcttgaaatcgatatcgtcgcagcccccctgctcccagagctggaagtccgtgcgcttcttgtaggcggggttgggcaaagcgaaagtaacatcgttgaaaaggatcttgcccgcgcggggcataaagttgcgagtgatgcggaaaggctggggcacctcggcccggttgttgatgacctgggcggcgagcacgatctcgtcgaaaccgttgatgttgtggcccacgatgtagagttccacgaatcgcgggcggcccttgacgtggggcagcttcttgagctcctcgtaggtgagctcgtcggggtcgctgagaccgtgctgctcgagcgcccagtcggcgagatgggggttggcgcggaggaaggaagtccagagatccacggccagggcggtttgcagacggtcccggtactgacggaactgctgcccgacggccattttttcgggggtgacgcagtagaaggtgcgggggtccccgtgccagcggtcccatttgagctggagggcgagatcgagggcgagctcgacgaggcggtcgtcccctgagagtttcatgaccagcatgaaggggacgagctgcttgccgaaggaccccatccaggtgtaggtttccacatcgtaggtgaggaagagcctttcggtgcgaggatgcgagccgatggggaagaactggatctcctgccaccaattggaggaatggctgttgatgtgatggaagtagaaatgccgacggcgcgccgaacactcgtgcttgtgtttatacaagcggccacagtgctcgcaacgctgcacgggatgcacgtgctgcacgagctgtacctgagttcctttgacgaggaatttcagtgggaagtggagtcgtggcgcctgcatctcgtgctgtactacgtcgtggtggtcggcctggccctcttctgcctcgatggtggtcatgctgacgagcccgcgcgggaggcaggtccagacctcggcgcgagcgggtcggagagcgaggacgagggcgcgcaggccggagctgtccagggtcctgagacgctgcggagtcaggtcagtgggcagcggcggcgcgcggttgacttgcaggagtttttccagggcgcgcgggaggtccagatggtacttgatctccaccgcgccgttggtggcgacgtcgatggcttgcagggtcccgtgcccctggggtgtgaccaccgtcccccgtttcttcttgggcggctggggcgacgggggcggtgcctcttccatggttagaagcggcggcgaggacgcgcgccgggcggcagaggcggctcggggcccggaggcaggggcggcaggggcacgtcggcgccgcgcgcgggtaggttctggtactgcgcccggagaagactggcgtgagcgacgacgcgacggttgacgtcctggatctgacgcctctgggtgaaggccacgggacccgtgagtttgaacctgaaagagagttcgacagaatcaatctcggtatcgttgacggcggcctgccgcaggatctcttgcacgtcgcccgagttgtcctggtaggcgatctcggtcatgaactgctcgatctcctcctcctgaaggtctccgcgaccggcgcgctccacggtggccgcgaggtcgttggagatgcggcccatgagctgcgagaaggcgttcatgcccgcctcgttccagacgcggctgtagaccacgacgccctcgggatcgcgggcgcgcatgaccacctgggcgaggttgagctccacgtggcgcgtgaagaccgcgtagttgcagaggcgctggtagaggtagttgagcgtggtggcgatgtgctcggtgacgaagaaatacatgatccagcggcggagcggcatctcgctgacgtcgcccagcgcctccaagcgttccatggcctcgtaaaagtccacggcgaagttgaaaaactgggagttgcgcgccgagacggtcaactcctcctccagaagacggatgagctcggcgatggtggcgcgcacctcgcgctcgaaggcccccgggagttcctccacttcctcctcttcttcctcctccactaacatctcttctacttcctcctcaggcggtggtggtggcgggggagggggcctgcgtcgccggcggcgcacgggcagacggtcgatgaagcgctcgatggtctcgccgcgccggcgtcgcatggtctcggtgacggcgcgcccgtcctcgcggggccgcagcgtgaagacgccgccgcgcatctccaggtggccgggggggtccccgttgggcagggagagggcgctgacgatgcatcttatcaattgccccgtagggactccgcgcaaggacctgagcgtctcgagatccacgggatctgaaaaccgttgaacgaaggcttcgagccagtcgcagtcgcaaggtaggctgagcacggtttcttctgccgggtcatgttggggagcggggcgggcgatgctgctggtgatgaagttgaaataggcggttctgagacggcggatggtggcgaggagcaccaggtctttgggcccggcttgctggatgcgcagacggtcggccatgccccaggcgtggtcctgacacctggccaggtccttgtagtagtcctgcatgagccgctccacgggcacctcctcctcgcccgcgcggccgtgcatgcgcgtgagcccgaagccgcgctggggctggacgagcgccaggtcggcgacgacgcgctcggcgaggatggcctgctggatctgggtgagggtggtctggaagtcgtcaaagtcgacgaagcggtggtaggctccggtgttgatggtgtaggagcagttggccatgacggaccagttgacggtctggtggcccggacgcacgagctcgtggtacttgaggcgcgagtaggcgcgcgtgtcgaagatgtagtcgttgcaggtgcgcaccaggtactggtagccgatgaggaagtgcggcggcggctggcggtagagcggccatcgctcggtggcgggggcgccgggcgcgaggtcctcgagcatggtgcggtggtagccgtagatgtacctggacatccaggtgatgccggcggcggtggtggaggcgcgcgggaactcgcggacgcggttccagatgttgcgcagcggcaggaagtagttcatggtgggcacggtctggcccgtgaggcgcgcgcagtcgtggatgctctatacgggcaaaaacgaaagcggtcagcggctcgactccgtggcctggaggctaagcgaacgggttgggctgcgcgtgtaccccggttcgaatctcgaatcaggctggagccgcagctaacgtggtactggcactcccgtctcgacccaagcctgcaccaaccctccaggatacggaggcgggtcgttttgcaactttttttggaggccggaaatgaaactagtaagcgcggaaagcggccgaccgcgatggctcgctgccgtagtctggagaagaatcgccagggttgcgttgcggtgtgccccggttcgaggccggccggattccgcggctaacgagggcgtggctgccccgtcgtttccaagaccccatagccagccgacttctccagttacggagcgagcccctcttttgttttgtttgtttttgccagatgcatcccgtactgcggcagatgcgcccccaccaccctccaccgcaacaacagccccctcctccacagccggcgcttctgcccccgccccagcagcagcagcaacttccagccacgaccgccgcggccgccgtgagcggggctggacagacttctcagtatgatcacctggccttggaagagggcgaggggctggcgcgcctgggggcgtcgtcgccggagcggcacccgcgcgtgcagatgaaaagggacgctcgcgaggcctacgtgcccaagcagaacctgttcagagacaggagcggcgaggagcccgaggagatgcgcgcggcccggttccacgcggggcgggagctgcggcgcggcctggaccgaaagagggtgctgagggacgaggatttcgaggcggacgagctgacggggatcagccccgcgcgcgcgcacgtggccgcggccaacctggtcacggcgtacgagcagaccgtgaaggaggagagcaacttccaaaaatccttcaacaaccacgtgcgcaccctgatcgcgcgcgaggaggtgaccctgggcctgatgcacctgtgggacctgctggaggccatcgtgcagaaccccaccagcaagccgctgacggcgcagctgttcctggtggtgcagcatagtcgggacaacgaggcgttcagggaggcgctgctgaatatcaccgagcccgagggccgctggctcctggacctggtgaacattctgcagagcatcgtggtgcaggagcgcgggctgccgctgtccgagaagctggcggccatcaacttctcggtgctgagtctgggcaagtactacgctaggaagatctacaagaccccgtacgtgcccatagacaaggaggtgaagatcgacgggttttacatgcgcatgaccctgaaagtgctgaccctgagcgacgatctgggggtgtaccgcaacgacaggatgcaccgcgcggtgagcgccagcaggcggcgcgagctgagcgaccaggagctgatgcacagcctgcagcgggccctgaccggggccgggaccgagggggagagctactttgacatgggcgcggacctgcactggcagcccagccgccgggccttggaggcggcaggcggtcccccctacatagaagaggtggacgatgaggtggacgaggagggcgagtacctggaagactgatggcgcgaccgtatttttgctagatgcaacaacagccacctcctgatcccgcgatgcgggcggcgctgcagagccagccgtccggcattaactcctcggacgattggacccaggccatgcaacgcatcatggcgctgacgacccgcaaccccgaagcctttagacagcagccccaggccaaccggctctcggccatcctggaggccgtggtgccctcgcgctccaaccccacgcacgagaaggtcctggccatcgtgaacgcgctggtggagaacaaggccatccgcggcgacgaggccggcctggtgtacaacgcgctgctggagcgcgtggcccgctacaacagcaccaacgtgcagaccaacctggaccgcatggtgaccgacgtgcgcgaggccgtggcccagcgcgagcggttccaccgcgagtccaacctgggatccatggtggcgctgaacgccttcctcagcacccagcccgccaacgtgccccggggccaggaggactacaccaacttcatcagcgccctgcgcctgatggtgaccgaggtgccccagagcgaggtgtaccagtccgggccggactacttcttccagaccagtcgccagggcttgcagaccgtgaacctgagccaggcgttcaagaacttgcagggcctgtggggcgtgcaggccccggtcggggaccgcgcgacggtgtcgagcctgctgacgccgaactcgcgcctgctgctgctgctggtggcccccttcacggacagcggcagcatcaaccgcaactcgtacctgggctacctgattaacctgtaccgcgaggccatcggccaggcgcacgtggacgagcagacctaccaggagatcacccacgtgagccgcgccctgggccaggacgacccgggcaatctggaagccaccctgaactttttgctgaccaaccggtcgcagaagatcccgccccagtacacgctcagcgccgaggaggagcgcatcctgcgatacgtgcagcagagcgtgggcctgttcctgatgcaggagggggccacccccagcgccgcgctcgacatgaccgcgcgcaacatggagcccagcatgtacgccagcaaccgcccgttcatcaataaactgatggactacttgcatcgggcggccgccatgaactctgactatttcaccaacgccatcctgaatccccactggctcccgccgccggggttctacacgggcgagtacgacatgcccgaccccaatgacgggttcctgtgggacgatgtggacagcagcgtgttctccccccgaccgggtgctaacgagcgccccttgtggaagaaggaaggcagcgaccgacgcccgtcctcggcgctgtccggccgcgagggtgctgccgcggcggtgcccgaggccgccagtcctttcccgagcttgcccttctcgctgaacagtattcgcagcagcgagctgggcaggatcacgcgcccgcgcttgctgggcgaggaggagtacttgaatgactcgctgttgagacccgagcgggagaagaacttccccaataacgggatagagagcctggtggacaagatgagccgctggaagacgtatgcgcaggagcacagggacgatccgtcgcagggggccacgagccggggcagcgccgcccgtaaacgccggtggcacgacaggcagcggggactgatgtgggacgatgaggattccgccgacgacagcagcgtgttggacttgggtgggagtggtaacccgttcgctcacctgcgcccccgcatcgggcgcatgatgtaagagaaaccgaaaataaatgatactcaccaaggccatggcgaccagcgtgcgttcgtttcttctctgttgttgtatctagtatgatgaggcgtgcgtacccggagggtcctcctccctcgtacgagagcgtgatgcagcaggcgatggcggcggcggcggcgatgcagcccccgctggaggctccttacgtgcccccgcggtacctggcgcctacggaggggcggaacagcattcgttactcggagctggcacccttgtacgataccacccggttgtacctggtggacaacaagtcggcggacatcgcctcgctgaactaccagaacgaccacagcaacttcctgaccaccgtggtgcagaacaatgacttcacccccacggaggccagcacccagaccatcaactttgacgagcgctcgcggtggggcggtcagctgaaaaccatcatgcacaccaacatgcccaacgtgaacgagttcatgtacagcaacaagttcaaggcgcgggtgatggtctcccgcaagacccccaacggggtgacagtgacagatggtagtcaggatatcttggagtatgaatgggtggagtttgagctgcccgaaggcaacttctcggtgaccatgaccatcgacctgatgaacaacgccatcatcgacaattacttggcggtggggcggcagaacggggtcctggagagcgatatcggcgtgaagttcgacactaggaacttcaggctgggctgggaccccgtgaccgagctggtcatgcccggggtgtacaccaacgaggccttccaccccgatattgtcttgctgcccggctgcggggtggacttcaccgagagccgcctcagcaacctgctgggcattcgcaagaggcagcccttccaggagggcttccagatcatgtacgaggatctggaggggggcaacatccccgcgctcctggatgtcgacgcctatgagaaaagcaaggaggagagcgccgccgcggcgactgcagctgtagccaccgcctctaccgaggtcaggggcgataattttgccagccctgcagcagtggcagcggccgaggcggctgaaaccgaaagtaagatagtcattcagccggtggagaaggatagcaaggacaggagctacaacgtgctgccggacaagataaacaccgcctaccgcagctggtacctggcctacaactatggcgaccccgagaagggcgtgcgctcctggacgctgctcaccacctcggacgtcacctgcggcgtggagcaagtctactggtcgctgcccgacatgatgcaagacccggtcaccttccgctccacgcgtcaagttagcaactacccggtggtgggcgccgagctcctgcccgtctactccaagagcttcttcaacgagcaggccgtctactcgcagcagctgcgcgccttcacctcgctcacgcacgtcttcaaccgcttccccgagaaccagatcctcgtccgcccgcccgcgcccaccattaccaccgtcagtgaaaacgttcctgctctcacagatcacgggaccctgccgctgcgcagcagtatccggggagtccagcgcgtgaccgttactgacgccagacgccgcacctgcccctacgtctacaaggccctgggcatagtcgcgccgcgcgtcctctcgagccgcaccttctaaaaaatgtccattctcatctcgcccagtaataacaccggttggggcctgcgcgcgcccagcaagatgtacggaggcgctcgccaacgctccacgcaacaccccgtgcgcgtgcgcgggcacttccgcgctccctggggcgccctcaagggccgcgtgcggtcgcgcaccaccgtcgacgacgtgatcgaccaggtggtggccgacgcgcgcaactacacccccgccgccgcgcccgtctccaccgtggacgccgtcatcgacagcgtggtggccgacgcgcgccggtacgcccgcgccaagagccggcggcggcgcatcgcccggcggcaccggagcacccccgccatgcgcgcggcgcgagccttgctgcgcagggccaggcgcacgggacgcagggccatgctcagggcggccagacgcgcggcttcaggcgccagcgccggcaggacccggagacgcgcggccacggcggcggcagcggccatcgccagcatgtcccgcccgcggcgagggaacgtgtactgggtgcgcgacgccgccaccggtgtgcgcgtgcccgtgcgcacccgcccccctcgcacttgaagatgttcacttcgcgatgttgatgtgtcccagcggcgaggaggatgtccaagcgcaaattcaaggaagagatgctccaggtcatcgcgcctgagatctacggccccgcggtggtgaaggaggaaagaaagccccgcaaaatcaagcgggtcaaaaaggacaaaaaggaagaagatgacgatctggtggagtttgtgcgcgagttcgccccccggcggcgcgtgcagtggcgcgggcggaaagtgcacccggtgctgagacccggcaccaccgtggtcttcacgcccggcgagcgctccggcagcgcttccaagcgctcctacgacgaggtgtacggggacgaggacatcctcgagcaggcggccgagcgcctgggcgagtttgcttacggcaagcgcagccgccccgccctgaaggaagaggcggtgtccatcccgctggaccacggcaaccccacgccgagcctcaagcccgtgaccctgcagcaggtgctgccgagcgcagcgccgcgccgggggttcaagcgcgagggcgaggatctgtaccccaccatgcagctgatggtgcccaagcgccagaagctggaagacgtgctggagaccatgaaggtggacccggacgtgcagcccgaggtcaaggtgcggcccatcaagcaggtggccccgggcctgggcgtgcagaccgtggacatcaagatccccacggagcccatggaaacgcagaccgagcccatgatcaagcccagcaccagcaccatggaggtgcagacggatccctggatgccatcggctcctagccgaagaccccggcgcaagtacggcgcggccagcctgctgatgcccaactacgcgctgcatccttccatcatccccacgccgggctaccgcggcacgcgcttctaccgcggtcatacaaccagccgccgccgcaagaccaccacccgccgccgccgtcgccgcacagccgctgcatctacccctgccgccctggtgcggagagtgtaccgccgcggccgcgcgcctctgaccctaccgcgcgcgcgctaccacccgagcatcgccatttaaactttcgcctgctttgcagatggccctcacatgccgcctccgcgttcccattacgggctaccgaggaagaaaaccgcgccgtagaaggctggcggggaacgggatgcgtcgccaccaccatcggcggcggcgcgccatcagcaagcggttggggggaggcttcctgcccgcgctgatccccatcatcgccgcggcgatcggggcgatccccggcattgcttccgtggcggtgcaggcctctcagcgccactgagacacttggaaaacatcttgtaataaaccaatggactctgacgctcctggtcctgtgatgtgttttcgtagacagatggaagacatcaatttttcgtccctggctccgcgacacggcacgcggccgttcatgggcacctggagcgacatcggcaccagccaactgaacgggggcgccttcaattggagcagtctctggagcgggcttaagaatttcgggtccacgcttaaaacctatggcagcaaggcgtggaacagcaccacagggcaggcgctgagggataagctgaaagagcagaacttccagcagaaggtggtcgatgggctcgcctcgggcatcaacggggtggtggacctggccaaccaggccgtgcagcggcagatcaacagccgcctggacccggtgccgcccgccggctccgtggagatgccgcaggtggaggaggagctgcctcccctggacaagcggggcgagaagcgaccccgccccgacgcggaggagacgctgctgacgcacacggacgagccgcccccgtacgaggaggcggtgaaactgggtctgcccaccacgcggcccatcgcgcccctggccaccggggtgctgaaacccgaaagtaataagcccgcgaccctggacttgcctcctcccgcttcccgcccctctacagtggctaagcccctgccgccggtggccgtggcccgcgcgcgacccgggggctccgcccgccctcatgcgaactggcagagcactctgaacagcatcgtgggtctgggagtgcagagtgtgaagcgccgccgctgctattaaacctaccgtagcgcttaacttgcttgtctgtgtgtgtatgtattatgtcgccgctgtccgccagaaggaggagtgaagaggcgcgtcgccgagttgcaagatggccaccccatcgatgctgccccagtgggcgtacatgcacatcgccggacaggacgcttcggagtacctgagtccgggtctggtgcagttcgcccgcgccacagacacctacttcagtctggggaacaagtttaggaaccccacggtggcgcccacgcacgatgtgaccaccgaccgcagccagcggctgacgctgcgcttcgtgcccgtggaccgcgaggacaacacctactcgtacaaagtgcgctacacgctggccgtgggcgacaaccgcgtgctggacatggccagcacctactttgacatccgcggcgtgctggatcggggccctagcttcaaaccctactccggcaccgcctacaacagcctggctcccaagggagcgcccaattccagccagtgggagcaaaaaaaggcaggcaatggtgacactatggaaacacacacatttggtgtggccccaatgggcggtgagaatattacaatcgacggattacaaattggaactgacgctacagctgatcaggataaaccaatttatgctgacaaaacattccagcctgaacctcaagtaggagaagaaaattggcaagaaactgaaagcttttatggcggtagggctcttaaaaaagacacaagcatgaaaccttgctatggctcctatgctagacccaccaatgtaaagggaggtcaagctaaacttaaagttggagctgatggagttcctaccaaagaatttgacatagacctggctttctttgatactcccggtggcacagtgaatggacaagatgagtataaagcagacattgtcatgtataccgaaaacacgtatctggaaactccagacacgcatgtggtatacaaaccaggcaaggatgatgcaagttctgaaattaacctggttcagcagtccatgcccaatagacccaactatattgggttcagagacaactttattgggctcatgtattacaacagtactggcaatatgggggtgctggctggtcaggcctcacagctgaatgctgtggtcgacttgcaagacagaaacaccgagctgtcataccagctcttgcttgactctttgggtgacagaacccggtatttcagtatgtggaatcaggcggtggacagttatgatcctgatgtgcgcattattgaaaaccatggtgtggaagacgaacttcccaactattgcttccccctggatgggtctggcactaatgccgcttaccaaggtgtgaaagtaaaaaatggtaacgatggtgatgttgagagcgaatgggaaaatgatgatactgtcgcagctcgaaatcaattatgcaagggcaacatttttgccatggaaattaacctccaagccaacctgtggagaagtttcctctactcgaacgtggccctgtacctgcccgactcttacaagtacacgccagccaacatcaccctgcccaccaacaccaacacttatgattacatgaacgggagagtggtgcctccctcgctggtggacgcctacatcaacatcggggcgcgctggtcgctggaccccatggacaacgtcaatcccttcaaccaccaccgcaacgcgggcctgcgctaccgctccatgctcctgggcaacgggcgctacgtgcccttccacatccaggtgccccagaaatttttcgccatcaagagcctcctgctcctgcccgggtcctacacctacgagtggaacttccgcaaggacgtcaacatgatcctgcagagctccctcggcaacgacctgcgcacggacggggcctccatctccttcaccagcatcaacctctacgccaccttcttccccatggcgcacaacacggcctccacgctcgaggccatgctgcgcaacgacaccaacgaccagtccttcaacgactacctctcggcggccaacatgctctaccccatcccggccaacgccaccaacgtgcccatctccatcccctcgcgcaactgggccgccttccgcggctggtccttcacgcgcctcaagaccaaggagacgccctcgctgggctccgggttcgacccctacttcgtctactcgggctccatcccctacctcgacggcaccttctacctcaaccacaccttcaagaaggtctccatcaccttcgactcctccgtcagctggcccggcaacgaccggctcctgacgcccaacgagttcgaaatcaagcgcaccgtcgacggcgagggatacaacgtggcccagtgcaacatgaccaaggactggttcctggtccagatgctggcccactacaacatcggctaccagggcttctacgtgcccgagggctacaaggaccgcatgtactccttcttccgcaacttccagcccatgagccgccaggtggtggacgaggtcaactacaaggactaccaggccgtcaccctggcctaccagcacaacaactcgggcttcgtcggctacctcgcgcccaccatgcgccagggccagccctaccccgccaactacccgtacccgctcatcggcaagagcgccgtcaccagcgtcacccagaaaaagttcctctgcgacagggtcatgtggcgcatccccttctccagcaacttcatgtccatgggcgcgctcaccgacctcggccagaacatgctctatgccaactccgcccacgcgctagacatgaatttcgaagtcgaccccatggatgagtccacccttctctatgttgtcttcgaagtcttcgacgtcgtccgagtgcaccagccccaccgcggcgtcatcgaggccgtctacctgcgcacccccttctcggccggtaacgccaccacctaaattgctacttgcatgatggctgagcccacaggctccggcgagcaggagctcagggccatcatccgcgacctgggctgcgggccctacttcctgggcaccttcgataagcgcttcccgggattcatggccccgcacaagctggcctgcgccatcgtcaacacggccggccgcgagaccgggggcgagcactggctggccttcgcctggaacccgcgctcgaacacctgctacctcttcgaccccttcgggttctcggacgagcgcctcaagcagatctaccagttcgagtacgagggcctgctgcgccgtagcgccctggccaccgaggaccgctgcgtcaccctggaaaagtccacccagaccgtgcagggtccgcgctcggccgcctgcgggctcttctgctgcatgttcctgcacgccttcgtgcactggcccgaccgccccatggacaagaaccccaccatgaacttgctgacgggggtgcccaacggcatgctccagtcgccccaggtggaacccaccctgcgccgcaaccaggaggcgctctaccgcttcctcaactcccactccgcctactttcgctcccaccgcgcgcgcatcgagaaggccaccgccttcgaccgcatgaacaatcaagacatgtaaaccgtgtgtgtatgtttaaaatatcttttaataaacagcactttaatgttacacatgcatctgagatgattttattttagaaatcgaaagggttctgccgggtctcggcatggcccgcgggcagggacacgttgcggaactggtacttggccagccacttgaactcggggatcagcagtttgggcagcggggtgtcggggaaggagtcggtccacagcttccgcgtcagctgcagggcgcccagcaggtcgggcgcggagatcttgaaatcgcagttgggacccgcgttctgcgcgcgagagttgcggtacacggggttgcagcactggaacaccatcagggccgggtgcttcacgctcgccagcaccgccgcgtcggtgatgctctccacgtcgaggtcctcggcgttggccatcccgaagggggtcatcttgcaggtctgccttcccatggtgggcacgcacccgggcttgtggttgcaatcgcagtgcagggggatcagcatcatctgggcctggtcggcgttcatccccgggtacatggccttcatgaaagcctccaattgcctgaacgcctgctgggccttggctccctcggtgaagaagaccccgcaggacttgctagagaactggttggtggcacagccggcatcgtgcacgcagcagcgcgcgtcgttgttggccagctgcaccacgctgcgcccccagcggttctgggtgatcttggcccggtcggggttctccttcagcgcgcgctgcccgttctcgctcgccacatccatctcgatcatgtgctccttctggatcatggtggtcccgtgcaggcaccgcagtttgccctcggcctcggtgcacccgtgcagccacagcgcgcacccggtgcactcccagttcttgtgggcgatctgggaatgcgcgtgcacgaacccttgcaggaagcggcccatcatggtcgtcagggtcttgttgctagtgaaggtcaacgggatgccgcggtgctcctcgttgatgtacaggtggcagatgcggcggtacacctcgccctgctcgggcatcagttggaagttggctttcaggtcggtctccacgcggtagcggtccatcagcatagtcatgatttccatgcccttctcccaggccgagacgatgggcaggctcatagggttcttcaccatcatcttagcactagcagccgcggccagggggtcgctctcatccagggtctcaaagctccgcttgccgtccttctcggtgatccgcaccggggggtagctgaagcccacggccgccagctcctcctcggcctgtctttcgtcctcgctgtcctggctgacgtcctgcatgaccacatgcttggtcttgcggggtttcttcttgggcggcagtggcggcggagatgcttgtggcgagggggagcgcgagttctcgctcaccactactatctcttcctcttcttggtccgaggccacgcggcggtaggtatgtctcttcgggggcagaggcggaggcgacgggctctcgccgccgcgacttggcggatggctggcagagccccttccgcgttcgggggtgcgctcccggcggcgctctgactgacttcctccgcggccggccattgtgttctcctagggaggaacaacaagcatggagactcagccatcgccaacctcgccatctgcccccaccgccggcgacgagaagcagcagcagcagaatgaaagcttaaccgccccgccgcccagccccgcctccgacgcagccgcggtcccagacatgcaagagatggaggaatccatcgagattgacctgggctatgtgacgcccgcggagcatgaggaggagctggcagtgcgctttcaatcgtcaagccaggaagataaagaacagccagagcaggaagcagagaacgagcagagtcaggctgggctcgagcatggcgactacctccacctgagcggggaggaggacgcgctcatcaagcatctggcccggcaggccaccatcgtcaaggacgcgctgctcgaccgcaccgaggtgcccctcagcgtggaggagctcagccgcgcctacgagctcaacctcttctcgccgcgcgtgccccccaagcgccagcccaacggcacctgcgagcccaacccccgcctcaacttctacccggtcttcgcggtgcccgaggccctggccacctaccacatctttttcaagaaccaaaagatccccgtctcctgccgcgccaaccgcacccgcgccgacgccctcttcaacctgggtcccggcgcccgcctacctgatatcgcctccttggaagaggttcccaagatcttcgagggtctgggcagcgacgagactcgggccgcgaacgctctgcaaggagaaggaggaggagagcatgagcaccacagcgccctggtcgagttggaaggcgacaacgcgcggctggcggtgctcaaacgcacggtcgagctgacccatttcgcctacccggctctgaacctgcccccgaaagtcatgagcgcggtcatggaccaggtgctcatcaagcgcgcgtcgcccatctccgaggacgagggcatgcaagactccgaggagggcaagcccgtggtcagcgacgagcagctggcccggtggctgggtcctaatgctacccctcaaagtttggaagagcggcgcaagctcatgatggccgtggtcctggtgaccgtggagctggagtgcctgcgccgcttcttcgccgacgcggagaccctgcgcaaggtcgaggagaacctgcactacctcttcaggcacgggttcgtgcgccaggcctgcaagatctccaacgtggagctgaccaacctggtctcctacatgggcatcttgcacgagaaccgcctggggcagaacgtgctgcacaccaccctgcgcggggaggcccgccgcgactacatccgcgactgcgtctacctctacctctgccacacctggcagacgggcatgggcgtgtggcagcagtgtctggaggagcagaacctgaaagagctctgcaagctcctgcaaaagaacctcaagggtctgtggaccgggttcgacgagcggaccaccgcctcggacctggccgacctcatcttccccgagcgcctcaggctgacgctgcgcaacggcctgcccgactttatgagccaaagcatgttgcaaaactttcgctctttcatcctcgaacgctccggaatcctgcccgccacctgctccgcgctgccctcggacttcgtgccgctgaccttccgcgagtgccccccgccgctgtggagccactgctacctgctgcgcctggccaactacctggcctaccactcggacgtgatcgaggacgtcagcggcgagggcctgctcgagtgccactgccgctgcaacctctgcacgccgcaccgctccctggcctgcaacccccagctgctgagcgagacccagatcatcggcaccttcgagttgcaagggcccagcgagggcgagggagccaaggggggtctgaaactcaccccggggctgtggacctcggcctacttgcgcaagttcgtgcccgaggattaccatcccttcgagatcaggttctacgaggaccaatcccagccgcccaaggccgagctgtcggcctgcgtcatcacccagggggcgatcctggcccaattgcaagccatccagaaatcccgccaagaattcttgctgaaaaagggccgcggggtctacctcgacccccagaccggtgaggagctcaaccccggcttcccccaggatgccccgaggaaacaagaagctgaaagtggagctgccgcccgtggaggatttggaggaagactgggagaacagcagtcaggcagaggagatggaggaagactgggacagcactcaggcagaggaggacagcctgcaagacagtctggaggaagacgaggaggaggcagaggaggaggtggaagaagcagccgccgccagaccgtcgtcctcggcgggggagaaagcaagcagcacggataccatctccgctccgggtcggggtcccgctcggccccacagtagatgggacgagaccgggcgattcccgaaccccaccacccagaccggtaagaaggagcggcagggatacaagtcctggcgggggcacaaaaacgccatcgtctcctgcttgcaggcctgcgggggcaacatctccttcacccggcgctacctgctcttccaccgcggggtgaacttcccccgcaacatcttgcattactaccgtcacctccacagcccctactacttccaagaagaggcagcagcagcagaaaaagaccagaaaaccagctagaaaatccacagcggcggcagcggcaggtggactgaggatcgcggcgaacgagccggcgcagacccgggagctgaggaaccggatctttcccaccctctatgccatcttccagcagagtcgggggcaggagcaggaactgaaagtcaagaaccgttctctgcgctcgctcacccgcagttgtctgtatcacaagagcgaagaccaacttcagcgcactctcgaggacgccgaggctctcttcaacaagtactgcgcgctcactcttaaagagtagcccgcgcccgcccagtcgcagaaaaaggcgggaattacgtcacctgtgcccttcgccctagccgcctccacccagcaccgccatgagcaaagagattcccacgccttacatgtggagctaccagccccagatgggcctggccgccggcgccgcccaggactactccacccgcatgaattggctcagcgccgggcccgcgatgatctcacgggtgaatgacatccgcgcccaccgaaaccagatactcctagaacagtcagcgctcaccgccacgccccgcaatcacctcaatccgcgtaattggcccgccgccctggtgtaccaggaaattccccagcccacgaccgtactacttccgcgagacgcccaggccgaagtccagctgactaactcaggtgtccagctggcgggcggcgccaccctgtgtcgtcaccgccccgctcagggtataaagcggctggtgatccggggcagaggcacacagctcaacgacgaggtggtgagctcttcgctgggtctgcgacctgacggagtcttccaactcgccggatcggggagatcttccttcacgcctcgtcaggcggtcctgactttggagagttcgtcctcgcagccccgctcgggcggcatcggcactctccagttcgtggaggagttcactccctcggtctacttcaaccccttctccggctcccccggccactacccggacgagttcatcccgaactttgacgccatcagcgagtcggtggacggctacgattgattaattaatcaactaaccccttacccctttaccctccagtaaaaataaagattaaaaatgattgaattgatcaataaagaatcacttacttgaaatctgaaaccaggtctctgtccatgttttctgtcagcagcacttcactcccctcttcccaactctggtactgcaggccccggcgggctgcaaacttcctccacactctgaaggggatgtcaaattcctcctgtccctcaatcttcatttttatcttctatcagatgtccaaaaagcgcgcgcgggtggatgatggcttcgaccccgtgtacccctacgatgcagacaacgcaccgactgtgcccttcatcaaccctcccttcgtctcttcagatggattccaagaaaagcccctgggggtgttgtccctgcgactggccgaccccgtcaccaccaagaatggggctgtcaccctcaagctgggggagggggtggacctcgacgactcgggaaaactcatctccaaaaatgccaccaaggccactgcccctctcagtatttccaacggcaccatttcccttaacatggctgcccctttttacaacaacaatggaacgttaagtctcaatgtttctacaccattagcagtatttcccacttttaacactttaggtatcagtcttggaaacggtcttcaaacttctaataagttgctgactgtacagttaactcatcctcttacattcagctcaaatagcatcacagtaaaaacagacaaaggactctatattaattctagtggaaacagagggcttgaggctaacataagcctaaaaagaggactgatttttgatggtaatgctattgcaacataccttggaagtggtttagactatggatcctatgatagcgatgggaaaacaagacccatcatcaccaaaattggagcaggtttgaattttgatgctaataatgccatggctgtgaagctaggcacaggtttaagttttgactctgccggtgccttaacagctggaaacaaagaggatgacaagctaacactttggactacacctgacccaagccctaattgtcaattactttcagacagagatgccaaatttaccctatgtcttacaaaatgcggtagtcaaatactaggcactgttgcagtagctgctgttactgtaggttcagcactaaatccaattaatgacacagtaaaaagcgccatagtattccttagatttgactctgacggtgtgctcatgtcaaactcatcaatggtaggtgattactggaactttagggaaggacagaccacccaaagtgtggcctatacaaatgctgtgggattcatgcccaatctaggtgcatatcctaaaacccaaagcaaaacaccaaaaaatagtatagtaagtcaggtatatttaaatggagaaactactatgccaatgacactgacaataactttcaatggcactgatgaaaaagacacaacacctgtgagcacttactccatgacttttacatggcagtggactggagactataaggacaagaatattacctttgctaccaactcctttactttctcctacatggcccaagaataaaccctgcatgccaaccccattgttcccaccactatggaaaactctgaagcagaaaaaaataaagttcaagtgttttattgattcaacagttttctcacagaaccctagtattcaacctgccacctccctcccaacacacagagtacacagtcctttctccccggctggccttaaaaagcatcatatcatgggtaacagacatattcttaggtgttatattccacacggtttcctgtcgagccaaacgctcatcagtgatattaataaactccccgggcagctcacttaagttcatgtcgctgtccagctgctgagccacaggctgctgtccaacttgcggttgcttaacgggcggcgaaggagaagtccacgcctacatgggggtagagtcataatcgtgcatcaggatagggcggtggtgctgcagcagcgcgcgaataaactgctgccgccgccgctccgtcctgcaggaatacaacatggcagtggtctcctcagcgatgattcgcaccgcccgcagcataaggcgccttgtcctccgggcacagcagcgcaccctgatctcacttaaatcagcacagtaactgcagcacagcaccacaatattgttcaaaatcccacagtgcaaggcgctgtatccaaagctcatggcggggaccacagaacccacgtggccatcataccacaagcgcaggtagattaagtggcgacccctcataaacacgctggacataaacattacctcttttggcatgttgtaattcaccacctcccggtaccatataaacctctgattaaacatggcgccatccaccaccatcctaaaccagctggccaaaacctgcccgccggctatacactgcagggaaccgggactggaacaatgacagtggagagcccaggactcgtaaccatggatcatcatgctcgtcatgatatcaatgttggcacaacacaggcacacgtgcatacacttcctcaggattacaagctcctcccgcgttagaaccatatcccagggaacaacccattcctgaatcagcgtaaatcccacactgcagggaagacctcgcacgtaactcacgttgtgcattgtcaaagtgttacattcgggcagcagcggatgatcctccagtatggtagcgcgggtttctgtctcaaaaggaggtagacgatccctactgtacggagtgcgccgagacaaccgagatcgtgttggtcgtagtgtcatgccaaatggaacgccggacgtagtcatatttcctgaagcaaaaccaggtgcgggcgtgacaaacagatctgcgtctccggtctcgccgcttagatcgctctgtgtagtagttgtagtatatccactctctcaaagcatccaggcgccccctggcttcgggttctatgtaaactccttcatgcgccgctgccctgataacatccaccaccgcagaataagccacacccagccaacctacacattcgttctgcgagtcacacacgggaggagcgggaagagctggaagaaccatgattaactttattccaaacggtctcggagcacttcaaaatgcaggtcccggaggtggcacctctcgcccccactgtgttggtggaaaataacagccaggtcaaaggtgacacggttctcgagatgttccacggtggcttccagcaaagcctccacgcgcacatccagaaacaagaggacagcgaaagcgggagcgttttctaattcctcaatcatcatattacactcctgcaccatccccagataattttcatttttccagccttgaatgattcgtattagttcctgaggtaaatccaagccagccatgataaaaagctcgcgcagagcgccctccaccggcattcttaagcacaccctcataattccaagagattctgctcctggttcacctgcagcagattaacaatgggaatatcaaaatctctgccgcgatccctaagctcctccctcaacaataactgtatgtaatctttcatatcatctccgaaatttttagccatagggccgccaggaataagagcagggcaagccacattacagataaagcgaagtcctccccagtgwgcattgccaaatgtaagattgaaataagcatgctggctagaccctgtgatatcttccagataactggacagaaaatcaggcaagcaatttttaagaaaatcaacaaaagaaaagtcgtccaggtgcaggtttagagcctcaggaacaacgatggaataagtgcaaggagtgcgttccagcatggttagtgtttttttggtgatctgtagaacaaaaaataaacatgcaatattaaaccatgctagcctggcgaacaggtgggtaaatcactctttccagcaccaggcaggctacggggtctccggcgcgaccctcgtagaagctgtcgccatgattgaaaagcatcaccgagagaccttcccggtggccggcatggatgattcgagaagaagcatacactccgggaacattggcatccgtgagtgaaaaaaagcgacctataaagcctcggggcactacaatgctcaatctcaattccagcaaagccaccccatgcggatggagcacaaaattggcaggtgcgtaaaaaatgtaattactcccctcctgcacaggcagcaaagcccccgctccctccagaaacacatacaaagcctcagcgtccatagcttaccgagcacggcaggcgcaagagtcagagaaaaggctgagctctaacctgactgcccgctcctgtgctcaatatatagccctaacctacactgacgtaaaggccaaagtctaaaaatacccgccaaaatgacacacacgcccagcacacgcccagaaaccggtgacacactcaaaaaaatacgtgcgcttcctcaaacgcccaaaccggcgtcatttccgggttcccacgctacgtcaccgctcagcgactttcaaattccgtcgaccgttaaaaacgtcactcgccccgcccctaacggtcgcccttctctcggccaatcaccttcctcccttcccaaattcaaacgcctcatttgcatattaacgcgcacaaaaagtttgaggtatatatttgaatgatggtttaaacgcggccgccaggcctacccactagtcaattcgggaggatcgaaacggcagatcgcaaaaaacagtacatacagaaggagacatgaacatgaacatcaaaaaaattgtaaaacaagccacagttctgacttttacgactgcacttctggcaggaggagcgactcaagccttcgcgaaagaaaataaccaaaaagcatacaaagaaacgtacggcgtctctcatattacacgccatgatatgctgcagatccctaaacagcagcaaaacgaaaaataccaagtgcctcaattcgatcaatcaacgattaaaaataattgagtctgacaaaaggacttgatgtg

SEQ ID NO: 41 - DNA, 2661 bp, Artificial Sequence
  Vector
ttaattaaccatcttcaataatatacctcaaactttttgtgcgcgttaatatgcaaatgaggcgtttgaatttggggaggaagggcggtgattggtcgagggatgagcgaccgttaggggcggggcgagtgacgttttgatgacgtggttgcgaggaggagccagtttgcaagttctcgtgggaaaagtgacgtcaaacgaggtgtggtttgaacacggaaatactcaattttcccgcgctctctgacaggaaatgaggtgtttctgggcggatgcaagtgaaaacgggccattttcgcgcgaaaactgaatgaggaagtgaaaatctgagtaatttcgcgtttatggcagggaggagtatttgccgagggccgagtagactttgaccgattacgtgggggtttcgattaccgtgtttttcacctaaatttccgcgtacggtgtcaaagtccggtgtttttacgcgatcgctagcgacatcgatcacaagtttgtacaaaaaagcaggctccaccatgggaacccgcgttttgagatttctgtcgccgactaaattcatgtcgcgcgatagtggtgtttatcgccgatagagatggcgatattggaaaaatcgatatttgaaaatatggcatattgaaaatgtcgccgatgtgagtttctgtgtaactgatatcgccatttttccaaaagtgatttttgggcatacgcgatatctggcgatagcgcttatatcgtttacgggggatggcgatagacgactttggtgacttgggcgattctgtgtgtcgcaaatatcgcagtttcgatataggtgacagacgatatgaggctatatcgccgatagaggcgacatcaagctggcacatggccaatgcatatcgatctatacattgaatcaatattggccattagccatattattcattggttatatagcataaatcaatattggctattggccattgcatacgttgtatccatatcataatatgtacatttatattggctcatgtccaacattaccgccatgttgacattgattattgactagttattaatagtaatcaattacggggtcattagttcatagcccatatatggagttccgcgttacataacttacggtaaatggcccgcctggctgaccgcccaacgacccccgcccattgacgtcaataatgacgtatgttcccatagtaacgccaatagggactttccattgacgtcaatgggtggagtatttacggtaaactgcccacttggcagtacatcaagtgtatcatatgccaagtacgccccctattgacgtcaatgacggtaaatggcccgcctggcattatgcccagtacatgaccttatgggactttcctacttggcagtacatctacgtattagtcatcgctattaccatggtgatgcggttttggcagtacatcaatgggcgtggatagcggtttgactcacggggatttccaagtctccaccccattgacgtcaatgggagtttgttttggcaccaaaatcaacgggactttccaaaatgtcgtaacaactccgccccattgacgcaaatgggcggtaggcgtgtacggtgggaggtctatataagcagagctctccctatcagtgatagagatctccctatcagtgatagagatcgtcgacgagctcgtttagtgaaccgtcagatcgcctggagacgccatccacgctgttttgacctccatagaagacaccgggaccgatccagcctccgcggccgggaacggtgcattggaacgcggattccccgtgccaagagtgacgtaagtaccgcctatagagtctataggcccacccccttggcttcttatgcatgctatactgtttttggcttggggtctatacacccccgcttcctcatgttataggtgatggtatagcttagcctataggtgtgggttattgaccattattgaccactcccctattggtgacgatactttccattactaatccataacatggctctttgccacaactctctttattggctatatgccaatacactgtccttcagagactgacacggactctgtatttttacaggatggggtctcatttattatttacaaattcacatatacaacaccaccgtccccagtgcccgcagtttttattaaacataacgtgggatctccacgcgaatctcgggtacgtgttccggacatgggctcttctccggtagcggcggagcttctacatccgagccctgctcccatgcctccagcgactcatggtcgctcggcagctccttgctcctaacagtggaggccagacttaggcacagcacgatgcccaccaccaccagtgtgccgcacaaggccgtggcggtagggtatgtgtctgaaaatgagctcggggagcgggcttgcaccgctgacgcatttggaagacttaaggcagcggcagaagaagatgcaggcagctgagttgttgtgttctgataagagtcagaggtaactcccgttgcggtgctgttaacggtggagggcagtgtagtctgagcagtactcgttgctgccgcgcgcgccaccagacataatagctgacagactaacagactgttcctttccatgggtcttttctgcagtcaccgtccttgacacgaagcttggtacc

SEQ ID NO: 42 - DNA, 37490 bp, Artificial Sequence
  Vector
gcggccgctcgagcatgcatctagagggccctattctatagtgtcacctaaatgctagagctcgctgatcagcctcgactgtgccttctagttgccagccatctgttgtttgcccctcccccgtgccttccttgaccctggaaggtgccactcccactgtcctttcctaataaaatgaggaaattgcatcgcattgtctgagtaggtgtcattctattctggggggtggggtggggcaggacagcaagggggaggattgggaagacaatagcaggcatgctggggatgcggtgggctctatggcttctgaggcggaaagaaccagctggggctcgaggggggatcgatcccgtcgagatatctagacccagctttcttgtacaaagtggtgatcgattcgacagatcgcgatcgcaagtgagtagtgttctggggcgggggaggacctgcatgagggccagaataactgaaatctgtgcttttctgtgtgttgcagcagcatgagcggaagcggctcctttgagggaggggtattcagcccttatctgacggggcgtctcccctcctgggcgggagtgcgtcagaatgtgatgggatccacggtggacggccggcccgtgcagcccgcgaactcttcaaccctgacctatgcaaccctgagctcttcgtcgttggacgcagctgccgccgcagctgctgcatctgccgccagcgccgtgcgcggaatggccatgggcgccggctactacggcactctggtggccaactcgagttccaccaataatcccgccagcctgaacgaggagaagctgttgctgctgatggcccagctcgaggccttgacccagcgcctgggcgagctgacccagcaggtggctcagctgcaggagcagacgcgggccgcggttgccacggtgaaatccaaataaaaaatgaatcaataaataaacggagacggttgttgattttaacacagagtctgaatctttatttgatttttcgcgcgcggtaggccctggaccaccggtctcgatcattgagcacccggtggatcttttccaggacccggtagaggtgggcttggatgttgaggtacatgggcatgagcccgtcccgggggtggaggtagctccattgcagggcctcgtgctcgggggtggtgttgtaaatcacccagtcatagcaggggcgcagggcatggtgttgcacaatatctttgaggaggagactgatggccacgggcagccctttggtgtaggtgtttacaaatctgttgagctgggagggatgcatgcggggggagatgaggtgcatcttggcctggatcttgagattggcgatgttaccgcccagatcccgcctggggttcatgttgtgcaggaccaccagcacggtgtatccggtgcacttggggaatttatcatgcaacttggaagggaaggcgtgaaagaatttggcgacgcctttgtgcccgcccaggttttccatgcactcatccatgatgatggcgatgggcccgtgggcggcggcctgggcaaagacgtttcgggggtcggacacatcatagttgtggtcctgggtgaggtcatcataggccattttaatgaatttggggcggagggtgccggactgggggacaaaggtaccctcgatcccgggggcgtagttcccctcacagatctgcatctcccaggctttgagctcggagggggggatcatgtccacctgcggggcgataaagaacacggtttccggggcgggggagatgagctgggccgaaagcaagttccggagcagctgggacttgccgcagccggtggggccgtagatgaccccgatgaccggctgcaggtggtagttgagggagagacagctgccgtcctcccggaggaggggggccacctcgttcatcatctcgcgcacgtgcatgttctcgcgcaccagttccgccaggaggcgctctccccccagggataggagctcctggagcgaggcgaagtttttcagcggcttgagtccgtcggccatgggcattttggagagggtttgttgcaagagttccaggcggtcccagagctcggtgatgtgctctacggcatctcgatccagcagacctcctcgtttcgcgggttgggacggctgcgggagtagggcaccagacgatgggcgtccagcgcagccagggtccggtccttccagggtcgcagcgtccgcgtcagggtggtctccgtcacggtgaaggggtgcgcgccgggctgggcgcttgcgagggtgcgcttcaggctcatccggctggtcgaaaaccgctcccgatcggcgccctgcgcgtcggccaggtagcaattgaccatgagttcgtagttgagcgcctcggccgcgtggcctttggcgcggagcttacctttggaagtctgcccgcaggcgggacagaggagggacttgagggcgtagagcttgggggcgaggaagacggactcgggggcgtaggcgtccgcgccgcagtgggcgcagacggtctcgcactccacgagccaggtgaggtcgggctggtcggggtcaaaaaccagtttcccgccgttctttttgatgcgtttcttacctttggtctccatgagctcgtgtccccgctgggtgacaaagaggctgtccgtgtccccgtagaccgactttatgggccggtcctcgagcggtgtgccgcggtcctcctcgtagaggaaccccgcccactccgagacgaaagcccgggtccaggccagcacgaaggaggccacgtgggacgggtagcggtcgttgtccaccagcgggtccaccttttccagggtatgcaaacacatgtccccctcgtccacatccaggaaggtgattggcttgtaagtgtaggccacgtgaccgggggtcccggccgggggggtataaaagggtgcgggtccctgctcgtcctcactgtcttccggatcgctgtccaggagcgccagctgttggggtaggtattccctctcgaaggcgggcatgacctcggcactcaggttgtcagtttctagaaacgaggaggatttgatattgacggtgccggcggagatgcctttcaagagcccctcgtccatctggtcagaaaagacgatctttttgttgtcgagcttggtggcgaaggagccgtagagggcgttggagaggagcttggcgatggagcgcatggtctggtttttttccttgtcggcgcgctccttggcggcgatgttgagctgcacgtactcgcgcgccacgcacttccattcggggaagacggtggtcagctcgtcgggcacgattctgacctgccagccccgattatgcagggtgatgaggtccacactggtggccacctcgccgcgcaggggctcattagtccagcagaggcgtccgcccttgcgcgagcagaaggggggcagggggtccagcatgacctcgtcgggggggtcggcatcgatggtgaagatgccgggcaggaggtcggggtcaaagtagctgatggaagtggccagatcgtccagggcagcttgccattcgcgcacggccagcgcgcgctcgtagggactgaggggcgtgccccagggcatgggatgggtaagcgcggaggcgtacatgccgcagatgtcgtagacgtagaggggctcctcgaggatgccgatgtaggtggggtagcagcgccccccgcggatgctggcgcgcacgtagtcatacagctcgtgcgagggggcgaggagccccgggcccaggttggtgcgactgggcttttcggcgcggtagacgatctggcggaaaatggcatgcgagttggaggagatggtgggcctttggaagatgttgaagtgggcgtggggcagtccgaccgagtcgcggatgaagtgggcgtaggagtcttgcagcttggcgacgagctcggcggtgactaggacgtccagagcgcagtagtcgagggtctcctggatgatgtcatacttgagctgtcccttttgtttccacagctcgcggttgagaaggaactcttcgcggtccttccagtactcttcgagggggaacccgtcctgatctgcacggtaagagcctagcatgtagaactggttgacggccttgtaggcgcagcagcccttctccacggggagggcgtaggcctgggcggccttgcgcagggaggtgtgcgtgagggcgaaagtgtccctgaccatgaccttgaggaactggtgcttgaagtcgatatcgtcgcagcccccctgctcccagagctggaagtccgtgcgcttcttgtaggcggggttgggcaaagcgaaagtaacatcgttgaagaggatcttgcccgcgcggggcataaagttgcgagtgatgcggaaaggttggggcacctcggcccggttgttgatgacctgggcggcgagcacgatctcgtcgaagccgttgatgttgtggcccacgatgtagagttccacgaatcgcggacggcccttgacgtggggcagtttcttgagctcctcgtaggtgagctcgtcggggtcgctgagcccgtgctgctcgagcgcccagtcggcgagatgggggttggcgcggaggaaggaagtccagagatccacggccagggcggtttgcagacggtcccggtactgacggaactgctgcccgacggccattttttcgggggtgacgcagtagaaggtgcgggggtccccgtgccagcgatcccatttgagctggagggcgagatcgagggcgagctcgacgagccggtcgtccccggagagtttcatgaccagcatgaaggggacgagctgcttgccgaaggaccccatccaggtgtaggtttccacatcgtaggtgaggaagagcctttcggtgcgaggatgcgagccgatggggaagaactggatctcctgccaccaattggaggaatggctgttgatgtgatggaagtagaaatgccgacggcgcgccgaacactcgtgcttgtgtttatacaagcggccacagtgctcgcaacgctgcacgggatgcacgtgctgcacgagctgtacctgagttcctttgacgaggaatttcagtgggaagtggagtcgtggcgcctgcatctcgtgctgtactacgtcgtggtggtcggcctggccctcttctgcctcgatggtggtcatgctgacgagcccgcgcgggaggcaggtccagacctcggcgcgagcgggtcggagagcgaggacgagggcgcgcaggccggagctgtccagggtcctgagacgctgcggagtcaggtcagtgggcagcggcggcgcgcggttgacttgcaggagtttttccagggcgcgcgggaggtccagatggtacttgatctccaccgcgccattggtggcgacgtcgatggcttgcagggtcccgtgcccctggggtgtgaccaccgtcccccgtttcttcttgggcggctggggcgacgggggcggtgcctcttccatggttagaagcggcggcgaggacgcgcgccgggcggcaggggcggctcggggcccggaggcaggggcggcaggggcacgtcggcgccgcgcgcgggtaggttctggtactgcgcccggagaagactggcgtgagcgacgacgcgacggttgacgtcctggatctgacgcctctgggtgaaggccacgggacccgtgagtttgaacctgaaagagagttcgacagaatcaatctcggtatcgttgacggcggcctgccgcaggatctcttgcacgtcgcccgagttgtcctggtaggcgatctcggtcatgaactgctcgatctcctcctcttgaaggtctccgcggccggcgcgctccacggtggccgcgaggtcgttggagatgcggcccatgagctgcgagaaggcgttcatgcccgcctcgttccagacgcggctgtagaccacgacgccctcgggatcgccggcgcgcatgaccacctgggcgaggttgagctccacgtggcgcgtgaagaccgcgtagttgcagaggcgctggtagaggtagttgagcgtggtggcgatgtgctcggtgacgaagaaatacatgatccagcggcggagcggcatctcgctgacgtcgcccagcgcctccaaacgttccatggcctcgtaaaagtccacggcgaagttgaaaaactgggagttgcgcgccgagacggtcaactcctcctccagaagacggatgagctcggcgatggtggcgcgcacctcgcgctcgaaggcccccgggagttcctccacttcctcttcttcctcctccactaacatctcttctacttcctcctcaggcggcagtggtggcgggggagggggcctgcgtcgccggcggcgcacgggcagacggtcgatgaagcgctcgatggtctcgccgcgccggcgtcgcatggtctcggtgacggcgcgcccgtcctcgcggggccgcagcgtgaagacgccgccgcgcatctccaggtggccgggggggtccccgttgggcagggagagggcgctgacgatgcatcttatcaattgccccgtagggactccgcgcaaggacctgagcgtctcgagatccacgggatctgaaaaccgctgaacgaaggcttcgagccagtcgcagtcgcaaggtaggctgagcacggtttcttctggcgggtcatgttggttgggagcggggcgggcgatgctgctggtgatgaagttgaaataggcggttctgagacggcggatggtggcgaggagcaccaggtctttgggcccggcttgctggatgcgcagacggtcggccatgccccaggcgtggtcctgacacctggccaggtccttgtagtagtcctgcatgagccgctccacgggcacctcctcctcgcccgcgcggccgtgcatgcgcgtgagcccgaagccgcgctggggctggacgagcgccaggtcggcgacgacgcgctcggcgaggatggcttgctggatctgggtgagggtggtctggaagtcatcaaagtcgacgaagcggtggtaggctccggtgttgatggtgtaggagcagttggccatgacggaccagttgacggtctggtggcccggacgcacgagctcgtggtacttgaggcgcgagtaggcgcgcgtgtcgaagatgtagtcgttgcaggtgcgcaccaggtactggtagccgatgaggaagtgcggcggcggctggcggtagagcggccatcgctcggtggcgggggcgccgggcgcgaggtcctcgagcatggtgcggtggtagccgtagatgtacctggacatccaggtgatgccggcggcggtggtggaggcgcgcgggaactcgcggacgcggttccagatgttgcgcagcggcaggaagtagttcatggtgggcacggtctggcccgtgaggcgcgcgcagtcgtggatgctctatacgggcaaaaacgaaagcggtcagcggctcgactccgtggcctggaggctaagcgaacgggttgggctgcgcgtgtaccccggttcgaatctcgaatcaggctggagccgcagctaacgtggtattggcactcccgtctcgacccaagcctgcaccaaccctccaggatacggaggcgggtcgttttgcaacttttttttggaggccggatgagactagtaagcgcggaaagcggccgaccgcgatggctcgctgccgtagtctggagaagaatcgccagggttgcgttgcggtgtgccccggttcgaggccggccggattccgcggctaacgagggcgtggctgccccgtcgtttccaagaccccatagccagccgacttctccagttacggagcgagcccctcttttgttttgtttgtttttgccagatgcatcccgtactgcggcagatgcgcccccaccaccctccaccgcaacaacagccccctccacagccggcgcttctgcccccgccccagcagcaacttccagccacgaccgccgcggccgccgtgagcggggctggacagagttatgatcaccagctggccttggaagagggcgaggggctggcgcgcctgggggcgtcgtcgccggagcggcacccgcgcgtgcagatgaaaagggacgctcgcgaggcctacgtgcccaagcagaacctgttcagagacaggagcggcgaggagcccgaggagatgcgcgcggcccggttccacgcggggcgggagctgcggcgcggcctggaccgaaagagggtgctgagggacgaggatttcgaggcggacgagctgacggggatcagccccgcgcgcgcgcacgtggccgcggccaacctggtcacggcgtacgagcagaccgtgaaggaggagagcaacttccaaaaatccttcaacaaccacgtgcgcaccctgatcgcgcgcgaggaggtgaccctgggcctgatgcacctgtgggacctgctggaggccatcgtgcagaaccccaccagcaagccgctgacggcgcagctgttcctggtggtgcagcatagtcgggacaacgaagcgttcagggaggcgctgctgaatatcaccgagcccgagggccgctggctcctggacctggtgaacattctgcagagcatcgtggtgcaggagcgcgggctgccgctgtccgagaagctggcggccatcaacttctcggtgctgagtttgggcaagtactacgctaggaagatctacaagaccccgtacgtgcccatagacaaggaggtgaagatcgacgggttttacatgcgcatgaccctgaaagtgctgaccctgagcgacgatctgggggtgtaccgcaacgacaggatgcaccgtgcggtgagcgccagcaggcggcgcgagctgagcgaccaggagctgatgcatagtctgcagcgggccctgaccggggccgggaccgagggggagagctactttgacatgggcgcggacctgcactggcagcccagccgccgggccttggaggcggcggcaggaccctacgtagaagaggtggacgatgaggtggacgaggagggcgagtacctggaagactgatggcgcgaccgtatttttgctagatgcaacaacaacagccacctcctgatcccgcgatgcgggcggcgctgcagagccagccgtccggcattaactcctcggacgattggacccaggccatgcaacgcatcatggcgctgacgacccgcaaccccgaagcctttagacagcagccccaggccaaccggctctcggccatcctggaggccgtggtgccctcgcgctccaaccccacgcacgagaaggtcctggccatcgtgaacgcgctggtggagaacaaggccatccgcggcgacgaggccggcctggtgtacaacgcgctgctggagcgcgtggcccgctacaacagcaccaacgtgcagaccaacctggaccgcatggtgaccgacgtgcgcgaggccgtggcccagcgcgagcggttccaccgcgagtccaacctgggatccatggtggcgctgaacgccttcctcagcacccagcccgccaacgtgccccggggccaggaggactacaccaacttcatcagcgccctgcgcctgatggtgaccgaggtgccccagagcgaggtgtaccagtccgggccggactacttcttccagaccagtcgccagggcttgcagaccgtgaacctgagccaggctttcaagaacttgcagggcctgtggggcgtgcaggccccggtcggggaccgcgcgacggtgtcgagcctgctgacgccgaactcgcgcctgctgctgctgctggtggcccccttcacggacagcggcagcatcaaccgcaactcgtacctgggctacctgattaacctgtaccgcgaggccatcggccaggcgcacgtggacgagcagacctaccaggagatcacccacgtgagccgcgccctgggccaggacgacccgggcaacctggaagccaccctgaactttttgctgaccaaccggtcgcagaagatcccgccccagtacgcgctcagcaccgaggaggagcgcatcctgcgttacgtgcagcagagcgtgggcctgttcctgatgcaggagggggccacccccagcgccgcgctcgacatgaccgcgcgcaacatggagcccagcatgtacgccagcaaccgcccgttcatcaataaactgatggactacttgcatcgggcggccgccatgaactctgactatttcaccaacgccatcctgaatccccactggctcccgccgccggggttctacacgggcgagtacgacatgcccgaccccaatgacgggttcctgtgggacgatgtggacagcagcgtgttctccccccgaccgggtgctaacgagcgccccttgtggaagaaggaaggcagcgaccgacgcccgtcctcggcgctgtccggccgcgagggtgctgccgcggcggtgcccgaggccgccagtcctttcccgagcttgcccttctcgctgaacagtatccgcagcagcgagctgggcaggatcacgcgcccgcgcttgctgggcgaagaggagtacttgaatgactcgctgttgagacccgagcgggagaagaacttccccaataacgggatagaaagcctggtggacaagatgagccgctggaagacgtatgcgcaggagcacagggacgatccccgggcgtcgcagggggccacgagccggggcagcgccgcccgtaaacgccggtggcacgacaggcagcggggacagatgtgggacgatgaggactccgccgacgacagcagcgtgttggacttgggtgggagtggtaacccgttcgctcacctgcgcccccgtatcgggcgcatgatgtaagagaaaccgaaaataaatgatactcaccaaggccatggcgaccagcgtgcgttcgtttcttctctgttgttgttgtatctagtatgatgaggcgtgcgtacccggagggtcctcctccctcgtacgagagcgtgatgcagcaggcgatggcggcggcggcgatgcagcccccgctggaggctccttacgtgcccccgcggtacctggcgcctacggaggggcggaacagcattcgttactcggagctggcacccttgtacgataccacccggttgtacctggtggacaacaagtcggcggacatcgcctcgctgaactaccagaacgaccacagcaacttcctgaccaccgtggtgcagaacaatgacttcacccccacggaggccagcacccagaccatcaactttgacgagcgctcgcggtggggcggccagctgaaaaccatcatgcacaccaacatgcccaacgtgaacgagttcatgtacagcaacaagttcaaggcgcgggtgatggtctcccgcaagacccccaatggggtgacagtgacagaggattatgatggtagtcaggatgagctgaagtatgaatgggtggaatttgagctgcccgaaggcaacttctcggtgaccatgaccatcgacctgatgaacaacgccatcatcgacaattacttggcggtggggcggcagaacggggtgctggagagcgacatcggcgtgaagttcgacactaggaacttcaggctgggctgggaccccgtgaccgagctggtcatgcccggggtgtacaccaacgaggctttccatcccgatattgtcttgctgcccggctgcggggtggacttcaccgagagccgcctcagcaacctgctgggcattcgcaagaggcagcccttccaggaaggcttccagatcatgtacgaggatctggaggggggcaacatccccgcgctcctggatgtcgacgcctatgagaaaagcaaggaggatgcagcagctgaagcaactgcagccgtagctaccgcctctaccgaggtcaggggcgataattttgcaagcgccgcagcagtggcagcggccgaggcggctgaaaccgaaagtaagatagtcattcagccggtggagaaggatagcaagaacaggagctacaacgtactaccggacaagataaacaccgcctaccgcagctggtacctagcctacaactatggcgaccccgagaagggcgtgcgctcctggacgctgctcaccacctcggacgtcacctgcggcgtggagcaagtctactggtcgctgcccgacatgatgcaagacccggtcaccttccgctccacgcgtcaagttagcaactacccggtggtgggcgccgagctcctgcccgtctactccaagagcttcttcaacgagcaggccgtctactcgcagcagctgcgcgccttcacctcgcttacgcacgtcttcaaccgcttccccgagaaccagatcctcgtccgcccgcccgcgcccaccattaccaccgtcagtgaaaacgttcctgctctcacagatcacgggaccctgccgctgcgcagcagtatccggggagtccagcgcgtgaccgttactgacgccagacgccgcacctgcccctacgtctacaaggccctgggcatagtcgcgccgcgcgtcctctcgagccgcaccttctaaatgtccattctcatctcgcccagtaataacaccggttggggcctgcgcgcgcccagcaagatgtacggaggcgctcgccaacgctccacgcaacaccccgtgcgcgtgcgcgggcacttccgcgctccctggggcgccctcaagggccgcgtgcggtcgcgcaccaccgtcgacgacgtgatcgaccaggtggtggccgacgcgcgcaactacacccccgccgccgcgcccgtctccaccgtggacgccgtcatcgacagcgtggtggcggacgcgcgccggtacgcccgcgccaagagccggcggcggcgcatcgcccggcggcaccggagcacccccgccatgcgcgcggcgcgagccttgctgcgcagggccaggcgcacgggacgcagggccatgctcagggcggccagacgcgcggcttcaggcgccagcgccggcaggacccggagacgcgcggccacggcggcggcagcggccatcgccagcatgtcccgcccgcggcgagggaacgtgtactgggtgcgcgacgccgccaccggtgtgcgcgtgcccgtgcgcacccgcccccctcgcacttgaagatgttcacttcgcgatgttgatgtgtcccagcggcgaggaggatgtccaagcgcaaattcaaggaagagatgctccaggtcatcgcgcctgagatctacggccctgcggtggtgaaggaggaaagaaagccccgcaaaatcaagcgggtcaaaaaggacaaaaaggaagaagaaagtgatgtggacggattggtggagtttgtgcgcgagttcgccccccggcggcgcgtgcagtggcgcgggcggaaggtgcaaccggtgctgagacccggcaccaccgtggtcttcacgcccggcgagcgctccggcaccgcttccaagcgctcctacgacgaggtgtacggggatgatgatattctggagcaggcggccgagcgcctgggcgagtttgcttacggcaagcgcagccgttccgcaccgaaggaagaggcggtgtccatcccgctggaccacggcaaccccacgccgagcctcaagcccgtgaccttgcagcaggtgctgccgaccgcggcgccgcgccgggggttcaagcgcgagggcgaggatctgtaccccaccatgcagctgatggtgcccaagcgccagaagctggaagacgtgctggagaccatgaaggtggacccggacgtgcagcccgaggtcaaggtgcggcccatcaagcaggtggccccgggcctgggcgtgcagaccgtggacatcaagattcccacggagcccatggaaacgcagaccgagcccatgatcaagcccagcaccagcaccatggaggtgcagacggatccctggatgccatcggctcctagtcgaagaccccggcgcaagtacggcgcggccagcctgctgatgcccaactacgcgctgcatccttccatcatccccacgccgggctaccgcggcacgcgcttctaccgcggtcataccagcagccgccgccgcaagaccaccactcgccgccgccgtcgccgcaccgccgctgcaaccacccctgccgccctggtgcggagagtgtaccgccgcggccgcgcacctctgaccctgccgcgcgcgcgctaccacccgagcatcgccatttaaactttcgccagctttgcagatcaatggccctcacatgccgccttcgcgttcccattacgggctaccgaggaagaaaaccgcgccgtagaaggctggcggggaacgggatgcgtcgccaccaccaccggcggcggcgcgccatcagcaagcggttggggggaggcttcctgcccgcgctgatccccatcatcgccgcggcgatcggggcgatccccggcattgcttccgtggcggtgcaggcctctcagcgccactgagacacacttggaaacatcttgtaataaacccatggactctgacgctcctggtcctgtgatgtgttttcgtagacagatggaagacatcaatttttcgtccctggctccgcgacacggcacgcggccgttcatgggcacctggagcgacatcggcaccagccaactgaacgggggcgccttcaattggagcagtctctggagcgggcttaagaatttcgggtccacgcttaaaacctatggcagcaaggcgtggaacagcaccacagggcaggcgctgagggataagctgaaagagcagaacttccagcagaaggtggtcgatgggctcgcctcgggcatcaacggggtggtggacctggccaaccaggccgtgcagcggcagatcaacagccgcctggacccggtgccgcccgccggctccgtggagatgccgcaggtggaggaggagctgcctcccctggacaagcggggcgagaagcgaccccgccccgatgcggaggagacgctgctgacgcacacggacgagccgcccccgtacgaggaggcggtgaaactgggtctgcccaccacgcggcccatcgcgcccctggccaccggggtgctgaaacccgaaaagcccgcgaccctggacttgcctcctccccagccttcccgcccctctacagtggctaagcccctgccgccggtggccgtggcccgcgcgcgacccgggggcaccgcccgccctcatgcgaactggcagagcactctgaacagcatcgtgggtctgggagtgcagagtgtgaagcgccgccgctgctattaaacctaccgtagcgcttaacttgcttgtctgtgtgtgtatgtattatgtcgccgccgccgctgtccaccagaaggaggagtgaagaggcgcgtcgccgagttgcaagatggccaccccatcgatgctgccccagtgggcgtacatgcacatcgccggacaggacgcttcggagtacctgagtccgggtctggtgcagtttgcccgcgccacagacacctacttcagtctggggaacaagtttaggaaccccacggtggcgcccacgcacgatgtgaccaccgaccgcagccagcggctgacgctgcgcttcgtgcccgtggaccgcgaggacaacacctactcgtacaaagtgcgctacacgctggccgtgggcgacaaccgcgtgctggacatggccagcacctactttgacatccgcggcgtgctggatcggggccctagcttcaaaccctactccggcaccgcctacaacagtctggcccccaagggagcacccaacacttgtcagtggacatataaagccgatggtgaaactgccacagaaaaaacctatacatatggaaatgcacccgtgcagggcattaacatcacaaaagatggtattcaacttggaactgacaccgatgatcagccaatctacgcagataaaacctatcagcctgaacctcaagtgggtgatgctgaatggcatgacatcactggtactgatgaaaagtatggaggcagagctcttaagcctgataccaaaatgaagccttgttatggttcttttgccaagcctactaataaagaaggaggtcaggcaaatgtgaaaacaggaacaggcactactaaagaatatgacatagacatggctttctttgacaacagaagtgcggctgctgctggcctagctccagaaattgttttgtatactgaaaatgtggatttggaaactccagatacccatattgtatacaaagcaggcacagatgacagcagctcttctattaatttgggtcagcaagccatgcccaacagacctaactacattggtttcagagacaactttatcgggctcatgtactacaacagcactggcaatatgggggtgctggccggtcaggcttctcagctgaatgctgtggttgacttgcaagacagaaacaccgagctgtcctaccagctcttgcttgactctctgggtgacagaacccggtatttcagtatgtggaatcaggcggtggacagctatgatcctgatgtgcgcattattgaaaatcatggtgtggaggatgaacttcccaactattgtttccctctggatgctgttggcagaacagatacttatcagggaattaaggctaatggaactgatcaaaccacatggaccaaagatgacagtgtcaatgatgctaatgagataggcaagggtaatccattcgccatggaaatcaacatccaagccaacctgtggaggaacttcctctacgccaacgtggccctgtacctgcccgactcttacaagtacacgccggccaatgttaccctgcccaccaacaccaacacctacgattacatgaacggccgggtggtggcgccctcgctggtggactcctacatcaacatcggggcgcgctggtcgctggatcccatggacaacgtgaaccccttcaaccaccaccgcaatgcggggctgcgctaccgctccatgctcctgggcaacgggcgctacgtgcccttccacatccaggtgccccagaaatttttcgccatcaagagcctcctgctcctgcccgggtcctacacctacgagtggaacttccgcaaggacgtcaacatgatcctgcagagctccctcggcaacgacctgcgcacggacggggcctccatctccttcaccagcatcaacctctacgccaccttcttccccatggcgcacaacacggcctccacgctcgaggccatgctgcgcaacgacaccaacgaccagtccttcaacgactacctctcggcggccaacatgctctaccccatcccggccaacgccaccaacgtgcccatctccatcccctcgcgcaactgggccgccttccgcggctggtccttcacgcgtctcaagaccaaggagacgccctcgctgggctccgggttcgacccctacttcgtctactcgggctccatcccctacctcgacggcaccttctacctcaaccacaccttcaagaaggtctccatcaccttcgactcctccgtcagctggcccggcaacgaccggctcctgacgcccaacgagttcgaaatcaagcgcaccgtcgacggcgagggctacaacgtggcccagtgcaacatgaccaaggactggttcctggtccagatgctggcccactacaacatcggctaccagggcttctacgtgcccgagggctacaaggaccgcatgtactccttcttccgcaacttccagcccatgagccgccaggtggtggacgaggtcaactacaaggactaccaggccgtcaccctggcctaccagcacaacaactcgggcttcgtcggctacctcgcgcccaccatgcgccagggccagccctaccccgccaactacccctacccgctcatcggcaagagcgccgtcaccagcgtcacccagaaaaagttcctctgcgacagggtcatgtggcgcatccccttctccagcaacttcatgtccatgggcgcgctcaccgacctcggccagaacatgctctatgccaactccgcccacgcgctagacatgaatttcgaagtcgaccccatggatgagtccacccttctctatgttgtcttcgaagtcttcgacgtcgtccgagtgcaccagccccaccgcggcgtcatcgaggccgtctacctgcgcacccccttctcggccggtaacgccaccacctaagctcttgcttcttgcaagccatggccgcgggctccggcgagcaggagctcagggccatcatccgcgacctgggctgcgggccctacttcctgggcaccttcgataagcgcttcccgggattcatggccccgcacaagctggcctgcgccatcgtcaacacggccggccgcgagaccgggggcgagcactggctggccttcgcctggaacccgcgctcgaacacctgctacctcttcgaccccttcgggttctcggacgagcgcctcaagcagatctaccagttcgagtacgagggcctgctgcgccgcagcgccctggccaccgaggaccgctgcgtcaccctggaaaagtccacccagaccgtgcagggtccgcgctcggccgcctgcgggctcttctgctgcatgttcctgcacgccttcgtgcactggcccgaccgccccatggacaagaaccccaccatgaacttgctgacgggggtgcccaacggcatgctccagtcgccccaggtggaacccaccctgcgccgcaaccaggaggcgctctaccgcttcctcaactcccactccgcctactttcgctcccaccgcgcgcgcatcgagaaggccaccgccttcgaccgcatgaatcaagacatgtaaaccgtgtgtgtatgttaaatgtctttaataaacagcactttcatgttacacatgcatctgagatgatttatttagaaatcgaaagggttctgccgggtctcggcatggcccgcgggcagggacacgttgcggaactggtacttggccagccacttgaactcggggatcagcagtttgggcagcggggtgtcggggaaggagtcggtccacagcttccgcgtcagttgcagggcgcccagcaggtcgggcgcggagatcttgaaatcgcagttgggacccgcgttctgcgcgcgggagttgcggtacacggggttgcagcactggaacaccatcagggccgggtgcttcacgctcgccagcaccgtcgcgtcggtgatgctctccacgtcgaggtcctcggcgttggccatcccgaagggggtcatcttgcaggtctgccttcccatggtgggcacgcacccgggcttgtggttgcaatcgcagtgcagggggatcagcatcatctgggcctggtcggcgttcatccccgggtacatggccttcatgaaagcctccaattgcctgaacgcctgctgggccttggctccctcggtgaagaagaccccgcaggacttgctagagaactggttggtggcgcacccggcgtcgtgcacgcagcagcgcgcgtcgttgttggccagctgcaccacgctgcgcccccagcggttctgggtgatcttggcccggtcggggttctccttcagcgcgcgctgcccgttctcgctcgccacatccatctcgatcatgtgctccttctggatcatggtggtcccgtgcaggcaccgcagcttgccctcggcctcggtgcacccgtgcagccacagcgcgcacccggtgcactcccagttcttgtgggcgatctgggaatgcgcgtgcacgaagccctgcaggaagcggcccatcatggtggtcagggtcttgttgctagtgaaggtcagcggaatgccgcggtgctcctcgttgatgtacaggtggcagatgcggcggtacacctcgccctgctcgggcatcagctggaagttggctttcaggtcggtctccacgcggtagcggtccatcagcatagtcatgatttccatacccttctcccaggccgagacgatgggcaggctcatagggttcttcaccatcatcttagcgctagcagccgcggccagggggtcgctctcgtccagggtctcaaagctccgcttgccgtccttctcggtgatccgcaccggggggtagctgaagcccacggccgccagctcctcctcggcctgtctttcgtcctcgctgtcctggctgacgtcctgcaggaccacatgcttggtcttgcggggtttcttcttgggcggcagcggcggcggagatgttggagatggcgagggggagcgcgagttctcgctcaccactactatctcttcctcttcttggtccgaggccacgcggcggtaggtatgtctcttcgggggcagaggcggaggcgacgggctctcgccgccgcgacttggcggatggctggcagagccccttccgcgttcgggggtgcgctcccggcggcgctctgactgacttcctccgcggccggccattgtgttctcctagggaggaacaacaagcatggagactcagccatcgccaacctcgccatctgcccccaccgccgacgagaagcagcagcagcagaatgaaagcttaaccgccccgccgcccagccccgccacctccgacgcggccgtcccagacatgcaagagatggaggaatccatcgagattgacctgggctatgtgacgcccgcggagcacgaggaggagctggcagtgcgcttttcacaagaagagatacaccaagaacagccagagcaggaagcagagaatgagcagagtcaggctgggctcgagcatgacggcgactacctccacctgagcgggggggaggacgcgctcatcaagcatctggcccggcaggccaccatcgtcaaggatgcgctgctcgaccgcaccgaggtgcccctcagcgtggaggagctcagccgcgcctacgagttgaacctcttctcgccgcgcgtgccccccaagcgccagcccaatggcacctgcgagcccaacccgcgcctcaacttctacccggtcttcgcggtgcccgaggccctggccacctaccacatctttttcaagaaccaaaagatccccgtctcctgccgcgccaaccgcacccgcgccgacgcccttttcaacctgggtcccggcgcccgcctacctgatatcgcctccttggaagaggttcccaagatcttcgagggtctgggcagcgacgagactcgggccgcgaacgctctgcaaggagaaggaggagagcatgagcaccacagcgccctggtcgagttggaaggcgacaacgcgcggctggcggtgctcaaacgcacggtcgagctgacccatttcgcctacccggctctgaacctgccccccaaagtcatgagcgcggtcatggaccaggtgctcatcaagcgcgcgtcgcccatctccgaggacgagggcatgcaagactccgaggagggcaagcccgtggtcagcgacgagcagctggcccggtggctgggtcctaatgctagtccccagagtttggaagagcggcgcaaactcatgatggccgtggtcctggtgaccgtggagctggagtgcctgcgccgcttcttcgccgacgcggagaccctgcgcaaggtcgaggagaacctgcactacctcttcaggcacgggttcgtgcgccaggcctgcaagatctccaacgtggagctgaccaacctggtctcctacatgggcatcttgcacgagaaccgcctggggcagaacgtgctgcacaccaccctgcgcggggaggcccggcgcgactacatccgcgactgcgtctacctctacctctgccacacctggcagacgggcatgggcgtgtggcagcagtgtctggaggagcagaacctgaaagagctctgcaagctcctgcagaagaacctcaagggtctgtggaccgggttcgacgagcgcaccaccgcctcggacctggccgacctcattttccccgagcgcctcaggctgacgctgcgcaacggcctgcccgactttatgagccaaagcatgttgcaaaactttcgctctttcatcctcgaacgctccggaatcctgcccgccacctgctccgcgctgccctcggacttcgtgccgctgaccttccgcgagtgccccccgccgctgtggagccactgctacctgctgcgcctggccaactacctggcctaccactcggacgtgatcgaggacgtcagcggcgagggcctgctcgagtgccactgccgctgcaacctctgcacgccgcaccgctccctggcctgcaacccccagctgctgagcgagacccagatcatcggcaccttcgagttgcaagggcccagcgaaggcgagggttcagccgccaaggggggtctgaaactcaccccggggctgtggacctcggcctacttgcgcaagttcgtgcccgaggactaccatcccttcgagatcaggttctacgaggaccaatcccatccgcccaaggccgagctgtcggcctgcgtcatcacccagggggcgatcctggcccaattgcaagccatccagaaatcccgccaagaattcttgctgaaaaagggccgcggggtctacctcgacccccagaccggtgaggagctcaaccccggcttcccccaggatgccccgaggaaacaagaagctgaaagtggagctgccgcccgtggaggatttggaggaagactgggagaacagcagtcaggcagaggaggaggagatggaggaagactgggacagcactcaggcagaggaggacagcctgcaagacagtctggaggaagacgaggaggaggcagaggaggaggtggaagaagcagccgccgccagaccgtcgtcctcggcgggggagaaagcaagcagcacggataccatctccgctccgggtcggggtcccgctcgaccacacagtagatgggacgagaccggacgattcccgaaccccaccacccagaccggtaagaaggagcggcagggatacaagtcctggcgggggcacaaaaacgccatcgtctcctgcttgcaggcctgcgggggcaacatctccttcacccggcgctacctgctcttccaccgcggggtgaactttccccgcaacatcttgcattactaccgtcacctccacagcccctactacttccaagaagaggcagcagcagcagaaaaagaccagcagaaaaccagcagctagaaaatccacagcggcggcagcaggtggactgaggatcgcggcgaacgagccggcgcaaacccgggagctgaggaaccggatctttcccaccctctatgccatcttccagcagagtcgggggcaggagcaggaactgaaagtcaagaaccgttctctgcgctcgctcacccgcagttgtctgtatcacaagagcgaagaccaacttcagcgcactctcgaggacgccgaggctctcttcaacaagtactgcgcgctcactcttaaagagtagcccgcgcccgcccagtcgcagaaaaaggcgggaattacgtcacctgtgcccttcgccctagccgcctccacccatcatcatgagcaaagagattcccacgccttacatgtggagctaccagccccagatgggcctggccgccggtgccgcccaggactactccacccgcatgaattggctcagcgccgggcccgcgatgatctcacgggtgaatgacatccgcgcccaccgaaaccagatactcctagaacagtcagcgctcaccgccacgccccgcaatcacctcaatccgcgtaattggcccgccgccctggtgtaccaggaaattccccagcccacgaccgtactacttccgcgagacgcccaggccgaagtccagctgactaactcaggtgtccagctggcgggcggcgccaccctgtgtcgtcaccgccccgctcagggtataaagcggctggtgatccggggcagaggcacacagctcaacgacgaggtggtgagctcttcgctgggtctgcgacctgacggagtcttccaactcgccggatcggggagatcttccttcacgcctcgtcaggccgtcctgactttggagagttcgtcctcgcagccccgctcgggtggcatcggcactctccagttcgtggaggagttcactccctcggtctacttcaaccccttctccggctcccccggccactacccggacgagttcatcccgaacttcgacgccatcagcgagtcggtggacggctacgattgagtttaaactcacccccttatccagtgaaataaagatcatattgatgatgattttacagaaataaaaaataatcatttgatttgaaataaagatacaatcatattgatgatttgagtttaacaaaaaaataaagaatcacttacttgaaatctgataccaggtctctgtccatgttttctgccaacaccacttcactcccctcttcccagctctggtactgcaggccccggcgggctgcaaacttcctccacacgctgaaggggatgtcaaattcctcctgtccctcaatcttcattttatcttctatcagatgtccaaaaagcgcgtccgggtggatgatgacttcgaccccgtctacccctacgatgcagacaacgcaccgaccgtgcccttcatcaacccccccttcgtctcttcagatggattccaagagaagcccctgggggtgttgtccctgcgactggccgaccccgtcaccaccaagaacggggaaatcaccctcaagctgggagagggggtggacctcgattcctcgggaaaactcatctccaacacggccaccaaggccgccgcccctctcagtttttccaacaacaccatttcccttaacatggatcaccccttttacactaaagatggaaaattatccttacaagtttctccaccattaaatatactgagaacaagcattctaaacacactagctttaggttttggatcaggtttaggactccgtggctctgccttggcagtacagttagtctctccacttacatttgatactgatggaaacataaagcttaccttagacagaggtttgcatgttacaacaggagatgcaattgaaagcaacataagctgggctaaaggtttaaaatttgaagatggagccatagcaaccaacattggaaatgggttagagtttggaagcagtagtacagaaacaggtgttgatgatgcttacccaatccaagttaaacttggatctggccttagctttgacagtacaggagccataatggctggtaacaaagaagacgataaactcactttgtggacaacacctgatccatcaccaaactgtcaaatactcgcagaaaatgatgcaaaactaacactttgcttgactaaatgtggtagtcaaatactggccactgtgtcagtcttagttgtaggaagtggaaacctaaaccccattactggcaccgtaagcagtgctcaggtgtttctacgttttgatgcaaacggtgttcttttaacagaacattctacactaaaaaaatactgggggtataggcagggagatagcatagatggcactccatataccaatgctgtaggattcatgcccaatttaaaagcttatccaaagtcacaaagttctactactaaaaataatatagtagggcaagtatacatgaatggagatgtttcaaaacctatgcttctcactataaccctcaatggtactgatgacagcaacagtacatattcaatgtcattttcatacacctggactaatggaagctatgttggagcaacatttggggctaactcttataccttctcatacatcgcccaagaatgaacactgtatcccaccctgcatgccaacccttcccaccccactctgtggaacaaactctgaaacacaaaataaaataaagttcaagtgttttattgattcaacagtttcacagaaccctagtattcaacctgccacctccctcccaacacacagagtacacagtcctttctccccggctggccttaaaaagcatcatatcatgggtaacagacatattcttaggtgttatattccacacggtttcctgtcgagccaaacgctcatcagtgatattaataaactccccgggcagctcacttaagttcatgtcgctgtccagctgctgagccacaggctgctgtccaacttgcggttgcttaacgggcggcgaaggagaagtccacgcctacatgggggtagagtcataatcgtgcatcaggatagggcggtggtgctgcagcagcgcgcgaataaactgctgccgccgccgctccgtcctgcaggaatacaacatggcagtggtctcctcagcgatgattcgcaccgcccgcagcataaggcgccttgtcctccgggcacagcagcgcaccctgatctcacttaaatcagcacagtaactgcagcacagcaccacaatattgttcaaaatcccacagtgcaaggcgctgtatccaaagctcatggcggggaccacagaacccacgtggccatcataccacaagcgcaggtagattaagtggcgacccctcataaacacgctggacataaacattacctcttttggcatgttgtaattcaccacctcccggtaccatataaacctctgattaaacatggcgccatccaccaccatcctaaaccagctggccaaaacctgcccgccggctatacactgcagggaaccgggactggaacaatgacagtggagagcccaggactcgtaaccatggatcatcatgctcgtcatgatatcaatgttggcacaacacaggcacacgtgcatacacttcctcaggattacaagctcctcccgcgttagaaccatatcccagggaacaacccattcctgaatcagcgtaaatcccacactgcagggaagacctcgcacgtaactcacgttgtgcattgtcaaagtgttacattcgggcagcagcggatgatcctccagtatggtagcgcgggtttctgtctcaaaaggaggtagacgatccctactgtacggagtgcgccgagacaaccgagatcgtgttggtcgtagtgtcatgccaaatggaacgccggacgtagtcatatttcctgaagcaaaaccaggtgcgggcgtgacaaacagatctgcgtctccggtctcgccgcttagatcgctctgtgtagtagttgtagtatatccactctctcaaagcatccaggcgccccctggcttcgggttctatgtaaactccttcatgcgccgctgccctgataacatccaccaccgcagaataagccacacccagccaacctacacattcgttctgcgagtcacacacgggaggagcgggaagagctggaagaaccatgattaactttattccaaacggtctcggagcacttcaaaatgcaggtcccggaggtggcacctctcgcccccactgtgttggtggaaaataacagccaggtcaaaggtgacacggttctcgagatgttccacggtggcttccagcaaagcctccacgcgcacatccagaaacaagaggacagcgaaagcgggagcgttttctaattcctcaatcatcatattacactcctgcaccatccccagataattttcatttttccagccttgaatgattcgtattagttcctgaggtaaatccaagccagccatgataaaaagctcgcgcagagcgccctccaccggcattcttaagcacaccctcataattccaagagattctgctcctggttcacctgcagcagattaacaatgggaatatcaaaatctctgccgcgatccctaagctcctccctcaacaataactgtatgtaatctttcatatcatctccgaaatttttagccatagggccgccaggaataagagcagggcaagccacattacagataaagcgaagtcctccccagtgwgcattgccaaatgtaagattgaaataagcatgctggctagaccctgtgatatcttccagataactggacagaaaatcaggcaagcaatttttaagaaaatcaacaaaagaaaagtcgtccaggtgcaggtttagagcctcaggaacaacgatggaataagtgcaaggagtgcgttccagcatggttagtgtttttttggtgatctgtagaacaaaaaataaacatgcaatattaaaccatgctagcctggcgaacaggtgggtaaatcactctttccagcaccaggcaggctacggggtctccggcgcgaccctcgtagaagctgtcgccatgattgaaaagcatcaccgagagaccttcccggtggccggcatggatgattcgagaagaagcatacactccgggaacattggcatccgtgagtgaaaaaaagcgacctataaagcctcggggcactacaatgctcaatctcaattccagcaaagccaccccatgcggatggagcacaaaattggcaggtgcgtaaaaaatgtaattactcccctcctgcacaggcagcaaagcccccgctccctccagaaacacatacaaagcctcagcgtccatagcttaccgagcacggcaggcgcaagagtcagagaaaaggctgagctctaacctgactgcccgctcctgtgctcaatatatagccctaacctacactgacgtaaaggccaaagtctaaaaatacccgccaaataatcacacacgcccagcacacgcccagaaaccggtgacacactcaaaaaaatacgcgcacttcctcaaacgcccaaaactgccgtcatttccgggttcccacgctacgtcatcaaaacacgactttcaaattccgtcgaccgttaaaaacgtcacccgccccgcccctaacggtcgcccgtctctcagccaatcagcgccccgcatccccaaattcaaacacctcatttgcatattaacgcgcacaaaaagtttgaggtatattattgatgatggttaattaaggatccttctatagtgtcacctaaatgtcgacggccaggcggccgccaggcctacccactagtcaattcgggaggatcgaaacggcagatcgcaaaaaacagtacatacagaaggagacatgaacatgaacatcaaaaaaattgtaaaacaagccacagttctgacttttacgactgcacttctggcaggaggagcgactcaagccttcgcgaaagaaaataaccaaaaagcatacaaagaaacgtacggcgtctctcatattacacgccatgatatgctgcagatccctaaacagcagcaaaacgaaaaataccaagtgcctcaattcgatcaatcaacgattaaaaatattgagtctgcaaaaggacttgatgtgtgggacagctggccgctgcaaaacgctgacggaacagtagctgaatacaacggctatcacgttgtgtttgctcttgcgggaagcccgaaagacgctgatgacacatcaatctacatgttttatcaaaaggtcggcgacaactcaatcgacagctggaaaaacgcgggccgtgtctttaaagacagcgataagttcgacgccaacgatccgatcctgaaagatcagacgcaagaatggtccggttctgcaacctttacatctgacggaaaaatccgtttattctacactgactattccggtaaacattacggcaaacaaagcctgacaacagcgcaggtaaatgtgtcaaaatctgatgacacactcaaaatcaacggagtggaagatcacaaaacgatttttgacggagacggaaaaacatatcagaacgttcagcagtttatcgatgaaggcaattatacatccggcgacaaccatacgctgagagaccctcactacgttgaagacaaaggccataaataccttgtattcgaagccaacacgggaacagaaaacggataccaaggcgaagaatctttatttaacaaagcgtactacggcggcggcacgaacttcttccgtaaagaaagccagaagcttcagcagagcgctaaaaaacgcgatgctgagttagcgaacggcgccctcggtatcatagagttaaataatgattacacattgaaaaaagtaatgaagccgctgatcacttcaaacacggtaactgatgaaatcgagcgcgcgaatgttttcaaaatgaacggcaaatggtacttgttcactgattcacgcggttcaaaaatgacgatcgatggtattaactcaaacgatatttacatgcttggttatgtatcaaactctttaaccggcccttacaagccgctgaacaaaacagggcttgtgctgcaaatgggtcttgatccaaacgatgtgacattcacttactctcacttcgcagtgccgcaagccaaaggcaacaatgtggttatcacaagctacatgacaaacagaggcttcttcgaggataaaaaggcaacatttgcgccaagcttcttaatgaacatcaaaggcaataaaacatccgttgtcaaaaacagcatcctggagcaaggacagctgacagtcaactaataacagcaaaaagaaaatgccgatacttcattggcattttcttttatttctcaacaagatggtgaattgactagtgggtagatccacaggacgggtgtggtcgccatgatcgcgtagtcgatagtggctccaagtagcgaagcgagcaggactgggcggcggccaaagcggtcggacagtgctccgagaacgggtgcgcatagaaattgcatcaacgcatatagcgctagcagcacgccatagtgactggcgatgctgtcggaatggacgatatcccgcaagaggcccggcagtaccggcataaccaagcctatgcctacagcatccagggtgacggtgccgaggatgacgatgagcgcattgttagatttcatacacggtgcctgactgcgttagcaatttaactgtgataaactaccgcattaaagcttatcgatgataagctgtcaaacatgagaattgatccggaacccttaatataacttcgtataatgtatgctatacgaagttattaggtccctcgactatagggtcaccgtcgacagcgacacacttgcatcggatgcagcccggttaacgtgccggcacggcctgggtaaccaggtattttgtccacataaccgtgcgcaaaatgttgtggataagcaggacacagcagcaatccacagcaggcatacaaccgcacaccgaggttactccgttctacaggttacgacgacatgtcaatacttgcccttgacaggcattgatggaatcgtagtctcacgctgatagtctgatcgacaatacaagtgggaccgtggtcccagaccgataatcagaccgacaacacgagtgggatcgtggtcccagactaataatcagaccgacgatacgagtgggaccgtggtcccagactaataatcagaccgacgatacgagtgggaccgtggttccagactaataatcagaccgacgatacgagtgggaccgtggtcccagactaataatcagaccgacgatacgagtgggaccatggtcccagactaataatcagaccgacgatacgagtgggaccgtggtcccagtctgattatcagaccgacgatacgagtgggaccgtggtcccagactaataatcagaccgacgatacgagtgggaccgtggtcccagactaataatcagaccgacgatacgagtgggaccgtggtcccagtctgattatcagaccgacgatacaagtggaacagtgggcccagagagaatattcaggccagttatgctttctggcctgtaacaaaggacattaagtaaagacagataaacgtagactaaaacgtggtcgcatcagggtgctggcttttcaagttccttaagaatggcctcaattttctctatacactcagttggaacacgagacctgtccaggttaagcaccattttatcgcccttatacaatactgtcgctccaggagcaaactgatgtcgtgagcttaaactagttcttgatgcagatgacgttttaagcacagaagttaaaagagtgataacttcttcagcttcaaatatcaccccagcttttttctgctcatgaaggttagatgcctgctgcttaagtaattcctctttatctgtaaaggctttttgaagtgcatcacctgaccgggcagatagttcaccggggtgagaaaaaagagcaacaactgatttaggcaatttggcggtgttgatacagcgggtaataatcttacgtgaaatattttccgcatcagccagcgcagaaatatttccagcaaattcattctgcaatcggcttgcataacgctgaccacgttcataagcacttgttgggcgataatcgttacccaatctggataatgcagccatctgctcatcatccagctcgccaaccagaacacgataatcactttcggtaagtgcagcagctttacgacggcgactcccatcggcaatttctatgacaccagatactcttcgaccgaacgccggtgtctgttgaccagtcagtagaaaagaagggatgagatcatccagtgcgtcctcagtaagcagctcctggtcacgttcattacctgaccatacccgagaggtcttctcaacactatcaccccggagcacttcaagagtaaacttcacatcccgaccacatacaggcaaagtaatggcattaccgcgagccattactcctacgcgcgcaattaacgaatccaccatcggggcagctggtgtcgataacgaagtatcttcaaccggttgagtattgagcgtatgttttggaataacaggcgcacgcttcattatctaatctcccagcgtggtttaatcagacgatcgaaaatttcattgcagacaggttcccaaatagaaagagcatttctccaggcaccagttgaagagcgttgatcaatggcctgttcaaaaacagttctcatccggatctgacctttaccaacttcatccgtttcacgtacaacattttttagaaccatgcttccccaggcatcccgaatttgctcctccatccacggggactgagagccattactattgctgtatttggtaagcaaaatacgtacatcaggctcgaaccctttaagatcaacgttcttgagcagatcacgaagcatatcgaaaaactgcagtgcggaggtgtagtcaaacaactcagcaggcgtgggaacaatcagcacatcagcagcacatacgacattaatcgtgccgatacccaggttaggcgcgctgtcaataactatgacatcatagtcatgagcaacagtttcaatggccagtcggagcatcaggtgtggatcggtgggcagtttaccttcatcaaatttgcccattaactcagtttcaatacggtgcagagccagacaggaaggaataatgtcaagccccggccagcaagtgggctttattgcataagtgacatcgtccttttccccaagatagaaaggcaggagagtgtcttctgcatgaatatgaagatctggtacccatccgtgatacattgaggctgttccctgggggtcgttaccttccacgagcaaaacacgtagccccttcagagccagatcctgagcaagatgaacagaaactgaggttttgtaaacgccacctttatgggcagcaaccccgatcaccggtggaaatacgtcttcagcacgtcgcaatcgcgtaccaaacacatcacgcatatgattaatttgttcaattgtataaccaacacgttgctcaacccgtcctcgaatttccatatccgggtgcggtagtcgccctgctttctcggcatctctgatagcctgagaagaaaccccaactaaatccgctgcttcacctattctccagcgccgggttattttcctcgcttccgggctgtcatcattaaactgtgcaatggcgatagccttcgtcatttcatgaccagcgtttatgcactggttaagtgtttccatgagtttcattctgaacatcctttaatcattgctttgcgtttttttattaaatcttgcaatttactgcaaagcaacaacaaaatcgcaaagtcatcaaaaaaccgcaaagttgtttaaaataagagcaacactacaaaaggagataagaagagcacatacctcagtcacttattatcactagcgctcgccgcagccgtgtaaccgagcatagcgagcgaactggcgaggaagcaaagaagaactgttctgtcagatagctcttacgctcagcgcaagaagaaatatccaccgtgggaaaaactccaggtagaggtacacacgcggatagccaattcagagtaataaactgtgataatcaaccctcatcaatgatgacgaactaacccccgatatcaggtcacatgacgaagggaaagagaaggaaatcaactgtgacaaactgccctcaaatttggcttccttaaaaattacagttcaaaaagtatgagaaaatccatgcaggctgaaggaaacagcaaaactgtgacaaattaccctcagtaggtcagaacaaatgtgacgaaccaccctcaaatctgtgacagataaccctcagactatcctgtcgtcatggaagtgatatcgcggaaggaaaatacgatatgagtcgtctggcggcctttctttttctcaatgtatgagaggcgcattggagttctgctgttgatctcattaacacagacctgcaggaagcggcggcggaagtcaggcatacgctggtaactttgaggcagctggtaacgctctatgatccagtcgattttcagagagacgatgcctgagccatccggcttacgatactgacacagggattcgtataaacgcatggcatacggattggtgatttcttttgtttcactaagccgaaactgcgtaaaccggttctgtaacccgataaagaagggaatgagatatgggttgatatgtacactgtaaagccctctggatggactgtgcgcacgtttgataaaccaaggaaaagattcatagcctttttcatcgccggcatcctcttcagggcgataaaaaaccacttccttccccgcgaaactcttcaatgcctgccgtatatccttactggcttccgcagaggtcaatccgaatatttcagcatatttagcaacatggatctcgcagataccgtcatgttcctgtagggtgccatcagattttctgatctggtcaacgaacagatacagcatacgtttttgatcccgggagagactatatgccgcctcagtgaggtcgtttgactggacgattcgcgggctatttttacgtttcttgtgattgataaccgctgtttccgccatgacagatccatgtgaagtgtgacaagtttttagattgtcacactaaataaaaaagagtcaataagcagggataactttgtgaaaaaacagcttcttctgagggcaatttgtcacagggttaagggcaatttgtcacagacaggactgtcatttgagggtgatttgtcacactgaaagggcaatttgtcacaacaccttctctagaaccagcatggataaaggcctacaaggcgctctaaaaaagaagatctaaaaactataaaaaaaataattataaaaatatccccgtggataagtggataaccccaagggaagttttttcaggcatcgtgtgtaagcagaatatataagtgctgttccctggtgcttcctcgctcactcgagggcttcgccctgtcgctcaactgcggcgagcactactggctgtaaaaggacagaccacatcatggttctgtgttcattaggttgttctgtccattgctgacataatccgctccacttcaacgtaacaccgcacgaagatttctattgttcctgaaggcatattcaaatcgttttcgttaccgcttgcaggcatcatgacagaacactacttcctataaacgctacacaggctcctgagattaataatgcggatctctacgataatgggagattttcccgactgtttcgttcgcttctcagtggataacagccagcttctctgtttaacagacaaaaacagcatatccactcagttccacatttccatataaaggccaaggcatttattctcaggataattgtttcagcatcgcaaccgcatcagactccggcatcgcaaactgcacccggtgccgggcagccacatccagcgcaaaaaccttcgtgtagacttccgttgaactgatggacttatgtcccatcaggctttgcagaactttcagcggtataccggcatacagcatgtgcatcgcataggaatggcggaacgtatgtggtgtgaccggaacagagaacgtcacaccgtcagcagcagcggcggcaaccgcctccccaatccaggtcctgaccgttctgtccgtcacttcccagatccgcgctttctctgtccttcctgtgcgacggttacgccgctccatgagcttatcgcgaataaatacctgtgacggaagatcacttcgcagaataaataaatcctggtgtccctgttgataccgggaagccctgggccaacttttggcgaaaatgagacgttgatcggcacgtaagaggttccaactttcaccataatgaaataagatcactaccgggcgtattttttgagttatcgagattttcaggagctaaggaagctaaaatggagaaaaaaatcactggatataccaccgttgatatatcccaatggcatcgtaaagaacattttgaggcatttcagtcagttgctcaatgtacctataaccagaccgttcagctggatattacggcctttttaaagaccgtaaagaaaaataagcacaagttttatccggcctttattcacattcttgcccgcctgatgaatgctcatccggagttccgtatggcaatgaaagacggtgagctggtgatatgggatagtgttcacccttgttacaccgttttccatgagcaaactgaaacgttttcatcgctctggagtgaataccacgacgatttccggcagtttctacacatatattcgcaagatgtggcgtgttacggtgaaaacctggcctatttccctaaagggtttattgagaatatgtttttcgtctcagccaatccctgggtgagtttcaccagttttgatttaaacgtggccaatatggacaacttcttcgcccccgttttcaccatgggcaaatattatacgcaaggcgacaaggtgctgatgccgctggcgattcaggttcatcatgccgtttgtgatggcttccatgtcggcagaatgcttaatgaattacaacagtactgcgatgagtggcagggcggggcgtaatttttttaaggcagttattggtgcccttaaacgcctggttgctacgcctgaataagtgataataagcggatgaatggcagaaattcgatgataagctgtcaaacatgagaattggtcgacggcgcgccaaagcttgcatgcctgcagccgcgtaacctggcaaaatcggttacggttgagtaataaatggatgccctgcgtaagcggggcacatttcattacctctttctccgcacccgacatagataataacttcgtatagtatacattatacgaagttatctagtagac

SEQ ID NO: 43 - protein, 24 aa, Foot-and-mouth disease virus
APVKQTLNFDLLKLAGDVESNPGP

SEQ ID NO: 44 - DNA, 143055 bp, Artificial Sequence
  Vector
tatttatttagtgtctagaaaaaaatgtgtgaccaacgaccgtaggaaactctagagggtaagaaaaatcaatcgctttatagagaccatcagaaagaggtttaatatttttgtgagaccatcgaaggagaaagagataaaacttttttacgactccatcagaaagaggtttaatatttttgtgagaccatcgaagagagaaagagataaaacttttttacgactccatcagaaagaggtttaatatttttgtgagaccatcgaagagagaaagagataaaacttttttacgactccatcagaaagaggtttaatatttttgtgagaccatcgaaggagaaagagataaaacttttttacgactccatcagaaagaggtttaatatttttgtgagaccatcgaaggagaaagagataaaacttttttacgactccatcagaaagaggtttaatatttttgtgagaccatcgaaggagaaagagataaaacttttttacgactccatcagaaagaggtttaatatttttgtgagaccatcgaagagagaaagagataaaacttttttacgactccatcagaaagaggtttaatatttttgtgagaccatcgaaggagaaagagataaaacttttttacgactccatcagaaagaggtttaatatttttgtgagaccatcgaagagagaaagagaataaaaatattttagtgacaccatcagaaagaggtttaatatttttgtgagaccatcgaagagagaaagagataaaacttttttacgactccatcagaaagaggtttaatatttttgtgagaccatcgaaggagaaagagataaaacttttttacgactccatcagaaagaggtttaatatttttgtgagaccatcgaagagagaaagagataaaacttttttacgactccatcagaaagaggtttaatatttttgtgagaccatcgaagagagaaagagataaaacttttttacgactccatcagaaagaccatcgaagagagaaagagaaagagatagttagtctagatatttttcttagtacaaaagtcaatgttttaaaatatatggacaagaatttgtctgtataaaaacttgtgtgaaattttgtaccaaagaaaaaatgtgagcagtatcccctacatggattttactagatcatttatataccaaaaaatattatacgatctacgttttattatatgattttaacgtgtaaattataaacattattttatgatatacaattgtctggtaacctagatgggcataggggatgagtatatgttgttggacgttattgtttaagaaatagttgatgcatcagaaagaggtttaatatttttgtgagaccatcgaagagagaaagagataaaacttttttacgactccatcagaaagaggtttaatatttttgtgagaccatcgaagagagaaagagataaaacttttttatgactccattgaagagagaatgagaataaaaatattttagtgacaccatcagaaagaggtttaatattttttatgagaccatcaaagagagaaagagaataaaaatattttatgactccattgaagagagaaagagaaaatgagaataaaaatattttagtgacaccatcagaaagaggtttaatattttttatgagaccatcaaagagagaaagagaataaaaatatttttgtaaaactttttttatgagaccatcaaagagagaaagagaataaaaatatttttgtaaaactttttttatgagaccatcaaagagagaaagagaataaaaatatttttgtaaaactttttttatgagaccatcaaagagagaaagagaataaaaatatttttgtaaaactttttttatgagaccatcaaagagagaaagagaataaaaatatttttgtaaaactttttttatgagaccatcaaagagagaaagagaataaaaatatttttgtaaaactttttttatgagaccatcaaagagagaaagagaataaaaatatttttgtaaaactttttttatgagaccatcaaagagagaaagagaataaaaatattttatgactccattgaagagagaaagagaataaaaatattttagtgacaccatcagaaagaggtttaatatttttgtgagaccatcgaagagagaaagagaataaaaatattttatgactccattgaagagagaaagagaataaaaatattttagtgacaccatcagaaagaggtttaatattttttatgagaccatcaaagagagaaagagaataaaaatatttttgtaaaactttttttatgagaccatcaaagagagaaagagaataaaaatatttttgtaaaactttttttatgagaccatcaaagagagaaagagaataaaaatatttttgtaaaactttttttatgagaccatcaaagagagaaagagaataaaaatatttttgtaaaactttttttatgagaccatcaaagagagaaagagaataaaaatatttttgtaaaactttttttatgagaccatcaaagagagaaagagaataaaaatattttatgactccattgaagagagaatgagaataaaaatattttagtgacaccatcagaaagaggtttaatatttttgtgagaccatcgaagagagaaagagaataaaaatattttatgactccattgaagagagaaagagaataaaaatattttagtgacaccatcagaaagaggtttaatattttttatgagaccatcaaagagagaaagagaataaaaatatttttgtaaaactttttttatgagaccatcaaagagagaaagagaataaaaatatttttgtaaaactttttttatgagaccatcaaagagagaaagagaataaaaatatttttgtaaaactttttttatgagaccatcaaagagagaaagagaataaaaatatttttgtaaaactttttttatgagaccatcaaagagagaaagagaataaaaatatttttgtaaaactttttttatgagaccatcaaagagagaaagagaataaaaatatttttgtaaaactttttttatgagaccatcaaagagagaaagagaataaaaatatttttgtaaaactttttttatgagaccatcaaagagagaaagagaataaaaatattttatgactccattgaagagagaatgagaataaaaatattttagtgacaccatcagaaagaggtttaatatttttgtgagaccatcgaagagagaaagagaataaaaatattttatgactccattgaagagagaatgagaataaaaatattttagtgacaccatcagaaagaggtttaatattttttatgagaccatcaaagagagaaagagaataaaaatatttttgtaaaactttttttatgagaccatcaaagagagaaagagaataaaaatatttttgtaaaaattataaacattattttatgatatacaattgtctggtaacctagatgggcataggggatgttgataagctcgacgagtatatgttgttggacgttattgtttaagaaatagttgatgcatcagaaagagaataaaaaatattttagtgagaccatcgaagagagaaagagataaaacttttttacgactccatcagaaagaggtttaatatttttgtgagaccatcgaagagagaaagagataaaacttttttacgactccatcagaaagaggtttaatatttttgtgagaccatcgaaggagaaagagataaaacttttttacgactccatcagaaagaggtttaatatttttgtgagaccatcaaagagagaaagagaataaaaatatttttgtaaaactttttttatgagaccatcaaagagagaaagagaataaaaatatttttgtaaaactttttttatgagaccatcaaagagagaaagagaataaaaatatttttgtaaaactttttttatgagaccatcaaagagagaaagagaataaaaatatttttgtaaaactttttttatgagaccatcaaagagagaaagagaataaaaatattttatgactccattgaagagagaatgagaataaaaatattttagtgacaccatcagaaagaggtttaatatttttgtgagaccatcgaagagagaaagagaataaaaatattttatgactccattgaagagagaatgagaataaaaatattttagtgacaccatcagaaagaggtttaatattttttatgagaccatcaaagagagaaagagaataaaaatatttttgtaaaactttttttatgagaccatcaaagagagaaagagaataaaaatatttttgtaaaactttttttatgagaccatcaaagagagaaagagaataaaaatatttttgtaaaactttttttatgagaccatcaaagagagaaagagaataaaaatatttttgtaaaactttttttatgagaccatcaaagagagaaagagaataaaaatattttatgactccattgaagagagaatgagaataaaaatattttagtgacaccatcagaaagaggtttaatatttttgtgagaccatcgaagagagaaagagaataaaaatattttatgactccattgaagagagaaagagaataaaaatattttagtgacaccatcagaaagaggtttaatattttttatgagaccatcaaagagagaaagagaataaaaatatttttgtaaaactttttttatgagaccatcaaagagagaaagagaataaaaatattttatgactccattgaagagagaatgagaataaaaatattttagtgacaccatcagaaagaggtttaatatttttgtgagaccatcgaagagagaaagagaataaaaatattttatgactccattgaagagagaatgagaataaaaatattttagtgacaccatcagaaagaggtttaatatttttgtgagaccatcgaagagagaaagagaataaaaatattttatgactccattgaagagagaatgagaataaaaatattttagtgacaccatcagaaagaggtttaatattttttatgagaccatcaaagagagaaagagaataaaaatatttttgtaaaactttttttatgagaccatcaaagagagaaagagaataaaaatatttttgtaaaactttttttatgagaccatcaaagagagaaagagaataaaaatatttttgtaaaactttttttatgagaccatcaaagagagaaagagaataaaaatatttttgtgagaccatcaaagagagaaagagaataaaaatatttttgtgagaccatcaaagagagaaagagaataaaaatatttttgtgagaccatcaaagagagaaagagaataaaaatattttatgactccattgaagagagaaagagaataaaaatattttagtgacaccatcagaaagaggtttaatatttttgtgagaccatcgaagagagaaagagaataaaaatattttatgactccattgaagagagaaagagaataaaaatattttagtgacaccatcagaaagaggtttaatattttttatgagaccatcaaagagagaaagagaataaaaatattttttatgagaccatcaaagagagaaagagaataaaaatattttatgagaccatcaaagagagaaagagaataaaaatattttttatgagaccatcaaagagagaaagagaataaaaatattttatgagaccatcaaagagagaaagagaataaaaatattttttatgagaccatcaaagagagaaagagaataaaaatatttttgtatgagaccatcagaaagaggtttaatatttttgtgataccctgaaaggaaataggaatagtgtcataatcgtatcacactattgagacagaaaaagaagaagtcgcgagaggtaactttttgttttgcaaaccggaatatagtgtccggtacacttttttaattcgtggtgtgcctgaatcgttcgattaaccctactcatccaatttcagatgaatagagttatcgattcagacacacgctttgagttttgttgaatcgatgagtgaagtatcatcggttgcaccttcagatgccgatccgtcgacatacttgacctcaagttcagatgattccttgcacatgtctccgatacgaacgctaaactctagattcttgacacattttgtatcgacgatcgttgaaccgatgatatcttcgtaactcactttcttatgagagatgttagacccgagtactggatgggtcttgatgtcgctgtctttctcttcttcgctacatctgatgtcgatagacacctcacagtctttccatcagcggattctgagatggatttaatctgaggacatttggtgaatccaaagttcattctcagacctccaccgatgatggagtaataagtggtaggaggatctacatcctcgactgattccacctcgggatctggatctgactcggactctgtaatttccgttacggattggcaaatcttatcatcggtcggtgtttggtcttgctttgtgactttgataataacatcgattcccatatgatgtttgttttcttcttccgtacacgatgaggatgattgctgaagactggcaggcacatgcatgccagtacgatatattgtttcatgattgctattgattgagtactgttctttatgattctacttccttaccgtgcaataaattagaatatattttctacttttacgagaaattaattattgtatttatgggtgaaaaacttactataaaaagcgggtgggtttggaattagtgatcagtttatgtatatcgcaactaccgggcatatggctacattacccacatgataagagattgtatcagtttcgtagtcttgagtattggtattactatatagtatatagatgtcgacgctagagttactgtctccgaatgcggcatgatagtatcattctttgctttcgttaactgtttggaggaagaatctttgttattgcatttaatctcgaaattcagagtgcacacctttctcctgtaaagaaacctgaagtcgctaccttattaagaagacgggatcgcagtctttatgattcatagtaatagttagttccgacgttgagatggattcgctgagaccggtagtggtcgtccgagtacacgatgtgtcgttaactggatacaggttaatttccacatcgatatagttaaaggtatttctgggtacgggttcgcatttatctgcggaagagacggtgtgagaatatgttccgagaccacacggagaacagatgacgtctccggatactccgtatcctattccacattttgtttgggaaacacatgccttgcatccatgatcgggagagcattcacagattctattgtgagtcgtgttacacgatcgcgtcgacattgttgacagaaacgtgaccttcattcttaccgtcgtccataaatacgttaggtatgtaccacatactgtcgcgaacgatgcgtccatctcataatgatttactttttcataattaaagatgtgaaagaaaaccgaacaatatatttttttagtaatgtttatgcgagacatataaaataaactccgtgtttatgatgccggtaaatgtttttatcatcttggacggaatcgattttgtaatatgccatggaaacaggacattatcactccatgataaattatttaatggagtcgatcctctcattgttctttgcgtatctcaatctgtggcgtttgcttcgtttaaataatatatcaaacatggagacgcctgatatgtaggcattcttcattctattaatgtctgctctatagcgctttagttccttatgacgaccggcgatatcatacttactttagaaggaaaatcatcatctaggattaaggcgtatctgatacaggcgaataatggttcaggatatagatagcgtatatctctattaaatgcgtcaatcatagtctctagagtgggatggtaactcagtaataaatcaactagcttctctttggtaactgcttttctggatggccgtattgattatcgagcgtgacactcgctccatattccaataaccgctttgcaaattgtatattattgacatcgaccgcgtaatatagtagagttatcgatcatatctatatcatccatgtacttgcttagtatatcaaatacatcttcataacagtgatacccgcaattattaaatctcgataatatcagaccgtacatacatagacggccattgttagatatgtgatttacagccgcgtgtccatattttccacgataaaccttacgacgtttacatcgacgagattattattaacaaagttgttgtccgtcgtcttatccaacatgcattgaatgataggtatacttaccatatcgccgtaatgtaagtagtttatcagtatggcttgtacgatggattcatcctgttgtctaaatctctttagaatgttatcgatgatgtagtggttatattctctggaatcgtacgaagtaatactacgcattacgtcgacaagagtatgacgtctctcaataagaagattaacgatttccatgtctacattatatggggttactctaaatcgcttgtttagataatacgcctctaatatagggctgacgtcgtatactctacacgtgtccacatcctttattaataatctctatatctatggttgagcaagaccagtagtattggatggaaacattgttatcgatcaaacatttaattacatccttggatagagattctctatgagacgatatatagtaatgaagagagttcttacacatatcactgttgtacatacaggtacgaaatacgtaaccggtgctgtaacattctgatttaagaagccatagcaatacttctggtctcggattaggcgtcgttacgtatatatccaccaatccgagaccattgattgcataattcgtattcttggacggacgtatccgtttatccacaattaggtattttagcagacgtaagtcgaaatcatttatattcgacttgagttcgttagaggaattcgaatagctggatatcagtagatgcacaatctgagattttacgtatctatgcttactgtatgctcctagcggagttaatccttcgttgtttctacaaagtctctcgactccgcgagagagtaacagtcgaacaatcttaatgtctgtatcgcatttattggagacgtaacaatgtagcgcattgtttcctcgtctatctatatgttttgataagttgtgacacgtttcaatttctagttttatttttttgtacgtcacatcttcatccagtagacgacatagaatacatgtgcaatccatagctattctggtgctaattattcctcataagatgataaaaagtgtagtgagagagcatgaaggagatttagtatttagcagtgcggatatgatccaagagggtgagatagtcgttctcgttcagaatctttcgcagcataagtagtatgtcgatatacttatcgttgaagactcttccagagacgatagctgattgagtacaaagtccaatgattgcacgaagttcttcggcggttttcatggagtcatttaatgatctccacggaagtgaatccttcaactcaccaccaaagagctccgttgcatcagttctgaaagagatgagaagcctgtagagagaccctgcgctttctctatgggtccatctatgagaaacccacaggatgtattcagtcagacaatgtctgacgtcggccacggtattcagggagtccttagtagcgtggcaatgacagggtctgaactgggcacaaggaaaggccattgtaaaggtagacctgtagccgtttatgctaatagagggctttaatttccattttttaatgggttgtggatgaggaatgagagtgatatcatattgagatacgtagttatgtagaggtgtatttcctatattatttactttcggtttcatattttaccaactctttaataaatttcttttcacgatgcatcttattaaatgacgttttctcataagtggacatatagatgcagaagtattacctctatcatctacataattagggtctgctcctaacttatacagtacgtagtagtagtttatcggttttaaatcaagtctagaatatatagtggattaatatatttttatattagctaaagcatatcattctcaacttcatcatgagttaaatatttgtgtctactagtttgtttatatcacagcattctacaaacagtctaaacaatagagaagacggacagactttaacgtataaatgacacatgttatcgatattcgttgataaatgattctaacgacatctctcgctagagataaaatctagtatcgtatcatactcgcatagcatagtttttcataattaatacaatatttaaaagacttattcggaaagtattttaatacatgtatcatcgatggagatccatatgaggagtcacttgtagttcttcagtagtgctatcatcgatagtataattatatgttgttgtaattggagtaactgttggtagttcttccgtggaatcaataattatactaacagcaatagtataattatataaatatgttccgttgatatcacatattttaatgaactcatttctaaagccgtacatccacatctattaggatctgatattttacacaactgtttaatagagtctacatttatatgttctctatcggtgagatacaaatacctagatagtcgcgttatagcacaaatacgatataaataataataataattattcagtaatgtatataaaaatgcattgtgtatttactccaatactactgtagttgtaagggttttttcaaaataatagttgtgtccacgacatttatatgtattacctatatattcttcagtaacattttcaaagtacaaggtcgcctcggtgataccgcctctactagttaaaacagagtatacatcaaaatcgaatcctataagccatccggatggattttcccattcaatcagtacatcgtcaatcaataatgacgttgacacagcagtgcatgttatattggcaggttctcctatcgttacgttgatttttggatctagtattagtttaaacctgtggtcttgcgacggtataaccgtaagtattttacatcttgattctaacgtcgtcgtaatgaacgtaacagttgtatcttccactatcttctaactctggattatgaataattaatttctttcccgtttgtgaatacttaatatcgtcgatattaatttccttattatctttataccaagttatattattataatgttttgcgtaaagaattccacagtataagtctatgccatacttatcatgagtacctagttcatatgtttttggaatgcatgaaggaggttttttaatatgagatctaactataccctgaacacagtcaccattctttgtagttacggtacacaaatacctacggttactgaatttagatgtatagttggctatccataaatcaccatgtttaacacgtttattagaaacctgtcgccgtctatttttttctagcctctcccatttaaccacatagtctttatatctgtgcgataaaagactgtcttcaataggaggacactttgcgctgaatggctctcctagagcggctatatcattcattgtgcctccgaacatacatgctggattcaaccatttagagtctttagctggtagagtatctctcattttattgaagaattctgtgatttcattttcgatgtctatggcgtaactgtggaatagcaataacaataatgatacgaaatatatatgtaccatcattttcatcgtcatcttcattatacggcactaaaatatttatataatatcagtttttttacacacatcgcatgagaaaaatacaactatactttggtaggtggatacgatatattataaagatcgttaattgtcagcatgtataatatttcgtatataatttctgaaggtagtaatgttagtagacaatttttatctgtgaaaacaggaaatagtttatcatatacctttgacacgtacatatctttataatatacattaaggtatctctcattcataatattagaatatattttaaaggacttatcgttattatatttttttaactcgttgaggtatcttcttaactttttcgaattatggcatcttaaaactgcatatagtgtagtgtctagaacagtggatagtttgagcaatattgtttctttatgacatttagttattataccatcgtatttatcaaacgacatgtattttgaaaatgcgtatcgatacgttttagaattgcgattcctaacgtgtctattgtaaaatgtgtcatctaaaagtatacagtaggatatgaatttctcaaatgattttatatcgaagataggtagagatggaagttgatccaccaacgatcttatcacattcttatctacaatatatctaagtatatacagtaaacaattaatggtatatggggaattttctttgttatctataatgagttgtgtagcgtgtttgttattgtcggttaacgcatttatatctccgttgatacgtataagataatctattacgtgtgtattattatattcacatgctacgtgtaataatgtctttccttcatagcgggtataaatatctatatttttaaacctattcatcaaataagttatcgaatctgccggacgtgtagaatatgttttgataaactcgaatacgattatacgacgctcatctatcggcatttctccaacatttgtttcatagtgatgtattaacataacaagaatatcgtgttgtatgtagtcggaagttatataacatagtataggcgttaatccatgattattacatattttgaaattcggattaaaagtcaacagcattttagtcatatgaatattattacacatttcaatactaagatacaaatggaatggtgtattaccacaattatctaacgcgtttagattagctccatgttgtataaacaaagaaataattcgcttggccttttttatcgttatcggttttctacactcacctggtttataaacgtgtgcgagacacaaataataataatgtaacgctgtatatccgtcttgtttaaagttaggatcgattcccttatctaataaagtggatactatgttctcatcgatatcctcttccttcaataacatgtaacgagattttatatactctagtagtaggttggaatagtctctatgcgataagtggtttttatctttgtctatcatatctatcactacatcatgtgaaatattacaacatctagtaagcaatatataaacaggcatacgtccgctactggttttcatcgttacatccactccatgatttaataatatcttcagtacatcgtttgtaaagtaattattatacaaatagcagtgtagtgcagtatacccagttacaggttgtcgtctgtttagatcatagtttttaactacaaaatcaagttctgtagaagtatggtctatattgcaatgactaaaatatgtatatatttcattctcttgtattttatgagttgattcgcggttgatatttaaaacataaatcagacgacgactcatttttatgatgctttgtggtaaaagtcctcatataattgtttaatattcattattatagacgattcccattaactaatctaacatctttgatatacccgtaaatatgtaaatatgatcctaaaataacacggattgtaagatgtctagaaagtttatgcaggtgtatgaatatgacagagagcaatatctcgatgagttcattgaagacagatataacgatagttttatcactagtccagaatactatagtgcggaaaaatacatgtgtagatatactacactaaatcacaattgtataaacgtacgacgatgcgcgttagactccaagttattacatgatatcataaccaattgtaaaatatataacaatatagaattagttagggcgacaaaatttgtttattatctggatctgataaaatgtaattgggtatctaaggtaggtgattcagttctatatcccgttatatttataacacatacaagcactagaaatttagataaagtctctgtaaaaacatacaagggcgttaaagtaaaaaaacttaatagatgcgcggatcatgctattgtaattaatccattcgtcaagtttaaactaacgttgccgaacaaaacaagtcatgcaaaggtattggttacattttgtaagttaagaacggatataacgcagatagaggcaccgctttcgggcaatgttttagtttatacatttcctgacattaataaaagaattcctggatatatacatgtcaacatagaaggatgtatcgatggaatgatttatataaattcttcaaagttcgcgtgtgttttaaaactacatagatcaatgtatcgcattccaccctttcctatagatatctgctcttgttgttcacaatatattaacgatgacatagaaattcccattcatgatttaataaaggatgtggcaatttttaaaaataaggagacggtatattatctaaaattaaataataaaactatagctagatttacgtactttaataatatagataccgcaattacacaagaacatgagtatgtcaaaatagcactaggtatagtctgcaagttaatgattaataatatgcatagtatcgtgggagttaatcatagcaatacgttcgtcaattgtttgttggaagataatgtataaaaattcttataaactcaattgacatggaaatgtaacaacatacattcacgttatactaacagtaactgttttgctgatgctaggaatagtaaacgccatacacgtaaacgttgtagcatcttcttccttgacaggattaatgtttaaccgggatgtaataacacgtctcttatcggtcatatagattttatttgctacacttattctaccgtctccgtccccatcatcttcttcgtaatacataccattacttatccaaaagacgtctgcatccgttgtgggaggtctcaacgatactctacacgcaatagtcaaattactacctattgaagttacaacaccttctggtaattgcatagtagaaggtattattttatcccgtacctctaattttacaattctggttacgttatatgttttgccaccgtatatatattctaaaacacatgtataataaccagcatcattttttctaacatcttctatggtaataattccaggtgtccgttgtttaagtctcttatttctaaggcgtcgatgcccgctccatataatatctgcgtttacgttactagcaataaatgcattaatattgggacataccatttcgccagtagatctctcatttactatttgtggatacgagataagatctatatttgattctgagacagacacgattgtcaaatttaacgacatcatgtcacagtaggtttcgttcgtggtaatgcatatataaataccagagtctgattgtgtcgggttcagaattagcatattgctaccattatctatcggtataattctatcattatccgctcctcgtttttcccataaaatatctaatatattatatccggatgatagcgtatttatttgaggacatggtaagattactggctcgttttctaactccatgaatgatgcaaaatattgccctttgtcgatacattcaggcgcgttaaaagtctgaacgaatgaagaataaaaaaatatagaaagaaatataacaggtagtatactcattttattttatagtgggtaaaaaaagtttgtttctgggaaagggagaagagaagaaagaagaaaatgtcaagatgtacaactcatcaattcatacgccggaatatgatgttataatccacgtaatttagcatctcaagcatcacaaacaatgcgttcagactgttactagtgggatggtcttcacctccccagtaagtagcagcatatgcacaaagtccgatgatggttttttgctcatccggtatataacaacggatgatttctacacaatctttgacatcatcccacggcatattttttaccagctcgcgaatgtcgatgaacactaattccgcatcatctctaaaagagaggagtgtggaatacaattgtccagcgcattgcctgttgcggtatgcataggacgaccaataaatatattcagtcaaacattgtttgacgtcatcaatactggtcagtctgtcacatccacagtgctgtggtgaaaagacgtgggtactaaagttggccgtcatcttaccaattgcaattggaagaataacgacctgcactaataccacatgttttttctatttttttaaaaaaaatggttaacaattagttgtcggagagcaatatctaccaacgaaaaaaatttttccatcaacatgcctaatcacatagatgaacggatgatctacacagaactcatttgtaattgttgatgcacagtctgacaccagtgcacaagttgctgcagctgcttctgtatactcttcattgacatctatatacgttttgtggatcatagcgtcgacactcacatctaaattacacatattgctataatctccagttgaaccgaacacctctgtcagtcctgactttactagagtatccaccagattatacgagcctgttaccttaaacttgggaatgtgaacatcgataaacgtagcttccagagagttacaccatttcttaaaatttgtatctgttagattttgttctatggattctaatccatcaatcttgtctggaagaatgaccatcatactagtatctccaacatatggcagttctatgattgaaaagttaccgaatgattcttttacagatgcgtgattaaatagctcgccgtacatagacatcatacttacgtctaccatttccgttggtgatacgtaaaagggataatcactggtaaattccttttcgaatggcgtcaaccattttgctttaaagtatacggcactaattgctaggagacaattgttcatccaatagtggattgattttcccctcagtaaagatatctacacacttgttgattgcatctatagtgcgacaatcagtgaagtcaacagtttgaaacttatcgccaatttttctcaaaaaggaatctttaaacacggcagaatatcgcccatatactttattcatggatttgaatgagatattctgagcgctaaccttatccgtgttctcctccttttctacatattttgatagctgttcagcagtggatccattagctccataatacagtattgtcaatactgacgagattgacgctggagaaatgaatacattctctcctttcatagaagatatccatagtaatcgatattggtcgtgtagcgcgatagagatagtctaatattaatattagatatccgtaacactaccacactctataaaaaaagaatatttcaatcttgtataaacagtctacgtagtctgtcataattaggagtttgagaataatctaacgtgtatactaattctatatatctaactaattccagaggttcatttccttcaggaaaacagtcctcaaagaaagtagctataaattttttatattcttttttttgttttattacttttatactactttcgtttttccatggaagtttgccaccgaaccattctatcatgcaatatcccaacatttctaaatctcctcgttttgaaactgttgctccaagatgattgtctacacacatataattgatatttcctgaagttatcatgtcctcgttgtaatctatatgtgagtttccactcttgtatagtttgttagttctagaatagtcaattagtgaaagacgtttatttctaatcagtatattcctcggttctatttttccatgggtaaatcctcgagagtgtataaactctaacgtgtttatcatagtgacgcatgcttcgaagactgattcagtatcctttggggcgaatactcttcccaaattctttataacgaagaacatataatcatcggtttctccaattccatacagatctggaatagccaaatactttataccacgttcccgtgtccagttgtcgatagtcaaaggatccaatacagatatatagaatcgtatttcagacaacaatggcttgtgtgatttgtgatctatcttcattacgtaattgtagaacgaactagtgaaattttttctgaccttatagagtattgaattaccagaatataaagtatttccgataatccatttcttgccatcgttatcaaaacaatacttgaaggattccatgcctgctatgtaataacgagttgttttttatgttttgtattgattataaaaattagtagatatgatctatattcctacatcgtgactgatacattctataacttctttatcaatggaatcactattactacttgtattaataacgagtgcttctctaatatattcattgggatgattcttgttaatgtttttattattttcaatttctacattttttagtatttcttctttctctctatctatttcattcatgatatcttctacatttgtaacatctgtatctgtatccatgttagtagtaagcaataaaactatagggtaatactgctatacataaaaactatttatattttcattttcaatcaataaggagaagttgataatgcctttatagcggggagaccatcatacttttccacatatccaatgtccttactaaatacatagaagacgttatttagtttacacaatgatgatatggatatcttataaatagtatatgaaatatcaaaccacttattcgttctaggattgtaacaagatatctcgttgtttttctctaaattaccatattgttcggtaacggatagacctccggcaaaatataacattccaaatgtcgagtcgatgccgtgatataccctagccataggcatttctataatcgaccattgtttgtctttataaatgtcaagtttttccatattgttaaccacgatcgtgctattagagttatttatgaataatccgccagttacgaaaatagtattattaacggaaacagcggacacattgctttttttataatttatcggtgtttcgtatatccctgaatccattgccttcacttgcagttgggagatgaacactgcaatcagttctttcgggatagaaatctttggcaattatacacaaccctattttcaatccccatgtttcctcttcagtcttctcacatcgtctaatagacatggagtagatgatagaggggaacagaaggactataatcagggacctcatcttgaaaatggttagagcctataagggcgttaaccagtgtataatatgcagttttatttcgtttttgtatcattaataaaaattagttatgaatatttagtcaagttaagcatgctaagaaaagtggtaacatcatttgatgtgctaccgagaaatttagttaaattttctcttgataactctggccattttgtccttgaaattgggaacatcttctttggatctaattgcgcatgtatatacactctttttaggtgtcagacatactttcgaactccatggagtaattttttcgagaaacccttctgtggctccctgtgctgtcacgcacactttttctgttgtgacaaagtctatgctgcaacctgtagacgtgcaatcgtagtcatcgatatcatatggtactggttctttagaatctccgaatgtgaagttagccgtatacaacaagtagatatcacacatgtcaccgcgtttgtaaataggaatctttttgctacctctagtagcatacggatggtcgtcgtattcagttaatgttacagtcggtggtcccgtacaatactcttccactttataatcgccttgttcaaatttaacccagaaagatacgaaatcattctttggaaatgcggatatgtcgtatgttccttctggtacatttgtatacattgtttgccacgtcttgatgccataatttttaagggatatattgtatagaccatccccagtccattcaattttggaatcaaaattgacggattcaaacttataactagttattttagcgtgtatactattaatgaacaaaactgcgagaattataatatatctcatggtgttgtttgttatttgactactgtcactgaagtgataatatattttaaatttttaaaaatcatattttgaataatatgtattactatgtccatgacgatcaaatatataagtagatccaattttaagagtatgttttctcaatagagtatcatcgttgatcatacttatttcatattttattcctttatagcattttccctctgcagtaatagaatattgtcgctcatcaccatcatatttgtgaatataagggtacttatcataatggcatgataatttggtagatattctacacgtgtgacctctgcgttgaatagtagacatatcaataattttatagtcgtttataacatctatatctatggaatcaaatccgacgtcgcatgactctgtaataatagaaattgtgtactctttaaaatttaacaccaattcattattatcatcagtatatgaattttctatattatctactccatctatatagagttttacactcagtttattaaacggagtgtactcattattcgaataggatgctaatgcacctattacaaataaaaacgttattagttttttatacatttaaaatcttaaaattttaactagtatattgaaataattatttatacaaactaactagatgcatcaacagataataacaaacacctccagcgatcgtgccaatagtagttagagatgcgtatccgtacaacttgttaatcatatttctacggatgtatataccatcgtcgttaaaagcgcttctatatctctcattagctagaattatagatacgctattaattatatcatacattagttgattgttgatactatttttattgtaatcgaaaaacatttccatgaatagtattccggtgccaacgcttacagaaacatcgcgttcattcatcattataccattaagtgtatccatcacccattgtttaacacgtgattcatttggcatagtacgtactatatcatcgaacggtataacggcgcatcttgtaaatagcctgtatatattatgtaatatggcgttacttcttccatacacaataaatctcttgttataatagtgcctgagtaaaaatgctctaacggcatcgtagatatcaacatccactgaagaagacatctcaattgattctagctataagtctttaatcttttgatacttgtttgttattaaattattaattattaattattcattattttaacggatttatattcacggtagcaatttatggaacttatattggtcattatttttgtcacaggaacaaactaatactataacggagattaaaaatatgacgcccataattgttaacgccactatgattatatgataagttgcttctaacgattctatttcttgttcatattgtacaacgtctttcgagagtttgctcaaatctgtctcatcgtcgggaccatcatccactggatcaaatttttcgttagatcgtacacatgttgggagtatgggattccatttaccgtcgatacatgtggatgatggagatcccgttagtataaaaccacttttacaactaagatgtataacgccaccgatagaaaatgtagatccggaaattaatccattagatagagacggtatatcacatttttgttgacatgatggaataacattccaagaattagctgtacaacttatgtacgaagcaccaataacctcatatccaacatcacagttgatagttatatattccccaaatgagtatttttctttaactggttgacacgatccgtgttctaattgaagaggttgacattccgcattaggacacgtaacagtatcattccaagaagtatttccatttttttcttcgcaacgaaaatattttgtttcgccgttgcaacttagtgtcatggtggaattcacttcgtatagcggtttattatatagttcagagatgtaatcagaaactgtgcacatttttttgcatggattttcgtatttccatttatctgtttcgcagacagcatttggatccgaagaatgatatccctgatcacatgtaaacgtaactttctggttattattaaacgatgtttcggtagacgttaatttagcgttattcatagtgggtacagtacatgttgaataaacaacagcaggtagtacgcataacaacgtaacaacggaaatcgttttcatttttatttatgagcgttaaaaatagtatacactgtcgagcactaaaaggaaacaatgatgtagtgtgattttatattttaatagtgtttataagatttttagatatgtggacagttcgttatcgttatattttatttcgttaggaaaacacgaccatttatctccaggatccagcttcttggataatagactaattaatctctgacgatatctaatagatgctatgatattacgtacacgacttccgtatacgtcgagactagtgcacttcacgaaagaaggatgtttaccgtatctcattaaagtattaatgtctttgatacaaaaaactaattggaatacagttttattttttatataacatctcttcatgatatctatttcatcgaaacatcttaaaatataccatttatattgctgtagtgattgtacatctataagagtatcataatcggtcatacacgcagtatattttatacacattttcaataaatctgcattatgctgtttatgtttagtaattgctatcatagactgtatcataattttcaaagatggtcgtttagacaatagtacttccattattattttgttgttgtttgcgactgcttccgaaatacatgtacatccactagtagtaatcgtctcaaaatcaccatttctgtttaatagatagaccaacgtattatacgcattataactgacagcgtcgtaaatagtacgatagttaatatcaataactcctctggataatagataatctaaagattcaacagcatcaaaaattattaaatgacgaactatatgttcattatctatttctaactctgtgtctgattccaaatatagttttataagcgagataccgtgtataattccacaataaaatggagtagttccgaatttattacgcgcattaacatttgctcctttagaaattaataactttacaaaatcatatttattacgacatgagacataatgaagaggtgtatatctattaaagtctacagagtctatattagcattctctaaacatatctcaaacaattccacgttgttgatatcgtgtttacataataggataaaaggtgtgtttccgtacgtatcttttttatctacatctgatccattatttaacaatatcttaattaattcattgtatgattctgattctgattctgatttcttatagtgatatatacatctatgtaataatgtacaaccgtaactgtcttcggcatctatataaaatacatatatagatattaactgtatctgatatataggacaaaaaatgtcttgttctacgtccattttcaagcattagtcttatcctattatctggatgatcattattaactaattgatatacatattcttttatattaatggatgatgataacctgagattgtgtataaatgacccgttcttattaatatttaatactctatctagaaaaaaaattataatattcgtattagcatcatccatagaataaatatgtagaatattttccccatattctaaaatatggaataaatttggcaacctagataaaaaatcaactattgttttatccactttctcgtatgttcgaacgagattataatcctgtattatatgggatgtggaaaaattggaaaacacgcgtgctatataatgaagagataaatatacactccagtcaagtatttcctttttaaaaaaaatccatatataatttatattctgtaacatgttatcccttttcaattaacaatgttggtttataaaaaattaaagaagcgaatcaatgattaatagatgttaagaactataattacgatgtattaataggtatagttagttagttaaaaagagataacagttactaattaattgttagttattgtctatatgatattacaacctattatttgttctctatagttacattaattaaaattttatatgtgacacctattcatctggagaatacttcttgataccatgattctggccaatctgcaaacacagcacaacagcatctttccactttgatagcgcacacgtatgtcgaggtagcctcatccccaggtttatataccttgatgaatcgacacgtgtacttgatgtcctctttcttctcacagaaatacacaacacaaagtcttttgatatgcttttctatatcattctctatcagtctgaggtagtcgtaacccaccgtgaatccaaatactttgtgtgtattattatcaactccaatgaacaaatatccaccctctgtgttggcaaaagatgagagtatacgtgttcttagttgcttagctgaaacagatgtatgtttaacattaatagatttaccagcctgaagttctgatctattgaagaactcctctaccaatctctcaattgattcagtgtcttccactccatctggatattcaaattcctgcatttctggtctgggactccatccacctgattccttcagttcgctaagatactcatttgaatgcatgatcccatagtcttcatgtacaaatttgtttttacagtactcggtataagattttgattagacaaatgcgtatgcacataacagcattctttaccattcacaatatcaaaatgatcatatacaacagaccacatatggcgtatagattccaaacgtttcatgagtacatgattcacactgtcttccagagaggtggttacctcgatggtgccgccgatatagtagaagaaagattttctgtatcattctccccaagtttaacttttaccagatttgggatcggaagcaccgcaccctttttgaatctcattctcataatttcctttccatgtacgtccacagcagtaacttgacagatacaatctcctatccagacgtggtaatcgatgataggtcctgaactgagtgcattcatttctttggccttctctttgatagtagaataatcatgttgaacttttccatatacagcgttttctgtttcaagtacgtgatgatgaatccctactccttccaaacacaagtctagactctcgtacccgattccgcttagagcatagtagtttttgtggcgatatgtgatttccttcttgatcatggatcggatctccaatttgtagatattcattgcactcaaacataggcagcagtgctccaatatatctcttgttcacctgactgtaacaccacatatatttgtcttttacaatgtcatacttgttattataaactgacatcattggcaacagtcgatgatattccaggaaaggcatgaagattctcgtcgtacccaccgagagcgtgtgcgtaaaacatcgccatgatttcggttgtacacacgagatcaataataaattaagttattttttaatttttatcgacaaaaattttacatcaaccaaacaccacacttaataatatacaccctgcattaatatgtgccgaaacttgtcgtaattgggttcctcaaaatatgtcaaagagtttaccatggtaatatattgcagcaattctctaggtgcatattgcaaactggtcattaacaaagtcgcagtattgttaacatatttctgttttgtggcacttactaatgcacaattctttgtttcagatatcttagtccatggcaagatacctcccaaccatctaatcatacaatatccaagtgtttctagatctccacgtctagatacaacgtatcctttatgcgaatctataggtgtaaattctagagtaccgttatccattttatttggatttcttataaatggaacatgttcgccattagacatgaatttagaaaccaatccgtaatccactagatataatttattcttatctatttgatccaagactatattactcgctttaatatctccgtgagaatatccttgctcgtgcataaattgtatggtatttaagatttcgattccgatcaacatcaccgacctttttggtaatctattattattggctctgatcaccgcatctagatctgcacctaatctattaattaccaagaatcgatattccacattaatggatttgtatagaccaaatgccttgcacgtgataagacctacgtgctttatattgtgagattttttccattcttcgataacggatggtttaagtactctagtataaaatgcctgttcggtaaataatgatccgttagctttgggctctatttttactacataattattgtcattagtagtataaatactaccaaatccaccttttcctattaatggtccaacgacccattgatttttgcaattgtcagttaacacaagtccttgaaagttcataatgtgtgatctatctgtcaatgaaatatcattttaaattttaagttttacgtggtaagttttaatatttaactaatacattagacgttgaaatagccacatataaaaacgagttatattattaattatcaagttttaagtcttaagtctctaattagtgttaaaatacattctaatacggtcctgtagtatctgaattaacttactatatgctaaattcacatcatcttcaatgataatagtgtcgaatagaccggcttcacctgcctcatccatgtcagtttttgccaacatcacacgacgatgaatctcatcatccgcttcagtgtttctacaacgaagcttggtctcaaccattttaagagaggtaggtcttatatacaccgagtaaggcattaggtaagtatttttaaaacttctaacaccgtcgatgtttagatccatcacacaaatacgattattaatagccgctgtattcacagcagttttagaagttccgtaaatatttcctaaaaactcagtatgttccggcggctattcccttccagatggcctctctgttaacgtaatggtaatcgacaccttctcgttccataggacgaggaaatctagtggtatgggacaccacaaatccaaatatattcccatagtcttttggctatggctgtctttcctaaaccagatggcccgctcaatatgatagattttactatcccagacatttatgtaagtcaaaaatctagactttgttctctgttttgtatttacgtgaacgtttattatatatataatatgtaatacagaatattgccacggccgacaatataattaatgcggtaataccaaatatttctacaaagtccttggttttataattgctaatagaggttgtactaccgcctacagtagttgatggtactgtatcattatcattgtacgtatcataaagatccgcatcatcggtggttgatttagtagtgacaattccagatgatgtacttactgtagtgtatgagacagtgtctgtaactgtatgatcttcttctttatcagtaattggttccggagtctcgtctgttgtggattctccagatgatgcacttactgtattaatgctatcactagtgtatgtgacggtgtctgtatgatcttctacattatcagtaattggttccggagtcgcgatttcgaataccgacgagcaattagaattatctatataatcaggtttctcagaactagtttccggtgaatgtgtagatccagatagtattatgtctatagtcgattcactatctgtatttacaatcaactctgtggagtattcttcataatctactttatcagtgtcatttgtaggcgatgtcataaagaatgcacatacataagtaccggcatctctagcagtcaatgatttaattgtgatagttgtaactagatcatcgtatggagagtcgtaagatattttatccttggtataattatcaaaatacaagacgtcgcttttagcagctaaaagaataatggaattgggctccttataccaagcactcataacaacgtagtcatttgtattatttcgattacatgataaagttgcatcatcacctatttttttagatgtctgaggaaaaggtgtagcgtatactaatgatattagtaacaaaagtattggtaatcgtgtcatattagtataaaaagtgatttatttttacaaaattatgtattttgttctatcaactacctataaaactttccaaataccagccaccgaaagagcaatcttaatcatgtcaggttcatatttccccaacatactagatccaaattcgcctacatcaggtaaattcatcataatacaatgtctgttcatatcacacgatgatccattgagcatctcatctctatcaagaatcctaatctgtggttcaaaataacagcatctacactcatcgttaattgtagtattgtctaatatatttttgctaatatttgcgtaagttctattatcagctattgcatgcatcacagatccatcaacaaccatatataatatagaacaatagtcggactttatacttatgtaaaacttgaaccaattggaactcggaagctcgtcatgtagacgctggtgtctagatataataacattattatcggttacacttcttaagagaggtgccgcatcgatagagaaatcaaacaggagaataatcaatgatgcatttcctttggtaaaaaaggaaacatccatgggaagaatggctactttatatgaatttaactctatacacgcacacgctttatcagatgagattaatagttcacaaacatctctatcctttcctatggatataataacaggaatggcatctttaggtttaaaataattatatacaccagtaggagtcttgtcatcgtcatctatctttatcaaattagcaaatctggatattcttgatacattctttttatacagtgaattgcatacatcggataccgcattatccatatatggcaaatctgcaatcactgtattgtttttagattgtccgccaatgtgaacgttcttgactttttcacaacatggtttaatcatgaaatcattttttatatgatttatttcctcgccatgttttactaacgcgtttagacagtatacaataacaccatccatggcgaccaccaactaaatagtgttattttaatttgtatgtaactattaagatttagtcaagtttactaaatcgtttagatgagtagattctttccacgttttatcctctcttatcctagtaaatctaggaaatctaatggatattccatttgcggtatgggacttggaagatgtaaactctgctcctgaaatttcccatatctgagattgttttggatcctctactacaaaatcgggaatatagattttattaactactaaccactctggaatttttttgggatccttgttaattttaatcatctttaattggtcttgcaactcccttaacgtattatcatcgtgtcctgaacacttggtaaccgtcttccatttaccggattcatcgtcgtaacaacccattagaaagactgccatgataccaccctttgctcctttaccatagtaagcacctagtactactaaatcggcagaatctgccatggaaccctcgttcaaatagtctcgctttatttttaaccatcttctctttcccggttcgtatactccattaatatcttttaagaccaatccttctaattttctcgttagtgcatcatccaatacgtcagttaactgagactcgttactaatattcgtcaactctgagaatactattctattgggtatttcaaccataacatctttgagaaaagatcttcgttcgtacaatggaatgtccgtcatatcgaatccatcaaagtacaaacagtcaaacacgaacaaacacatgttagagtttttatattctttctttttgtgtatacctaaacttccaaacgggagcggtacattatgttcgtctacaagaacaatttcagaatccaatacgatagacgtagcttttttaaatgctttcggtatgtattctttgagataatccactttatgagagagtactggtttcatgtttctactaaagaaggcaaactcgttattatttttatgaacttgtactctttcaccatcgtatttgacttccgcaaacattcctgatggaaattttttaaacgccttattgacagaatcacacgattccgctaacatgggattaattggagtcataacagaaatagatatagagtctagattttgtttagatgcattttctattatctctttcaagttattagattttctaaacacatcataggcatgaggactaatagcgttaagtacgtaccgagggcccgctttaatttttagatctttatcaataagcatgactacacattttaaatcattacatgtacaaacggatgcgatatcagtcaataattttatttgatgcgattctttagttacggatgataacgtagttaaaaaactatccacttcttctaaagttaaaatgcttttatctcgtggacggatttctgtgttctctttgaagaaagtcctaatagtgtctcctatatatccgtatcctaaatcttgtagcatatcttcctgagattgtttaaatattatactatataattttataatttgtttatcgttcatgttataaattctatcgtctaatccgggaagcaatagcttaatgatcaaatatttatcatccctatctgttataaagtctctaattaatttagatttttctttatatcctgatgcgtgatatatatcacagcataattttctaaattcgcgaagcgacgtcatttaataaaaaaagtatttttttttaatattttcacaaatatcgttcgcggatattattagacaattgtagtatattctcacgtatcacttgtttaatatctatatccgctattctggaaccgagtacttcggcatacgtagttttaaaatctggattattcattatatattttagagtaatgatagcatctactatattttctaggttatccttataaaagctcataaacttgttaactatacaatcgataatttcattgtcgtctaatgaattaatcaattcggtctgatagatctcttgatctataatagtatatacagtatctaggaaagagataaatggattatccaagtttgatctacacatgataaaatttacaatgtccttgtttaatatatcattatctatagtttctatcttggcaataactaattgagatattgatgcgagttcggtatgcatatcggacacgtatccgagtactgattccaagttgccagagtaatatgcttcatccatttataaaaaatgtaatttcactattacatccacagttgccccactggtccagtaaccgtgtgtatagcctctataactatattcttaatcaactccttctttacatcttcctcgaattcagaagaaataatttgccaatgaatatctccttcttcaatcatttttttatattcttgtaataccttttgttggaatgtaacatcttcataaatttcctcgccgacgtttctattaatttctttgctaccagattccaagaatataactaagtcgggtttaggcaatccagattcataactcttactgagagtcattgacgcgcctttagcggcggcatacgctactccagagaatgcgtatctatcaactattaaagtaattccctgttctagttgttcttgtataaaagatgcaaactcccatctatttgcacaaaataatagattaactatatgatcattataggtttttttacgagttagatagtcatctatcatctttccagtgacagtggatctctgaggaaagttaagatattttatcgtgtttgccggtatagattccatgatgttcatacattgtgttgtttttccagatttgtccaatccttcaaaaacgattaatgccccacgagacatttttgtaaacctaacatattttttacaatttatgcgtataataaaactgaaaataaatatatggtcatccgagacgattaggtctacctttatagatcatgggtaacaaaaatattaaaccatctaaggaaaatagactgtccatcttgtccaaggataagatggattcatttaagagaggatcctttagagaaaagtcgcgtgcaaccatccaaagattttcatctcttagacgagaacatattaaagtagaccatcctgacaagttcctggagttaaagagagggatatatgaaataattcagaaatcgtcgtctatagatgtggacaaacggactaagctcatgtccaacataaaaacgatgatgataaatccattcatgatcgagggtttaatgacatctttagaaaacttggatcccgataacaagatgagctactcatcggtgatgatattgggagaattcgacatcatcaatataagcgacaatgaggcggcattcgagttcataaacagtctgttgaaatctcttctcttggaatactccattagtaatgacttgttgtatgcccacataaatgcgttggagtatatcataaaaaatacatttaatgttccagaacggcaactgattctgagaggtcaatacctaactccaattttcagtgatttgttaaagtatgcgggtctaaccataaagtcaaacatacttatgtggaataaacagtttatcaaaccagtatctgacctctatacatctataagactccttcattgtgttacagaatcatataaggtgattggaatgggataaatacaacaattatattttttatcatatccttcacgctataaaaaaaattatacatccgtttccctgtcggttacggcagaacatgtagacgaatcatcgtcttcaaaataatcaaattcatcctctatgctctcagtgtgcccgcgtagatacttacatagattgtatcgtagtctagatagctcagatattggaatactatcagatatatgttcggctaatgccatacacctatattttttatttgtcaattcccaatgtttagatactagactagatagagctactactattctagaatcacaacatatcatatcctttacaaagttgacaaagtcaaatagtcccgaatcggagtctactttaagtttctcattaaataatagatcaatgtctccatactgtttaatagccaaatcatctagtgtcatcaatgccgaataaatattgccggatatagtatttctgtgtcttatatattctgctaaaatcagtttaaaactatacttattatacaagtaagtcatactaaccggcgtattaaccgcgcaaccaatattagtttcctctggaagcacccctcttatctctatggagtcattatgtctattatatgaaataaacgtgtcaactactttgtccctatcaaattcgacagtgtagtgtgtatcattaacttcattacgtatgactaatttattttgctgagtagaaaagtaaactaatgcatttattgttttagacgcattaactgatatatcaaacgccattctcgttaattgtaagaaaatgtattatcttttcatttatgtaagaaataccaataactccacacgctaatctctgatcattttttgaaatagataacgcctttccaataattgtagatatatttacatctgtatctaaataaacatatgctacaccatatctgtttacaaagatgttaccgataaatatttctggactgcctatggaatcacatccttgactaatatctccgtaacgatgaattatcaaactatacgttccggattttaatccaataactttatcttttccatggactggttcaaagtaaataactcctctgatattatcgtggtctattatacaaacagccattatttagtaaaatagaataagtagtctgatattatgagtggcagcaatggccgtgtacgcggttactggtggtgccggatttctaggcaggtatatagtaaaactgttaattagtgcagatgatgttcaagaaatcagagtcatagatattgtagaagatccacaaccaataacctcgaaagttaaggttataaactatatacaatgtgatataaacgactttgataaggtaagagaagcgctagatggggtaaatctgattattcatacagctgctctagtggatgtatttggaaaatacaccgataatgaaatcatgaaagtaaactattatggaacacagactatattggcagcttgtgtggacctaggaatcaagtatttgatctatactagtagcatggaagcaataggacccaataaacacggtgatccattcatcggccatgagcataccctttatgatatatcaccaggacatgtatacgcaaaaagtaaacgtatggccgagcaactggttatgaaagccaataattccgtaatcatgaatggagcaaaattgtatacttgttgcctaagacccactggaatttacggagaaggagacaaattgatgaaagtcttttacgagcaatgtaagcaacacggtaacattatgtatcgtacagtcgatgataacgcggtacatagccgggtatatgtaggaaatgctgcatggatgcacgtgttggctgcaaaatatatccagtatccgggatctgagattaaaggaaatgcttacttttgctacgattactctccatcgtgttcgtacgatatgtttaatcttctattgatgaaaccattgggaatagaacaaggatctaggattccaagatggatgctaaaaatgtacgcgtgcaagaatgatatgaagagaattctatttagaaaaccatcactactcaacaactatacgttgaagatatccaacactacatttgaggtgcgtaccaacaatgcagaactagatttcaactactcccctatctttaacgtcgatgtggcattcgaacgaacacggaaatggctagaagaatcagaataagtatttttttttaaaaaaataatcgagtagggtatcaccactacacagtaagagtacagtaaataaaaagtatttatatacttatttttatagatcgtattatgcgctttctacatccatatcatcgtcatcttcaatatcgataatatttttttcttctaccttgacatcttttgcctcttcgacagcaactgattgcgctaataatacatccttttcttttttctttttaggtgtgacatcaatagttatcttttccaagttatacgatatggtaacaacattaccaatttttgaatcaaccgtaattttgattttatccatttctaatagcatagcataattaagagttcatttttatttttttaaacacgtatatggtcactatcaatgtagacgctattagcatacatattgcagtaaaatcatagatgtcatttatatctttataccatataatagaatcgtatcctattatagtaatacacgtggaccgatgtagagaataagtcttatgtttagatgttaatatagtagatgtactcgttgccaaatttttaatgagacacgatacatttactgagcattgtatatcattatattttaagtttcctgataatgagacaatcaaactaggattaagtgaaccatatttgtgttttaaaaaataaccatgtgtaaaaaagacattatcgtctagttcatctacggttaacgtgcgattaataaaattatatctatatggaatatgcggattatattttatatttactacattatagatcctatcaaaatacaaatgcccataacataattccacatcctctgaatgaaatctaaaaatcgatgaactgtatgccaataccggcattattgacatcgtcaatatggatattatccatttcatcatcatcatttaaaattgacactacatatgaatattactttttattttaattaccagttgcacgtacacgggtagcgtgatctctacacgttctatacacgtcacgtctggatgttgttggcttacccatcaaaaatataagtgcggtatgagttctcgctataacgatcggagatacaggggcgtacccagtaagcaactccatagcatacgtgttctcatccattagagagttagtatatacaatacaatatttctgaccaataagaggttttagaatattacgattagtgatgagaggattaatcttggcaaatgttctgttaggaatagcagctagaacattctttgtagtcttgtaatcaacgatggcggcatcctcgaacttattattttttgagatatcctcgataattttatgccattcagccattgttatttattatatatgttttttaataagacatctattggaataaacttgacattagcattctattcttactacaaaatataaaatataaaataaaatatacaatccaatactcacataatccaactcactcgaacactatttttccaattacgataacaatattgcagaatgtactcgttattatttattattttgatgtgtataccatttagttttcaaacagtgtatgatgataaatcggtatgcgattctgacaataaagaatatatgggaatcgaagtttacgtagaagcaacactagacgaacacctcagacaaacaacgtgtgaatccgaaatccataaatatggcgcatctgtatcaaacggaggattaaatatttctgttgatttattaaactgttttcttaattttcatacagttggtgtatacactaatcgcgataccgtatacgcgaagtttgctagtttggatccatggactacggaacctataaattctatgacccatgacgatctagtaaaattaacagaagaatgtatagtggacatttatttaaaatgtgaagtggataaaacaaaggatttcatgaaaactaatggcaatagattaaaaccaagagactttaaaactgttcctccttctgatgtaggaagcatgatagaactacagtctgactattgcgtaaacgatgtgactgcatacgtcaaaatatacgatgagtgcggaaacattaaacagcattccattccaacactaagagattattttaccaccaagaatggtcaaccacgtaaaatattaaagaaaaaatttgataattgttaattgttatttttataaaaacaagaacggtacggcgatatttatttttttctaaaacatctaaccgaagtagtggtatgataaaaatgtagtttgggagtattcgttgtactacaaatatatttccgttttttagttccattcttcgtggcatttttagctataaaattatatggggttgtctggtttaatatttcggattctcctacccaatatccgcgtctaatgcttcttaaaaaacttaactcgtttggagtctctatcttaattagatccgaatttggatttagagctttgcatgcattacgtccttcctcccaggtttttcgatcagtagataaatggatacatttattattatagcttatccagtcagtaggacaatcttctctaatatatgcatcttttatcgttttatctattgatggtgtatgaactaatttacgttctacaacttttaatagtgtcgctgtaaaaataattccaacaattagaccgcatattacgcagcaagcataaccagcataatctgtcttatgtttgttcattgtcgtgcggtgtactcgattaagattacattttaagtatttttttcatttgtggcattcctactcctatccctatatctgctataaataacggtttcgaagttaccattactgaaaatagtcgcgcatcgacttgcgagctacgagtttgtttagattttgtatcgaacgaatatatagaattttcttttatgaagtatattctatattcccgatgttcattttccttctcctttatatcgaaccatttaacaccagacggtccttcgaagataggttggttagataaaggctttataatatcatctagtacattatatttttctatgacttcaaacgtggtatgtggaacaacttttccagctggtaaacatataccaggagctggagacggcaattgctttgtatatccttccaattttgacgtagaaaaagattgtttaatggtattcatagaataggtacataatgcggacttggaataaggactatcgaagaatacatatagtatcgtatcattatctgtttttatagttctagaatgaataatttgtctataacttcttccgtcgatatcacattctaattcgactttgagaaacgtcgaccatctatgactagacaatgatgatggaccaccttcgtcgtttaggcacatttgtgctatatacggaattttgacaattctctttgagccgatagtatcagtgaaaagaatgtaaactttgtcataagtaccatctttatcgacgaatgctcctcgtaaaccatcttttggaattacgttatccgccgtgtataaatcataaccacatggtccgtcaaatcttctccatcgtttaattccttcttttgatatgtttatgtcagatagtacacatccgttgtgactgattatcgttactttgctattttgataaggagcgtatcctctacctctatgttttgggtcgtctgaaccgtctattttccaacatttgggatttccgttattggttccgcatcctctacttttatagatgttgttatataattattattagttaaaccagttttgtttagtttattatttgaaaatgtgtataccgccccattaacacccgtgtataatacgtcgtctaataagtaagtagaaattatttcttcactcgtttcaaacttatgccattcaataccgttagcaaaatagaataaaataaataacaaaggtatcattttaaataaataaaaaatgtcaagagttagaatatcgttgatatacctctatacgttggttgttataacaactacaaagaccatagagtatacagcatgtaatgataccatcattattccgtgtactatagataatccgacaaagtatattagatggaaattggataaccatgatattttaacttataataaaacttccaagacgacaatattaagtaaatggcatactagtgctagacttcattcgttatcagatagtgatgtctcattgattatggaatataaagatatcttaccaggtacttatacatgcggggataatactggaataaaatctactgtgaaattagttcaacttcatactaattggtttaatgattaccaaacaatgttgatgtttatctttacgggcattactttattcttattatttctcgagatcacttatacatcgatatccgttgtattttctactaatttaggaatcttacaagtatttggttgtgttattgccatgatagagttatgcggagcatttttgttttatccgtcaatgtttactctccggcatattattggattgttgatgatgacgttaccatctatatttcttataattactaaagtattttcattttggttactgtgtaaatcatcatgcgctgtacacctcattatctactatcaattggccggatacattttaacggttttgggtttgggattgagtttaaaggaatgtgttgatggtactctgttattatctgggttgggaactattatggtgtctgaacattttagcctgttatttctagtctgctttccgtcaacgcaaagagactattactaggcatgtgtataataccacgagctagtagacgtggaagaggaaccaggaactattgttattttataataatccttgatcttattcttattctttttatcagattttttgcttccagttttatcagtagatatacaacagagtttcataaaaagagaagagaatgaatccattccgtacagtatttgataatagcttttttttcgttttatgaggtatttagagattagagatgattaatgatccccatactagaaatctattaatccacagaaatactaatgctcatatttatattatcaattctaccgtacaatatttgttccttgataggtacagaattgtacgactgcatttttttgtatactaagtcgaatggatgctcgaggttacaaacatgtattaaagtatcttgctcgatgctagaatttatgtacttggcagaggacatacctatacagtttgatggaataggaaactgcttattgtcgatggttataatggaataccacttattattcgcaaatatctgatcgcatatgtgtctatccaaatagtcggtaactcgtctaataatgaatacagacaacggcgaataattaatcagtgatagattgtttacatacagtatgtcgtttgtaaacgatgttaccaatcgtttgctaggtatatccgctttaacaaccaatatggttgtaggacccttgctaactacgacacatttactcagtggggatatgattacagcatgatcaatgggaaaggttagaatatttttgccattgacgtcattatctatagagataacacatcctccgacagaactaatacagagtataatcgtcgataatctatgaggaataagatggtacatctcattgtcatttacaacttctacgcttaagatgttggtaagaagtaccgtttcatccatctgtctattgatctcatcagatataattttttgatgttctgtatctatataatatctacagtcattattagcaataaaattgctaattttagaaatgccgaatacagggaatatctccatttgtacaacgtgacggcagcaataatactaaatattacttcaattttataaaaaggaaactaatcacaccaatgattctatatcatcgtgttcatgatcttgttcttgcttattaagataatcatcgctatgtgctcgtctaaacggattattctcactaaatttattgttgagttctgtaatgaacggatttgacttgctacaaatactggttttattataatttacgaaaggattggatgaatagttaggattctgtttggtatcttcattaagtactactgtagtgttctgataaatagtctgttcattacgatcattatttattagcagcgtgcttccagcaacactatcgtaaatgtgttctgtgctaggcgccataacattggattcgttatcccatattaaactaccagcgaagctatcatcgtccaatatctcattcctagaaatattatctacgtcattgttttgttccatagcactacagtgatcctcccagtctgattcgctatcagttgatttactagatttgctggaattagaactctttatcttttttaattttgtcatgataattttattgtcattatagacagtacgtatctttttcctacaaatatataatatataacatactaatattgttcccgcaactacggtcaccgtgataagaggtaccagcatcatttctgattgctcaatatacgtactactagttcaatatttattgttttattatttactttacaacttttatgataaaaaattactattgcatttcccatcaattatgatccatccattgccgtctgatatgcagaatgaagaattaaacgacaatttcattttcagattatctgaaggattgatgattagatgataatctccagctgtatacaggttatacgcttctatgattgtagcgttaaaaacatcaatagatgggaatagataaaatggctgatgtttatcttctatatctaacatgatatcatagtcgcatgctatgatgatggtattttttgatctgtatgcggcacaaatgctataaatgttgaatctagccaaatcattagaatcctgaggaactattttacccttatagctaaagtagcatttttgcatgtcggaatattttatatcccgtacatctatttggacagtttttatgttacctataatgtatggtcctataaagtccatgattgagatatcgagatcatcatacaatgtatctgttatagtcaacacacccattggagtaataacaaacgcggcgtccatggcggcgtacgttaacgacttattattaattcattttttgttgtcacttgtagaattttttaacacatagtacagattgagtacttttacatactgttttaaccagttttccagacttgtatatataacacgcttcagcatccgtcgtactgtttagttgtttaaaatttgttaatttactaatatctatatctttatcattattaatatctaaccatttatcattggtcttttttaaacttacccaataatctttataaaaaatactaaacaatactctcagatgtctagtatccggtctaggcaatctggctcgtaatttacgacactgataaaccgcattatctgtagacattttaatgttagtatctaaataacaatgtttatcgtattgtatccatccattggcgcaagcactaggcatcagttcttctttgtaatgcagaaatgttcctatgccactaataatggttgagagtatcatcattatagcgaccggcaccgacaacttcttaaacctacttacagtttgtctattaagcgatttcatttattaatgtacaaaaataaatattagttcattgttttaacacaaaaatactttctaacttcttgtgatacatcagaatcttgataatcggatgtagtttttgtaattggattaccatcagatccccatgtatccttaacataatcaatgagccaggtagtcaagacatcggatttattgggtagtgttgatgattccgcagtgcaatttgctttagcatccgagaataactggtagtctgaatgtaatatataacaagaaccctggtaatataaaccattacagctttctttgtgatcatattgcgtagtgctagacgcaacctttctatgagtagatgatgcagcagcaacggcaacagcggcgtcagtaatagcagcctcgttagcagacatgcattgatttaggcgcactatgagaaacgcggacatggtaatcatagatagtagtgaaataaccatagatattctaatacatagaccaatcacgcgtttgcgtttattctttccctgaattttgtctctgtaaacagtagcggagaacacagatgtctgctcttcgtcgttttctggtgtcatcatgataataaatgttatttatgtcacgatgtgccttctttgttctcctccctactaacgaccttagttttccatattttgatttattatcaaattaatttagtaactgtaaatataattatgaattgtttccaagaaaaacaattttcaagagaaaatttattaaaaatgccgtttagaatggttttaacgggaggatctggatctggaaaaactatctatttactatctctgttttctacactagttaaaaaatataaacatgtattcttgtttacacccgtttataatccagattatgatggatacatttggccaaatcatattaatttcgttagtagtcaggaatctctagaatataatctgatacgaactaaaagtaacatagaaaaatgtattgctgtcgcacaaaatcataaaaaatcagcacactttttacttatttttgatgatgtaggcgataaactatcaaaatgcaatactctaatagaattcttaaactttggaaggcatttaaacacgtctattattctactatgccaaacttatagacacgtaccaatattaggacgggctaacattacgcatttttgtagttttaacatttccatctcagacgcggaaaatatgctacgatcgatgcctgtaaaggggaaacgaaaggatatattaaacatgttgaatatgatacagacagctagatccaataatcgattggctattattatcgaagactccgtattttgtgaaggtgaattacgtatatgtaccgataccgccgataaggacgttatagaacaaaagttaaacatagatattttagtaaatcaatattcgcacatgaaaaagaatctaaacgctatattagaaagtaaaaaaacaaaattgtgcaatagcgatcaatcatcatcgtcaaaaaatgtatcataattataattattaacttttgtaacaatagtcctatttagagaaagtctatcgatagacgatcccaatttgtaaattgttccactacttgtcactccatgatatgataaatccatgtaaaatagcatcatctttagatcattaattgttaccttccccaatacaaccaaatcatcatgatatatacctcctccagacaagtatttaacaacggtagaatgctttggcttataaaatacaaatgacattcccttatgtttaatcttaatcttttctttagttattgaatcgttacaattataaaatgatgttttttccaaaaacctaagtgtatttaaaatagatgccatgttaaaaatgtccgccgtcgactttttggaacgattgataaaagctggtgtttatatttatgttttacggacaaagtgtgtaattgcagctttactagtaaaaaactattccataaaagacgaataagatacaaacacaaatgtttatataatatttaaatggaagaccttaacgaggcaaacttctcacatttattgataaatttatctaataataaagatatcgatgcgcaatacgcgtctacattatccgtggtacatgaattgctatccgctataaattttaaaatatttaatataaacaaaaagtcgaaaaagaattccaaatcaatcgaacaacatcccgtcgttcatcatgcagcatccgcgggaagagaattcaatcgtcgttgaactcgaaccctcattggctacatttatcaaacaaggatttaataatctcgtaaaatggcccttgttaaacattggaatagttttgtctaatacatctaccgctgtcaatgaggaatggctaactgcggtagagcatattcccaccatgaagatattttacaaacatatacataagatacttactagagaaatggggtttttagtctatttgaaaagatcccaatctgaacgcgataattatataactttatacgattttgattattatattatagataaggatacaaattctgtaactatggtagataaaccgaccgagttaaaggaaactttgttacatgtatttcaagaatatcgtttaaagagttctcaaacaatagagcttatagcgtttagttcaggtacggtaataaacgaagacatagtttcaaaattaacatttttagatgtggaggtatttaatagagaatataataatgttaaaactatcatagatccggattttgtatttagatctccatttatagttatttctcctatgggtaaactaactttcttcgtagaagtatattcgtggtttgattttaaatcgtgtttcaaagatattatagatttcttagaaggtgctctaatagccaatattcataatcacatgattaaggtaggtaattgtgacgaaacagtatcgtcttataatccagagtctggaatgttgtttgttaatgacttaatgactatgaacatagtcaactttttcggatgtaattctaggttagaatcataccatcggttcgatatgacaaaagtagatgttgaactatttattaaagcattgtctgatgcgtgtaaaaaaattttgtcagcttctaatagattataaatgaactctctatcaattttttttattgtggtagctacggctgcggtgtgtttactttttatccagggttactcaatatatgaaaattatggcaatattaaggaatttaatgctactcatgcagcattcgaatattcaaaatctataggtggaacaccggcattagataggagagttcaagatgtcaacgacacaatttctgatgtaaagcaaaagtggagatgtgtggtttatccaggaaacggttttgtatccgcttccatatttggatttcaggcagaagttggacccaataatactagatccattagaaaatttaacacgatgcaacaatgtatagactttacattttctgatgttattaacatcaatatttataatccatgtgttgtaccaaatataaataacgcagagtgtcagtttctaaaatctgtactttaaatggacggaactcttttccccggagatgacgatcttgcaattccagcaactgaatttttttctacaacggctgctaaaaagccagaggctaaacgcgaagcaattgttaaagccgatgaagacgacaatgaggaaactctcaaacaacggctaactaatttggaaaaaaagattactaatgtaacaacaaagtttgaacaaatagaaaagtgttgtaaacgcaacgatgaagttctatttaggttggaaaatcacgctgaaactctaagagcggctatgatatctctggctaaaaagattgatgttcagactggacggcgtccatatgagtaacttaactcttttgttaattaaaagtatattcaaaaaatgagttatataaatggcgaacattataaatttatggaacggaattgtaccaacggttcaagatgttaatgttgcgagcattactgcgtttaaatctatgatagatgaaacatgggataaaaaaatcgaagcaaatacatgcatcagtagaaaacatagaaacattattcacgaagttattagggactttatgaaagcctatcctaaaatggatgagaataaaaaatctccattaggagccccaatgcaatggctaacacaatattatattttaaagaatgaatatcataagaccatgctagcgtatgataatggatcattgaatacaaaatttaaaacgttaaacatttacatgattactaacgtgggtcaatatattttatatatagtattttgtataatatctggtaagaatcacgatggtactccttatatatacgattctgaaataacgagcaatgataaaaatcttattaatgatcgtatcaagtatgcatgtaagcaaatattacacggtcaattaactatagctctgagaattagaaataaattcatgtttataggatcacccatgtatttatggtttaacgtaaacggatcacaggtatatcacgacatatatgatcgtaatgccggttttcataataaagagataggtagactactatacgcatttatgtactatctatctatctataagtggtagatttttgaatgatttcgcactattaaagtttacgtatttaggagaatcctggacatttagtttgagtgttcctgaatatatattatatggtttaggatattctgttttcgatactattgaaaaatttagcaatgatgctatactcgtttatattagaacaaacaatagaaatggatatgattatgtagagtttaataaaaaaggaattgctaaggtgacagaagctaaacccgataacgataagcgaattcatgctataagacgcatgaaggctgaacgtgaaatcgctcgtaaaaactgcggaggtaacccatgcgaacgtgaagaggttggaatatcaactagatgcggagaaagaaaaagttaagttctacaaaagagaactagaacgtgatcggtatctttctagtagatatcttacctcttcttcagatccacatgagaaaccattaccaaattatacatttcctcgcattgaagtagctccgttgatgactgaggataaagaaccagaacctgtagaagtggtgcctccatcgtccacagacgttaccgaaccgattagtgatgtgacaccatcggtggatgtcgaaccagaacatcccccagctttctgaatatcagacttcagtatcccaagtagcagttacacctccaccaaaacctaaaactccacagattttcgaatatcagacgtccgattctatagttaacaatccacgcccattttataattcggatctcgaatttgatgatattgatatgtatctactaccaaactagaatattacaccagaaaagacggtttgagatcaactttatctaatggtttataaaacgaaggaggccttcgttcgaaatctaatttaacttttacgcctctggcgttcatttgagtaagaaatactttagatacgtgcgtggtatcaatttttgttaagagaggagagagattaagttttgaacatctaagacatgtattaatacccttgatttgtgctgctatgtctccacaattttcacaaacatacacatcttgataatcttcttccgaatctttcaaaacttctgtaatagtattggctgcaccatgcgctattaaacagtctctctccatttctccgaacttgatacctcctccacgttttcgtccctcattcgcctgtctaatgagcttcgtctttttacctctacatctaacggttgccttgtcctgagttaaatgcctcagacgcaagtaataaattggtccaaaaaatactttggatgcataaggcttatccgtttcaggatcatagagaatcttttcacaaaagattttatccgataattcttcatcagacaatttcggatttgaatgctcataacattgtttagcgaattgcatatatgtatcgatggatgtttcgttactactaggaaaacagacaggtcggttttctcccttattgttgtacggcttagcagaatatgcggctgttaaaataacctctatcaacatagatatagtttttctagagaagatggatgtagaattaataatgacatctggtgtgataccattttcatcgtatggaagttccgtttcatccgcgatatacgcgactgttcccttttgactcgttctagtggtaaatttgtctcctagaatgggtcttctttctttcatggttaatactcgtaccttaactttgtcagtaagttctacttgtactcgttcaacgcgagatttgtacatatcggtatatttttcggaaacatcaaagctaatctgattatctctagcaaaatcatcttcaagagttcttgatgagatatttcgtgctatagcgtctccggattccaagaaagcattcagtctaactaatccattactttctaattttgaataggcgttagacctatctctttctttgttattaaagttttccaacggaatttctacttgatgtttcttggctgtaacaatatcgagaccgcctctctgaataaattgttttttgatgataattccatcctcttgattgatacctttgtacgacattaatgctatagtaacatgttggccgaagcaattagccgcaatctttgaagtttctaaagccttactaatcacgattggcctctctggatacatcaaatgaattccattgtctattttatttcgtatatccgagctcagacaagagatagcttgtttagcttgagcacatccaagaatagctctgggtccagaattgtgattgattcccactagtgaagatgctacatatccatctctaaattcggcaggaaagtcacataaatcgtattgctttctttcatcctttgacatcattctaaatttttgaaccgattcacatacgttactaaaagtaaattgttctatatctaccatttcgatgacatgcggaaactctttctgaatgtcagagaatgtcatgtcgtctaatctgctttctaactccggacacacatccatcatgagctctccgttatccacaaccaagaatggtctgactaatcttcccgctccaatattaatgcgaatttcattcatgtgatccctaactaaagtaatacctacctccaagttaccgaagaatcccatccgttttctacgtctaaagtcagttacaaaatcacatatcatatttggattaagagatgcgactagagcattttctatagtgattggaaatcctgtttcaaagtaacttatatcatctttataatatgatctgatatactcacaaattttcttttccaaatccaaatactcagacgttagtatatttgtaatggaactcaagacagacaattgagatactaaacctacctgaggacctctttccggaacgtccgatgaacaaaagtaaagatattgacttggatggtattttctgacagaaaacatctttgaaatctttacttgatccggataaaatccaacactcctaggaatagaaatattctgcatccatgaatagtgaggatgtgttcgataactaccgtctgactttttgaactttccactcaatagactagaaaatgcatgattaagtccaggagttgttagtacatgaatgtttaccgcgtaagtgcctctgttcttgtgattgttcatgatatcgtttcggatgttgcctatgtaattctctaattcatcatgtgccaacgtctcaaaatatttgccgtacgttaggatgcgatgacaaaccatcgaatctctatctggatatctagaagtgtggtagatacagtagagaaactttcttagtaaagatatcatataaaatccctttagttgatcgggtgtatagttcatatgaggtaaaaagttatgcagcatttcatatttgaactcgttgatcgttaactgagatttttgtttaatgtgttcagcttccaccaggtcattaatgtatgtatcaatattaaagtcagtaatagattcagtaattcgtttagcactatctattatcgcgtttactagatagacaacttctggaggcatatcgtatgataaactacgtctaatgaattctagactcactctagataaatattgagacagcaaaacaatattgaccgttataaatgtctttgtcgatgatatattcaacgcttccaattgtgatatatccagagatatcttgtaatggcgatatcttgtcggtaatacattaggaggggatacggaggaaaacgagaaagtgaatgagtttggcttaacaaccctaaattttggccatgttgtaatcttttctactagattaattcctactttttcgacagattgtttattgataaagactccacctatgacattaggaacaagatacttggctgtatcaagtggatttttattcccgtatcctattagtagcggaatttttatcaaatgagaatcttttccctcataactacttattttagtgatggatataccctctttggtcattacctctttaaagatatttacagtgaacgtggctaatgcgtcataactcttacctttaatactcgcgattataggtgagtaatctggaggagtcactttaacattgctaatttctatcataattcgttctgtattattcttaaacgataagagtggccgcttgacggtcaagatttcatgcaatcgatgcaatataaaattagaatacgatacatattggaaatgtaacggtctataaaaaactccggctttaggatcaggcaccaaaaacttatatccgagtcgttgatccatttctgaattagtgtttttttttcattttagaagcaattcttttagacgatctaccgattccgtttctatatctatgctatttaaaatagtcgatctttccttcatcatttctatcatattctcggatttagtcacgtaatttatacaatcctccagagatcgtaatgctacaatattgagctttttccccttaaaaaactttattttgctatcctcatctaacagagaggggaaaacggtatgatccaacgacttaataaatgtcaggttaaacatccctattttgaaattgctaactccataaacatcgtgttcagccattttcttaattaggaataatttctcatctaatgccgtagccgtgagtacgtggtttacaacattagctacttctttaaagtactcgttttggatgatatcctcgaacaacagaaataaattataatagacatagaataatttgtcaatcatgtgtatacaccccttttcatccttgtccttggatagaataatgtgcatagtagaatccttgaatattttcacacatgttctattagtaaaaataatttctatagtttgtaatatagagctttttccacgcgttactatagagtgattaatgatatctactctcattctcttagaaatggttttgatccaaggttgattaatgttggacctgactgtagtgctcagatactcatcagactttttaccggaaaagtaatttgcattagtgcctccatgtacagttttctttatttccccataattgacctttctcttcttattggtagttttaatatatgatacaagagatgacttttccctctcaaatatctctactgtacgagagctaatattgctattatctgagtttatatcgaaataatgacaacatttcacttgtgaagaatcgttaaataccggatacgtattctgattaataatgtgtttagtaagttggatgtcgcaatacactagtttcttaatggcatgatgtatatctttattatacactatattatcaaacatatcctctgaggaaatgcgttctttcataagaccatatatatctcctatttcatcgcaacttattagatgaaagttaaaaatagttctggcatatctatcttctatttcatgtagaaaggtaaatagattatccataatggcgttactaacgttattacattttttttatgtaatttctagatttacacctattataaggtgtataattagtattccatttatctaatacgtatctcatagccaaattgaaactatccgctacatcgtctaatttgcgtctatccggaacggagtctcgcaatccgaatgtgtccatccaatcaagaaatgcttcgaccgatctcttttttcgatctctatatgaattaccagacatgacaggcgagacgcaaataactttggcagccgatgtatgatataaaaagcctttaataaaatagataaatttgacgtacggcgaccttctaggctgacgttctagaagaactgtagtgtattcatattgtgacaaatctttagctatgtgcctttcccaatcagaactccagtctaattttgatatatccaataccctaacggagttatccttgacttctaaaacagttctggcaggattttttgcacctatatcaaaggcgcatattatttcactcgaataatctttttttgacatcggtgacgatattaaagattgagacgaactggttaaagtttccatatatagtctcaatactcgggttatttaaacaattagtattttcaatattgaaatttacaaccttacaattttctattttgaaccgcatgttattaactaacgttataaaatccgcttctggatatcccaaacattctctgcttaaatcaaatgctgattggttttttatttttcgttttacagttccggatttattaatctcatcaactaactcatcgacagttgcgcactcattaatatctaatttattagtcaattgctttaagcctgcactaccaaccttagagaaatactttccgttaacataatagtctcgtcctatagtgtctataattcgttttattacttctcctctagtttctgttccgtttccatcatagtcgtataaaatggaaaatgtgtttttcttttttacttttacaaatgtatgttctctaaccttggatcgtattaaatggtctacatcttttactaatatcttttttcctgattttgttataacgctaggaataaaaatattatctcctatacgatctaccttgatggactcaatatacatgaatgagaatttgaaaaagtctacaacttgccgcctaagttctcccaacttaatatacgatatggatatttttggaaatttatcatcgaaagagcgttctataatagagtataactcgtcgtcaaataatgtgtcttcctctatttcaatttctaaatatttgggtatgtttaatccgtactcactagctagtttaaatatattaactggagactgatattttgatatagcatcttccattatccatctattgtttaacaaaacaaatctcagaaagtctattccgttatcgctgtctaatactttgttacacgcacttcgcatatcatctggtatttgaaaagagtttccagatccaagttctaccatatttttacccttcgaataaataaagacgctcccaaaatataccggtaagaaaatgtaatagcccggatcaatattaaacggtttattttttacctcatcataataatcagatattgacgtctcgacattagctaccttttgcacgcctattttccagtaagtagatgttccccattctaccaaagaattatacttttctatagccgcagaatctgaaaatttcaaacttttgtacagactaagtaattcttttaagttagttaaatcagcgctagaagtcatgataactttatttttaatcctatgttatttcattcttatttttaatattatagtacctgcaatatctgaaaaaatgagacgcgaacgagccgcatacgtaaactacaaacgtctaaacaagaatttcatttgtgtcgatgatagactgtttagttataattttacaacatctggaattaaggcaaaggtggccgttgataacaaaaatgttcccattccatgttccaagataaacgaggtcaataataataaagatgtcgatacactatattgtgataaagatagagacgatataccaggttttgcacgatcgtgctatagggcatattctgacttattttttactacctaaatggatagcaccaatgtgcgttccggaatgaagagccgcaaaaagaagcccaagactacagttatcgatgacgatgatgattgcatgacgtgttctgcctgtcagtctaaattggttaagatttccgacatcacaaaagtatcattggattatattaatactatgaggggtaatacactggcctgcgcagcatgcggatcgtcgcttaaacttcttaacgattttgcgagttaaatattctatttaatacacgttcttctctggaggatgttgtacatacagaagtgggatcggattcttgatgtttccgataacttttttgtttaaatcctagtttatctacagacagactaataattcgttgaacgaaatttcctatcatgtactttatttctttgatggatgtgctaggaaatacatataccgtcctatctaatagttctgtttctcgacataccctccctagtaattgctctatttgcatattgttgattactgccgagcaaatgaacaaagaatccaaactaggaatatctaaaccagtaccggaataaaataaggtggatacgaatataaatctatttagttccttgattgatttgaccatatctggagtacgtctattttgggcgtctcctataaatacaacctctgatccgaaaaaatctaataatcgtttgtagaagaataccatatgttcacgtagtttagtaataactaaaatgcgattaatagttcctgacttgaattcttctaccagggtattaagaataagttgatttctaggctcgtctacagataataacttctcggtatatatatgatatttattagatggtccatctaatcgttttatcatatgtctaatattatctgtggaatatggctcaaaaaaactatctactgcatagatagttttttttagatcggataacttggcaatattaataatactgttacaataaattctgttagatggtctaggtgtagcagttaaaaaataacacatcatcggaggataatacgctaaaaatcttgtaactgctgtattgttcatcagattatacgtatgtgattcatccaagatgaacaaatcataatgcttattgatatatttacaaaaggcatcgtttgtcagatgtctactgactactattaatacatccggactttgagtctttagttcctttaatagactacttactccatctatggatatcttatgttccaatccgactgcctctacctgtgtcttccattgatgtattaacattttattgggtacgcaaatgacggtttttctaccgtgtgtagccataagataacacgtggtaatagtcttaccaaatccacacgccaagtgaagagtgatgtatagaggacgttttgattcgatcattttcctcatattagaaactacttcagatacgactttgcgttgaagaggatataactttggcgcatttgttggattgatactagtaattttattatcggtcgttgttaatgtttcaaatactagactcgtctttacggaaggagaggcgtaaaatcccttaggtatcagaaacttaaaggatgatcccggttcaacttctacgaaatccccgtcttcgttaaaaagacttaggggttgaccacaagtcattttttttagttcggcataaagattatactccatctttaatagtgacattttttaatatataaatgagttatttaagatattacaatatgcttgacgacttctctgcgggtgctggagtgcttgataaagatttatttacagaggaacagcagcaatcgtttatgcctaaagatggaggtatgatgcaaaacgattatggaggaatgaatgattatttgggaatcttcaaaaataatgatgttagaacgttactcggtttgattttgttcgtcttggctctatatagccctcctctaatctctatattgatgatatttatctcatcttttctattgcctcttactagcttagttattacctattgcttagtaactcaaatgtatcgtggaggtaatggcaacactgtgggaatgtctattgtatgtattgtagctgctgtaattattatggcaatcaatgtatttacgaattcacagatatttaatattatttcttacattattttgtttattctgttctttgcatatgtgatgaacatcgaaagacaggactatagaaaaagtataaatgtaaccattcctgaacagtatacctgcaacaaaccttatactgcgggaaataaggtaaatgttgatataccaacatttaacagtttaaatactgacgattattaaaaatgggggcagccgttactcttaatagaatcaaaatagcaccaggaatagcagatatacgagacaaatatatggaattaggttttaattatcctgaatataatagagctgttaagtttgcagaagaaagttatacgtactattatgaaacatctccgggagaaattaaacccaagttttgtttgatagatggtatgtcgatagatcattgtagtagttttatagttcctgaatttgctaaacaatatgtattaattcatggagaaccatgtagttctttcaaatttcgtcctggatcattaatctattatcagaacgaggtaactcctgaatatattaaggatttaaaacacgctactgattatatagcatccgggcaacgatgtcattttataaaaaaggattatctcctgggcgatagtgatagcgtggcaaaatgttgttctaagacaaataccaaacactgtccaaaaatatttaataataattacaagacagaacattgtgatgatttcatgactggattttgtagaaacgatcctggaaaccccaattgtttagaatggttacgtgcaaaacggaaaccggctatgtctacttattccgatatttgctccaaacatatggatgcgagatattgttctgagtttattagaattattcgtcctgattattttacttttggggatacggcattatacgtcttttgtaacgatcataaaggaaatagaaattgttggtgcgcgaattatccaaaatctaattccggagataaatatttaggacctagggtatgttggttacatgagtgcaccgacgaatctagagatagaaaatggttatattataatcaagatgttcaaagaactagatgtaaatacgttgggtgcacgattaacgttaactctttagcgttaaaaaattcccaagcggaacttacgtctaattgtactagaactacgtccgccgttggtgacgtacatccaggagaacctgtagtaaaagataaaataaaactgcctacctggttgggcgcggccataacattggttgtaatatctgttattttctattttatatctatttattcgcgtactaaaattaaaacaaatgatataaatgttcgtagacgataattcgttgataatttattctacatggcccagtacattgtccgattcatcgggtagagtcatcgttatgccagataatagatcattcacgtttaaggaagggtttaaattagatgaatcgataaaatctatattgttggtaaacccgtcgtctatagatctattaaagattagagtatataaacatcgcataaaatggatgggtgatatattcgtattatttgagcaagaaaatatcccaccaccttttcgtctagtaaatgataagtaattacgagccgttgctgctgttagttataacatgctgtgtactactatttaattttaccatatcttcgaaaacaaaaatagatattatttttgcagtacaaactattgtttttatatggtttatattccactttgttcattcggcgatttaaaatttttattagttaaatggatatgatgcttatgattggaaattatttttccggcgtgctaatcgctggaatcattcttttgattctttcgtgtatcttcgcctttattgactttagtaagtctaccagtcccactcgtacatggaaagtattgagtattatggcgtttatacttggtattattatcacagtcggaatgctaatttattctatgtggggaaagcactgcgcgccccacagagttagcggagtcattcataccaatcatagcgatatttccatgaactaaattattatcgtccatatatctcgacattgttgaatcattattactacttatttagtgaaaagatgatatattgcatacttgatcaatagtgaagttattgtcaataaatgattggtattcttttgttgatcggtatttgcgtagcagttaccgtcgccatcctatatgcgctgtataataagatcaagaacccacaaaatccaaatccaagtccgaatttaaattcgcctcctccagaaccaaaaaataccaagtttgtaaataatctggaaaaggatcatattagttcattgtataatctagttaaatcttctgcataaataaaaatatttttagcttctaaatggcggataaaaaaaatttagccgttagaagcagttacgatgattatatcgaaacagttaataagattacaccacagcttaaaaatctactagcgcaaatcggtggagatgcagccgtcaaaggaggcaacaataatcttaattctcaaacagatgtgactgccggcgcatgtgatacaaaatgtattacatgtaaaccaaaatcaaaatcctcgtcttcttctacatcaacatccaagggctccaaaaatacttctggtgctcctagacgtagaacaacagttactactacatcgtacaatgcgatggatggtcagattgtccaagctgttactaatgctggtaaaatagtttatggtaccgtcagagacggccaattagaagttcgtggaatggtcggagagatcaatcacgatcttctaggtatcgactcagttaatgctgggaaaaagaaaccatctaaaaagatgcctactaataaaaagattaatatgtcgtccggtatgagacgacaggaacagattaatccagacgattgttgtctggatatgggaatgtattaaattaaataattttaattcgtttaacgaatatcttgagtataaacaatacaatattaagaaccggactgttaccgattcctagttttgatgctacagcatcgcagtcatctccgatctccacatcgataatttctgaagtgatatcggtactcagtcctttgatttcttcaaatccgagttttagcaatgcttgctcgataatatttatgacaataataatcacgttagtgacgataatttttcgttttctactttcgtgatattgtttaatcgttttatagattctatctatttcatcctctgaacaaacatccaagtcctcgactgataagggagacccgttcaaatttgcataattaacgatggctatacgcttattaacttctgttgatttatacggagtcttaccaaatagtattctggtaaaattatctaaattatcagatgattttgtattagatcgttgatttctaagattaaccacttcatcctccaacatctgaattcttttatctttatcataaactactcccaaggatggtgtttgtgttggcatagaagatatcatagatctagattccattattgcttcagcatttttcgatactgtaatattaaatcttttttctcgttgttgacgttgttccgatatcaataactctctacgaaacgtaggaggtggagtatcgtcaataatagtagtatgaggttgtactcgttcgataatagtggccggagaatcatcatctggaaatagatcttcattaagttgtgaggatatttcctctggagatgacactacggcggcattatgttctctatctaccacgttgttaacgtgagttagaatagacatttgacgaagagttatttcataatttttgttagatggataattatcttctgaaaactctgtaattaaatcgttttgtatatccgtcactggtacggtcgtcatttaatactaaataaatgatgcctattaagtcaatagttactcttgatcaattagaggactctgaatatttatttcgtatagtttctaccgttcttccgcatctatgtctagattacaaagtatgtgaccaacttaaaacaaccttcgttcatccgttcgatatattgcttaataactcattaggatccgtaactaaacaagatgagcttcaggctgctatatccaaattgggcattaattatttaattgataccacgtcacgtgaattaaaactgtttaatgttacacttaacgctggaaatatagatattattaataccccaattaacattagttcggaaactaatcctatcattaatactcacagcttttacgatcttccacctttcactcaacaccttcttaatattagattgacggatacagaatacagagctagatttatcggtggttatattaaaccagatggctccgactcaatggatgttctagcagaaaagaaatatccagatcttaactttgataacacttatttgtttaacatcctctataaggatgttattaatgcaccaataaaagaattcaaggcaaaaattgttaacggtgtattaagcagacaagattttgataatcttataggtgttagacaatatataacagcacaagatcgaccccgctttgacaacgcttataacatcgcagatgctgctagacattatggagttaatcttaatacattgccattaccaaacgtagatctcactactatgccaacatataaacatctcatcatgtttgaacagtacttcatttatacatatgacagagtggatatttattacaatggtaacaaaatgctcttagatgatgagattatgaacttttgtatttctatgcgatatcaatctcttattcctagactggtagaattctttccagatataccagtaaacaataacatcgtacttcatactcgcgatcctcaaaatgctgcagtgaatgtaaccgtggcgcttccaaacgtgcaatttgtagacataggtagaaaccacaaattctttattaatttctttaacctgttggcgaaggaacaaagatctacggctatcaaagttaccaaatccatgttttgggacggtatggattacgaggaatacaagtctaaaaaccttcaggacatgatgtttataaattctacctgttatgtattcggtctttataatcacaataatactacttattgctctatcctttctgatattatctccgcagagaaaacacctattagagtttgtttgttacctagagtagtcggaggtaagactgttactaatcttatttcagaaactttgaagagtatttcatctatgactatacgagagtttcccaggaaagataaatctatcatgcatataggactttctgagacaggattcatgagattcttccaactactcaggctcatggctgataaacctcatgaaacggctattaaagaggttgttatggcttatgtgggtataaagttgggtgacaaaggtagtccgtactatattagaaaggagtcataccaagactttatctatctgctatttgcatcaatgggctttaaggtgactactagaagatccattatgggaagtaataatatctctatcatcagtattagaccaagagtaactaaacaatacatcgtcactacattgatgaaaactagttgtagtaaaaacgaggcagaaaaattaattacttcagcgtttgatcttctcaatttcatggtatcagttagtgactttagagattatcagagttacagacagtatagaaactattgtcctagatatttctatgcaggatctcccgaaggagaggaaaccattatctgtgactcggaaccgataagtatcttggatagaattgatactcgtggtatcttttctgcgtatactattaatgaaatgatggacactgatatcttttctccagagaataaggcatttaagaataatctgagtagatttatcgagagtggaaatattacaggagaagatattttctgcgcaatgccatacaacatcttagataggattattacaaatgctggtacgtgtaccgtatccataggtgatatgttggataacattacaacccagtcagactgtaatatgactaacgaaatcacagatatgataaacgcctcattgaagaatacaatttctaaagataataatatgctagtcagccaagcattggactctgtagctaatcgttctaaacaaacgattggagacttgaggcaatcatcgtgtaaaatggcattgttgtttaaaaatcttgctacatccatctacacaatagaacgtattttcaatgctaaagtaggcgatgatgttaaggcatcgatgttggagaagtataaagtattcacagatatttccatgtcattgtataaagacttgatagctatggagaatctcaaagcgatgctatacattattcgacgaagcggatgcagaatagacgatgcacaaattactactgacgatctagtcaagtcttactcattgatccgtcctaaaattctaagtatgataaactattataatgaaatgagtagaggatactttgaacacatgaaaaaaaatctaaatatgacagatggtgactctgtctcttttgatgatgaataaatgtcatgttatacagctatattaaaatctgtaggaggactggcgctatttcaagtagccaatggcgccatagatttatgtagacatttctttatgtatttttgtgaacaaaagctacgaccaaattcattttggttcgtcgttgttagagccattgcaagcatgataatgtatttagtattaggcatagcattgctgtatatttctgaacaagataacaagaagaatactaataatgataaacgaaatgagtcgtctataaattctaactccagtcctaagtaaaatattttagtagcgtatccttatcgcgtttgcttatcttgaatgaactggtcttttttaactcgttgatgaattttgtaaataattcatttctatctttaagtaattttattggaagttttgattccacagccaatgaacatgtaaattgtgaatcattttctatgaccagttgtaacttttcatacactgtaatcaatacagtatttaccatttgattaattacagcgcccgtactagcactccattgaacaagatcagattttagattaattagataaaatctatatgttatttcagataatgaacttaccagataactctcttgacggatattaaaaatgccagatgaatgttcatctcgaatagccagagctactgtagagtaatacggttcaaaatcataaacgtgatagtttccaaactggtatccgagtttttcttggatgatggatacttgagagttgaatttaaatttcttactatgttcattatatagttctggaaagaatgcttcaatcattgtttctgtaagtttgcatccttttgatgcgatagttaaaagtgctatataaggcgccacgataatgttattttttttggtaatagtgacgtcttttacagcgtcaacgcatctgaacaaataatgaatctctctatgatctaaaaaataaagtctttgtaaaaagaatcgtagtgctagttttctctcatcatccttagatctatgggcgaatagacgtctactacgggatataaaaccgctattttcctttatcataggtgttgtttgatctatatttacctcccctagttctacggaggcctccaaattaagatctggtactggttcgaacattgtaagacttacatcatcggtagtagattttcactttaccccacgatataaatatgcgatatatagtaagtccgcaattggtattacaggtgggtaaggggcaggaggtagaacgagccctatatctcactccatatgattacatagatgagaagtcgcccatatattattttttacgaagtcatttaaatatacaacagccggaaatagttaagagacatattctattgacgcttcgaatgactcaattaaagggatatttaggaaatttgttagatattaaggacgatattattatctattctcataagaataatttggaatatagttacgttgataatactatttttaatcccttcgtatatactcagaaaaaaacactactaaaaaacgatagctttttatacaatgtatatcctggagcgtgtgactttttggttatctgggtggccagagcgtgcgatacatctattccggaatttggatcgtatgaagatgtagataataatattatcaagtttgaaacaatgttgatggaagtatttccacaactagatttggacattactgtagaatcaaagtttaacaatatatttcgtaccaatctaaaactaactgggttaaaaaagatcattcagcgagttcaagacttggacattaattataagtcgttgttatctagatacgatgaacactttattaatatgaccggtaatcattttattctaaacgatgaacagttaaatctctccatttgggacttggatggtacattagcgttatctagcgacggcgataccgtgatgattaataacgtaaaactatttacagatcttgtgtccgatatagatacacaaatggaacgcatcaagggagatataacgtataaggtacatttggcgactcctatcaattctagaataaaattggatatcgagactagcttcatttttatagagacggcgactaataatattttactatcctcggataaaaaaatatctatcattttggccaaaaaccatatatctattaaagtgaaaaaccatattcctaacatagaaaaatattttacatttttagttattgccattaatgccatgtttaatagcgttcaaaagtctgctgattttaccaaagtggaaactgtttactggtctaggatatgccaaaatacaaagaataagaatagaaaacccatcattattaattatctagatcctggaatgaaaaaaatcagtaacaacttttacagatccgatgagaaagaagtctttattaatgataacggcataatgtttacatgcatggatcctttggggaaatataataaggtgggatttcttaatatatttcatgatatgtggaaatattgtatcccttgttgttttctacatgatcaatctcatcgaagtacattttcatcgtgtgttcatcaaatcgacgttgagaaaaagatagtaagtccgtatatccttaattttggtaaagttgtaacagaatccaaaatgtcatttctccctattatctttgacgccttcttaaatgatggaatgactgctaatatggaacaagataataaacgactaaaggaaactagtggatatcatatagttagatgttgtgctggtgatgatatagttcgtttacgaactacatctgatattattcagtttgtaaacgaggataaaaatattcttatagttaacgacatggtatattttccaatgaacgcgtccgatataggaaagaaaatacatatactcattcaagaaatagttcatgaggtaatgatagtaaaaaagaaagagtctagtgataaaatcgattttttcccacccaactataagttattgaaggatctatttccaaaacaaactattcaaactcctattcaatctgacgcgggaatggtgttaacaaccgatggattctacatagatggaaaactttttaacgaagatctgtcgtctaaatacgttacatttacaaaaaatgttattgcgtctgatgccgtagctaaatatttttctcctttgtttaaatacgttatttcagaagctaaagatagatttatcaaaacgtggatgattaatattatgatacatatgaacgtagatcctaataatataataccgacgttagaaaaatactatcccaactctggaagagcacaaataaattaaacaactaaatctgtaaataaataatggacaaacttagagttctatacgatgagttcgtcaccattagtaaagataatcttgaacgcgagactggtcttagcgcatcagatgttgatatggattttgatttaaacatttttatgacgttggttccagtcttggagaaaaaggtatgcgctattacaccaactatagaagatgataaaatcgtaactatgatgaaatattgtagttatcagagtttttcattctggttccttaaatctggtgccgttgtgaaatcggtatataataaactagatgatgtggaaaaggaaaagtttgcagccacatttagagacatgttgcttaatgtacaaactctaatttctcttaactctatgtatactagattgcgtcaagataccgaagatattgtatccgattccaaaaaaataatggagattgtttcccatttgagagcgtcgactacagagaacgcggcgtatcaagttctccaacaaaacaatagttttatcatatctacactaaataaaatcttatctgatgaaaactatctcttgaaaattattgcagtattcgactctaaactaatttctgaaaaagagacattgaatgaatacaaacaattgtacaccatttcttctgaaagtttggtatatggaatcagatgcgttagtaatctggatatatcatctgttcaactgagtaacaataaatacgttctctttgttaagaaaatgctacctaaaatcatactgtttcagaataacgacatcaatgcacaacaattcgctaatgttatttctaaaatttatacgttgatttatagacaattgacgtcgaatgtcgatgttggatgtctattgacagatacgatagaatctgccaaaactaaaatatctgtagaaaaaattaaacagacgggtatcaataatgttcaaagtcttatcaaattcatatctgataacaagaaagaatataagacaataatctctgaagaatatctatcgaaggaagatagaatcattactattttgcaagatatcgttaatgaacacgatataaagtacgacaataaattgctgaacatgcgagacttgattgtgacatttagagaacgatattcgtataaattctaatatcgtttttgaagtttccaaattttgataatatagtctagatggaattttagaccatctttgtcaaaatcgtttaccgacaacaattctccgttcttttcgatgactataggacaagaaccctcctctatctcttgtataattacatgtagcatattttgcttcatcgtttcgtcagaaaattctgaaactagaggtaatcttcctcgttgaagcaagttatagctttctgctattatacccgctatttcaaatagacttatacgtctagtatagcgtcgtttaagagcagatatatgattccctatatgtttaagattggaatgcgcatcttctatatgagtggatgctgattctacaatcttataagaagatttgggatctatatcactagtttctagtgactctccatcttcttcctcttcttcatcatcctcgtattcggtgagatcatcggattcatagtcgataatatcgtctgtgtctgccatttaatcttataatcgcaattcaattttaaagccttaaatggacttctttaacaagttctcacaggggctggcagaatcctctacaccaaagtcgtcaatctattattctgaagaaaaggatccggatacgaaaaaggatgaagcgattgaaataggactaaagtctcaagagtcgtattatcaaagacagttgcgagaacaactagctagagataatatgatggccgccagcagacagcctatccaaccgctacaaccaactattcatataactccacagccggttccaacagctacaccggctcctacaccaaaaccacgacaacaaactaatacatcatctgatatgtctaatctttttgattggctgtctgcagatactgatgcgccggcgagttcactccttccagcgttgacgccgagcaatgctgttcaggatattatctctaaatttaataaagatcaaaagacgacgacgccgccatctacccaaccttctcagacgttaccaacaactacatgtacacaacaatcggatggaagtatttcttgtactactccaacggttacacctcctcaacctcctattgtggccactgtatgtactcctacacctactggtggtacagtatgtacaacagcacaacaaaatccaaatccaggagcagcatctcaacaaaatctagacgatatggcccttaaggatctcatgtcgaatgttgaaagagatatgcaccaacttcaggccgaaacaaacgatctggtgacgaacgtatatgatgcaagggagtatacgcgtagggcaatagatcaaattctacaattagtcaaaggttttgaacgattccaaaagtaataagattgaatattaaaatcacgctttcgagtaaaaactacgaatataaataatggaagccgtggtcaatagcgatgtttttttaacatctaacgcaggactaaaatctagttatactaatcaaactctttctttggtagatgaagatcatattcacacttctgataaatctttgtcttgtagtgtatgcaattcattatccaaaattgtagacgatgactttatatccgcaggggctagaaatcaacgtaccaaacctaaacgtgcaggaaataatcaatctcaacagcctatcaaaaaggattgtatggtttccatcgacgaagtagcatccacgcatgattggagtacgagattgagaaatgatgggaatgcaattgctaaatatctaactactaacaagtatgacacatctaactttactattcaggatatgcttaacattatgaataaactaaatattgtcagaacaaatagaaacgagctatttcaactccttacccatgtaaagagcacattgaacaatgctagtgtttctgtgaaatgtactcatcctttagtacttattcattctcgagctagtcctagaatcggtgaccaactcaaagagttagataaaatatactctccatctaatcatcatattcttctgtcgactacacgattccaatccatgcattttaccgatatgtctagttcacaagatttgtcttttatttatagaaaaccagaaactaattactatattcatcctattctgatggcactattcggtattaaacttcctgcgctcgagaacgcgtatgtacatggagacacctatagcctaatccagcaactttatgaatttagaaaagtaaagtcttataattatatgttgttggttaatcgtcttacggaggataatccgatagtgattacaggtgtatcagatctaatttccacagagattcagagagcaaacatgcataccatgattagaaaagcaattatgaacattagaatgggaattttttattgtaacgatgatgatgcggtagatccccatctaatgaagattattcatactggatgctctcaagttatgacagatgaagaacagatattggcttctattttgtctatagttggatttagacctacgttggtttctgtggctagacctataaacggcatcagttacgatatgaaacttcaggcggcaccatacatagttgttaatcctatgaagatgatcacaacatccgacagtccgatttctatcaattccaaggatatttattctatggcattcgatggcaatagtggaagagtggtgttcgctcctcctaacataggatatggaagatgttctggagttacacacattgatccattgggaactaatgtgatgggtagtgctgttcattcccctgttatcgttaatggagcaatgatgttttatgtagaacgacgtcagaataagaatatgtttggtggagaatgttacaccggctttagatctctaatagatgatactccgattgacgtatcaccagaaatcatgctaaacggtatcatgtataggttaaagtccgcagtttgttacaaactcggagaccaattctttgattgtggatcgtctgatatcttcttgaagggacattatacgattctatttacagaaaatggaccctggatgtacgatcctctttctgttttcaatccgggagctagaaatgctagattgatgcgagctctcaaaaaccagtacaagaaattatcaatggattcagacgatggtttttatgaatggttgaatggcgacggttcagtatttgctgcctcaaaacagcaaatgttgatgaatcacgttgctaactttgacgacgatcttctaactatggaagaagccatgtcgatgatttcgagacattgttgtatcttaatttatgcacaggattatgatcaatatattagcgctagacatattacagaactattttagattatgatatttaaatgagttggtacgaaaaatataacattgtactgaatccgcctaagcggtgttcttctgcatgtgcggataatttaactactatattggcggaggacggtaaccatattagggcgatactttattcacagcccaaaaaactaaaaatattacaggattttctggcaacgtctagaaataaaatgtttttatataaaatattggacgacgagatacgtagagtgttaacatgaatctacgattatgtagcggttgtagacacaacggtatagtatctgaacaaggatatgaatattgtattttttgcgagtctgtatttcaaaaatgtacaaaggtacaaaaaaagtcaaacttccatgtgtctaataaacttattcatttgagaaatgtattgcggagattattgtctcatcaatgttctggagaaattatctcggaactcttggatatcatggaaaaaaatcaaatatccacggatgatgtagatgcaaattttgtatctagttttcttaaggctaacgagagaataaataaaaaggattataagttagtctttgaaataatcaatcaagtaaaagatgagaaactgaatctgagtacagaaaagattaatgaagtagtagaaatatttaagcacttggtattcttttgccaagaaaacactccttctaagacaattaattattcattctttttggataaaatattcgatatcacttctgtaactaaaaatctaaaacctcaaactgttaaaaattatacgaaaaataatagtaaccaattagtatgggaaaactttttagcacatatgagatctaaaaaacgtgtaactatggtagaggattatggacacgagtatgtttttgtagatgagaggttttctacttgctcattagaagtataaaaaaatagttccgtaattaaatggctaagcgagtaagccttccagatgtggttatttcagcacctaaagcagtctttaagcccgctaaagaagaagcactcgcttgtatactaccaaagtattataaatctatggcagatgtgtctattaagacaaatagtgtaattgataagtgttggttttgtaatcaagatttggtttttagacctattagtattgagacattcaagggtggtgaagttgggtatttctgttctaaaatatgtagggattcgttggcttctatggttaagtctcacgtagctcttagagaagaaccaaaaatttctttgttgcctttagtattctatgaagataaggaaaaggtcataaatacaataaacctactaagagataaagacggcgtttacggaagctgttactttaaggaaaactcacaaattatagatatttctctacggagtttattgtaagctttttccattttaaatagaaaatgaataatactatcattaattctttgatcggtggggatgactctattaaacggtctaatgtcttcgcagtcgatagtcaaattccaactttgtatatgccgcaatatatttctctatccggagttatgacaaacgatggtccagacaatcaggctatcgctagcttcgaaattagggatcagtatattactgcgcttaatcatttggttctgagtttggaacttccagaagttaaaggtatgggaagattcggttacgtaccatatgttggatataaatgtattaatcacgtatctatctcttcgtgtaacggtgttatttgggaaattgagggcgaagaattatataataattgtatcaataatacaattgctttgaaacactctggatattctagtgaacttaatgatatttctattggcctaactcctaatgacactattaaagaaccatctacagtatacgtttatattaaaactccgtttgatgtggaagatacattcagcagtcttaaactatccgattcaaaaattaccgtaacggtaaccttcaatccagtatccgatatcgttattcgtgactcttcgttcgactttgaaacgttcaacaaagaatttgtttatgttcctgaattgagctttattggatatatggttaagaatgtacaaattaaaccatcgtttatagagaaacctaggagagtaataggtcaaataaaccaaccaacggcgactgtaactgaagttcatgcggcaacatcgctctctgtttatactaaaccttattatggaaatacggataataaatttatttcgtatccagggtactcacaagatgaaaaagattatatagatgcatatgtgagtagattgttggatgatctagttattgttagtgatggcccaccgactggttatccggagtctgccgagattgttgaggttccagaagatggtatcgtttctattcaagatgctgatgtgtatgtaaaaattgataatgttcctgataatatgagtgtttatcttcatactaatctgctaatgtttggaacacgaaaaaattcttttatatataacatttctaaaaagttttccgccattactggaacatatagtgatgccactaagagaacaatctttgctcacatatcacatagtatcaacatcatcgatacatctattcctgtaagtctttggactagtcaacgtaacgtctataacggagataatagatcagccgaatcaaaggccaaggatttgttcattaacgatcccttcatcaagggaatagattttaagaataagaccgatattatttctagactagaagttagatttggaaatgatgttctatattcagagaacggacccatctcgagaatttataatgaactactgacaaaaagcaataatggaacaagaaccctaacttttaactttacaccaaagatattctttaggccgacaactattacggccaatgtatctagggggaaagataaactatctgttcgagtagtttattccaccatggatgtcaaccatccaatctattatgtacaaaaacaattggtagttgtatgtaatgacctgtataaggtatcttacgatcaaggggtaagtattaccaagattatgggagataataactaataataatgaaaacaaactatagagttgtaaatggatgaaattgtaaaaaatatccgggagggaacgcatgtccttcttccattttatgaaacattgccagaacttaacttgtctttaggtaaaagcccattacctagtctggaatacggagctaattactttcttcagatttctagagttaatgatctaaatagaatgccgaccgacatgttaaaactttttacacatgatatcatgttaccagaaagcgatctagataaagtctatgaaattttaaagattaatagcgtaaagtattatgggaggagtactaaagcggacgccgtagttgccgacctcagcgcacacaataaactgttcaaacgtgaacgagatgctattaaatctaataatcatctcactgaaaacaatctatacattagcgattataagatgttaaccttcgacgtgtttcgaccattatttgattttgtaaacgaaaaatattgtattattaaacttccaactttattcggtagaggtgtaatcgatactatgagaatatattgtagtctctttaaaaatgttagactgctaaaatgcgtaagcgatagctggttgaaagatagcgccattatggtggctagtgatgtttgtaaaaaaaatttggatttatttatgtctcatgttaagtccgtcactaagtcttcttcttggaaggatgtgaacagtgttcaatttagtattttaaacaatccagtggatacggaattcattaataagttcttagagttttcgaatagagtatacgaagctctctattacgttcactcgttgctttattctagtatgacttctgattcaaaaagtatcgaaaacaaacatcagagaagactagttaaactactgctgtgatttttaaaacatagttattacttatcactcataaatgagtaaatcacacgcggcctatatcgattatgcattgcgcagaactactaatatgcctgttgaaatgatgggaacagacgtagtacgcctcaaggattatcaacattttgtagcaagagttttcttaggattagacagtatgcattctcttttattgttccatgaaacgggtgttggtaaaacaatgactactgtatatattctcaaacatcttaaggatatttatacgaattgggctattatcttattggtgaaaaaggctttgatagaagatccttggatgaacactatactcagatacgctccagagataacgaaggattgtatttttattaattacgatgatcaaaattttagaaataaattttttactaatatcaaaactattaattccaagagtagaatatgcgtcattattgatgaatgtcataacttcatttctaaatcattaatcaaagaagatggtaagatccgtcctactcgttcagtatataattttttatctaagaccatcgcattaaaaaaccataagatgatttgtttatcggctacacctatcgttaatagtgtgcaagaattcaccatgttggttaacttactacgaccaggatccttacaacaccaatcgctatttgagaataaacgtctagttgatgagaaagaattagtctccaaactaggaggcctatgttcgtacatagttaataacgagttttctatttttgatgacgtagaagggtctgcatcattcgctaagaaaacagtattaatgcgatacgttaatatgtcgaaaaagcaagaagaaatttatcaaaaggctaaactcgctgaaataaaaacaggtatatcatcatttagaattctgagacgtatggctactacgtttacgttcgatagctttcctgaaagacaaaatcgtgatccgggcgaatacgcgcaagagatagcaacactatataatgattttaaaaattcattaagagatagagagttttctaaatccgcattagatacctttaaaaagggagaactattgaaaggggatgctagtgcggctgatatctctctatttactgaattaaaagagaaaagcgtcaaatttatagatgtatgtttgggaatattagcatcccatggtaaatgtctagtctttgaaccatttgttaatcagtcaggaatagaaatcttattactatatttcaaagtctttggtatctctaatatagagttctcatctagaacaaaagatactagaatcaaggcggtggctgagtttaaccaagaatcaaacactaacggagaatgcattaaaacatgcgtattctcttctagtggaggcgagggtattagttttttctcaattaatgatatcttcattttagatatgacatggaacgaggcgtctcttcgtcagatagtaggaagagccattcgtctcaatagtcacgttcttactcctccagaacgtagatatgtaaacgtgcactttataatggctagattatctaatggtatgcctactgtagacgaagacctatttgaaatcattcaaagcaaatcaaaagaatttgtccaattgtttagagtgtttaaacatacatcattagaatggattcatgctaatgaaaaagacttctcaccgatcgacaatgagtccggttggaaaaccttggtttcaagagccatcgatctatcgtctaaaaaaaatattaccaataaactaattgagggtactaatatttggtattccaattctaatagattaatgtcaataaatagaggatttaaaggcgtagatggtcgagtatacgatgtagacggtaactatctacatgatatgccggacaatcccgttataaaaatacacgatggtaaattaatttatattttctaatcaatcatcctcagttaatttttttaatgattcgtaataacatcctctatggccataacatttgagttttgcagtatctagagcatattttgcaatttcgtattggagtccattacctgaattcggatctaaaaatattagatccttgatttcatgattacttttaaatgtatcaatgatttgatcactcgttaaagatattcttccgacaaagaagattacctcaaaaaatttattaataatggtatcttctatgatgccatgaataaaaaaccgagtgtctatgaatacaaaagaattgtctatattaacttcttctttaatttccctggataaacactctggaacattctcaccccttttgggtatgccacccggataaatagcatctattctatcattatcagtagtagctggatctagagaaaaaaatgacgatagtatacttctttcctgtttggacaaataattggaataattcagaaataatcgtttctttctagacatgtttctagttctaattatttcagaatagagaaaactatctcgtctgttacatactaatattttgttatcagtagttaataaaatagcggacacggatactcgtttatgacaccataggcattggttaacgaatgccgtgagtgtaataatttgagagtcatcctcgcaaataatagacttagctagtcgtctattatacttaataatctgactaattatactagatctgtaaaagttcatttactattaactagcatattataaatataagacagatattcgtatttatcgtcgttaatacaatcatttaatgatttaatctttctaatttctacattgtaaatactagtatgcgataaatcctccaacgattgattaataaaacacgccatgcaataacttatatatactttattaaataatttatcccgtgttgtaagttttagaattacatttccaaattcttttactgttatacgttcatcactttcctcttttaattctcttcttaaacaatctttaatagattcctttttatctagtttaccacccaataatattaactcttcaaagtgaggatcgatatcgttgatagaaccttttctcaaccgtctaaagatttctcttagttcattgtagtacataaaccgtaatagtttagtggatactctaaagatagaatctgaattttgttgagataatatcgcttggaatgcgaatgaagttcttctagctcctattaacggatatccgtcacttgttatacacgcagcaaacacatgcgtgtcttttgatcttggaatatcttttattcgtttaatagatattaattctctaggagtttcaaatatcacttcctcatccattgtaattcccatactaagagctatttttaaacagttatcatttcatttttactatgccgcaacaactatctcctattaatatagaaactaaaaaagcaatttctaacgcgcgattgaagccgttagacatacattataatgagtcgaaaccaaccactatccagaacactggaaaactagtaaggattaattttaaaggaggatatataagtggagggtttctccccaatgaatatgtgttatcatcactacgtatatattggggaaaggaagacgattatggatccaatcacttgatagatgtgtacaaatactctggagagattaatcttgttcattggaataagaaaaaatatagttcttatgaagaggcaaaaaaacacgatgatggacttatcattatttctatattcttacaagtatcggatcataaaaatgtatattttcaaaagatagttaatcaattggattccattagatccaccaatacgtctgcaccgtttgattcagtattttatctagacaatttgctgcctagtaagttggattattttacatatctaggaacaactatcaaccactctgcagacgctgtatggataatttttccaacgccaataaacattcattctgatcaactatctaaatttagaacactattgtcgtcgtctaatcatgatggaaaaccgcattatataacagagaactatagaaatccgtataaattgaacgacgacacgcaagtatattattctggggagattatacgagcagcaactacctctccagcgcgcgagaactattttatgagatggttgtccgatttgagagagacatgtttttcatattatcaaaaatatatcgaagggaataaaacattcgcaattattgccatagtattcgtgtttatacttaccgctattctcttttttatgagtcaacgatattcgcgagaaaaacaaaactagattcgataccttgttgagcctccattagaacggcagtgacttcgctgccattgtcatacgcattaccatttcgaaaaaagcagtactttgaatcgctaaatgatacagtacccgaatctctacttagtttacagattaaatctccacattgaatagttacatttgattcatcttcgatgtttaatgttcctctgactatatccccaacgtgataatacgcgtaggttattacacacggaacgtttataactacagaattattaactatttcgccgagaggtaattccacgtcttcacgaatttctattttcttggccattttaccactaatttctctatggagatacgtcttatatacggcattcctaatattagtttttatgtctaacgtcagctcgtgtggctccaatgtaactggaaggtatccattggtaacaaagctcgacatttatttctttatatatctcatcagttttatggagaagataccacgttatattctttacgaaagttaactccccaaacaaatggttcgtaggaaagtctaaacggtactgtaataatatcgttttcgtatttgtataaaagagatttatcaaatactttattcgatacaaagaagtgaccgtttacaatatcatctatgtaattcctagcgtcttctttattttttataactgatgtaaccattttaagtaacttggtatcgttatacttaatacgagaattattataaaaaaattgtctgaccaattctcccaataaaacttttacaattgatggatgtggtggaagagaatacgtttcagacatctcttgaagaatagagtatattctattcgtttctttagtcttaaattttagatacaacagctttttgatgtcaaatggtaaaacattaattaattcatcctgtgtgtaatcgtttaatgacgtcacttcgtcattgaaatcggaatatacggcggctaaaagatatacattaactggttcagaaatatcggcgtaagagaattttctaatagatcgtccaagaatttggttgtattgagaaaaagtatctgggatagtcataaaccaaatatgccttacctctttcagagtataggattcggacataatgtttgacgaaaacaaaaacatcaattgactgccatcatcgttttcaggagaattatacacatctaatagatcctctaaagacgatttcattttactagtaacgatagcaaatgtttttggtttgccgtttatcatatgtggattagttccctgagaaccattatattcagaatatccattactgagcatgatatatttaattaccaatccgccatatgtagaattagaaaagtatataaaatgttttccgttgagtgtctgtatccgattaataaagtatttaaatttggaactaatgtttaacgttaccaattcttctccgtataacacgccattatttattttcagatttgggtacaattccttatcctgttcctgaaataaagtatctaaattattcatcagattaagttgtcccaatactgccattgacacgttatacatatttttatcaaacatttcatgataacatagctgtcgtctagtaatcatataatctctctcttgaagtttagacatgtgacaatatactactctagtatctagaaacttacgtccgtgatatcttatcgttggtagatctttatcaggcatttcgtaatatgatattcttcctttaagcaaatccttaagtacattcacacctcgttcgttaagaagtgtctgaattactttcttaccacgactaataatttcaccaaaatctatcgtctcttcggacattaaatctataatatgacccagagtattaggtgtgttagtaatgggagatccagacaatagtaaaaaaggaatcttgtttttattttttatcacggtcataagttctccagtattattcccaaagatattatgtgcctcatcaacgataaaaatagagttattgtagcgagataatccgttataattaatgacgttatcgttataattaagagaataaaaacttgttgtggaatgaataaagatattctcagctatgaattcgtcattaaacaagttcatagctacacccatattataattaaaaattttcaaaatgttaatattaggcactagaatgtaaacctttttaaatctggaagctaccaaggcgaacaacaaagcgattattgttttacctgatcccataatatggaacaataacacgcttctgttctcatctatgatagttctaactagataatctagagtagctaactgatgaggtaatatagttggtatactatcaacatgattatcaaataaatctatgattccggtattcatttagatatgtgatatcttctataaatatatgagcatatatttacggagatgaaatatcctctatgaatatatattgcagatattcatcactaacattggcaaatttcttatgtctattgatgaagctctctatatcgtgtccaaatagtctagaattaaaatacttggatattttctgttggaaagtagtcaacggaagagtaaccacattatcgtacaatatatatccctttttggagaggtccgtcattaatggaatatgctttacagagctagatactaacagagtacctattttgagatagaatgcaaagtccggaatctcttccggtgtaggatatagtttcataataggaacatgatattttttgtaccatttcaccaacaagtatagaaatgcgaatctatatctattattttgtattttaccatctaacccctcgtctaatagtttgactttatcgtacgcgtcattattttcagcagcctctctaccagaaggttgagaaaagtgtgttctgaatcgcacgacggcaattcttctcattaatgcgttatctatcctatcaaagacaggtttgtaattagtatcgataatgattgtcgcatggtttctattattaattttattggagaaacacggtcttccaatgacacaaggttctgtcaactttttaatattgtcagatctaattttctttgatccactacaggcaaaatcaggtagttcgctacagaatacagatcttttcaaatgcatgttagcgataaatggattaggtcctttatccaatacatctgttaaaattgtttgacccgtctcaacaaacaggtcaccgatagcagactttaacaaacgtttggttgtcgactttccagttgcagtttctccaaaaaagaatgttaaacatcctttggtagcaccgcataaacaactagataaagttttttcgtacaactctctatttttcttattttcatccgttaatggttggatatcgttaatgatattcattaactcttccatttctggactgtcttcgacgaactttgtatcgtcaaatttaaatccggttgatacagtacacgtatattttttagcatcatctccagagtaaaacattccgtctaccaggtccaatacaccatttttaaacggaagtttatccggataggtatcggtctccactgaatctattaacatgtctcgtatgttagcttctacagtctttcgtttcctcggacagagtaattcgcttgaatattccttaggtagttgatgtcttattgacagaattagttttgttatcaagggttcttcgctgttaaatttccatgaattattaatccaaactatatggtctcctcgttcggttaataaaacagagttagtgtctaaaattctttgtgcaatattaaacagtttattaccatccaacggaacaattttaactttacaactatgtggattaccagttttgtaaattctaatagcaccattttccaacgatagttgatgcggatgtttatgcgatcgttttttacataatgcacaaggtgttacgtaatctatgaccagtggtaccgttgtaaaattattttcatcgagatcattaaagtttattatagaattaatgaatatttttgaaactctttttatagcgtcttcgaatgaaataaaccctggttcccataacttatcaggaactaaatcctccaatcgtcgttgtagagaaaagtaataactattgttgttcatatccacgtaagtgaataggtaatcttctatattatcatgcggtggttgcattacatgaatagtgtcgcaatttggatttttcctagtacctacaacccgaagagttgtttttctcctatatacggcagtgtctatcgatctggttagtggattttcagatgatctacttaattctaatagtgttcgtttcatagctatcaatgtatccatagtggtatacgtgtctaaaaagataatatgaaaacttgttttatctctatttgtagacttagtcaatgaaaaattagatctcatggattttattacattttcatgaatggcaccgcattctgtaaacgcgaatctagctacacagtttgacacctcgataataaaatcttgaatagccgttaaataatctatttcgtctagacacgcgtctaaatctacatccatgaaaattctgactatagagtatgcttcctcatccctaagactttcgaatagtgtacattctggattattctcaatatatctttctaactcgtcgcatttaaatgcttctacaaatcttggatcttcattttgtctgcacgctgacgggacacctatagtcttaagaacaaagataacatcattacctctaatagttgcatccatttagaacacaagttaaaatttcactaaagcattaataaataaacccttgagcccaatttataggtgccttgttgtctaattccagtaaaacgttgataatttcaaatgatctatctttctcgaattggcggtctctagccgctggatgatatccgactatggtagttaccggggattctaactttgcccgtatattcgagaaatctgttttacccaaacaataaagaacactaacgtgtttagttatatgctgcagcagtaacttggaaatcttatcccagtagatcgcgtgactttttgtttctcctaatttacaacttaagtaataattccagggtataaccccgtctattatattaaggttataacctttataatcaattactccggttaatctagatatagatgaagctatctccttaattgatttttttgtaaaatttggtgattcgaacggtacaccagttccatctttcggatacggatctataccacacacacatactcgtttatttctaagcggttgtttcaactgtataaagaacttatcaggaataggcgacgtctcgtctcgtagcagccaactggctacttcgttataaaactctaccaattgactcattactggttcccaatcatcgtgataagtaatagtatatggcgcgtgtgatacagtcactgaattcattatatcaaattagatacctttttatacgtatctagtaccttttcattttccgaaacgccgttaaaccaagcgaatacaaacgccttaaacttatctctattataacatattctcgttagatttaattcttcggtatccttgtatctaactattgttatatgtttagaaactctatagtggcttctaatcagatgttctaataaatattttaaaaatgaatcttgattaaaaatcatatcattgaccatttgtctggctactgaattacgataatacggagacaataacggattagtcaaatagctatcatctcctaatgatggaggcacctgtacaaataccaatcgtttattcttgaacgaatcaaacgtataaatatcataaatgacaaatttatcagtgtgcatatcttcagatatatgattggatgtagaacaccatctaacttgtcttccagcatctataaattcctccacctctatatatctaccaccgtgctgaaaactagacccatttaattcgacgcataaagatccatatgtatctggagtcacaatatattcagaaaaaaatacatgctcctttaattttgttaattttgatctgataaagtcattgtgatttcctaaaagtataaatacttcgttatcgtcgttatcgactttgggatacttattatccttaactataaaaatgtccatcaatatcgatataaaaaaaataactgatttactcaacagtagtattttattcccagatgatgtgcaagaacttcttcgagagaaatatatagtattagaaagaaaatcaaatggtacacctacagtagctcacatctataagacaatggctagatttgataataagagtatatatagaatcgccaagtttttatttatgaacaggccagatgttatcaaacttttatttttagaagacgtagaacctctgttacccgacaaaagtattaatatatctattaacaatacagagtatccacagttggaaggtcctataggaacaaaaatcgctctattggaattatttaatgcatttagaacggggatatcagaacccataccatattattatttaccgcttagaaaagacataaacaacatagtaactaagtaagtcttcgacatctaaaccttcacatttaatggctcctctatttagttcgaaaaagttttttgtagacggtctatcttccattgtagatgcgccattaataaactttttacttcgttctataattgtagcgaaatcaacgttatctacaagaacaaatccgtattcgttaaacactctgactatatcgttctttttgataatgtattcagtcattggagtagacattgttgatggattatataccactattctatcatcagctattttttctacagacatatagttttcgctactaggtaaattcttatgaattataaaagtctttttatctgttaattttgataatttgtctccgtccatggtagtgattaataccttgcctccagaagcagttagttcggataagttattcatgacggtagcataatgtctcggatgaaaagaataatggatagcaaactgccagtcgatgatattaaactttccaaaatagaatacttctctgacactagagacaaatgtatcggatcgaatagtttcctgaatgtagtcaaatttgtagtacttggttttaattccagagtttaatttgttgtatctttcatttcctctagctatagcatcagcatccggatccgtcgctaccaataacgcaatctctccataaaagtatttttccaggtccgcaccgtttccaaaatcaatcgccaatacctttcgtttgttggaatcgtctaaaaatgttttggaacaatacatagaaataagaagagtcttgacgtagtttgataaaattcccaacggtcctctagttcgtttattcgtaaaataactaacttctggatttaatctaaatttatcattattggcgtattgatgtcccacatccgatagtttatcctcgttaaagatatctcctattttgatgctttgatctcttaaatgttcgactatgatattatgttgatttccataataatcttctgagttaatatatttcatggttttatcaattctaggtttaagtatttctccattaactaagaattctgctataaacttaataggtacaaccacggacttaatacccacttcattatgtgtattaatatattccaaacaatagatattatttagataattaacgccgttatataacacaatcttaccagaaccatattctttaggaaagcctttatcgttgctaaatttcttatactctacaaagatagacgattctccaaagataattggttcactggacatgtacctaaatactacatttgcagtttggtctatagtattttcctttttaattttaaaatcaatgttagatttaggtccctttgaatagaacagaataacaccttctggttgctttggtaaatatgtagataacatatcgacgacttcactagttgtagtaaacggaccttcgtatttctttgacttgaatactatccgatcacaaatatccactagtttagattcaacatacttactttcttctagtctatcattgattgcattcacaggctctattagcttaatgagatatacggtccagttcttatccttaactgcctcaccaaagactactacttcggaatctattattctcttaacaggatatctaataatataaccaagatgtgtaaaataacaatacaacccttttgatgtaactctgatagttataggaattccgtcagtcttagttacggcatatagattttccagatccaaacctactatatcttgtttaggcaacataaaggtttttataggcgcgttaataggcggagaaagaattacattctctggagaagccataaatatatgacgtgatagagtcgtcaattcctttattagttcatcatatggaactttttcattgtctctaggtgtgaattctatttccagagatgtattaggccttgactttggatgattaatagcgtgtaataaagaacttttagactgggcaccggatcctagaaaatattttagcttaaagtctatcgtaaagttttttgtttttgcttgaataagattgactaattctagtcggatagaggatccatatttcttgtaatccaaaaatatatgacgttcctctgtcgatagtctcaacaagcattctttgtgaagacgattttccgtcactaatgatttcttttcccaaactatgttatctatagcatctactaactgtacattttttacatctagaccatgtaccttagataatggaatcttagttctaattttaacaccttccttattagtaacggtaaatcgaataaacgattcctgaatcgtagagatattcactacatttgtcaaagtaattaatggcggcttaataaatactagttccaattcattatttatttcgtatgcggtagacctctgttctaattctgaagcattcttcgctaaagcgtctatatacgttgcaatagtagaagatgatactatgttggcatccatattgtgttttattataaacgactagttttttttcatttacttattaacaagcgtcttttatatattcgtaatctatgcctttagctagagctattttaagcttttctgtatctcgactgatacgagtatctgatctattgcggtatttttttataaatcgtttaagacggggagtagttttgatatattcgctaatatcctctttaataatatccacacacgccaattgttcggctatactcgatgcgtgagtcttgcattcatctccagatatcggagtgagggtcagatccaaatattgagaagccttataattatcgtattcgaaatcaatcataaactgaccatccttatccactgaaaaaatggtattgtttggatggcgtttaaatatagacattatcaatgccataatatctaatgtgtttagctctccgaagaaagctgtcattgcgagagatttcatacgcttatccatttccatttatcggtcttgtaattatttgtgtaaagatctatatcatccatccgtagatgatttaacgtgatctacgactatagataggaattcatcgaacgtagttttagatactacatctaaaaaatttttatcctttaccatttctaaaatagtcgttgccatataagctctttttgaaattgatggagtatgacctaccacttcagcagtttgtttgatagttaacgctattaacttttttggtgacggaagaggagatatggactttacatttgtccaaaaattatataaaaacgtataattgactccatacgttcggagatccttgattctaataccaaactgtttgatacattcgtatacctttcgttcacttagtttgttgaacagaaattcttcgggactagaatcatccgtcagtttcaatagcggtttatatagtctattagacttatgaacaacaaattcatgtgaaactttgtcctttcctacaaacttgataactatttcatcgggacttatttctatgtgtttattttttagtgttaataaccctactgtttcattctccttaagatatttcattttaccaaatctaataaaaaacatagtttccattaacataaaaaccgccaactgataattggaatctgtggacgatttctttatatttttgtttataaaacaattaattcgtttcataacgttatatactctaacaaaaatacgatctcttttagcgttgcgattctgtacatgcatttttccgtaaaagtattgtctacgtccttttgaatcacttcccacaaaaattaatctagttaacgcctcctcccacgtttgttcatatactactacatctgttaaatgagtaggaattttaacatgttgcaaaacctcatacgctggattatcgtctgatacaggatttaaaaaattattatcggtaaagagtttaccatctttataaaaaagtgcacgcatttacttcttacaagttttaacttttttacgaacaactttagattttccctcggtgactagatcagatagtgttgtaatagctttagtcatagaagtaaattgtctagagataccagctgcttgaacatcctctagaaccgtcgatactgcagagattctagtaataattttcttaagatctttaacgatattgtcggtagccacctttaggtcagaaagatcgcttctagcactatgatttactttaccagcttcaacttgtaccataggttcatcatccccgtcgctatcatcgagctctacagcagccacgctttctacaatgtcgctgactccaggagatggagaatttttttcagttgtttgatgatattcctctataactacttcttcttccacttcctcctttttggttgatcttttagtagccgctggtttacgaggagtagtggctcgtttggttttgggcttagtagatggaattattacatcttccgggaaaatatcctcgtttttatctttattttcagcgctattttttagatgagctctgatttcagccatctttgtgaagctactagtatccgctttatttgtaattgaccacgccattacgatacaaacttaacggatatcgcgataatgaaataatttatgattatttctcgctttcaatttaacacaaccctcaagaacctttgtatttattttcattttttaagtatagaataaagaatctataaaaactaaaaaaattatacatcataaaccaatttcctagttgtttgtaactttaaatggactctaaagagactattctaattgagatcattccaaaaataaaagcatatctactagacgcgaatataagtccaaaatcctacgatgactttatctcacgaaataaaaatattttcgttatcaacctttataacgtatcgactatcacagaagaagatatacgattgttatacactacgatagaacagaatattgacgcggatgatcaaacactggttgctattttttcgtatataggatataaatttgaacaggctgttaaagaagagattagtacgagtttatccttcaatgacaagaataccacagatgaaatgacgtataacttgtatgatcttttttttaacacattagacatgtatttacgacaaaagaagatcagtattctggtaaatgatgatgttagaggtgatgtaatcgttagttataaaaatagtgacttagtttcatcatttaatgcggaactagaaccagagattaagaagataccgttcaatatgaaaaatctattaccgtacttggaaaagaatttggaccaactaagattctctaaaaaatatttagactttgcatatttatgtagacacatcggtattcccatttccaaaaaaaagtataatgtgcgatatgtatttctttataaaatagacggattatccattcctattatcattaaggattttttagatgttaagtacgtatatttggaaaatactggaaaaatttataaaaattctttttccgaagaccataacaacagtctatctgattggggtaaagtcatcatacctctcttaaaggatcgtcatctatatagctacatctttctatctagttatcatttacatagttactatacagatctcatcgcgagagacgagcctgtgtttgtgaaacgcaaaaaactagatattatagagatcgatgaacctgaggcatggaaaagggatgttagagtggaattcgcaccgtgtgagcatcaaattagattgaaggaagctatgaaagttgacgctaactatttcactaaaattaataattttgctaacgaatttatttattatgaagatggtgtggcatattgtagagtgtgtggaataaatatacctatatttaatttagatgccgctgacgtgattaaaaatacagttatcgtttccacgtttaacaagactatattcttgagcgaaccatatagctatttcgttcatagtcagcgctttatctttaatattatcatgtcttttgataatattatgaaatctcaaacttgggtaatgaaatacaacattaaccgactaattcttaactttcttattgatataaactctagacgtcaggaatacgaaaaaaagttttcttctgaaattaagagaggtctgttctttcttcgtttgtctgcaaacttattcgaaagtcaagtatcgtctacagagttattttatgtttccaagatgcttaatttaaactatatagttgcgttagtaatcattcttaacagtagtgcggactttatagtttcttatatgaaatccaagaacaaaacggtagaagaatccactcttaaatacgccatctccgtggttatatacgattttttggttaagactagaatttgcgagaagggatcgttggatactatagttttatttaccgatgtatacacatctataatgccggaggaattggatttacattttcagagaatcacattagaacttagaaaactagtatccattcagagatcggcgttagaacccaattacgatgtagaaagtcgcggcgaagagcttccattatctgcattaaagtttttcgatacaagcaccattatagttaagacaatggctccagtacatacatacatcgaacaaaaaattgttgcacctactccatcggtcgaaccaactgatgcatctcttaaaaacttcaaagaactaacgtgtgacgaagatattaagatctcgattagagttcatgatactaatgctacaaaattagtcatttttccatcacatctaaaaatagaaatcgagagaaaaaaactaattataccgctaaagagtttatatattaccaatactctcaaatattattattctaactcctatttatacgttttcagattcggagatcctatgccattcgaagaagaactcatagatcacgaacatgtgcaatacaaaataaattgttacaatattctaagatatcatttattgccagacagtgacgtgtttgtatattttagtaattcattaaacagagaagcattggaatacgcattttatatctttttgtcgaaatatgtaaatgtgaaacaatggatagacgaaaatataactcgtattaaagagttgtatatgattaatttcaataactaaatggcggcggtgaaaactcctgttattgttgtgccagttattgatagacctccatcagaaacatttcctaatgttcatgagcatattaatgatcagaagttcgatgatgtaaaggacaatgaagttatgccagaaaaaagaaatgttgtggtagtcaaggatgatccagatcattacaaggattatgcgtttatacagtggactggaggaaacattagaaatgatgacaagtatactcacttcttttcagggttttgtaacactatgtgtacagaggaaacgaaaagaaatatcgctagacatttagccctatgggattctaatttttttaccgagttagaaaataaaaaggtagaatatgtagttattgtagaaaacgataacgttattgaggatattacgtttcttcgtcccgtcttgaaggcaatgcatgacaaaaaaatagatatcctacagatgagagaaattattacaggcaataaagttaaaaccgagcttgtaatggacaaaaatcatgccatattcacatatacaggagggtatgatgttagcttatcagcctatattattagagttactacggcgctgaacatcgtagatgaaattataaagtctggaggtctatcatcgggattttattttgaaatagccagaatcgaaaacgaaatgaagatcaataggcagatactggataacgccgccaaatatgtagaacacgatcctcgacttgttgcagaataccgtttcgaaaacatgaaaccgaatttttggtctagaataggaacggcagctgctaaacgttatccaggagttatgtacgcgtttactactccactgatttcattttttggattgtttgatattaatgttataggtttgattgtaattttgtttattatgtttatgctcatctttaacgttaaatctaagctgttatggttccttacaggaacattcgttaccgcatttatctaacactattccatattactaaaatcggaacaccaatgcggtgacataaaataaccgctataacctaattcatttaacatctcattaccacaagtaataacattattagacttgtgttttatcaaatactgacaaaattgttgagcagatggatcgacctttgccgcctttttaaccatccacgcgtctccagtacctcgcctaatagcttgcggcagatatgttttcttatccaatcgcatagctataaaataggcgccgaaatccacacatttgaattcgaatatatcatccttaccagcggctagaagtctacctctatcactttctaattttgttttgctatccgttaatgatttccaatcgttaaccgtatttttaattcgcatatatctcgttaattcattaaagactggattatcagacgtctgaaaccagagtaatagcgcactaattgccaatataataacaaagaatataagtgttgatgttttggctgcttgtacgcctactatagccttttctctaacgtattctaaattacacgcgtttaccgataaagtagttttatccatttgtacgttataaatggataagaaaagtttgtataaatacttactactacgttcaactggagatatgcacaaagccaaatctcccactataatgacaagagtaaccaataatgtgtatttgggaaattataaaaatgctatggatgcaccatcatctgaagttaagttcaaatatgttttaaatttgacgatggataaatatacattacctaactctaatattaatattattcatataccgttggtagatgatacaactaccgatattagtaaatattttgacgacgtaaccgcctttttatctaaatgtgatcaacgaaacgagcccgtgttggttcattgtgctgcgggagtaaatagaagcggggctatgattttggcatatctaatgtctaaaaataaggagtcattgcctatgctatattttttatacgtgtatcattctatgagggacttgagaggcgcatttgtggaaaatccatcgtttaaaagacagatcatagaaaaatatgttattgataagaattaaaagtcttctgtttcttccatttccttgatcttttgagaagatatcttatcagatagtttcctttccattctcatgagaagacccaagtcgataaagtatttgtaatatccagttcctatattagggaccttgctaaaaaagtggcagctactattatcgttaataggttctgactttttatgaagagccgcgtttaacaatgctttattgtctccgaacgtagctctcttaagagtactagctgcgccgaacttgaatttattcactgattctggttcgtaactagcacatagtaaactagcgagaagatcacaaggctgatacagataatcgaacccttctccataggtgtttaacatggcttcgcacaagtattcacgagcggcctcgataccgaagatatcgtatgtattccatactccaggatacacgttgacgttttccaaatcgaaagaacccaattcttttagattcatgagttctacagtcatcttattgagcttttttgtttgattgaagtcgtcatatcccgtataatcagagataggaatcttgaatttactaatcttgcccttgttggcggcacccggaagaaccatcataaacttactaagattcaattcttccggttcaacgaaatttaggtagacagtaaatctaatattatcctcatcctcaatgaatgtttccataccccattcctttacaatgacgctaaaggagatgaatcgttcaatcatatattcgacgactaattcggtaatttctgctctcttgatgtataatctattgactattatatctactacatacctatctgtttcttttcgaagagtgatgtttggatttaattctcccaaacatacaaattcgaaattaatcttaacagattgaagtttagagatatcatcggataccagagtgataatttcggtcttattcttactcaaattagtcaagttattaaactcgttgaaaccaagtttttgtttgacggcaccacttttttcagtagtgtgaaaactggacagggcttgttgtgtaaacttctcagacaatacctgtgcagaaataattccaataggagttccaccacctagagtataattgagtttttcatagaacttttcaaagatagtgatagccgtttcttttgtaattctaattctagaaggattaagatgcgtcaagaatatatactccataaaatctatattagataccgtaaagaagtatttctctctcacatcatcaatgacgttatgaatcatatcgtacagatccttaaccttaatagcattatcctcagtggtgggtttgacgaatactaggaaattaaacggcgccaatgtcttttttgcaagtttctgtttctgagagtaaacgaatccctgttttattttattccacagagcactaatttccaaataccaagtcatggactcatctggatagataagatctacaggtttacatactgagcctagaattttggtataattggcggcgtacttgatgagcgtattacctataactacttgtccgtatccgtcgaccaccatatcctccatctttttaatgatttttctagccagtgttccggtacgtgatgtttcacagacgatatcagtagattgagatcttgcaaccagcatcgaaaagtaatattgagaacccgttaatccttttgttaaagaattaagaatgtaacctcttccttctggatccttagagtctggaagatagtaaggtaagactctacccaatactcgagtctctgctggttcaccatcaatcctctgttgtccataagtacctagaatatacattagttctgtgggatttactttataacccgctttggccattttcaggaggttattatctggatcatctatcagcgtttgtctcatatgttcttctatctctcggatattaagatttgtcaagttggataacatggattccacatagtccgcctctaaagctttagataatggaactattttcccgtctcttacatcgttgagatatttggcgtatgcttctttgataagttctattttttctacgttgatggcctccaatttattagtgaacgtcgaatttggtctcagatctttgaatgtcaccccaaaaccgtaaatagatagatatctcttaaaaacataagatgacttgataataaagttgataccttccacgttcgacttatgatcggataagagtccagccaatgacagatgcctcatagccacaacaaaattactatctacgtcgtttgcaataatttcaccatcctttaagagacccggataattaatcttttcacctatcaagtaagtatagatatctttaccgctgaatttacatttacctttaggatcgaactctcttccatatttccccaagatgttcaatacttcatctaaacaaagatcttgtatcctaaacaatgaatacgctgctacgatttcatcttgaatagatccataaacgggggctccatgaatatcgtgtttgagtaacgtcgtcggatacataagaatactttgttcaattacggctttaggattttgctccaatatcatccattcttcatctccgtcgaaatcagcattttgagagttgacaattccgggagatattttgatagtatctccttcggtagctctgatagatgaagcgatgacgttgtatctatgtagagacggctgtcttccaaaaataatacttgtatattcttgaacagctacttctacccaatcaccaggcaataaatgtattttatttttgataaactttccttggcgtattcttgttaattggtttaatcgtttattaaagtaaaatttaacttggtttgacgctaatagttgtttaactttatccactgtaaaggcattaacaaatatcttttctgtaagtgtatttctaatatatgcgggcattcctacctcattaacggtgatagatgtactgggaccaattacagatctagcggtctgatcttttcgccgggcgacgatataacttctaatcatattatttttgccggatgtgatatatgataaattgatactggaagtgttattagaaataattttaatatcatcgtattctattaccgccttctggataacctgttcatcagcattcaagttacaattcttaacgatcatacctaataagtaagttaattcattggtttctttgggtatactatctatccaaaaactaatagccggtctaataatcaacggagggatgggaaagtagtctgtataaaataagttagctggatattgatgaatttctaataatggccaaaacttttcatgaatagaaattaacttttgatagatgagagaattaggaacgttaatatcatccaacttgttgacgaaacaaacctttttctttgaaaaagtaattttttgatacggttgcatacattcactgttccaacatgactttttcttggataatattttatcctttaatctcctaagagcgtgtcccgataactcttttaggttaatatcgtcggaatacggttctcgtgaacgcaataatccgcagtgaatacatatataattcagtaaacgaataatttctgaaataaattcaggcttaactatatgagttttataaatacttactttaccccagtgaccgaaacattccaattccgttttcccacaagttttacataatgccccatccatagcacctagtctaccatctttaacggtaccgatatcgtcgtcatttttaacatgactaatgataatatctgtagcattaatctctttttgatcatatagactatacgtaaccttagagattacagccatttttatcaagtcagtttcttttaaagaaccgaaagtatacaatcaaatttccctttttattacaactataaaataatagttatatttacactttaaatttttatcatgacggacgaacaaatttatgcattctgtgatgctaacaaagacgatatacgatgtaaatgtatttatcctgataaaagcatagtacggataggaatagatacaagattaccctattattgttggtacgagccatgtaaacgaagcgatgcgttgttaccagcctctttaaaaaaaaatataacaaaatgcaatgtatcggattgtaccatttcattgggaaacgtttccattacagatagtaaattagatgtaaataatgtttgtgattccaaacgagtagctaccgagaatatagctgtccgctatctgaatcaggaaattagataccctattatagatatcaaatggcttccgattggattactagcgttagctattttaatattagcatttttctaaacaagatataagatataaaatatattattgattattataatgttcttatctcatctctactaattgattaatcagcgactgaaataacagatctatcggctatctctactccagttaccatgttattgcggaaaaatctaacaatttttaatggtatattaggacggtagagaatcttgacaactatttccgtctctaacattttgggaagacgaagagtctttttaccatcgcctgtttgtagtacactattaactatattagtttctgtagtatctagtctaacaaagctaggaaataagtcagatattaccacatctatgtatagaaaatttacaggaaacttgttatgacctttttgaagatacgatgttataatgattggttctccataatcatcatcaaccggagtataatttatggatgattcgttaaatacctgaaacacagttttcatagaatcaattttatgtctaacggttattaaagtaactaaatcattatactctatatcggtagtatatctcagtagtacgtttctatttattactgcgtacggatctcttgctatttctgtttttagacatagaatttttgctagatattttacgttgtattggttcatgactaactttttcagttgatgttgttggaatatttaagaaacgaaatatagattgttgtagaaatagtacctttgctttagtagtaggaaatgttttattgcagtacacggtcctcagcataaagtacatgtgaaaatagtcatattcctgattaggataatcaaagttaacaactactttgttacggacgatcttattaaggtagtacatctttttttcataatttacagcgtctgatttggtaactcgagtcagtctcatgttctcaccggtataaatacttaataatctcatttcagctgaatatgaaggagcaaaaggttgtaacattttattaccgtgtgggatataaaagtccttgatccattgatctggaaacgggcatctccatttaagactagacgccacggggtttaaaatactaatcatgacattttgtagagcgtaattacttagtaaatccgccgtactaggttcatttcctcctcgtttggatctcacatcagaaattaaaataatcttagaaggatgcagttgttttttgatggatcgtagatattcctcatcaacgaaccgagtcactagagtcacatcacgcaatccatttaaaataggatcatgatggcggccgtcaattagcatccatttgatgatcactcctaaattatagaaatgatctctcaaataacgtatatgtgtaccgggagcagatcctatatacactacggtggcaccatctaatataccgtgtcgctgtaacttactaagaaaaaataattctcctagtaatagttttaactgtccttgatacggcagtttttttgcgacctcatttgcactttctggttcgtaatctaactcattatcaatttcctcaaaatacataaacggtttatctaacgacacaacatccatttttaagtattatattaaaatttaatcaatgtttatttttagttttttagataaaaaatataatattatgagccgacgtaacactttctacacaccgattgatacatatcattacctcctattatctctatctcggtttcctcacccaatcgtttagaaaaggaagcctccttaaagcatttcatacacacagcagttagttttaccaccatttcagataatggaataagattcaaaatattattaaacggtttacgttgaaatgtcccatcgagtgcggctactataactatttttccttcgtttgccatacgctcacagaattcaacaatgtctggaaagaactgtccttcatcgatacctatcacggagaaatctgtaattgattccaagacatcacatagtttagttgcttccaatgcttcaaaattattcttatcatgcgtccatagtcccgttccgtatctattatcgttagaatattttatagtcacgcatttatattgagctatttgataacgtctaactcgtctaattaattctgtacttttacctgaaaacatggggccgattatcaactgaatatgtccgccgttcatgatgacaataaagaattaattattgttcactttattcgactttaatatatccatcacgttagaaaatgcgatatcgcgacgaggatctatgtatctaataggatctattgcggtggtagctagagaggattcttttttgaatcgcatcaaactaatcacaaagtcgaacaaatatcctttattaagtttgacccttccatctgtaacaatagggaccttgttaaacagttttttaaaatcttgaaagtctgtgaattttgtcaattgtctgtattcctctgaaagagattcataacaatgacccacggcttctaatttattttttgattggatcaataataataacagaaagtctagatattgagtgatttgcaatatatcagataatgaagattcatcatcttgactagccaaatacttaaaaaatgaatcatcatctgcgaagaacatcgttaagagatactggttgtgatccatttattgatcgcaaaagctttgcacaatctttatacactatcggtttactatttattgataacgcagatgtttgagttgtcatccatggtaatccatagatcattaatttatcgtcttcacacgctagattagcacgtcgtaatctatcaataggatcgggtatttttcgtttaggcatgaagaacatatttaattcagatctaaaaaatacatatattagaatgaatacaatgaatacttcaaataaaactattaatctgtgtttataaacacttaataaagaatgtttaaacgtgggctctataaacacaggattaaagtatacattaggaacattctccatttatagtaatcaatcctttgtcggaatatctgttagaggaatattctttttaacacattccaatagtcccagaaaatcatttaacctaatgggttcttgaagagggctagaactatacgattctagttccttattagtactaagtttctctagtttatttttattggtgaatccgtaaatggcattcaatctcatggatgtggaaggagaatacacattcaggacattaattcccgcatatttagatatcaaagccttgttgtctccgataggtgtatactcagtcgacgcggattccatattttctttataaatattaatctttttacgagtttcgaaaatacacaagataggtgatgatccttgacggaaaataaccatgttcttattctttctcctaccactttttttaggaatgacggcagtcatatccgtattattaatgataagaggcataacctcattgttaggatccaagaaatagttttcaatggcttcaatagttagtttatcatctcctagacccaaattgtttcttatattatacattgtggtaaacattgcccctgtgatattctcgttatgaatcaactccaactcatattttgacatcgttctaggtactatattaaaaatagaaagcatagatcttggaaatttggattttgcgccggcaataaccatttgtaaatcatcatactcagatatacttcctgcaaaaaatatggtatcttcttcgatgaggttttctagcagtagactcatttagagaagttttttttgtgataaatgaatacccgtaccgatgttacaaacgataatatagacaaaaatccaaccaaacgaggtgatagaaatataccaggaagaaatgaaagatttaatgaccaaaatagattcaacaacgatataccaaagcctaaaccaagactacagcctaatcagccaccgaaacaagataataaatgcagagaagagaatggagattttatcaatattagattgtgtgcctacgaaaaggaatattgcaatgacggatatctatctcctgcctattatatgttaaaacaggtggatgatgaagaaataagttgctggtcagaactatcgtcgttggtgagatccagaaaggcggtgggatttcctctattaaaggcggctaaacgtatttctcatggatcgatgctatattttgaacagtttaaaaacagtaaagttgtgaaattaaccccgcaagttaaatgtttaaatgatactgttatttttcaaactgtagttattttatattccatgtataaacgtggcatatattctaacgaattttgttttgatctggtttctattcccagaacgaacattgttttttctgttaatcaattaatgtttaacatttgtacagacatattggtagttctatctatttgcggcaaccggctctatagaacaaatctaccacagtcgtgttacttaaatttcatacacggccatgagacaatagcccgtagaggatatgaacactccaattacttttttgagtggttgataaaaaatcacatatcgctattgaccaagcaaacgatggatattctcaaggtaaagaaaaagtatgctacaggagcaccagtaaataggttgttagaacctggtacactggtatatgtgcccaaagaagattattactttataggcatatcactcaccgatgtgtcaattagcgataatgtcagagtattattttccacagatggaatagtgttagaaatagaagactttaatatcaagcatttatttatggcaggtgagatgtttgttagaagtcagtctagtactattatagtataaagtaataaaaaatagttaatgtgatgactagcgccaccaacgccaacaacatttgataatttctacttactagacgtaccgtaaaaatataaattactataacaaataatagtatatcaataaacaacctaattaatggtcgaagtatagcaggacattgatgctctagaccgtgtataacaaaatctacaaatttttcatccgctatattttgtttcactatatcgtctagacgatcagcgataacttccatgttaatctattaaaatattatcaatatattttcagttttgcatatccgtggtagcaataaccatcggagaagttctaaagaatgtgtccatgtaagtagtccaatggacgttttccttattggctaaaataagtttgattttatcattggtggatgtgaacaacatacgcttggcatagtacataaacaacgctgccaatattataacaccgataacaatcatataaaactgaactcctgtaccagcaacttgtctaggtgctatttgagtagtggccttagtcgtcaattgcatcaacgctttaatggcacaatttcctttgctagatcctgtattaataaattccaaatttgttggagatcctggggctccgtaacattcatctatgattacgttttgtatctttaatttgttatcgacgaccgcgctagaattacaagtctgtttcacataattttcaaaatctctaacaacagtgtttacactcgtctgaatgtttaacgcagcagtaaacatagctggtacgtatgctttttgttccggtgttaatccactatatgtttctgtagcggctgataacacagcatccaactgagcatccgcgtccgcagagcacatatttttaacagtgaggttacatccatggttttgtcggatataaaaatttccgatttctatatcacattttgtttgagcactagcgttcgcttcttgttctaatttagacgagatacgttcgctgagtgtattcaccgtcgtctgtatgcttgccgcggcacccatttaaatagctacaattagtatccatattaccaagagagataataaactgatcaaatgcaattttaggtcgaacgaatgtttaatattatgttgaactacttttgctctattgacgggaacagtagaaaatctatcactattgcttaatccacatgacaatcttaatgaggaagttttatccatctgtaagttgttcacgctagtattacatcgtacaatattgcaaagtcctaaattattataattacgtgttagtaagaaattaacattggcattcgaacactctggatcccaacattctcgaggttccgcatattttaatgactcttctaacttatctctagtgggataactacatctcatatatttctgtttaaagtccgcagactgttgtcttagaatataatcgatcatctctttgctatcttctgtattgtgtgcgcgtaaatgatgcaaaaatgattcacatattggtacactagcatctttactacataatgtttgcatcttattatacagatttattaacgattgttgaccctctacagttctatcactcctattaaaggctgaaccgatccactgatggcatatgtttctatcgaacgtatccccctgacaccagtcgaataaatcaacatcgcattttccagtgtcgtgaacgtctggccaacacgattctaatactgcaccctcttcatacttatctgatatctttccatcctttttccaataatgagtacgattaaaagtgcgacagcaattgggtgcggttccattatacgattgtcttaacaatgccgaaagaccaccgggtcctgtgttgactaatctaaactctggatatcttttctttactttatcctctttatcttttgctagtggtcctatatgcacatattctaaaagcttagcgggagctatcacgtcatgcattttatccacgtttaataacatctcatcagtgggtactcccggaggcggatcccgtttagggagctcaacacttactctgccacccatatttatctcattgaaagtattaatctaaaaacgtcataaagatgttgatcttaaaggattgaactctatccgaaaacaacattcctagaatgttatcgtcattatccattacgattctagtttcaaaaacattgactctctttttgaatcctcgtagtttgttgagagacgagatagctattttgaaagaaaacttttgtagttcttgagaacattcagtcatagaatattccctggaaaacgcatcagtattaccaggagtcttcataataatattgtcatctttaaacataatagccaaatgctgatgctgactaatacacttgataaagcccaacaaccattctaaatgaatgacggttctaccacaacatttttcttcatacttgtgaaaattaaacacgtaagatttcttttgatctatacttagacaaatagtagtatctgtcctaataggcatcagttccttgttacaatcgacacttactacatgataactagaaagttttactagattattttccagatcaggttctatatctatgatggcatcattgtgaaaactacacaaacacgattttaccttggacacaggaagattaaacacaatgttttcggctccgcggtagaacactgatgcactgagaggtataatggcccaaatgtttacagatccgcccaaggcggcaaaaatatacattaactcatccgtcgagtctacatttatagatacttcttcactgaactctgaaaaatatgccacaatttggcgcagtttatcgatttttatacggatgctcattttaaatttttgtaaattatttaaagttaaatggctgcagaacagcgtcgttctacaatttttgacatagtttcaaaatgtatagtgcaatctgtattgagagatatatctattaattctgaatacatagagtccaaagctaaacaattgtgctattgtccggcatcgaaaaaggaatcagtgattaatggtatctacaattgttgcgagtcaaatatagaaataatggacaaagagcagctattaaaaatattggacaatcttcgatgtcattcggctcatgtatgtaacgccacagatttctggagactatataattcgttaaaacggtttactcatactaccgcattctttaatacatgcaagcccactattctagccacgctaaacactttgataaccctgattttatctaacaagttattgtatgcggcagaaatggtagagtatctagagaaccaactagattcatcaaataaatcaatgtctcaagaactagcagaattattggaaatgaaatatgctctcattaatctggtacaatataggattttgccaatgatcatcggtgagcctattatagtagctggattttctggtaaagaaccaatttctgattattctgcagaagtggaaaggctaatggaactaccagttaaaactgatatagtgaataccacatatgacttcttagccagaaaaggtattgatactagcaacaatatagcagaatatatagccggcttgaaaatagaagagattgaaaaggtagaaaaatatttaccagaagttatatctacaattgccaatagtaatataataaaaaataaaaaatctatctttccggccaatatcaacgataaacagatcatggaatgctctagaatgttagacacgagtgagaaatactctaaaggatataaaactgatggagctgtgactagtccattgacgggaaataatacaattacaacatttataccaatttctgcgtccgatatgcaaaagtttaccattttagaatatctttacattatgagagtgatggcaaacaacgttaagaaaaagaacgagggaaaaaacaacggaggagtagttatgcatattaactcaccctttaaggtaatcaatttgccaaaatgttaaattattagaatcatatatctttatccatctattatcatctgtgaagttttggctcagaaaaatatctttacctaatattcgtttagacgatgtatcaataccggcatttttataacattcagctaccaatttaaaacaatacattctattatgaccaaatccatacggaatacccaataaagttaatgacgtatcagctgctattttcataacttgaatattctctaacatgtatacttttgcactaagatatccttcaaaaaaactatccaatgggactattcgaactccttttctataggtagattcaactaccaagtgttccgataataacgtaccataataaatacccacatgtttttctatcgatggattcaaatgacttgttaatgacatggtataattaataaaaataatagaacctctaggcgcatatgtcttgataaaattaaccggatccatattagtttatatccaatagaggttgcactgttaagttacgttgaggttctatttgtgtagataattttaacctacaacattcgttctttacactgacgagtacatcctttaatgatttttttcgtataatcaatttatatcgttcgtgagaaatatctttgccgcacgtagagcacacgagttggaacaccatttttaatctagtaacctatatttattatattatcacttttagtattggttattaacagactatcgttaaagtaaaatgaactatttatactcagtagtaaattatccttatagatgccgaacactatagtgttacagttttcgttagaatatccgaagatcgaagatatagattttataacatcgatatctgatttagtattttcgaaatctatataagatgataaagttttaacttctgaaacatcaatctccttgcgtggttctaatgcatacattaattggcagggtaacggaacggtctctaaataagatgatttaaaattgttccatttttcatctaatgcggaaaatataaattcttgaacagtgcattgacaaggaggaacatacgagtagacatcgtctaaattagcgtaatcgtttataaacgtaacaatattacgcacgtctacggtagagttagtctttctataataatttttaattgccaaactagtgactatattatcgattgtaaaatcactaaacaattgtattttgtttaagttggtgggtgttatagatgccccatagagtccaggaaagaaatcacatccattcactaacgccgttaattttgctaaatagttatcctctgccgagggaacaaatttaaacagttgagttaagttttttatcatcttaggatgattatcagtagatgcaaatagcatagtatcctgatcggtacttattatcaacggccattctcctgtggtagagaaatgtgttttagcctcgagacacataacgaattctgcgtctcgttcatcacaataaaataatgtaacattctcattattgttgaaatgtgttagtatctcattcaatgatatttttatgttatcagaatcagataaatatatttgaaatgtgagtttatcgatttttaattgcatttctgcctttatttcttcttccataaatccggtaacattttgtatttcggatgtacacttttctaattctagcatttttctgtccttggttaatttagaatatttacgtctcttgtctctaacgtcttgtttaatttttatacttcctctatcgataaaaagggttacatgccctcccttttttacccatccgtttacgtattttatgaataccgtagttaactcttctaagtttctgacacaattggcgacggctatataaatactcattgtatccacaaatattccattgtatactttgtataaattatcatctaatatcgtcagtgatttattttccagcagtaacgattttaagtttttgatacccataaatgaagaacgtactgattattttcggtaaaccgtattgtagtatttgtgaaaatgtcagtgatgcagtagaagaattaaaatccgagtatgatatactccatgttgatatcttatcattttttttaaaggatggtgattcaagtatgctgggtgacgtaaagcgcggaaccctaataggaaactttgcagcgcatctatctaactacatcgtttccattttcaaatacaatccacagacaaaacaaatggcatttgtggacattaataaatccttggatttcaccaaaaccgataaatcgctggtgaatttggaaattctaaaatccgaaatagaaaaagcaaattatggagtttggccaccggttaccgaataaaatatcttcctgagtattttgtttattgttccgcttcctttatcaaataaattttgaagtatttgataatttattggatcgactagttcatctatacattttttggaaacgagaacatctacctttttatttgttgttatatgcgacgttgtatacgccataaatgtaacttgagaaaatccacaaagaattaattttgaaccagttatggggacgcgctcattagaatatgtataaatctgaggagtgtattccttgaggagatattctatcaagtcatcatttgcttctctaatataaatattcctgtcctttataacaactatgccttttagattatctcctaatttataacacggccgtatacacttggaatacttgtacaatctaagatagactaaatctctcagagttgtatcatggaattccatacttaattcctccgataaatctacatgttcaaatactttagaaatatatttatggtatttcctatctggaaagtaagttatcaagtcatcataagatatttcaaatcctctacataaggaagacactatctccaacgattcctcatcttctgtaagtaggaatttggacaagttaaacaaaattagatctctaaatggcatctttattatatcttattttatttttgttattcgtatgtatttcttattattttacatattatccgaccaataaacttcaggcagctgtaatggaaacagatagagaaaacgctattattagacagcgaaatgatgaaataccgactagaacattagatacagctatatttaccgatgcatcaaccgtcgcgagtgcgcaaatacacctatattataattccaatattggtaaaattataatgtcacttaatggtaaaaaacacacctttaatttatacgatgataacgacatacgaacattacttcctattttactccttagtaaatgattgtcttaccgaataaagttcgtattttcatcaacgatcggatgaaaaaggatatctacttgggaatttctaatttcggattcgagaatgatatagatgaaatcttgggaattgctcacttgttggaacatctacttatatcctttgattctactaattttttagcgaatgcttctacatctagaagttatatgagtttttggtgtaaatccattaattcagcaacggaatcggacgcaatcagaacattagtttcgtggttcttttctaacggaaaactcaaagataatttttccctttctagtatacgatttcacattaaagaattagaaaacgaatactattttagaaatgaagtattccattgtatggatatactaacgtttcttagcggaggcgatttatataacggtgggagaatagacatgatagataatcttaatatagttcgtgatatgctggtaaatagaatgcaaaggatatcgggatcgaatatcgtaatttttgttaagagattaggacctggaacattggatttcttcaaacagacatttgggtctttaccagcatgtccggagattattccttcgtctattccagtaagtacaaacggtaaaatagttatgactccgtctccattttatacagttatggtaaagattaatccaacattagataatattttagggattctgtatttgtacgaaacttaccacttaatagactatgagactatcggcaaccagttatatttaacggtatcctttatcgatgaaactgaatacgagagctttcttcgtggcgaggctatattacaaattagtcaatgtcaacgtattaatatgaattatagcgacgattatatgatgaacatctatttaaattttccttggctatcgcatgatttatatgattacattacacgtattaatgacgatagcaagtcgatactaatatccttgacaaatgaaatatatgcatctataattaatagagatatcatagttatttacccaaactttagtaaggccatgtgtaacactagagatacccaacaacatccgatagtagttcttgacgcaaccaatgatggactgattaagaaaccttatagaagtatacccctaatgaagcgtctaacatctaatgaaatatttatacgatacggagacgcgtctctcatggacatgataactttatcattgtctaaacaagatatatcattaaaaagaaatgccgaaggaatacgtgtaaaacatagtttttcagctgatgatatacaggcaattatggaatctgattcgtttttaaagtatagtagatcaaaaccagctgcgatgtatcaatatatatttctatcattttttgctagtggtaattccatagatgacatattggcaaatagagattctaccttagaattttctaaaagaactaaaagtaaaattttgtttggtaggaataccagatacgacgtcactgcaaaatctagttttgtatgtggtatagtacgaggtaaatcattggataaaacgtctctggttgaaatgatgtgggatctcaagaagaaaggattaatatattctatggaatttaccaatctattgagcaagaataccttttatctgttcacatttactatctacactgatgaagtatacgattatctaaacactaataaacttttttctgcaaaatgtttagtcgtgtctacaaaaggagatgtggaaaatttttcatctctaaaaaaagatgtggtcattagagtttgatttttagttattatctacaggaacaaatatagtatctgaaatcatattcatatatcccgttagaggtctatgataatatatagtagcgtttgttccgttatagacaccgaataatattttacaaaagtgtatatacgtatcatcatctttatgtttaaaatttaaaatcttaattcgtaaatttagagataaaatggcttcttgtacaatactagttaattctcccgtcctctcaaaattatccaactcctcagcgagaataggacttagtacataaagtttagcatactctatcatcttcatataataattggataataatttattccatgtttctgtactaatatcgaacgagtctatatattcctttgtacgccatagaatatccaaatttgtagggattataaacaaatcttcggggagtgttagattaaacttattagcgtacaatatataattatgtagaaattctgaatctattcgctgtatagacttcatataagacagatcatagaaatatacgtatgtcccaggattaactcttcctactcttccttttcgttgatctctcatagatttagaaataaattcttgcgatcctccaaaaggagcggggacaaaaactctacccatatcataaatgtgtgtaacattgcgtatagtaacgctggattccaaataaggagtagaaataattatcgatacattaggtgatgaatacactttttctaatatttcgtctatatctaagaccttaccatgaataatatacatatcatacggtaatcttttttctaaatatgatttatattcgtgacactgtgcaacggatgccacaaagactataccggatgatccatcaggaggagtatacatctgtatagcagtaactaaatttctcttttcttcttctatgtatgccattctggaagatggatttatcttattatgaataaatacctcgctaattttaaacagtgtatctccaggaatatgtataaatgcgggattaggtaaaaatacttttagccgttccctgtcatcctctaacgtggcagtcattaaaaacatagaatctattttcgtatgatgctttctcgctactgctataataatatctcctatttgatcatgctcatgaacttcgtctataataagagtgccataactaaatagttttgttagagataacttatgggtagaaaatacaattccatatttttttggttgtttgtttattaattcttccggtatagatccgtaccgtaaagaaataggagatccatctagtaccttaaatcccaatgattttaaaatggtattgctatgcaatctaactaaagctatcctaggaagagatagaatgactggtctttcgtgaaagtcagtgattttatctagagtagagaatccaccaaataaataattaaaccaaagcaataacttgggtacctgtgacgtcttacccactccagttcctccagttaaaactacaggtctatgagaaatccacgctgaaaatatctctcgttgtgctttaggagttaatgaggccaatggaattttgctaaatggatacttattccctagtacacctatagtatctgttcgtttacctacggaattggaaaatatctgtaaactattaccagcttctaatagtcctcttaatatatactcatcgaacgaattgatttctgtatttgttatacattttagaaaactataacattcaaagcttattgtgtgttcactgtatatatattgcttcgcggttaggtttatgtgtgcgggttttcctagtgatggaggagatactttttttccacgtgcttctgtactaactttgtatattcctttatgttttacaacgtgtgcgttatgccatctatgttttataactggaaacaccgccaatgagaaactatcacgttccgttttactcatattactgaattcatcttgtgaatatttgtaagagaatacattaacgcagtttggaaaaaagaagatatctggtaaattcttttccatgataaatggaaagatatacagatttagtaattagtaaaataccagaactaggatttaccaatttattatgtcatatatattcactagctggattatgtagcaatatagatgtatctaaatttttaacaaattgtaacggatatgtagtggagaaatatgataaatctacaaccgccggcaaagtgtcttgtattcctatcggtatgatgttggaactagtagagtcggggcacctgagcagacccaatagtagcgacgaactcgatcaaaagaaagagttaaccgacgagttaaagacgcgttaccattctatatatgatgtctttgagttacctactagtataccgttagcgtatttctttaaacctcgactacgggaaaaagtatctaaggcgatagacttctcacaaatggatttgaaaatcgatgatttatcacgtaaaggaatacatactggtgaaaatccaaaggtcgtcaagatgaaaatagagcctgagagaggagcctggatgagcaatcgaagtattaagaacttagtctctcagtttgcttatggatccgaagtggattatataggacaatttgacatgagattcttaaactccttagcgattcatgaaaaatttgacgcgtttatgaataaacatatcttatcgtatatacttaaagacaaaattaaaagttctacctctagatttgtaatgtttggattttgttatttgtctcattggaaatgtgtaatttatgataaaaaacaatgtttagtatccttttatgactccggaggcaatattccaactgaattccaccactataataatttttatttttattccttctccgatggttttaacacgaatcacaaacattctgtattggataatacaaattgtgacatcgatgttttattcagatttttcgaatgtacatttggagcgaaaataggctgtattaatgtagaagttaatcagctgttggaatctgaatgtggaatgtttattagtttgtttatgatattgtgtactaggacaccacctaagagtttcaaatctctgaaaaaggtttatacattctttaaatttttagcggataagaaaatgacattatttaagagcattctatttaacttgcaagatctatccctggatataacggaaacggataacgcaggattaaaagaatataaacgtatggaaaaatggaccaaaaagtcaattaatgtgatatgtgataaattaactacaaaattaaatagaatagtaaacgacgatgaataactttgttaaacaagtagcttcaaagtctctaaaacctaccaaaaaattgtctccgtcagatgaggtgatatctttaaacgaatgcataatatcctttaacttggataacttttattattgcaacgatggactgtttactaagcccattaatactccggaggatgttcttaaatcactcttgatcatggaatcattcgcctacgagaagatgataatcaaaggattgataaaaatactaatatctagagcatatattaatgatatttattttactccattcggttggttgacgggcgtcgacgatgatcctgaaacacacgtggtgataaaaataattttcaattcatcactaatatctatcaagtctcaagttatagaatatttaaaaccatacaatgtcaataacctatcggtacttaccacagaaaaagaattaagtattaatacgttcaatgttccagattctatacctatgtcgataatttcgtttttcccattcgatacagattttatactagttattttgttttttggagtatataatgactcgtattgtggaataagctatataagtccgaaagagagactaccgtatatcatcgaaatattaaaaccgttggtgtcggaaattaacatgttatcggatgaaataggtagaacatcatccattagaatcttcaattccactagcgtcaaaaaatttcctactaatacattaacatccatttgtgaaattgtttattcgtttgatgaatcatcctttccgacgcctaagacgttcactcctctaaacgcgagtccatacattcctaaaaagatagtttcactattggatttaccatctaatgtggaaataaaagcgatatctagaggcggtgtggatttcatcactcatattaataataagcgtctaaacacaatcttggtaatagcaaaagataactttttaaaaaattctacattttctggaacttttatcaaagagaatattatttggaagggtatctatacttatagaataatcaagtctagttttccagttcctactattaagtcggttactaataaaaaaaaaatatgtaagaaacattgtttcgtcaattctcagtatacaactaggactttgtcacatattctttgatctaatttttagatataaatggtggatgctataaccgttctaactgcgatcggcataactgtattaatgcttttgatggtaatttctggcgccgccatgatagtcaaggagttaaatcctaatgatatattcactatgcaatcattaaagtttaatcgagccgtaacgattttcaaatatataggactctttatctatataccaggaacgataattttgtacgctacatacgtcaaatccctattaatgaaaagttaaataattttttttattacaccaacaaaaatgtttgtcattaaacgaaatggatacaaggaaaatgtcatgtttgataaaatcacgtctcgtattagaaaattatgttatggcttaaacacggatcatatagatcctattaaaatagctatgaaggttattcaaggaatatataatggagtaacaacggtagaattggacactctggcagccgaaatagcagccacttgtactacacaacatccggattatgccattctagccgccagaatagccgtatcaaatctacacaaggaaacaaaaaaactatttagtgaagtgatggaggatttattcaactatgttaatcctaaaaatgggaaacattctccgattatttcaagtatcaccatggatatagttaacaaatataaggataaactcaactcggttattatttacgaacgagacttttcatacaactattttggttttaaaactttggaaaaatcctacttgttgaaaataaacaacaagatcgttgaaagacctcagcacatgttaatgcgtgtcgcagtaggaattcatcaatgggatatagactcagctattgagacgtacaatctactttctgaaaaatggtttacgcacgcttctcctaccttatttaatgcgggaactagtcgtcaccaaatgtctagctgttttctacttaacatgatcgatgatagcatagagggtatctatgacacgttaaaacgatgcgcattaatctctaaaatggcagggggaataggtctatcaattagtaatattcgtgccagtggaagctatatctccggtaccaatggtatatcaaacggtattattccaatgttgagagtttataataacaccgctagatacatagatcagggaggaaacaaacggcctggagttatggccatatacttggaaccgtggcattctgatattatggcgttcctcgatcttaaaaagaatacaggaaacgaggaacatagaaccagagatctatttatagctctttggattcctgatctctttatgaaacgagtgaaggatgacggagagtggtcgttgatgtgtccggatgaatgtcctggattggacaatgtttggggagacgagttcgaacgattgtatacactatacgaaagagaaaggagatacaaatctataataaaggctcgagtcgtctggaaagcgattatagaatctcagattgaaactggtactccattcattctttataaggatgcgtgtaacaaaaagagtaatcaacaaaatttaggaactatcaagtgtagtaatctttgcactgagataatacaatatgcggatgctaatgaggtagccgtttgtaatctggcatctgttgccttgaacatgtttgtaatagatgggcgatttgattttctcaaactgaaggatgtggtcaaagtaattgtcagaaatctcaataaaattatagatattaattattatcctattccagaagctgaaatctctaataagagacatagacctatcggtattggtgttcaaggattagcggacgcgtttattctcttaaattatccatttgatagcctggaagcacaagatctaaataagaagatcttcgaaaccatttattacggtgcattagaggcgagttgtgaactagctgagaaggaaggaccatacgatacatatgtaggatcgtacgccagtaacggtattctacaatatgatctttggaatgttgtaccgtcggatctttggaattgggaacctctaaaagataaaatcagaacatacggtcttagaaatagtttattggtggcacctatgccgactgcatcaactgctcaaattttgggaaataatgagtcggtggaaccgtataccagtaatatttacactcggagagtattgtctggagaatttcaagtagttaatccgcatctccttagagttttaaccgagagaaaattatggaatgatgagatcaagaataggattatggcagatggtggatccattcagaatacaaaccttccagaagatattaagcgagtttataaaactatttgggaaattccacaaaagacgatcataaaaatggctgcagacaggggagccttcatcgatcaaagtcaatctatgaatatccatatagcagatccgagttattccaaactaacgagtatgcatttttacggatggagtctcggtctaaaaacgggaatgtactatctacgtacgaaacccgcatccgctcccattcaattcacattggacaaggataaaataaaaccactggtggtttgcgattccgaaatctgtacatcatgcagtggttaaacaaaaacatttttattctcaaatgagataaagtgaaaatatatatcattatattacaaagtacaattatttaggtttaatcatgagtaaggtaatcaagaagagagttgaaacttcaccaagacctactgcatctagcgattctctacagacttgtgcgggtgttatagagtatgcaaaatcgattagtaaatctaatgcaaaatgtatcgaatacgttacactaaatgcttctcaatacgctaattgttcgtctatctctataaaacttactgatagtttatctagtcaaatgacttccacttttattatgttggaaggagagactaaactttataaaaataaatctaaacaagatagaagcgatggatactttctaaaaataaaagttaccgcggctagtcctatgttgtatcaacttctagaagccgtctatggaaacattaagcacaaggaacgcattccaaattctttgcatagtctttcggtggaaactattacagagaaaacatttaaggatgaatccatcttcatcaacaaattaaacggatccatggtagaatatgtttcgactggagaatcatccattctcagatctatagaaggtgaactagaatcactcagtaaaagagaaagacaattggccaaggcaattatcacacctatcgtcttctatagatccggaacggaaacaaaaattacattcgcactcaagaaactaatcattgatagagaagtggtggctaacgttatcggactctctggagatagtgaacgtgtatcaatgactgaaaatgtagaagaagatctggctcgtaatctgggacttgttgatattgatgatgaatatgatgaagatagcgataaagaaaagccaatattcaatgtataaatggataagttgtacgccgctatatttggtgtatttatggggtctccggaagatgatttgacagactttatagaaattgttaaatctgttctaagtgatgagaaaacagtcacatcaactaataataccggttgttggggttggtattggttaattattattttttttatagttcttattctactactattgatatatttgtatttaaaagttgtttggtgaacttaaatggcggaatttgaagatcaactcgttttcaatagtatcagtgcccgtgcattgaaagcttatttcactgctaaaatcaatgaaatggtagatgagttggtcacaagaaaatgtccacaaaagaaaaaatcacaagctaagaaacctgaattacgcattcctgtagatcttgtaaagtctagttttgttaaaaagtttggattgtgcaattatggaggaatccttatcagtcttattaatagtctagtagaaaataatttctttacaaaggatggaaaactggatgatacaggcaaaaaggaattggttttgacagatgtcgaaaaacgaattcttaataccatagataaatcatctcctttgtatatcgatattagtgatgttaaagtattggctgctagactaaaaagaagcgctacacaatttaactttaatggacatacatatcatctggaaaatgataaaatagaagatctcattaatcagttggttaaggacgaatccattcaactggatgaaaagagttctattaaagatagtatgtatgtcattcccgatgaacttatcgatgttctcaaaactagattgtttagatctcctcaagtcaaggataatattatttcgcgtactagattgtatgattattttactagagttactaagagagacgaatcgtcaatctatgtgattctaaaggatcctaggatcgctagcattttgtcactagaaactgttaaaatgggcgcctttatgtatacaaaacatagtatgttgacgaacgctatttcatctagagtcgatagatattctaaaaagtttcaagaatctttttacgaagatattgtagaatttgttaaagaaaatgagagagttaatgtatcgagagtggttgaatgtttgactgtgcctaatattactatatcaagtaatgctgaataaaaatatttataaatatgctcgtcgtaattatgttttttatagcgtttgccttctgtagttggctatcatatagctatctgcgtccatatatctcgactaaagagttaaataagtcgagatagttttatatcacttaaatattaaaatggccgaggaatttgtacaacaaaggttggccaataacaaagtgacaatttttgtcaagtatacatgtcctttttgtagaaatgcactggatattctaaataagtttagtttcaaaagaggagcgtatgaaattgtcgatattaaagaatttaaacccgaaaatgaattgcgtgactattttgaacaaattactggtggtagaactgttcctagaatcttttttggaaaaacttctattggtggatatagcgacctgttggaaatagacaacatggacgcattgggtgatattctatcatctattggggtattgagaacttgttgagaaaataatgaaaaaacaatacttaatcatgtcgccgacatgttcatgtatccggaatttgcgaggaaggctttatcaaagcttatttcaaaaaaattaaacattgaaaaggtgtctagcaagcaccagctcgtgttactggattatggattacacggactattgccaaaatcactgtatctggaagctattaattccgatattctcaatgttagattctttcctcctgaaataataaacgtcactgatatcgttaaggctctccaaaattcttgtagagtagatgagtacctaaaatctgtttccttatatcataagaattctttaatggtatcgggaccaaatgtagtcaagcttatgatagaatataatcttcttacacacagtgacttggaatggttaattaatgagaatgtagtcaaggctacataccttttaaaaatcaatgcctatatgattaactttaaaatagatctaacggttgatgaaatcattgacttagttaaagatattcctgtaggagctacgctacatctatataatatattaaacaatatagatttggacattgttcttcgtatatctgatgaatataatataccacctgttcacgatattctgtctaaacttaccgatgaagagatgtgtataaaactagttacaaagtatcctatggacaatgttataaattttattaatcaagatgttagatatagtcccaccttcatcaagacaattaaagattttgtcaacaagcatcttccaaccatgtacgatggattaaatgattatctacattctgttattatcgacgaggacttaatagaggaatataaaattaaatccgttgccatgtttaatttggaatacaaaactgatgtagatactctaacattggacgaacagatatttgtagaggtaaacatctcatattatgattttagatatagacaatttgccgatgaatttagagattacattatgataaaagaaagaagacaaatcaccatgcaatctggtgatagaataagaaggtttagacgtcccatgtcattgagatccactatcatcaaaaaggatactgattctctagaggatattctcgcacatatagataatgccagaaaaaatagcaaggtatccattgaagatgttgagagaatcatttcatctttccgtcttaatccttgtgttgtcagacgcaccatgctgtctgatatagatatcaaaacaaagattggaaatcttgtgctctgacactatcagccatcaaaggaattatggtaacagataccatcaataccgtgttatccaaaattctgcatcatcataggaatgtcttcaagtatcttacatctgtagagaataaagaaattgctgtctgtcgctcttctatagagaattaaaaagtgtacgatgtgatctacgcacagatgatggattattggataggctatacgatctgactagatacgccttacacggaaaaatcaatcaaaacttaatcggtcaacgatgttggggtccgttgacagaaatgctgtttaacgagaataaaaagaaaaaactaaataatttaatggaatacatcaaaatatcagacatgttggtatacggacactctatcgagaagacgcttattccaattactgattctctttcattcaagctatctgttgataccatgtctgtgttaaatgatcaatatgccaagattgtcatcttcttcaataccatcatagaatatattatagctactatctattatagattgacagtcttggacaattatactaatgtcaaacattttgtatccaaagtgttacacactgtcatggaagcatgtggcgtactgttttcatacattaaagttaatgacaaaatagagcatgaattggaggagatggtggacaaaggtaccgtaccttcttatttgtatcatctgtccatcaacgtcatttcaataatattggatgatataaatggaactcgttaatatttttttagaaacggatgctggaagagtaaagtttgccataaaaaataccgacgatgtatgtgcctcggagttaataaataaatttgtggaactgttaagtgaatacattcacattgaccaatcagaattttatttggtggtaaaggataaggatattttttattttaagtgtgatagggggtctatttcgattgtaaacaatgagttttatgtctttgacgaacccttgctgtttgttaaagatttcactaatgtaacgggggttgaattcatagttacagaaaccatgccgtgtagaattataccaaaaaataatcacgcggttatttcagtcgtgactaatcataagttttataatgggttaagtttataaagggttaacctttgtcacatcgatcgcgtatttgggatcagatgccaaattgttaaataatctgatgaaaaaataataaatataattcagatcatcgctagacatgacattattgtcctctatagcgatagtcgcgtgccgtctacatgcaggacatggaagagtgctgactatagtatatagttttcgtttacacgcttctatgttgccgtctaaacccgcttgcgaaagtactataaaaataatggtccatacggctcttccccaatgtttgggattcatttaaatgaaaatatatttctaaattctataaatggatgttcggtgcattaattggtttgaaagtcacggtgaaaacagatttttatatctgaaatccagatgtcgaaatggcgagaccgtatttatacgatttcctcattacttttattacgtagttacggacgaaatatatcagtcattgtctcctcctccatttaatgcgaggccgttgggaaagatgagaactatagacattgacgagacaataagttataatctagatattaaagatagaaaatgctccgtcgcagatatgtggttgatagaagagccaaagaaacgcagcatacaaaatgccaccatggatgaatttctcaatattagttggttttatatttctaacgggatatctccagacggatgttactcgttggacgagcaatatttgacaaagattaacaatggatgttatcattgtgacgatccacgtaactgtttcgctaaaaaaatacctagattcgatatcccaagatcgtacttatttctagatatagagtgtcacttcgataagaagtttccttctgtatttattaacccaatctcgcatacaagttactgttatatcgatttaagtggtaaacgattattgtttacgctcattaatgaagagatgttaacggaacaggaaatacaagaagccgtcgatagaggatgtttgaggatacagtcactaatggaaatggattacgaacgagaactagttctatgttctgaaatagttttgttacgaatagctaaacaattgttggaactaacgttcgactacgtcgttacctttaacggacataactttgatctgagatatattactaatcgtctagagttattaacaggagagaagattatctttagatctccggacaaaaaggaagctgtacatctctgtatttatgagagaaatcagtctagtcataagggagtaggcggcatggccaatactacgtttcacgttaataacaataatggaactatatttttcgatctatattcattcattcaaaaatctgaaaaattggattcgtacaaattggattctatatccaagaacgcgttcagttgcatgggtaaagtattaaatagaggagttagagaaatgacgttcatcggtgacgatactacggacgcgaaaggcaaagccgctgcatttgcaaaggttttaaccacaggtaattatgtgactgttgatgaggatattatatgtaaagtaattcgtaaagatatttgggaaaatggatttaaagtcgtactatcatgtcctactttacctaatgatacatataaattatctttcggaaaggatgacgttgatttagctcagatgtataaggattataatctaaacatagctttagatatggctagatactgtattcatgatgcttgtttgtgtcagtatttgtgggagtattatggagtagaaacaaaaacagacgcgggtgcgtcaacatatgtgcttcctcaatccatggtattcgaatatagagcgagtacagtcatcaagggtccactgttaaagctattgttggaaactaaaactatcttagttagatcagaaacaaaacaaaagtttccttatgaaggcggtaaggtatttgctccaaaacaaaaaatgtttagtaataatgtattaatctttgattataacagtctgtatcctaatgtgtgtatctttggaaatctatctccggaaacattagtcggtgtcgttgttagtaccaatagattggaagaagaaataaataatcagctcttgcttcagaaatatccacctcctagatatattacggttcattgtgaacctagactaccgaacctcatctctgaaatagcaattttcgatagatcgatagaaggaaccattcctagactattaagaacatttttggcagagagagccagatataaaaagatgctaaaacaggctaccagttcaactgaaaaggccatctatgattccatgcaatatacgtacaagatagtagccaactcagtatatggtctgatgggatttagaaatagtgctctatactcatacgcttcggctaagagttgcacatccataggacgtagaatgatcttgtatctagaatcggtactaaatggagcagagttatctaacggtatgttacggtttgccaatccattaagtaatccattttatatggacgatagagatattaatccgattgtgaaaacatcgttgcctatagattacagatttcgttttcgtagcgtgtatggagataccgactccgtgtttacagagatagacagtcaagatgtcgataagtctatagaaatagcgaaagagttagaacgactgattaataatagagtattgtttaataattttaaaatagagtttgaggcggtatataagaatctgattatgcaatcgaagaagaaatatacaacgatgaaatactcagcatcgtcgaattcaaaatctgtacctgagagaattaataaaggtactagtgaaactagaagagatgtttccaagtttcataagaatatgattaagacatacaagaccagactgtctgagatgttgtctgaaggacggatgaattctaatcaggtatgtatagatattctccgttctttagaaacagatttacgatccgaatttgatagtagatcgtctcctctagaattatttatgttgagtcgaatgcatcactcaaattataaatccgcagataaccctaatatgtatttggttactgaatataataaaaataatccagaaactatagaacttggagaacgatattattttgcatatatttgtccggctaatgtaccatggaccaaaaaacttgtaaatattaaaacatatgaaacaattatcgatagaagttttaaactcggcagtgatcaaagaatattttacgaagtttactttaaacgattgacgtccgaaatagtcaatctattggataataaagttttatgcatctcattctttgaaagaatgtttggttcaaaacctacattttacgaagcataaaataatttacaacagttgtacgtcgctctttgttagattcagtttatccattagatattctacggctggagtaatttttgtagtaattgaatacccaggtacgtaaaacaataaaaacattaataccggatcatacttggtaaagtacaatatagtactaatattagctaatgtctcataatcggatggacttcttgctctactaagattagggtgatctatatctttgatacttattggaacgggaccggtaaatatataattctctttgagacgactaaacaaaggcttatagtctcctgtttgatgcatatacctagccaacgccaggtgtttggcattatctgtatagacgtatctgaataatgtgtgtttagtaatatcaaactgagtatttttaaaccagaacaagatattatagattggaatggaagtcagtaacaaaaaactaataaactcgtttgttggaagggcagaaaactttcgaagatatgatacgtatctaccagagaacgatccattagcaatgaattcagtatttactttttcttcatatacgggaataggacctttatatagagacatgagaaactcgaactttttaagtaatcccaacgaaatgggataatagtcacttgcatctaagtttgcgtatctactactccaaattgcagtttctggtatccatccatacgcgtaattatcaaatagatatgtgtttttcattaacggtctacttagacctctactaaaaaatgtttcttgatctagaattcttctttgtgcatttttgtacacgtcgtcaaaacgcggaacggtggcagccataatatttatatcctaccgctttttatcaactatgttatgtcttttagttaggttaatattctaataagatgcaggtaatacatcaggttaaagtattagaatgggattatacttatatatttagtttatctttcatcagataactaaaaaatgtataaaacagacgcgttacattgcctatgctacatgagttccatgtgcggagattgttaaagtttagggtagagagttgttctagcatccattcattgtctttacatccgttatatgtaattatgtcacccatggacattataggttttaatagtacttcagatactggaataagatattgttcgtatatgtgtttgataatcatttgttgcgtttctggagaacttttctctgcatgatttttacatagctttacaaactcgtgatcactttttataatgagagatctatagtcttcgtatctgttacgaaaatcaatatattcaggattattttctgaatcacttgattcgtcactaatatacataactatatgatcaacaattttttccaaaatcatttctgcattttctttattcattaatttggtgggagtctgaattgttgcagcagttcccatttatcaaaaatgtgtgataattatatctatgtatatacaaattattaataatatatttggtctgttctatgatctaccgtgtcttatcaattgaagtatatatttcttatccgtcttggttagatggatgcttttatccaagaattcttctacatgatatagattatctctcaaaaacctttgaaataagacgatgatggaaatattataactagctaaaatagttttgattagcgatggaagaatactagggtttttatctgtagaaaatcgaacgaatgcggatacatcctccacagacttaagatggtttatcattttaactaacaagtctcctttataatcatctaacacaagacctagacgagccaattgtccgtctaaataatattttaaaatgtttttgctaaacaagttcagccgtctactcttggattttatagatgacagtttctttagtattccgttctctatgaccatgggatccgactcgtgcaaaaacaggtatgtattgtattccttaacataatacgacgtatcctcgttaaagatttgacacttcttcatatcatccattgtatctaatgtgatatcgttcacctcataaattatattagatatataactgttattaatatctaactcatcaaatcgtttaatgtccgcagcactcgtagagaataaagacataattcgttcattatcgaaatattcgggatctatttgaacaacaactctgaataagtcctcgttaaacgttctatcactaataaatgtattaccgttaataaaattagctttataaaaactaataaaatattttttccaatcgtcgttttttgcatcaataatagataggatatctccaggaatatcatatatgatttctagcagaagttctctgatatctttttcaggctcaaagatataaactaacttaagcatgtttttattaacgcgtccttgttttatctcagagtatatataactaagaattttatcatacatggtaatggcgtgtctattaagaacaatatccgcatcattagctatactttcgtttaaccacacccaatagctagtcttatctccgggaaagatataatctctaaacgtttctgttagattgctatggactattctaccagtttgttgaaatagagtgtatatatcttgtctatcattatccgcaaactctatgcctgtatctttcttgcttaggtaagcccaaataagtaatcttataacacttaattttttaacaactttgaagtctgttttcttaaacagttttaaaaaaatgatttccatatctttgatgggttcccctccgtgaaataatggattaagaactaagtcataatttacgcctataagttctcctaattcgtccatgtattcggcaacctctaaaaatttttcatcttgtgttagtttatgcacggtttccttgtacgattgtattgcgttactaaacgataaataattcttagtcaatgctttaacgtacaacgtgggtgcatcaaatgcgtgtcgtaaaaccgcttcgtacactttacaacatcgtaccatatgtatgaaaacaaaaaaattggtattagctaatacatccttagtaataacgtgttgaggaaaattgctaactagatacttgagagctagtacatgattgagggtaaaattgtttactttacttaatgtatcatcctttaaaaaatctatattattttctactgtgtatataagatactttctacgaataaaatccatttttatagaagagagttatctatgatactacactcttattctaataattatttttactattttatcactaataactatttatactatccattattaatttaacaatttgaattagtattggagaaagatgaaatgcctattcactaacaaagtcaatgcactcttgaagatttttaccaataatatgtagcggattctcaaagtatttatttaccatttctttacacagtatcttagccactggcctacgaacaggcatacatggttcaactatatcatgaacaatgtttaattttagtgtatccaatccaataaatccattttctacatcatcatcgtatctgtacgctttgtattctccactcttgaacaaatctctaaacagtatcttcaacactttttccaccaattcctgggatgtcacacattgttctaccatctgtttgataaagagggtatcttcttcagattttcccttgattctatacatgggttttaggttataccttgcatctattgtatatttatcagattcagctatcaacattttatcaacttgtgttccaattattctccatttattagatctgcattcattattatagaatctttcttccactaatattctaataagattaagtttgaaaggagagaagatcttgtgtttgattttactcattggatgcattctataacgaatgaatctatgatcatctccaaacaaattgggaaacatgtaaagcagcagagcatataccatcttactcggattctgtgatgctttgccgatggctgaaatgtccgagaatagtttataagttttctgattatttggaatagatggtgctatatcttctagagtagtagtcctaatcattctcttaaattttatgtatcctagtttcaatgtctcgtaatgagtttgtgctgctcttattgtctgatttatttcttttaccattttggctctattctgaaactttatcctcttcttatccatttttattgttgactccgcactatcgatttgatactttcttttcagagtaaagctatcgtcattgatcatcggacactgacttccactcattatgaaattgtagccgtataaccacaatacaattattaacatatatattcacttttgttaatatcaacataataatgaaaaaatataaatgaacaaagttaatacataagtgttataaatggaaaatgtatacattagtagttactcatccaatgaacaaacatcaatggcggtagccgctactgatatccgagaattactatcacaatatgtggatgatgccaacttggaagacttaatagaatgggccatggaaaaatcatcaaagtactacatcaagaatataggtaatacaaaatctaatatcgaagaaactaaattcgaatcaaagaataatattggtatagaatactcaaaggattccagaaacaaactatcgtatagaaataaaccgtctattgccacaaatttggaatataaaacactatgtgatatgattaagggtactagcggcaccgaaaaagaattccttcgctatctcttattcggtataaaatgcattaagaaaggagtagaatacaatatagataaaataaaggatgtgagttacaacgattattttaacgttctcgacgagaaatacaatacaccgtgtcctaactgtaaaagtaggaatactacgccgatgatgattcaaactagagccgctgacgaacctccactagttagacatgcgtgtagagattgcaaacaacactttaagcctcccaaatttagagcatttcgcaatcttaatgttacaacgcaatcgatacatgaaaacaaggaaataacagagattcttccagataataatccatctcctccagaatctccagaaccagcatcacctatagatgacgggttaatcagatccacattcgatagaaacgacgaaccaccagaggatgatgaataaaaaaatgataaaataaattagttttattgctggttgtgttagttctctctaaaaatgtctaagatctatattgacgagcgttctgacgcagagattgtgtgtgcggctattaaaaacattggaatcgaaggagctactgctgcacaactaactagacaacttaatatggagaagcgagaagttaataaagctctgtacgatcttcaacgtagtgctatggtgtacagctccgacgatattcctcctcgttggtttatgacaacggaggcggataagccggatgctgatgttatggctgacgccataatagatgatgtatcccgcgaaaaatcaatgagagaggatcataagtcttttgatgatgttattccggctaaaaaaattattgattggaaagatgctaaccctgtcaccattattaatgagtactgccaaataactaagagagattggtcttttcgtattgaatcagtggggcctagtaactctcctacattttatgcctgtgtagatatcgacggaagagtattcgataaggcagatggaaaatctaaacgagatgctaaaaataatgcagctaaattggcagtagataaacttcttggttacgtcatcattagattctgattctagttatcaataacagttagtagtttagttatacattgaatcatacatattaatttttttattgagatagattaaaaaatacaaattgtagtactattaacgcgactagtatattctctaaagatgatatctgtcacagatattcgtagagcgtttctagacaatgaatgccatactatcacaaaagcgtttggatatctgcacgaggacaaggctatcgcattaattaaaataggatttcatcccacttatctacccaaagtcctttataataatgttgtagaattcgttccagaaaaactatatctgtttaagccaagaactgtagctccattggatttgatatctactataacaaaattaaagaacgtggacaaatttgcctcacacataaattatcacaagaatagtatattgataacaggagacaagtctctaattgttaaatgtatgccttacatgattatttcagatgatgatatacgattcataagagaacagtttgttggtacaaattctattgagtatattctatccttcatcaacaaggaaagcatatatagaatgagttaccaattttcagagaatgaaatagtcactatcatcaatagagatcatttcatgtatgaaccaatatatgaacatcaggtcttagattctgactttcttaaaactatgttagatagatacggaatagttcccattaattctggtataatagatgaattatgtccagaagctataatagagatattaatggcagtagttcgtcctagggacgctatccgtttcttagatatagtgaataagaatcaattgacagaagatagtgtcaaaaactatatcattaatgatatcagaagaggtaaaatagattattatattccatacgttgaagattttttagaagatagaactgaagacttgggaatatatgcgaatatattttttgaggatgctatagatattacgaaactagacatcacaaagacagagttggaacatatatcgaaatacatgaattattacactacttatatagatcacatagttaacatcatcttacaaaataattatatagatatcttggcatctataatagattacgtgcaagacgtattaacagaagaattatgtattagaatagtttgcgaatcaacaaaccctgttcccgttacatctcttcctatacattctacgttagtaatggttatgtgtatacaaatgaaatatgtcgatatagttgaattcttagacgagatcgacatcgatactttaatagaaaaaggagcagatccgataaccgaatacacatttacaacaagatggtacaataaacacaatgatttgatcactctttacattaagaaatatggattctgtccaatgatgatgaaacggttaatgttcgaatatccattgactaaagaagccagtgatcatttacttaaaaccatggatgaaaacaggggagctattatgttttttccgcgtactatttgcacacttccttatctattatgttgtaattataaactaattcaaaaacctattccattcaaagaagaaaatcgtaacatcgtatataagaaaaccaacagagtattatgctttgactcgttggagaactctgcgtttaaaagcctcattaaaatagattctattccaggattaaaaacttataacatgaaagacattacatacgaaaagtctaataatataatttgtgttaggtttatacctcaagaatcaattcataatgaagagcgaagaataaaattacagttattcgacattgctagattggcatcctatggactatattatattccctctagatatttatcatcgtggacaccagtagtgaacatgatagagggaagagagtacactaatccacaaaaaatagaatgtctagttattttggatttattttcagaggaattcatagaatatcaaaatctgggcaatgcggtatctaataaatatgaactggaatatactatatctaattatcaagctgccataaactgcctaatgagcacgttattaatatatctagttctaggatcaatcagatcgatatcaaaaactgaagattttgtattatctatattaaatatcttctataaaggactgaaaattaatgaattactttctgaaccagtatcaggagtttgtatcgaattaaataaaataaaagatagagcgagctctggagacagtagttttatatttcttaagaaaaacgagttatcaaaaactctatcgctctgtgaaaaagtttgtgttgagaccatattagacaataatcagagttttaaatcctcaaaatgaataggaatcctgatcagaatacttttcctaatattacattaaagattatagaaacctatttaggcagagtacctagtgtgaacgaatatcatatgttaaaattacaagctagaaatattcagaaaataactgtttttaacaaagacatatttgtatctttagtaaaaaagaataaaaaaagatttttttccgatgttgatacatctgcatcagaaataaaagatcgtatacttagctacttttctaaacagactcaaacatataatataggtaaattatttacgattatagaactacaatctgtattagtgaccacatacacggacatattaggagttcttactattaaagctccaaatgtaatttcatctaaaatttcttataatgtaacatcaatggaagaattggcaagagatatgctaaattctatgaacgtcgcagtaatagacaaggcaaaagtaatgggacgtcataatgtatcttccctagtcaaaaatgttaataagttgatggaagaatatcttagacgccataataaaagttgtatatgttacggatcatattctctatatctaattaatccaaatatacggtacggcgatatagatattcttcaaactaattcgaggacttttcttatagatttggcatttctaataaaatttattacgggaaataatattatattaagtaaaatcccatatcttagaaactatatggtgataaaagatgaaaacgataatcatatcattgatagttttaatattcgccaggataccatgaacgtagttcctaaaatctttatagataatatctatatagtggatccgacgtttcaactattgaacatgataaaaatgttttctcaaatagatagattggaagatctatccaaagatcctgaaaagtttaatgcgcgtatggcaaccatgctagaatacgttagatatacacatggtatagtctttgatggtaagcgtaataatatgccgatgaaatgtatcatcgatgaaaataatcgcatagttactgttactactaaagactattttagctttaaaaaatgtctagtgtatctagatgaaaatgtgttatcgagtgatatattagatcttaacgccgacacatcgtgtgatttcgagagtgttacaaattctgtatatctaattcatgataatatcatgtatacatatttctcaaatactattctccttagtgataaggggaaggtacatgaaataagtgccagaggtttatgtgcacatatattgttgtatcagatgctgacatctggagaatacaaacaatgtttatcggatctcttaaattcgatgatgaatagagataaaatacctatctattcacatactgaaagagataaaaaacctggacgacacggatttattaatatcgaaaaggatataattgtattttaggacaaaagtctagaagctacattatcgcgattagccgcgaacatattttgtagcatgtccgtcctcataaacggaacttgttttcctgggttattcattctctcgcatctggaaggggacgaaggtcttctctcacacgcgggtgatgagggtttatctactttgagtacgcaggaagctttacttccttcgcattctacagttctaacatcgcatactttaacggcttttagaaccagatatcttccttctttggtattgatataaaacggagtatgagcagatgcaaaatgagaattcatttatagcatagaaaaaaaacaaaatgaaattctactatatttttacatatatatattctaaatatgaaagtggtgattgtgactagcgtagcatcgcttctagacgcatctattcagtttcaaaaaacggcatgtaggcatcactgtaattacctatctatgcaagtagttaaagagatagaagaatttggtactatcaatgaaaaaaatttggaatttgacacttggaaagacgttatacaaaacgatgaaatagatgcattagtattttatagagtaaaacaaattagtatttctacgggtgttctatataaatctatgatgcgcaatagaacaaaacctatttccatgtactttgtacgtgattgtctggcatttgatggagatcctccgtcttttagaatgacgtcttgcaatatcaacgcatacaatcgtagtaagattaaagatttaataatcctaatgaatatgaaaacatgtaataaaaaaattatcggtgagtttataatagacaattttggaagcgtcgatgcattactatcgatagttaattccaatgttacgtggattacatcagttataaataatagtaacggcaggggtattaatatcagggtatcaaataataaaatgttaactataactagttttcgacgattcgtcaataaacttaaaatgtacaaaactactaaatgcgcttctcaattggataatctatgtaccgagatgaacaaaatggatattatagacaaaaaatgaaacgtaatgaggagtattgcggggctacataaattaaaaatggaaatttttaatgtagaagaattgataaatatgaaaccttttaagaatatgaataaaataacaattaatcaaaatgataattgtatattagcaaatcgatgctttgttaaaatagatactcctagatacataccatcgacatccattagcagttctaatatcatcagaatacggaatcatgattttacattatctgaattattgtattcaccgtttcattttcaacagcctcagtttcaatatctccttcctgggtttgtattaacgtgtattgataaagtttcgaaacagcaaaaaaaatgtaaatattgtatctctaatcgtggagatgatgatagtttaagcattaatctatttattccgactattaacaagtctatatatattattatcggtttacggatgaaaaatttttggaagcctaaattcgaaatagaataatgtttttatattatacatgttctaaaagaataatcgatacagtttaagtgaaagctagagaggggtttttaaatggtcatcggtttagtcatattcgtgtctgtggcggccgccatcgtcggtgtgttgtctaacgtattggacatgtttatgtacgtagaagaaaataatgaagaggatgctagaatcaaggaggagcaagaactactgttgctatattgatacataattgaaaatctaccaacttaaatacaccgcctataaatttacaatgaaacacagattgtattctgaaggattgagtattagtaatgatttaaactcgataatcggtcaacaatctacaatggatacggatatagaaatagacgaagatgacatcatggaacttcttaatatattgactgagttaggttgtgatgtcgactttgatgaaaattttagcgatatagccgatgatattctagaatcgttgatagaacaggatgtataagtttttatgttaactaaatgtggccatttgcaccggtacctgcgggagcaaaatgtaggctggtagaaacactaccagaaaatatggattttagatccgatcatttaacaacatttgaatgttttaacgaaattatcactctagctaagaaatatatatacatagcatctttttgttgtaatcctctgagtacgactaggggagcgcttatttttgataaactaaaagaggcatctgaaaaagggattaaaataatagttttgctagatgaacgagggaaaagaaatctgggagagctacaaagtcactgcccggatataaattttataaccgttaatatagataaaaaaaataatgtgggactactactcggttgtttttgggtgtcagataatgaaagatgttatgtaggaaacgcgtcatttactggaggatctatacatacgattaaaacgttaggtgtatattctgattatcccccgctggccacagatcttcgtagaagatttgatacttttaaagcctttaatagcgcaaaaaattcatggttgaatttatgctctgcggcttgttgtctgccagttagcactgcgtatcatattaagaatcctataggtggagtgttctttactgattctccggaacacctattgggatattctagagatctagacactgatgtagttattgataaactcaagtcggctaagactagtatagatattgaacatttggccatagttcccactacacgtgtcgacggtaatagctactattggcccgacatttacaactccattatagaagcagccattaatagaggagttaagatcagacttctagttggtaattgggataagaacgacgtatattctatggcaaccgccagaagtctagacgcgttgtgtgttcaaaatgatctatctgtgaaggttttcactattcagaataatacaaaattgttgatagtcgacgacgaatatgttcatatcacttcggcaaatttcgacggaacccattaccaaaatcacggattcgtcagttttaatagtatagataaacagcttgtaagcgaggctaaaaaaatatttgagagagattgggtatctagccacagtaaatcgttaaaaatttaaaaaatagaaacgtatagaacgccatcatgttaaacaggatacaaaccttgatgaaaacagctaacaattatgaaactattgagatattgcgtaactatttaagactgtatatcattttggcacgaaatgaagaaggtcatggtatactaatatacgatgataacatagatagtgttatgtcgatgatgaatattacaatattagaagttataggattgacgactcattgcacaaaattaagatcatcgcctccaattcctatgtctagattgtttatggacgaaatagatcatgagtcatattattctccaaaaacttcagattatccgttgatcgatattatacgaaagcgttctcacgaacagggagatatagcactggctttagaacgatacggtattgagaatacagattccatatcagaaattaatgaatggttgtcgtcaaaaggtttagcatgttatagatttgtaaaatttaacgattataggaaacagatgtatcgtaagttctctaggtgtactatagttgacagtatgataatagggcatataggtcatcattatatttggattaaaaatttagaaacatatacgcgtcccgaaattgatgtgttaccgtttgatattaaatacatatctagagatgaattgtgggcgcgaatttcttcctcgttagatcaaacacatataaaaaccatcgccgtatcagtttatggagctattactgataatggaccaataccatatatgatatccacgtatccgggtaatacctttgttaactttaacagtgtaaaaaatctaattttaaatttcttagattggattaaagatattatgactagtacacgaactatcattctagtaggttacatga

SEQ ID NO: 45 - DNA, 31690 bp, Artificial Sequence
  Vector
tggctggaatcattaacaagaaaataaaaaacaatttcaaagttaaacataactggtattacgatttccatttctttgttcatactttattaaaaacatatccagaaatcgaaaaagatatcgaatttagtacggcattggaagaattcatcatgtgtaccaaaacagactgtgataaatatagattaaaggtttccattcttcacccaattagtttcttggaaaaatttattatgagagacattttctcagactggataaatggcggaaactaaagagtttaaaactttgtataatctttttatagatagttatttacaaaaattagctcaacattctatccctactaatgtcacttgtgctattcatataggagaggttataggacagtttaaaaattgcgcgctccgaataactaacaaatgcatgagtaattctcgacttagtttcacactcatggttgaatcatttattgaagtgatttcattgcttccggaaaaggatagaagagctatcgctgaggaaataggaatagatctagacgatgtacctagtgcggtatccaagctagaaaagaactgtaatgcgtatgcggaggttaataatattatagatatacagaaattggatatcggagaatgttcggctccgcccggtcaacatatgcttttacagatagttaatacaggatccgcggaagcaaattgtggtttacagacaattgttaagtccttaaataaaatatacgttccacctattatcgaaaaccgattgccgtattacgatccgtggtttctagtgggtgtagcaattattctagttatttttactgtagctatttgttctattagacgaaatctggctcttaaatacagatacggaacgtttttatacgtttaattaataaaaaaatttaattacaaggtataaaatagtactccatctacgcaatcgcgataatggagggatctaaacgcagacacgacagtcggcgactacaacaagaacaggagcagcctcgtccacgtacaccgccatcatatgaagaaattgcaaaatatggacactcatttaacgtgaaaagatttacgaatgaagaaatgtgtcttaagaatgattatccacgaattatatcatataatcctccaccaaaatagagtatatatatatcatcatttcatgatgtatactactgacatagtttcaatgtgaacttttcactttcttgccggttatgaagaatatttttattttaatggtcattactaatcgtatattataattgaaaatggattagtttaatatgacgctcgtcatgggatcctgctgtggtagattctgtgacgctaagaataagaataagaaggaagatgtagaagagggaagagaaggatgttacaattataagaaccttaatgatctggatgaatccgaagcacgtgtagaatttggaccattatatatgataaatgaagaaaaatcagacataaatacattggatataaaaagaagatatagacacacgatagagtctgtatatttctaaaagtttttataaaaaatgagtaaaatactcacgtttgttaaaaataagataattgacttgattaataatgaccaaattaaatattctagagttataatgatagaagagtccgatagtcttttaccggttgatgaggtgcatgctaaccacggatttgactgtgtggagatgatagatgaaaatataagcaatgagaatatcgaacagtataaaaccgaatctttttttacaataaattgaaatcaaaacatttattaaaccgcatcaagatgggtacgaacggcgttagagtatttgtcattttatatttgttggctgtatgcggatgtatcgaatacgacgtagacgataatgtacatatttgtacccacactaacgtgtcacatattaatcacactagttggtattataatgataaggttatagcgctagccaccgaggataaaacttctggttatatatcatcattcataaaacgcgttaatatctcattaacttgtttaaatatatcgagtttgaggtacgaagattctggtacatacaaaggagtatcgcatctaaaagatggagtcatcgttacgactactatgaatatatctgtaaaggctaatatcattgacttgactggtagagtgcgttatctaaccagaaattattgcgaagttaaaatacgatgcgaaataacatctttcgcgcttaatggttctactacaccaccacatatgatattaggaacagtagataaatggaaatatcttccatttcctacagatgattatagatacgtaggggaactgaaaagatatatatctggaaacccatatccaacagagtcgctagcgttagaaattagctcgacgtttaatcggtttactatcgttaaaaatttgaacgatgacgagttttcttgttatctgtttccataaaatgttgaacgcgcgccatatttgtgaatccgaatgggaggctttaaataataataacgataattcatcctccatgcccgcttcccacaacaatctcgcaaacgatttatctagtatgatgtcacaattacaaaatgataataacgataatttaattatgatagtactaataacaatgctatcaataatacttgtaattattgtagtgattgcggcgatatcgatgtacaaaagatccaagtacaggcatatagataactgaaaaaaaatttattgttattgttaatttagttatggaacccatccttgcaccaaatccaaatagatttgttattttcccaatccaatatcatgacatctggaacatgtataaaaaggcagaggcatcattttggacagtggaagaagtagatatatctaaagatatcaatgattggaataaactaacaccagacgaaaaatattttataaaacatgtattggcgttttttgcagccagtgacggaatagtgaatgaaaatttggcggaacgattttgtacagaagtacagattaccgaggctagatgtttctacggatttcagatggccattgaaaacattcattcggaaatgtatagtcttttgatcgatacttatgttaaagatagtaatgaaaaaaactatctctttaatgccatagaaacgatgccttgtgtaaaaaagaaggccgattgggctcaaaagtggatacatgacagcgccggttatggagagagacttattgcctttgctgcagtagaaggaatcttcttttccggatcattcgcttccatattttggcttaaaaagcgtggcctaatgcccggactcacgttttccaacgaattgattagtagagacgagggtctacactgcgacttcgcatgtttgatgtttaaacatttattgcatccaccgagtgaagaaaccgttagatctattataacagatgcggtatccattgaacaagaatttcttactgcggctcttccagttaaacttataggaatgaattgtgaaatgatgaaaacatatatagaattcgtcgcggatagattgatttctgaattgggatttaaaaaaatttataatgttaccaatccgtttgatttcatggaaaatatatcattagaaggtaaaactaattttttcgaaaaacgtgtgggtgaataccaaaaaatgggagttatgtctcaagaagataatcatttttctttagatgttgacttttaaagaaacataaatgccgatatttgtcaatactgtgtactgtaagaatatattagcattgtctatgactaagaaattcaaaacaattattgatgccataggaggcaatataatagtcaattctacgatattgaaaaagttatctccttactttcgcacacatttacgtcaaaaatacacgaaaaataaagatccagttacgagggtttgtctagaccttgacattcacagtctaacttctatagttatttactcatatactggaaaggtatatatagatagtcataacgtcgtcaatttattacgtgcttctatattaacctctgtagaatttatcatctacacttgtataaactttatcctacgagattttagaaaggaatattgtgtcgagtgttacatgatgggtatagaatacggactatccaatctcttatgtcatactaaaaactttattgccaaacactttttggaactggaagatgacatcatagacaattttgattatctatctatgaaacttattctagaaagcgatgaactaaatgttccagatgaggattttgtcattaagtggtatataaagcgaagaaataaattaggaaatctgctactccttatcaaaaatgtaatcaggtcaaattatctttctcccagaggtataaataatgtaaaatggatactagactgtaccaaaatatttcattgtgataaacaaccacgcaaatcatacaagtatccattcatagagtatcctatgaacatggatcaaattatagatatattccatatgtgtacaagtactcatgttggagaagtagtatatctcatcggtggatggatgaacaatgaaatacataacaatgctatagctgtaaattatatatcaaacaattggattccaattcctccgatgaatagccccagactgtatgctagcgggatacccgctaacaataaattatacgtagtaggaggtctaccaaatcccacatctgttgagcgttggttccacggggatgctgcttgggttaatatgccgagtcttctgaaacctagatgtaatccagcagtggcatccataaacaatgttatatacgtaatgggaggacattctgaaactgatacaactacagaatatttgctacccaatcatgatcagtggcagtttggaccatccacttattatcctcattataaatcatgcgcgttagtgttcggtagaaggttattcttggttggtagaaatgcggaattttattgtgaatccagcaatacatggactctgatagatgatcctatttatccgagggataatccagaattgatcatagtggataataaactgctattgataggaggattttatcgtgaatcgtatatagatactatagaagtgtacaatcatcacacttattcatggaatatatgggatggtaaataattttgaaataaaatattagttttatgttcaacatgaatattaactcaccagttagatttgttaaggaaactaacagagctaaatctcctactaggcaatcgccgggtgctgccggatatgatttgtatagcgcttacgattatactatccctccaggagaaagacagttaattaagacagatattagtatgtccatgcctaagatttgctatggtagaatagctcctaggtctggtctgtcactaaaaggcattgatataggaggtggtgtaatagacgaagattataggggaaacataggagtcattcttattaataatggaaaatgtacgtttaatgtaaatactggagatagaatagctcagctaatctatcaacgtatatattatccagaactggaagaagtacaatctctagatagtacaaatagaggagatcaagggtttggatcaacaggacttagataataaacaatagtatgttgtcgatgtttatgtgtaataatatcgtagattatgtagatggtatagtacaggatatagaagatgaggctagcaataatgttgatcacgactatgtatatccacttccagaaaatatggtatatagatttgacaagtccactaacatactcgattatctatcaacggaacgggaccatgtaatgatggctgttcgatactatatgagtaaacaacgtttagacgacttgtatagacagttgcccacaaagactagatcatatatagatattatcaacatatattgtgataaagttagtaatgattataatagggacatgaatatcatgtatgatatggcatctacaaaatcatttacagtttatgacataaataacgaagttaatactatactaatggataacaaggggttgggtgtaagattggcgacaatttcattcataaccgaattgggtagacgatgtatgaatccagtaaaaactataaaaatgtttactctactatcgcatactatatgcgatgattgttttgtagattatataacggacatttcaccaccagataataccatccctaacactagcacgcgtgaatatctaaagcttattggcatcacagctatcatgtttgctacatataaaactctcaaatacatgataggataattttttttaacacggatatagaatgctaacgtaataattatgcgttatgaagacccctatatcatcaattcaattttttttctagaaaaagtatcaagatgtttatattatcgtcggtcatcagatctgtaatgtttcccaatgattggaatctagattctgaaatctttttgtatccccaatgttcagtgattttagcacatattcctatggtagcgaataaactttcctgatcatggacttttgtaaaattgatgtagtggtctccttcgctcatagcttcgacaatctcattaattttatcaataccatagtaccgtatagcgacatcatcgaacttcatcaattccttgtacagtcttccacaactggtaatatctttgttaaacactataacatgatttctccacgtaatatattcatctattagatcgatgatggagtcgcgactacatattttatcatcatccacaaagtaaaaaacagcatcctcataatctaatttagtcgccatgactatctcacaaaagacagtagccgtctccttcctctatattgatttaattgtatgtttttacaattatcaataaaacataaaaataatatgatcatcaaacgaactgttaatattgatagttatataacgtgaatcatgagtgcaaactgtatgttcaatctggacaatgattacatatcctaaggcattagtattcataagtcatggagctggtaaacattctggacgttatgacgaactagctgaaaacatatcatcgttaggaattttagtattctcacatgatcatattggacatggaagaagtaatggtgaaaaaatgatgattgatgactttggtacagcacgtggtaactattaaatctacttattgggtcattccatgggagcaacaatttctatactagcctcttacgataatccaaacttgtttacagcaatgattctaatgtctcctctagttaatgcagatgctgtttcaagactgaatctgctagctgccaaacttatgggaaccatcacaccaaatgcgccagtcggaaagctatgtccagaatcagtatctagagatatggataaagtttataaataccaatacgacccattaatcaatcatgaaaaaattaaggctggatttgctagtcaggtcttgaaggctaccaacaaggttagaaaaataatttccaagattaacaccccgactctcatactccagggaacaaacaatgagattagcgatgttttaggtgcatattatttcatgcaacatgcaaattgtaatagagaaataaaaatttatgaaggtgccaaacatcatcttcataaggaaacggatgaagttaaaaaatcagtcatgaaagaaatagaaacttggatttttaatagagtgaagtgatataggattattcttttaacaaataaaatgaatccggataatacaatcgcagtgattacagagactattcctataggtatgcaatttgataaagtatatttgtctacatttaacatgtggagggaaattctatccaataccacaaaaacactagatatatcatctttttattggagtttatcggatgaagtgggtacgaatttcggcacgataatattaaacgagattgtacaattacccaaaagaggagtacgagttagagtagccgtcaataaatctaacaaaccattaaaggatgttgaaagactacaaatggccggagttgaagtacgatacatagatattacaaatatcctaggaggagttcttcatacaaaattttggatatctgataatacacatatttatttaggaagcgctaacatggattggagatcactaactcaggtcaaagaattgggtattgcgatcttcaataataggaacttggcagcggatctcactcaaatttttgaggtatactggtatcttggagttaacaatctaccatataattggaaaaacttttatccgtcgtattataatacagatcatcctcttagtattaacgtaagtggtgttccacactctgtatttattgcttctgcaccgcaacaactatgtactatggaaagaaccaatgatttaaccgctttattgtcatgtattagaaatgcgagtaaattcgtttatgtatctgttatgaactttatccctattatttattcgaaggcgggtaaaattttgttttggccttatatagaagatgaattaagaagatccgctatagacagacaagtatccgttaagctattgattagttgctggcaacgatcttcgtttatcatgagaaactttttaagatctatcgctatgctaaaatctaaaaacataaatatagaagtaaagctatttattgtaccagatgctgatcctcccattccgtattctagggtaaaccatgccaaatatatggtaaccgataaaacggcctatataggtacctcaaattggacaggaaattactttacggatacatgtggagcatctattaatattacaccggatgatggattaggtcttcgtcaacaattagaagatatttttatgcgtgattggaattcaaaatacagctatgaattgtacgatactagtcctactaaaaggtgtaaactattaaaaaatatgaaacaatgtacaaatgatatatactgcgatgagatacaaccggaaaaagaaattcctgaatattctcttgaataaaatagatataaaaacataatttttatcccaatttacgagcccgttaacaagatgcttgcattttgttattcgttgcccaatgcgggcgatgtaataaagggcagagtatacgagaatgattatgctctatatatttatctttttgactatcctcactctgaagctatcttggcagagagtgttaagatgcatatggatagatatgttgaatatagggataaactggtagggaaaactgtaaaagttaaagtgattagagttgattatacaaaaggatatatagatgtcaattacaaaaggatgtgtagacatcaataatttttataccgaacataaaaataaggttaattattaataccataaaatcatgattgcgttattgatactatcgttaacgtgttcagcgtctacctatcgtctacaaggatttaccaatgccggtatagtagcgtataaaaatattcaagatgataatattgtcttctcaccgtttggttattcgttttctatgtttatgtcgctattgcctgcatcaggtaatactagaatagaattattgaagactatggatttgagaaaaagagatctgggtccagcatttacagaattaatatcaggattagctaagctgaaaacatctaaatatacgtacactgatctaacttatcaaagtttcgtagataatactgtgtgtattaaaccgtcgtattatcaacaatatcatagattcggcctatatagattaaactttagacgagatgcggttaataaaattaattctatagtagaacgtagatccggtatgtctaatgtagtagattctaatatgctcgacaataatactctatgggcaatcattaatactatatattttaaaggtatatggcaatatccgtttgatatcactaaaacacgcaatgctagttttactaataagtacggtacgaaaacggttcccatgatgaacgtagttactaaattgcaaggaaatacaatcacaatcgatgacaaagaatatgacatggtacgccttccgtataaggatgctaatattagtatgtacctggcaataggtgataatatgacccatttcacagattctattacggctgcaaaattagactattggtcgtttcaattagggaataaagtgtacaatcttaaactccctaaattttctatcgaaaataagagggatattaagtcgatagccgaaatgatggctcctagtatgtttaatccagataatgcgtcgtttaaacatatgactagggacccattatatatttataaaatgtttcagaatgcaaagatagatgtcgacgaacaaggaactgtagcagaggcatctactattatggtagctacggcgagatcatctcctgaaaaactggaatttaatacaccatttgtgttcatcatcagacatgatattactggatttatattgtttatgggtaaggtagaatctccttaatatgggtacggtgtaaggaatcattattttatttatattgatgggtacgtgaaatctgaattttcttaataaatattatttttattaaatgtgtatatgttgttttgcgatagccatgtatctactaatcagatctattagagatattattaattctggtgcaatatgacaaaaattatacactaattagcgtctcgtttcagacatggatctgtcacgaattaatacttggaagtctaagcagctgaaaagctttctctctagcaaagatgcatttaaggcggatgtccatggacatagtgccttgtattatgcaatagctgataataacgtgcgtctagtatgtacgttgttgaacgctggagcattgaaaaatcttctagagaatgaatttccattacatcaggcagccacattggaagataccaaaatagtaaagattttgctattcagtggactggatgattcgtattcgatgattatttttaacaaaataacataaaaataatatatttttttaggatgcgatcatgacgtcctctgcaatggataacaatgaacctaaagtactagaaatggtatatgatgctacaattttacccgaaggtagtagcatggattgtataaacagacacatcaatatgtgtatacaacgcacctatagttctagtataattgccatattggatagattcctaatgatgaacaaggatgaactaaataatacacagtgtcatataattaaagaatttatgacatacgaacaaatggcgattgaccattatggagaatatgtaaacgctattctatatcaaattcgtaaaagacctaatcaacatcacaccattaatctgtttaaaaaaataaaaagaacccggtatgacacttttaaagtggatcccgtagaattcgtaaaaaaagttatcggatttgtatctatcttgaacaaatataaaccggtttatagttacgtcctgtacgagaacgtcctgtacgatgagttcaaatgtttcattgactacgtggaaactaagtatttctaaaattaatgatgcattaatttttgtattgattctcaatcctaaaaactaaaatatgaataagtattaaacatagcggtgtactaattgatttaacataaaaaatagttgttaactaatcatgaggactctacttattagatatattctttggagaaatgacaacgatcaaacctattataatgatgattttaaaaagcttatgttgttggatgaattggtagatgacggcgatgtatgtacattgattaagaacatgagaatgacgctgtccgacggtccattgctagatagattgaatcaaccagttaataatatagaagacgctaagcgaatgatcgctattagtgccaaagtggctagagacattggtgaacgttcagaaattagatatagagaaaatagctccagaatacagacaatgcttacaggatctataccatatgaaaattacgcgtcctagacactttgataactagttatgtcattctcgtttttatagagtgtactcgttactaaatattaattaatgaaataataacaattattaagacatactattcatccaacttaaacaacgaaaaacatttttcattaagtttatcatgaatgcgtataataaagccgattcgttttctttagagtctgattctatcaaagatgttatacacgattatatttgttggctcagtatgactgatgaaatgagaccatctatcggaaacgtctttaaagcgatggaaacgtttaagatagacgcggttagatattacgatggtaacatatacgatttagctaaagatataaatgcgatgtcattcgacagttttataagatctctacaaaatatctcttcaaagaaagataaactcactgtttatggaaccatgggactgctgtctattgtcgtagatattaacaaaggttgtgatatatccaatatcaagttcgctgccggaataatcattttaatggagtatatttttgatgacacggatatgtctcatcttaaagtagcactctatcgtagaatacagagacgtgatgatgtagatagatatttttttttcctaaactgatttctctgtttaaattcgtagcgatatataaaacaacatgtaattaattaataaactttaagacatgtgtgttatactaagatggttggcttattccatagtagcttgtggaatttataaacttatgatagtaaaactagtacccaatatgtaaagatgaaaaagtaaattactattaacgccgtcggtattcgttcatccattcagtatgggtatacagcacgaattcgacatcattattaatggagatatcgcgttgagaaatttacagttacataaaggggataactacggatgcaaactaaaaattatttcgaatgattacaagaaattaaagtttagattcattatacgcccagattggtcggaaatcgacgaggtcaaaggattaaccgtatttgcaaacaactatgcggtgaaagttaataaggtagatgacacgttctattacgtaatatatgaggctgtaatacatctgtataacaaaaaaacagagatattgatttattctgatgatgagaacgaactctttaaacactattacccatacatcagtctaaatatgattagtaaaaagtataaagttaaagaagaaaactactcatccccgtatatagaacatccgttaatcccgtatagagattatgagtccatggattaatatgagtatagtgttaaatgacacttactaaatagccaaggtgattattcgtatttttttaaggagtaaccatgtccgcaattagatttattgcatgtctatatctcatttccatcttcggaaattgtcatgaggatccatattatcaaccatttgataaattaaacattactctagatatatacacttatgaggatctagtaccatacaccgtagacaatgacacaacttctttcgttaagatatactttaaaaatttttggattacggttatgactaaatggtgtgctccgtttattgataccgttagcgtatacacatctcatgataatctgaatatacaattttatagtagggacgaatatgatacacaaagcgaggataaaatttgtaccattgatgttaaagcacgatgcaaacatctaacaaaacgagaagttacagtacaacaagaagcctacagatattcattatcttctgacctatcgtgttttgattctatagatctagagattgatcttattgaaactaatagtactgacactacagtactgaaatcatatgagctcatgcttcccaaacgtgctaaatccatacataactgaaatgaaagaaaccaaaaaatgcgatagcatcaacaaccaatcatggttaacgataagatactctatgatagttgtaaaacatttaacatcgatgccagcagtgcacaatcattgatagaaagtggtgcaaatccattatatgagtatgatggtgaaactccattaaaggcatacgttaccaagaaaaataataatatcaaaaacgatgttgtgattttgttattgtcgtcagtcgactataaaaatatcaatgattttgatatactcgaatatctatgttctgataacatcgatatagacttattgaaattactaatttcgaaaggtatagaaataaatagtatcaaaaatggtattaatattgtagaaaaatacgctacaacatcaaatcccaatgtagatgtgtttaaactattattggataaaggaatacctacatgtagcaacatacagtatggatacaagatcaaaatagaacagattagacgtgctggtgaatattataattgggatgatgaattagacaattacgattacgactacaccactgattatgatgatagaatgggtaaaacagttctctattattatattattactaggtcacaagatggttatgctacatctttggacgtaataaactatttaatttcacacgaaaaagagatgcgttattatacttatcgtgaacataccacactctattattatcttgacaaatgcgatattaaacgggaaatatttgacgcgttattcgatagtaactatagtggtcatgaactaatgaatattctatctaactatttacgtaaacagtttaggaagaaaaatcacaaaatcgataattatatagttgatcaactattattcgaccgtgatacgttttatattttagaattgtgtaatagtttacgtaataatatccacaattcttaaaagatatacagattctatacaagatctattgttagaatatgtatcttatcatacagtatacatcaatgttattaaatgtatgattgatgaaggagctacattatatagatttaagcatataaataaatattttcaaaaatttggcaatagagatcctaaagttgtcgagtatattttaaaaaatggaaacttagttgtagataatgacaatgatgataacctaataaatattatgccattattccctaccttctctatgcgtgagttggatgtgttatcgatactaaaactttgtaagccgtatattgatgatataaacatggatgtagtatactttatcattgtattaagtcgcatagtgtcagcctagtagaatggttaatagataatggcgcagacattaatataataacaaaatatgggtttacatgtattactatttgtgttatactggcagataaatatatcccagaaatagcagaattatatattaagatattggaaattattctgagtaaattaccaaccatcgaatgtattaagaaaacagttgattacctagacgatcacaggtacttattcataggtggtaataataaatcgttactgaaaatatgtatcaagtacttcatattagtcgattataagtacacatgtagcatgtatccatcatatatagaatttataaccgactgcgaaaaagaaattgcggatatgcgtcaaattaaaataaatggtacggacatgcttacagtgatgtacatgttaaataaacctacaaagaaacgatatgttaataatccgatatttacagattgggctaataagcaatataagttttataatcaaataatatataatgctaataagttaatagaacaaagtaagaaaatagacgacatgatagaggaggtatccattgacgataatcgtttatcaacactaccgttagaaattagacatttgattttctcgtacgcgttcctataaaaatagaaactataatcatataatagtgtaggttggtagtattgctcttgtgactagagactttagttaaggtactgtaaaaatagaaactataatcatataatagtgtaggttggtagtagggtactcgtgattaattttattgttaaacttgtccttaagtcttattaatatgtcttctaaagggggtagtggcggcatgtggagtgtctttatccatggacatgatggtagtaataaaggatctaaaacttatacatctggtggcggtggaatgtggggaggaggatcgtccagtggtgtaaaaagtggggttaacggaggtgtaaaatctggaactggtaaaatttaaacactaaattatttttattaataattgtacaagtttttgacatgatatttaatgacattagttgtgtgggtgtatagagttcacagtagctcattcagtcaaaatgtttgactatttggaaaatgaggaggtggctctcgatgaacttaaacagatgttgagagacagagatcctaatgataccaggaaccaattcaagaataatgctttacacgcatacctttttaatgagcattgtaataatgtcgaggtcgtcaaactactactagacagtggcactaatccattacgcaaaaattggagacagctaccccattagaagaatacacaaatagtagacatgttaaagttaaaggatatagcgatggctctactagaagccactggatttagcaacataaatgactttaatatattcagctatatgaaatccaaaaatgtagacgttgacttgataaaggtgttggtagaacatggatttgacttgagtgttaaatgtgaaaaccatcgttcagttatagaaaattatgtaatgacagatgatcctgttcctgaaattattgatttgttcatagaaaatggctgcagtgttctttatgaggacgagtactgatacgcgtatgatgattatcaactacgaaattgcggtaccgtattgcatctgtatatcatctctcatctgtattcagagtcggatacgagagcatatgtgcgtccggaagttgttaaatgtctaattaatcacggaatcaagccgtcttttatagataaaaactattgtacagctcttcaatattatattaagtcatctcatatagatatagacatcgttaaattgttaatgaaaggaatagataacacggcttattcatatatagacgatctaacatgttgcactcgagtaattatggctgattatctaaatagtgattatagatacaataaagatgtagatttggtcaaattgtttttggaaaatggaaagccgcacggaataatgtgtagtattgtaccactatggagaaatgataaggaaaccatctttttgatattgaaaacaatgaactcggatgtcctccaacatatactaattgagtatatgacattcggcgatatccctctagtggaatatggaactgtggtaaataaagaggctatacacggatactttagaaatattaatattgattcttacacgatgaaatatctactaaaaaaggaagggagatgccatcaattatctcgatgatggagagatcccgattggacacctatgtaaatccaactatgaatgttataatttttacacttatacatacaaaaagggtctttgtgacatgtcttatgcttgcccaattcttagtactataaacatttgcctaccttatcttaaagacattaacatgattgacaaacgaggagaaacacttcttcacaaggctgttagatataataaacaatctctagtatctttactgctagaatccggttcagatgtcaacattagatcaaataacggatatacatgtatagccattgccatcaacgaatctaaaaacattgaactgctgaaaatgctattatgtcataaacctacattagattgtgtgattgattcattgagagaaatatctaacatcgtagataacgactatgctataaaacaatgtattaaatatgccatgattatagatgactgtacatcgtctaagattccagagtccataagtcaacgctataatgattatatagatctttgcaattaagaattgaatgagatgaaaaaaataatggtaggtggtaatactatgttctcattaatatttactgatcatggagctaaaattattcatagatatgtcaataatccagaattacgtgagtattatgagttaaaacaaaataaaatatatgtggaagcatatgatattatttccaacgcaatagtgaaacatgatagaatacataaaaccatagaatcagttgatgataatacctacatttctaatcttccgtataccatcaaatacaaaatattcgagcaacaataagtattttttatacctttaaaattgataaataaattttttctagtgatattttggcaagatgaaaatcctatttctcatcgctttcatgtatgggtgtgttcactcatatgttaacgcggttgaaaccaaatgtccaaatctagacattgtaacatcttctggagaatttcattgttcaggatgtgtggaacatatgcctgagtttagctatatgtattggttggcaaaggataccaagtttatagaacatctgggtgatggcatcaaagaagatgaaaccgttcgtaccacagatagtggaatcaccactctacgtaaagtccttcatgtaaccgatactaataaatttgctcattataggttcacttgtgtcctcactacgatagatggcgtttcaaaaaagaatatttggctgaagtagtgcgtgctactatttttatttatgatataatctaatggaattaatttgaattgatatttatccaatactaaagattatattagaatcaaattaatcttttatacgagaaaaaataacgacatacgtcgtcaacaaattaaactttttatttattagttaacttgctcattgttatgtttctaaaacgggtacgacatataggacaattatccgacgcaccggtttctcttcgtgttctatgccatatattgatgcatgttatgcaaaatatatgattacacgaatccaataaaccaaagtatctatcgttttgagtaaacaacttcatagcaaatttcacattctttttctttacttactctatacacgtcctcgtatttatccagtattttgatgatatccaactcagaaatggttgttgtattattgggtgtataggtattattagctatgtaccaatttaccaaccttcttaatattgattgataatcacatcggttatccaattaataactaaattgtagtgtatatatagaccatatatgtttctatttttttgacagtttcagtaagttttgattgttgtattcctgtatctctagataagttagtcatatagtcccttccggcgatacgttttttccaagcccgaaattgattagccaaatgtggatttatttttgtgataatgcatactgttagtcttatatcatttggttcatctatgtattgtaatattgttacatgatctatagatgatgtattgattttggcaggatcgaattccatatccgcgactaaacagtgaaaaaaatgtaaataattttaaattagtaaaacttttttttattttttatgattccaaaaaaactgaatacaaagtcctaaattataaatatggagatcatactaccacaacttattattatgtatacaaggccggtgtaatagatagatatatataattctattacaccggcagacaattaccgatcggtatttgtcgttaccaacataccgtataatatgtaatatacaattccataacccattgacagttgttatacatcaaaattgcaattcttttgattacgatgttataagaatgtagttaattgatgtatgatgttaatgtgtcctctttcctcttataacatcgtaatcaaaaacttttttataatatatacctaataatgtgtcttaatagttctcgtgattcgtcaaacaatcattcttataaaatataataaagcaacgtaaaaacacataaaaataagcgtaactaataagacaatggatatttacgacgataaaggtctacagactattaaactgtttaataatgaatttgattgtataaggaatgacatcagagaattatttaaacatgtaactgattccgatagtatacaacttccgatggaagacaattctgatattatagaaaatatcagaaaaatactatatagacgattaaaaaatgtagaatgtgttgacatcgatagtacaataacttttatgaaatacgatccaaatgatgataataagcgtacgtgttctaattgggtacccttaactaataactatatggaatattgtctagtaatatatttggaaacaccgatatgtggaggcaaaataaaattataccaccctacaggaaatataaagtcggataaggatattatgtttgcaaagactctagactttaaatcaacgaaagtgttaactggacgtaaaacaattgccgttctagacatatccgtttcatataatagatcaatgactactattcactacaacgacgacgttgatatagatatacatactgataaaaacggaaaagagttatgttattgttatataacaatagatgatcattacttggttgatgtggaaactataggagttatagtcaatagatctggaaaatgtctgttagtaaataaccatctaggtataggtatcgttaaagataaacgtataagcgatagttttggagatgtatgtatggatacaatatttgacttttctgaagcacgagagttattttcattaactaatgatgataacaggaatatagcatgggacgatgatacagatatatggactcccgtcacagaagatgattacaaatttctttctagactagtattgtatgcaaaatctcaatcggatactgtattcgactattatgttcttactggtgatacggaaccacccactgtattcattttcaaggtaactagattttactttaatatgccgaaataaaaaatttttgtataatatctagaggtagaggtattgtttagataaatacaaataacatagatacatcgcatatttagcatttttataaatatacataagacatacactttatacatttttgtaaaaatactcataaaaaaaatttataaaaattatggcacaaccatatcttgtataggtagtttagttcgtcgagtgaacctataaacagataatagacaacacgtaataataataatgcctactaatacaagcataataccgggagatgggatatatgacgttgtagtgtttggtttttctgaacgttgatagtctactaatactacatgctgacatctaatgcctgtataaccatgagagcatctacaatacataccgtcgatatctctagcgtggatacagtcaccgtgtaaacaatatccatctccctctggaccgcataatctgatagctggaatatctgttgtagcgtttgtaatttctggcgatgtcgtttcgatagcgttaccactatcggcgaatgatctgattatcatagcagcgaacaacaacatcagataatttatcaacatttttgatggattttgtgtttatgctgtttctcagtgtgtgtttatgacaagattgggaattttatattattaattcagtaatataaactaataatatattgttaattgtgtaaataatataaaaataacaatacaatattgaatgtgttgctgttaaaaatgtatgtgttaatataatagaataaaataaatgagtatgatcattttagataacgattgattttatcattaccgcttcattcttatattctttgcttacggaacctatatttagaaacatctactaacgattttttatgcttgcattattaatggtatgtaataccaatttgttaagtatgaatacggggtacaaacataaactgaaatttagatcattaaatgtttcatcagaaatgactccatgaaaaccgccgaagaacttcgtgcaatcattggactttgtactcaatcagctatcgtctctggaagagtcttcaacgataagtatatcgacatactacttatgctgcgaaagattctgaacgagaacgactatctcaccctcttggatcatatccgcactgctaaatactaaatctccttcatgctctctcactacactttttatcatcttatgaggaataattagcaccagaatagctatggattgcacatgtattctatgtcgtctactggatgaagatgtgacgtacaaaaaaataaaactagaaattgaaacgtgtcacaacttatcaaaacatatagatagacgaggaaacaatgcgctacattgttacgtctccaataaatgcgatacagacattaagattgttcgactgttactctctcgcggagtcgagagactttgtagaaacaacgaaggattaactccgctaggagcatacagtaagcatagatacgtaaaatctcagattgtgcatctactgatatccagctattcgaattcctctaacgaactcaagtcgaatataaatgatttcgacttacgtctgctaaaatacctaattgtggataaacggatacgtccgtccaagaatacgaattatgcaatcaatggtctcggattggtggatatatacgtaacgacgcctaatccgagaccagaagtattgctatggcttcttaaatcagaatgttacagcaccggttacgtatttcgtacctgtatgtacaacagtgatatgtgtaagaactctcttcattactatatatcgtctcatagagaatctctatccaaggatgtaattaaatgtttgatcgataacaatgtttccatccaatactactggtcttgctcaaccatagatatagagattattaataaaggatgtggacacgtgtagagtatacgacgtcagccctatattagaggcgtattatctaaacaagcgatttagagtaaccccatataatgtagacatggaaatcgttaatcttcttattgagagacgtcatactcttgtcgacgtaatgcgtagtattacttcgtacgattccagagaatataaccactacatcatcgataacattctaaagagatttagacaacaggatgaatccatcgtacaagccatactgataaactacttacattacggcgatatggtaagtatacctatcattcaatgcatgttggataagacgacggacaacaactttgttaataataatctcgtcgatgtaaacgtcgtaaggtttatcgtggaaaatatggacacgcggctgtaaatcacatatctaacaatggccgtctatgtatgtacggtctgatattatcgagatttaataattgcgggtatcactgttatgaagatgtatttgatatactaagcaagtacatggatgatatagatatgatcgataactctactatattacgcggtcgatgtcaataatatacaatttgcaaagcggttattggaatatggagcgagtgtcacgctcgataatcaatacggccatccagaaaagcagttaccaaagagaagctagttgatttattactgagttaccatcccactctagagactatgattgacgcatttaatagagatatacgctatctatatcctgaaccattattcgcctgtatcagatacgccttaatcctagatgatgattttccttctaaagtaagtatgatatcgccggtcgtcataaggaactaaagcgctatagagcagacattaatagaatgaagaatgcctacatatcaggcgtctccatgtttgatatattatttaaacgaagcaaacgccacagattgagatacgcaaagaacaatgagaggatcgactccattaaataatttatcatggagtgataatgtcctgtttccatggcatattacaaaatcgattccgtccaagatgataaaaacatttaccggcatcataaacacggagtttattttatatgtctcgcataaacattactaaaaaaatatattgttcggttttctttcacatctttaattatgaaaaagtaaatcattatgagatggacgcatcgttcgcgacagtatgtggtacatacctaacgtatttatggacgacggtaagaatgaaggtcacgtttctgtcaacaatgtcgacgcgatcgtgtaacacgactcacaatagaatctgtgaatgctctcccgatcatggatgcaaggcatgtgtttcccaaacaaaatgtggaataggatacggagtatccggagacgtcatctgttctccgtgtggtctcggaacatattctcacaccgtctcttccgcagataaatgcgaacccgtacccagaaatacctttaactatatcgatgtggaaattaacctgtatccagttaacgacacatcgtgtactcggacgaccactaccggtctcagcgaatccatctcaacgtcggaactaactattactatgaatcataaagactgcgatcccgtcttcttaataaggtagcgacttcaggtttctttacaggagaaaggtgtgcactctgaatttcgagattaaatgcaataacaaagattcttcctccaaacagttaacgaaagcaaagaatgatactatcatgccgcattcggagacagtaactctagcgtcgacatctatatactatatagtaataccaatactcaagactacgaaactgatacaatctcttatcatgtgggtaatgtagccatatgcccggtagttgcgatatacataaactgatcactaattccaaacccacccgctttttatagtaagtttttcacccataaatacaataattaatttctcgtaaaagtagaaaatatattctaatttattgcacggtaaggaagtagaatcataaagaacagtactcaatcaatagcaatcatgaaacaatatatcgtactggcatgcatgtgcctgccagtcttcagcaatcatcctcatcgtgtacggaagaagaaaacaaacatcatatgggaatcgatgttattatcaaagtcacaaagcaagaccaaacaccgaccgatgataagatttgccaatccgtaacggaaattacagagtccgagtcagatccagatcccgaggtggaatcagtcgaggatgtagatcctcctaccacttattactccatcatcggtggaggtctgagaatgaactttggattcaccaaatgtcctcagattaaatccatctcagaatccgctgatggaaagactgtgaggtgtctatcgacatcagatgtagcgaagaagagaaagacagcgacatcaagacccatccagtactcgggtctaacatctctcataagaaagtgagttacgaagatatcatcggttcaacgatcgtcgatacaaaatgtgtcaagaatctagagtttagcgttcgtatcggagacatgtgcaaggaatcatctgaacttgaggtcaagtatgtcgacggatcggcatctgaaggtgcaaccgatgatacttcactcatcgattcaacaaaactcaaagcgtgtgtctgaatcgataactctattcatctgaaattggatgagtagggttaatcgaacgattcaggcacaccacgaattaaaaaagtgtaccggacactatattccggtttgcaaaacaaaaagttacctctcgcgacttcttctttttctgtctcaatagtgtgatacgattatgacactattcctatttcctttcagggtatcacaaaaatattaaacctctttctgatggtctcatacaaaaatatttttattctctttctctctttgatggtctcataaaaaatatttttattctctttctctctttgatggtctcataaaatatttttattctctttctctctttgatggtctcataaaaaatatttttattctctttctctctttgatggtctcataaaatatttttattctctttctctctttgatggtctcataaaaaatatttttattctctttctctctttgatggtctcataaaaaatattaaacctctttctgatggtgtcactaaaatatttttattctctttctctcttcaatggagtcataaaatatttttattctctttctctcttcgatggtctcacaaaaatattaaacctctttctgatggtgtcactaaaatatttttattctctttctctcttcaatggagtcataaaatatttttattctctttctctctttgatggtctcacaaaaatatttttattctctttctctctttgatggtctcacaaaaatatttttattctctttctctctttgatggtctcacaaaaatatttttattctctttctctctttgatggtctcataaaaaaagttttacaaaaatatttttattctctttctctctttgatggtctcataaaaaaagttttacaaaaatatttttattctctttctctctttgatggtctcataaaaaaagttttacaaaaatatttttattctctttctctctttgatggtctcataaaaaatattaaacctctttctgatggtgtcactaaaatatttttattctcattctctcttcaatggagtcataaaatatttttattctctttctctcttcgatggtctcacaaaaatattaaacctctttctgatggtgtcactaaaatatttttattctcattctctcttcaatggagtcataaaatatttttattctctttctctcttcgatggtctcacaaaaatattaaacctctttctgatggtgtcactaaaatatttttattctcattctctcttcaatggagtcataaaatatttttattctctttctctctttgatggtctcataaaaaaagttttacaaaaatatttttattctctttctctctttgatggtctcataaaaaatattaaacctctttctgatggtgtcactaaaatatttttattctctttctctcttcaatggagtcataaaatatttttattctctttctctcttcgatggtctcacaaaaatattaaacctctttctgatggtgtcactaaaatatttttattctcattctctcttcaatggagtcataaaatatttttattctctttctctctttgatggtctcataaaaaaagttttacaaaaatatttttattctctttctctctttgatggtctcataaaaaaagttttacaaaaatatttttattctctttctctctttgatggtctcataaaaaaagttttacaaaaatatttttattctctttctctctttgatggtctcataaaaaaagttttacaaaaatatttttattctctttctctctttgatggtctcataaaaaatattaaacctctttctgatggtgtcactaaaatatttttattctcattctctcttcaatggagtcataaaatatttttattctctttctctcttcgatggtctcacaaaaatattaaacctctttctgatggtgtcactaaaatatttttattctcattctctcttcaatggagtcataaaatatttttattctctttctctctttgatggtctcataaaaaaagttttacaaaaatatttttattctctttctctctttgatggtctcataaaaaaagttttacaaaaatatttttattctctttctctctttgatggtctcataaaaaaagttttacaaaaatatttttattctctttctctctttgatggtctcataaaaaaagttttacaaaaatatttttattctctttctctctttgatggtctcacaaaaatattaaacctctttctgatggagtcgtaaaaaagttttatctctttctccttcgatggtctcacaaaaatattaaacctctttctgatggagtcgtaaaaaagttttatctctttctctcttcgatggtctcacaaaaatattaaacctctttctgatggagtcgtaaaaaagttttatctctttctctcttcgatggtctcactaaaatattttttattctctttctgatgcatcaactatttcttaaacaataacgtccaacaacatatactcgtcgagcttatcaacatcccctatgcccatctaggttaccagacaattgtatatcataaaataatgtttataatttttacaaaaatatttttattctctttctctctttgatggtctcataaaaaaagttttacaaaaatatttttattctctttctctctttgatggtctcataaaaaatattaaacctctttctgatggtgtcactaaaatatttttattctcattctctcttcaatggagtcataaaatatttttattctctttctctcttcgatggtctcacaaaaatattaaacctctttctgatggtgtcactaaaatatttttattctcattctctcttcaatggagtcataaaatatttttattctctttctctctttgatggtctcataaaaaaagttttacaaaaatatttttattctctttctctctttgatggtctcataaaaaaagttttacaaaaatatttttattctctttctctctttgatggtctcataaaaaaagttttacaaaaatatttttattctctttctctctttgatggtctcataaaaaaagttttacaaaaatatttttattctctttctctctttgatggtctcataaaaaaagttttacaaaaatatttttattctctttctctctttgatggtctcataaaaaaagttttacaaaaatatttttattctctttctctctttgatggtctcataaaaaaagttttacaaaaatatttttattctctttctctctttgatggtctcataaaaaatattaaacctctttctgatggtgtcactaaaatatttttattctctttctctcttcaatggagtcataaaatatttttattctctttctctcttcgatggtctcacaaaaatattaaacctctttctgatggtgtcactaaaatatttttattctcattctctcttcaatggagtcataaaatatttttattctctttctctctttgatggtctcataaaaaaagttttacaaaaatatttttattctctttctctctttgatggtctcataaaaaaagttttacaaaaatatttttattctctttctctctttgatggtctcataaaaaaagttttacaaaaatatttttattctctttctctctttgatggtctcataaaaaaagttttacaaaaatatttttattctctttctctctttgatggtctcataaaaaaagttttacaaaaatatttttattctctttctctctttgatggtctcataaaaaatattaaacctctttctgatggtgtcactaaaatatttttattctctttctctcttcaatggagtcataaaatatttttattctctttctctcttcgatggtctcacaaaaatattaaacctctttctgatggtgtcactaaaatatttttattctctttctctcttcaatggagtcataaaatatttttattctctttctctctttgatggtctcataaaaaaagttttacaaaaatatttttattctctttctctctttgatggtctcataaaaaaagttttacaaaaatatttttattctctttctctctttgatggtctcataaaaaaagttttacaaaaatatttttattctctttctctctttgatggtctcataaaaaaagttttacaaaaatatttttattctctttctctctttgatggtctcataaaaaaagttttacaaaaatatttttattctctttctctctttgatggtctcataaaaaaagttttacaaaaatatttttattctctttctctctttgatggtctcataaaaaaagttttacaaaaatatttttattctctttctctctttgatggtctcataaaaaatattaaacctctttctgatggtgtcactaaaatatttttattctcattttctctttctctcttcaatggagtcataaaatatttttattctctttctctctttgatggtctcataaaaaatattaaacctctttctgatggtgtcactaaaatatttttattctcattctctcttcaatggagtcataaaaaagttttatctctttctctcttcgatggtctcacaaaaatattaaacctctttctgatggagtcgtaaaaaagttttatctctttctctcttcgatggtctcacaaaaatattaaacctctttctgatgcatcaactatttcttaaacaataacgtccaacaacatatactcatcccctatgcccatctaggttaccagacaattgtatatcataaaataatgtttataatttacacgttaaaatcatataataaaacgtagatcgtataatattttttggtatataaatgatctagtaaaatccatgtaggggatactgctcacattttttctttggtacaaaatttcacacaagtttttatacagacaaattcttgtccatatattttaaaacattgacttttgtactaagaaaaatatctagactaactatctctttctctttctctcttcgatggtctttctgatggagtcgtaaaaaagttttatctctttctctcttcgatggtctcacaaaaatattaaacctctttctgatggagtcgtaaaaaagttttatctctttctctcttcgatggtctcacaaaaatattaaacctctttctgatggagtcgtaaaaaagttttatctctttctccttcgatggtctcacaaaaatattaaacctctttctgatggagtcgtaaaaaagttttatctctttctctcttcgatggtctcacaaaaatattaaacctctttctgatggtgtcactaaaatatttttattctctttctctcttcgatggtctcacaaaaatattaaacctctttctgatggagtcgtaaaaaagttttatctctttctccttcgatggtctcacaaaaatattaaacctctttctgatggagtcgtaaaaaagttttatctctttctctcttcgatggtctcacaaaaatattaaacctctttctgatggagtcgtaaaaaagttttatctctttctccttcgatggtctcacaaaaatattaaacctctttctgatggagtcgtaaaaaagttttatctctttctccttcgatggtctcacaaaaatattaaacctctttctgatggagtcgtaaaaaagttttatctctttctccttcgatggtctcacaaaaatattaaacctctttctgatggagtcgtaaaaaagttttatctctttctctcttcgatggtctcacaaaaatattaaacctctttctgatggagtcgtaaaaaagttttatctctttctctcttcgatggtctcacaaaaatattaaacctctttctgatggagtcgtaaaaaagttttatctctttctccttcgatggtctcacaaaaatattaaacctctttctgatggtctctataaagcgattgatttttcttaccctctagagtttcctacggtcgttggtcacacatttttttctagacactaaataaatatttaaaatataatattaatatactaaaatttatgtattattaatttataatattaatatactaaaatttatgtattattaatttatctaactaaagttagtaaatcatatacataattttataattaatattatatacataattttataattaatttaatcttac

SEQ ID NO: 46 - DNA, 4590 bp, Artificial Sequence
  Vaccine construct
cccgccgccaccatgtctctgctgtggggcggagtgacagtgctggccgccatgctgattgctggccaggtggcctccgtggtgttcctcgtgaaaggcggaggacctggcggcggaatgcagctgtttcacctgtgcctgatcatcagctgtagctgccccaccgtgcaggccagcaagctgtgtctgggatggctgtggggaatggacatcgacccctacaaagaattcggcgccagcgtggaactgctgagcttcctgcccagcgacttcttcccctccatccgggacctgctggatacagccagcgccctgtatagagaggccctggaaagccccgagcactgcagccctcatcacaccgctctgagacaggccatcctgtgctggggcgagctgatgaacctggccacttgggtgggaagcaacctggaagatcccgccagccgggaactggtggtgtcttacgtgaacgtgaacatgggcctgaagatccggcagctgctgtggttccacatctcctgcctgaccttcggccgggaaaccgtgctggaatacctggtgtccttcggcgtgtggatcagaaccccccctgcctacagaccccccaacgcccctatcctgagcaccctgcctgagacaacagtcgtgcggcggagaggcagaagccccagaagaagaacccccagccccagacgcagaagaagccagtcccctcggcggagaagatcccagagcagggaaagccagtgtggcggaggctctgggggaggcatgccactgagctaccagcacttcagaaaactgctgctgctggacgacgaggccggacccctggaagaggaactgcctagactggccgacgagggcctgaacagaagagtggccgaggacctgaacctgggcaacctgaacgtgtccatcccctggacccacaaagtgggcaacttcaccggcctggcctccagcaccgtgcccgtgtttaatcccgagtggcagacccccagcttcccccacatccatctgcaggaagatatcatcaaccgctgccagcagtacgtgggccccctgaccgtgaacgagaagcggagactgaagctgatcatgcccgccagattctaccccaacctgaccaagtacctgcccctggacaagggcatcaagccctactaccctgagcacgccgtgaaccactacttcaagacccggcactacctgcacaccctgtggaaggccggcatcctgtacaagagagagacaaccagaagcgccagcttctgcggcagcccctacagctgggagcaggaactgcagcacggccggctggtgtttcagaccagcacaagacacggcgacgagtctttctgcagccagagcagcgggatcctgtccagatctcctgtgggcccttgtgtgcggagccagctgaagcagagcagactgggactgcagcctcagcagggaagcctggccagaggcaagtctggcagaagcggcagcatccgggccagagtgcaccctaccaccagacggtcctttggcgtggaacctagcggcagcggccacatcgataacagcgccagcagcacctccagctgcctgcatcagtctgccgtgcgcaagaccgcctacagccacctgtccaccagcaagagacagagcagctctggccacgctgtggaactgcacaacatcccccctagcagcgccagaagccagagcgagggccctatctttagcgcctggtggctgcagtttcggaacagcaagcccgccagcgactacgccctgacccacatcgtgaacctgctggaagattggggccctgccacagagcacggcgagcacaatatccggatccccagaacccctgccagagtgacaggcggcgtgttcctggtggataagaatccccacaacaccaccgagagcaggctggtggtggacttcagccagttcagcagaggcagcacccacgtgtcctggcccaagttcgccgtgcccaatctgcagagcctgaccaacctgctgagcagcaacctgagctggctgagcctggacgtgtccgccgccttctaccacatcccactgcatcctgccgctatgccccatctgctcgtgggcagttctggcctgcctagatatgtggcccggctgtctagcaccagcagaaacatcaattaccagcacggcaccatgcaggacctgcacgacagctgcagccggaatctgtacgtgtccctcctgctgctgtacaaaaccttcggcagaaagctgcacctgtactcccaccccatcatcctgggcttcagaaagatccccatgggcgtgggcctgagcccattcctgctggcccagtttaccagcgccatctgtagcgtcgtgcggagagccttccctcactgcctggcctttagctacatggacgacgtggtgctgggcgccaagagcgtgcagcacctggaatccctgtttacctccatcaccaactttctgctgtccctgggcatccacctgaaccccaacaagaccaagaggtggggctacagcctgaacttcatgggctacgtgatcggcagctggggcacactgcctcaggaacacatcgtgctgaagatcaagcagtgctttcggaagctgcccgtgaaccggcccatcgactggaaagtgtgccagcggatcgtggggctgctgggatttgccgccccttttacccagtgcggctaccccgctctgatgcccctgtacgcctgcattcagagcaagcaggccttcaccttcagccctacctacaaggcctttctgtgcaagcagtatctgaacctgtaccccgtggctcggcagagaagcggcctgtgtcaggtgttcgccgatgccacacctacaggatggggcctggccatcggacacagagccatgagaggcaccttcgtggcccctctgcctattcacacagccgagctgctggctgcctgtttcgccagatctagaagcggcgccaagctgatcggcaccgacaactctgtggtgctgagccggaagtacacctccttcccttggctgctgggctgcgccgccaactggatcctgagaggaaccagcttcgtgtacgtgccaagcgccctgaaccctgccgccgatcctagtgctggaaggctgggcctgtaccggccactgctgcatctgcctttcagacccaccaccggccggaccagtctgtatgccgtgtctcctagcgtgcccagccatctgcccgacagagtgcatttcgccagccctctgcatgtggcctggcggcctccaagaaaaagacgggcccctgtgaagcagaccctgaatttcgacctgctgaagctggccggcgacgtggaaagcaaccctggccctatgggcggctggtccagcaagcctagacagggcatgggcaccaacctgtccgtgcctaaccccctgggattcttcccagaccaccagctggaccctgccttcggagccaacagcaacaaccccgactgggatttcaaccctaacaaggaccactggcccgaggccaaccaagtgggagctggcgcatttggccctggcttcacacctcctcatggcggactgctggggtggtcacctcaggctcagggcatcctgactacagtgcctgccgctcctcctcccgcctccaccaatagacagagcggcagacagcccacccccatcagccctccactgagagatagccacccccaggccatgcagtggaacagcaccacctttcaccaggccctgctggacccaagagtgcgcggcctgtattttcctgccggcggaagctctagcggcaccgtgaatcctgtgcctaccaccgccagcccaatcagcagcatcttctccagaaccggcgaccctgcccccaacatggagaacaccacctccggctttctgggcccactgctggtgctgcaggccggcttttttctgctgacccggatcctgaccatcccccagtccctggactcttggtggacctccctgaactttctgggaggcgcccctacatgtcccggccagaatagccagagccccacctccaatcacagcccaaccagctgcccccctatctgccccggctatcggtggatgtgcctgcggcggttcatcatctttctgttcattctgctgctgtgtctgatcttcctgctggtgctgctggactaccagggcatgctgcctgtgtgccctctgctgcctggcacctctaccacaagcaccggcccttgcaagacttgcaccatcccagcccagggcaccagcatgttccccagctgttgctgcaccaagccctccgacggcaactgtacctgcatccccatcccaagcagctgggccttcgcccggtttctgtgggaatgggccagcgtgcggttctcctggctgagtctgctggtgcctttcgtgcagtggttcgtgggactgtcccctaccgtgtggctgagcgtgatctggatgatgtggtactggggcccctccctgtacaatatcctgtcccccttcctgcccctgctgcccatcttcttttgcctgtgggtgtacatctga

SEQ ID NO: 47 - DNA, 4578 bp, Artificial Sequence
  Vaccine construct
cccgccgccaccatgtctctgctgtggggcggagtgacagtgctggccgccatgctgattgctggccaggtggcctccgtggtgttcctcgtgaagggcggatctatgggcggctggtccagcaagcctagacagggcatgggcaccaacctgagcgtgcccaatcccctgggattcttcccagaccaccagctggatcctgccttcggcgccaacagcaacaaccccgactgggacttcaaccccaacaaggaccactggcccgaggccaaccaagtgggagctggcgcttttggccctggcttcacacctcctcatggcggactgctgggatggtcacctcaggcccagggcatcctgacaacagtgcctgctgctccacctcccgccagcaccaatagacagagcggcagacagcccacccccatcagccctccactgagagatagccacccccaggccatgcagtggaacagcaccacctttcaccaggccctgctggaccctagagtgcggggcctgtattttcctgccggcggaagcagcagcggcaccgtgaatcctgtgcctaccaccgccagccccatctccagcatcttcagcagaaccggcgaccctgcccccaacatggagaacaccaccagcggctttctgggccccctgctggtgctgcaggccggcttttttctgctgacccggatcctgaccattccccagagcctggactcctggtggacctccctgaacttcctgggcggagcccctacatgccctggccagaatagccagagccccaccagcaaccacagccctaccagctgccctcctatctgccccggctacaggtggatgtgcctgcggcggttcatcatctttctgttcatcctgctgctgtgcctgatctttctgctggtgctgctggactatcagggcatgctgcccgtgtgccctctgctgcctggcaccagcacaacaagcaccggcccttgcaagacctgcaccatccctgcccagggaaccagcatgttccccagctgctgctgcaccaagcccagcgacggcaactgcacctgtatccccatcccttccagctgggccttcgccagattcctgtgggagtgggccagcgtgcggttcagctggctgtcactgctggtgcccttcgtgcagtggttcgtgggcctgtctcctaccgtgtggctgagcgtgatctggatgatgtggtactggggcccctccctgtacaatatcctgagccccttcctgcccctgctgcccatcttcttttgcctgtgggtgtacatccggaagcggagagcccccgtgaagcagaccctgaatttcgacctgctgaagctggccggcgacgtggaaagcaaccctggccctatgcagctgtttcacctgtgtctgatcatcagctgtagctgccccaccgtgcaggccagcaagctgtgtctgggatggctgtgggggatggacatcgacccctacaaagaattcggcgcctctgtggaactgctgagcttcctgcctagcgacttcttcccctccatccgggacctgctggatacagccagcgccctgtatagagaggccctggaaagccccgagcactgcagccctcatcacaccgctctgaggcaggccatcctgtgttggggcgagctgatgaacctggccacttgggtgggaagcaacctggaagatcccgcctcccgggaactggtggtgtcttacgtgaacgtgaacatgggcctgaagatccggcagctgctgtggttccacatctcctgcctgaccttcggccgggaaaccgtgctggaatacctggtgtccttcggcgtgtggatcagaaccccccctgcctacagaccccccaacgcccctatcctgtccaccctgcctgagacaactgtcgtgcggcggagaggcagaagccccagaagaagaacccccagccccagacgcagaagaagccagtcccctcggcggagaagatcccagagcagggaaagccagtgtggcggaggatctggcggcggaatgcctctgagctaccagcacttccggaaactgctgctgctggatgacgaggccggacccctggaagaggaactgcctagactggccgacgagggcctgaacagaagagtggccgaggacctgaacctgggcaacctgaatgtgtctatcccctggacccacaaagtgggcaacttcaccggcctggcctccagcaccgtgcccgtgtttaatcccgagtggcagacccccagcttcccccacatccatctgcaggaagatatcatcaaccgctgccagcagtacgtgggccctctgaccgtgaacgagaagcgcagactgaagctgatcatgcccgccaggttctaccccaacctgaccaagtacctgcctctggacaagggcatcaagccctactaccctgagcacgccgtgaaccactacttcaagacccggcactacctgcacaccctgtggaaggccggcatcctgtataagcgggaaacaaccagatccgccagcttctgcggctccccctacagctgggagcaggaactgcagcacggccggctggtgtttcagacctctaccagacacggcgacgagtctttctgcagccagagcagcgggatcctgagcagatctccagtgggcccttgtgtgcggtcccagctgaagcagagtagactgggcctgcagcctcagcagggctctctggctagaggcaagtctggcagaagcggcagcatccgggccagagtgcaccctaccaccagacggtcctttggcgtggaacctagcggcagcggccacatcgataacagcgcctctagcacctccagctgcctgcatcagtccgccgtgcggaaaaccgcctacagccacctgagcacaagcaagagacagagcagctccggccacgccgtggaactgcacaatatcccccctagcagcgccagaagccagagcgagggccctatctttagcgcctggtggctgcagtttcggaacagcaagcccgccagcgactacgccctgacccacatcgtgaacctgctggaagattggggccctgccacagagcacggcgagcacaacatccggatccccagaacccctgccagagtgacaggcggcgtgttcctggtggataagaaccctcacaacaccaccgagagcagactggtggtggacttcagccagttcagccggggctctacccacgtgtcctggcctaagttcgccgtgcccaacctgcagagcctgaccaacctgctgtccagcaacctgtcctggctgtccctggatgtgtccgccgccttctaccacatcccactgcatcccgccgctatgccccatctgctcgtgggaagtagcggcctgcctagatacgtggccagactgagcagcacctcccggaacatcaattaccagcacggcaccatgcaggatctgcacgacagctgcagccggaacctgtacgtgtcccttctgctgctgtacaagaccttcggcagaaagctgcatctgtactcccaccccatcatcctgggctttagaaagatccccatgggcgtgggactgtccccattcctgctggcccagttcaccagcgccatctgttccgtcgtgcgcagagccttccctcactgcctggcctttagctacatggacgacgtggtgctgggcgccaagagcgtgcagcacctggaatccctgtttaccagcatcaccaactttctgctgagcctgggcatccacctgaaccctaacaagaccaagcgctggggctacagcctgaactttatgggctacgtgatcggctcctggggcacactgcctcaggaacacatcgtgctgaaaatcaagcagtgctttcggaagctgcctgtgaaccggcccatcgactggaaagtgtgccagcggattgtgggcctgctgggctttgccgccccttttacacagtgcggctaccccgctctgatgcccctgtacgcctgcattcagagcaagcaggccttcaccttcagcccaacctacaaggccttcctgtgcaagcagtacctgaatctgtaccccgtggcccggcagagaagcggcctgtgtcaggtgttcgccgatgccacacctacaggatggggcctggccatcggacacagagccatgagaggcaccttcgtggccccactgcctattcacacagccgagctgctggctgcctgtttcgccaggtctagaagcggcgccaagctgatcggcaccgacaactctgtggtgctgagccggaagtacacctccttcccttggctgctgggctgcgccgccaactggatcctgagaggcacaagcttcgtgtacgtgccctccgccctgaatcctgccgccgatcctagtgctggacggctgggactgtaccggcctctgctgcatctgcccttcagacccaccaccggcagaaccagcctgtatgccgtgtcccctagcgtgccaagccatctgcccgacagagtgcatttcgcctcccccctgcatgtggcttggaggcccccttaa

SEQ ID NO: 48 - DNA, 4704 bp, Artificial Sequence
  Vaccine construct
cccgccgccaccatgtctttgctttggggcggagtgacagtgctggccgccatgcttattgctggacaggtggccagcgtggtgttcctggtcaaaggcggaggacctggcggaggcatgcagctgtttcacctgtgcctgatcatcagctgtagctgccctacagtgcaggccagcaagctgtgtcttggatggctgtggggcatggacatcgacccctacaaagaattcggcgcctccgtggaactgctgagcttcctgcctagcgacttcttcccctccatccgggatctgctggatacagccagcgcactgtatagagaggccctggaaagccccgagcactgttctccacatcacacagccctgagacaggccatcctgtgttggggcgagctgatgaatctggccacatgggtcggaagcaacctggaagatcccgccagcagagaactggtggtgtcctacgtgaacgtgaacatgggcctgaagatccggcagctgctgtggttccacatctcctgcctgaccttcggcagagaaaccgtgctggaatacctggtgtccttcggcgtgtggatcagaacccctccagcctacagacctcctaacgctcccatcctgagcaccctgcctgagacaacagtcgtgcggagaagaggcagaagccccagaagaagaaccccatctcctcggaggcggagatctcagtcccctcggagaagaagatcccagagcagggaaagccagtgcggtggtggaagtggtggcggaatgcctctgagctaccagcacttcagaaaactgctgctgctggacgacgaggccggacctcttgaggaagaactgcctagactggccgacgagggcctgaatagaagagtggccgaggacctgaacctgggcaacctgaatgtgtctatcccctggacacacaaagtgggcaacttcacaggcctggccagctctaccgtgcctgtgttcaatcccgagtggcagacccctagcttccctcacatccatctgcaagaggacatcatcaaccggtgccagcagtacgtgggccctctgaccgtgaacgagaagcggagactgaagctgatcatgcccgccagattctaccccaacctgaccaagtacctgcctctggacaagggcatcaagccttactaccctgagcacgccgtgaaccactacttcaagacccggcactacctgcacaccctgtggaaggccggcatcctgtacaagagagagacaaccagaagcgccagcttctgcggcagcccttactcttgggagcaagagctgcagcacggcagactggtgttccagacctctacaagacacggcgacgagtctttctgcagccagagcagcgggatcctgtctagatctcctgtgggaccttgtgtgcggagccagctgaaacagagcagactgggactgcagcctcagcagggatctctggctagaggcaagtctggcagaagcggcagcatcagagccagagtgcaccctaccaccagacggtcctttggcgtggaacctagcggcagcggccacatcgataatagcgccagcagcaccagcagctgtctgcatcagtctgctgtgcgcaagaccgcctacagccacctgagcacaagcaagagacagagcagctctggccacgccgtcgagctgcacaatatccctccaagcagcgccagaagccagagcgagggccctattttttctgcctggtggctgcagttcagaaacagcaagcccgccagcgactacgccctgacacacatcgtgaacctgctggaagattggggccctgccacagaacacggcgagcacaacatcagaatccccaggactcccgccagagtgaccggcggagttttcctggtggacaagaaccctcacaacaccaccgagagcaggctggtggtggacttcagccagtttagcagaggcagcacccacgtgtcctggcctaaattcgccgtgcctaacctgcagagcctgaccaatctgctgagcagcaacctgagctggctgagcctggatgtgtccgccgccttctatcacatcccactgcatcctgccgctatgccccatctgcttgtgggaagttctggcctgcctagatatgtggcccggctgtcctctaccagccggaacatcaattaccagcacgggaccatgcaggacctgcacgatagctgctcccggaacctgtacgttagcctgctcctgctgtacaaaaccttcggccggaagctgcacctgtactctcaccctatcatcctgggcttcagaaagatccccatgggcgtgggactgagcccatttctgctggcccagtttaccagcgccatctgcagtgttgtgcggagagcctttcctcactgcctggccttcagctacatggacgatgtggtgctgggcgccaagtctgtgcagcacctggaatctctgtttacctccatcaccaactttctgctgtccctgggaatccatctgaaccccaacaagacaaagagatggggctacagcctgaacttcatgggctacgtgatcggcagctggggcacactgcctcaagagcacatcgtgctgaagatcaagcagtgctttagaaagctgcccgtgaacagacccatcgactggaaagtgtgccagcggattgtgggcctgctgggatttgccgctcctttcacacagtgcggctaccccgctctcatgcctctgtacgcctgcatccagtccaagcaggccttcacattcagccctacctacaaggccttcctgtgcaagcagtacctgaatctgtaccccgtggctagacagagaagcggcctgtgtcaggtgttcgccgatgccacacctacaggatggggactcgccattggacacagggccatgagaggaacctttgtggcccctctgcctattcacaccgccgaattgctggctgcctgtttcgccagatctagaagcggcgccaagctgatcggcaccgacaattcagtggtgctgagccggaagtacaccagctttccatggctgctgggctgtgccgccaactggattctgagaggcaccagcttcgtgtacgtgcccagcgctcttaaccctgccgctgatcctagtgctggacggctgggactctacagaccactgctgcatctgcccttcagacccaccacaggcagaaccagcctgtatgccgtgtctcctagcgtgccaagccatctgcctgatcgggtgcactttgcctctccactgcatgtggcttggcggcctccaaagagccccaacagcaacaaccccgactgggatttcaaccctaacaaggaccactggcctgaggccaatcaagttggagccggcgcttttggccctggctttacacctcctcatggcggactgcttggatggtcacctcaggctcagggcatcctgactacagtgcctgctgctccacctcctgccagcaccaatagacagtcaggcagacagcccacacctatcagccctccactgcgggatagtcacccacaggccatgcaatggaacagcaccaccttccatcaggccctgctggatcctagagtgcggggcctgtattttcctgccggcggatctagctccggcaccgtgaatcctgtgcctacaaccgcctctcctatcagcagcatcttcagccggacaggcgaccctgctcctaatggctctaagggcaagagaaagcggagggcccctgtgaaacagaccctgaatttcgacctgctgaagctggccggcgacgtggaatctaaccctggacctatgggcggctggtccagcaaacctagacaaggcatgggcaccaatctgagcgtgcccaatccactgggattcttcccagaccaccagctggaccctgccttcggcgccaatagcaacaatcctgattgggactttaatcccaacaaagatcattggcccgaagctaatcaagtcggcctggaaggcggaagcggcggcatggagaataccacatctggctttctgggcccactgctggttctccaggccggcttttttctcctgacacggatcctgacaatccctcagagcctggactcttggtggacctctctgaacttccttggcggagcccctacctgtcctggacagaatagccagtctcctaccagcaatcacagccccacaagctgccctccaatctgccctggctatcggtggatgtgcctgcggcggttcatcatctttctgttcatcctgctgctgtgtctgatcttcctgctggtcctcctggactaccagggcatgctgccagtttgtcctctgctgcctggcacctccacaacatctacaggcccttgcaagacctgtacaatccccgctcagggaaccagcatgttccccagctgttgctgcaccaagccaagcgacggcaactgcacatgcatccccattcctagcagctgggcctttgccagatttctgtgggagtgggcctccgtgcggtttagctggctgtctctgctcgtgcctttcgtgcagtggttcgtcggactgtctccaaccgtgtggctgagcgtgatctggatgatgtggtactggggccctagcctgtacaatattctgagccccttcctgcctctcctgccaatcttcttttgtctgtgggtgtacatctga

SEQ ID NO: 49 - DNA, 4800 bp, Artificial Sequence
  Vaccine construct
cccgccgccaccatgtctttgctttggggcggagtgacagtgctggccgccatgcttattgctggacaggtggccagcgtggtgttcctggtcaaaggcggaggacctggcggaggcatgcagctgtttcacctgtgcctgatcatcagctgtagctgccctacagtgcaggccagcaagctgtgtcttggatggctgtggggcatggacatcgacccctacaaagaattcggcgcctccgtggaactgctgagcttcctgcctagcgacttcttcccctccatccgggatctgctggatacagccagcgcactgtatagagaggccctggaaagccccgagcactgttctccacatcacacagccctgagacaggccatcctgtgttggggcgagctgatgaatctggccacatgggtcggaagcaacctggaagatcccgccagcagagaactggtggtgtcctacgtgaacgtgaacatgggcctgaagatccggcagctgctgtggttccacatctcctgcctgaccttcggcagagaaaccgtgctggaatacctggtgtccttcggcgtgtggatcagaacccctccagcctacagacctcctaacgctcccatcctgagcaccctgcctgagacaacagtcgtgcggagaagaggcagaagccccagaagaagaaccccatctcctcggaggcggagatctcagtcccctcggagaagaagatcccagagcagggaaagccagtgcggtggtggaagtggtggcggaatgcctctgagctaccagcacttcagaaaactgctgctgctggacgacgaggccggacctcttgaggaagaactgcctagactggccgacgagggcctgaatagaagagtggccgaggacctgaacctgggcaacctgaatgtgtctatcccctggacacacaaagtgggcaacttcacaggcctggccagctctaccgtgcctgtgttcaatcccgagtggcagacccctagcttccctcacatccatctgcaagaggacatcatcaaccggtgccagcagtacgtgggccctctgaccgtgaacgagaagcggagactgaagctgatcatgcccgccagattctaccccaacctgaccaagtacctgcctctggacaagggcatcaagccttactaccctgagcacgccgtgaaccactacttcaagacccggcactacctgcacaccctgtggaaggccggcatcctgtacaagagagagacaaccagaagcgccagcttctgcggcagcccttactcttgggagcaagagctgcagcacggcagactggtgttccagacctctacaagacacggcgacgagtctttctgcagccagagcagcgggatcctgtctagatctcctgtgggaccttgtgtgcggagccagctgaaacagagcagactgggactgcagcctcagcagggatctctggctagaggcaagtctggcagaagcggcagcatcagagccagagtgcaccctaccaccagacggtcctttggcgtggaacctagcggcagcggccacatcgataatagcgccagcagcaccagcagctgtctgcatcagtctgctgtgcgcaagaccgcctacagccacctgagcacaagcaagagacagagcagctctggccacgccgtcgagctgcacaatatccctccaagcagcgccagaagccagagcgagggccctattttttctgcctggtggctgcagttcagaaacagcaagcccgccagcgactacgccctgacacacatcgtgaacctgctggaagattggggccctgccacagaacacggcgagcacaacatcagaatccccaggactcccgccagagtgaccggcggagttttcctggtggacaagaaccctcacaacaccaccgagagcaggctggtggtggacttcagccagtttagcagaggcagcacccacgtgtcctggcctaaattcgccgtgcctaacctgcagagcctgaccaatctgctgagcagcaacctgagctggctgagcctggatgtgtccgccgccttctatcacatcccactgcatcctgccgctatgccccatctgcttgtgggaagttctggcctgcctagatatgtggcccggctgtcctctaccagccggaacatcaattaccagcacgggaccatgcaggacctgcacgatagctgctcccggaacctgtacgttagcctgctcctgctgtacaaaaccttcggccggaagctgcacctgtactctcaccctatcatcctgggcttcagaaagatccccatgggcgtgggactgagcccatttctgctggcccagtttaccagcgccatctgcagtgttgtgcggagagcctttcctcactgcctggccttcagctacatggacgatgtggtgctgggcgccaagtctgtgcagcacctggaatctctgtttacctccatcaccaactttctgctgtccctgggaatccatctgaaccccaacaagacaaagagatggggctacagcctgaacttcatgggctacgtgatcggcagctggggcacactgcctcaagagcacatcgtgctgaagatcaagcagtgctttagaaagctgcccgtgaacagacccatcgactggaaagtgtgccagcggattgtgggcctgctgggatttgccgctcctttcacacagtgcggctaccccgctctcatgcctctgtacgcctgcatccagtccaagcaggccttcacattcagccctacctacaaggccttcctgtgcaagcagtacctgaatctgtaccccgtggctagacagagaagcggcctgtgtcaggtgttcgccgatgccacacctacaggatggggactcgccattggacacagggccatgagaggaacctttgtggcccctctgcctattcacaccgccgaattgctggctgcctgtttcgccagatctagaagcggcgccaagctgatcggcaccgacaattcagtggtgctgagccggaagtacaccagctttccatggctgctgggctgtgccgccaactggattctgagaggcaccagcttcgtgtacgtgcccagcgctcttaaccctgccgctgatcctagtgctggacggctgggactctacagaccactgctgcatctgcccttcagacccaccacaggcagaaccagcctgtatgccgtgtctcctagcgtgccaagccatctgcctgatcgggtgcactttgcctctccactgcatgtggcttggcggcctccaaagagccccaacagcaacaaccccgactgggatttcaaccctaacaaggaccactggcctgaggccaatcaagttggagccggcgcttttggccctggctttacacctcctcatggcggactgcttggatggtcacctcaggctcagggcatcctgactacagtgcctgctgctccacctcctgccagcaccaatagacagtcaggcagacagcccacacctatcagccctccactgcgggatagtcacccacaggccatgcaatggaacagcaccaccttccatcaggccctgctggatcctagagtgcggggcctgtattttcctgccggcggatctagctccggcaccgtgaatcctgtgcctacaaccgcctctcctatcagcagcatcttcagccggacaggcgaccctgctcctaatggctctaagggcaagagaaagcggagggcccctgtgaaacagaccctgaatttcgacctgctgaagctggccggcgacgtggaatctaaccccggacctatggacgccatgaagaggggcctgtgttgtgtcctgctgctgtgtggcgctgtgttcgtgtctcccagccaagagatccacgccagatttcggagaatgggcggctggtccagcaagcctagacaaggcatgggcaccaatctgagcgtgcccaatccactgggattcttcccagaccaccagctggaccctgccttcggcgccaatagcaacaatcctgattgggactttaatcccaacaaagatcattggcccgaagctaatcaagtcggcctggaaggcggaagcggcggcatggagaataccacatctggctttctgggcccactgctggttctccaggccggcttttttctcctgacacggatcctgacaatccctcagagcctggacagttggtggacctctctgaacttccttggcggagcccctacctgtcctggacagaatagccagtctcctaccagcaatcacagccccacaagctgccctccaatctgccctggctatcggtggatgtgcctgcggcggttcatcatctttctgttcattctgctgctttgcctgatcttcctgctggtcctcctggactaccagggcatgctgccagtttgtcctctgctgcctggcacctccacaacctctacaggcccttgcaagacctgtacaatccccgctcagggaaccagcatgttccccagctgttgctgcaccaagccaagcgacggcaactgcacatgcatccccattcctagcagctgggcctttgccagattcctctgggaatgggcctccgtgcggtttagctggctgtctctgctcgtgcctttcgtgcagtggttcgtcggactgtctccaaccgtgtggctgagcgtgatctggatgatgtggtactggggccctagcctgtacaatattctgagccccttcctgcctctcctgccaatcttcttttgtctgtgggtgtacatctga

SEQ ID NO: 50 - DNA, 2100 bp, Artificial Sequence
  Promoter
tgagatttctgtcgccgactaaattcatgtcgcgcgatagtggtgtttatcgccgatagagatggcgatattggaaaaatcgatatttgaaaatatggcatattgaaaatgtcgccgatgtgagtttctgtgtaactgatatcgccatttttccaaaagtgatttttgggcatacgcgatatctggcgatagcgcttatatcgtttacgggggatggcgatagacgactttggtgacttgggcgattctgtgtgtcgcaaatatcgcagtttcgatataggtgacagacgatatgaggctatatcgccgatagaggcgacatcaagctggcacatggccaatgcatatcgatctatacattgaatcaatattggccattagccatattattcattggttatatagcataaatcaatattggctattggccattgcatacgttgtatccatatcataatatgtacatttatattggctcatgtccaacattaccgccatgttgacattgattattgactagttattaatagtaatcaattacggggtcattagttcatagcccatatatggagttccgcgttacataacttacggtaaatggcccgcctggctgaccgcccaacgacccccgcccattgacgtcaataatgacgtatgttcccatagtaacgccaatagggactttccattgacgtcaatgggtggagtatttacggtaaactgcccacttggcagtacatcaagtgtatcatatgccaagtacgccccctattgacgtcaatgacggtaaatggcccgcctggcattatgcccagtacatgaccttatgggactttcctacttggcagtacatctacgtattagtcatcgctattaccatggtgatgcggttttggcagtacatcaatgggcgtggatagcggtttgactcacggggatttccaagtctccaccccattgacgtcaatgggagtttgttttggcaccaaaatcaacgggactttccaaaatgtcgtaacaactccgccccattgacgcaaatgggcggtaggcgtgtacggtgggaggtctatataagcagagctctccctatcagtgatagagatctccctatcagtgatagagatcgtcgacgagctcgtttagtgaaccgtcagatcgcctggagacgccatccacgctgttttgacctccatagaagacaccgggaccgatccagcctccgcggccgggaacggtgcattggaacgcggattccccgtgccaagagtgacgtaagtaccgcctatagagtctataggcccacccccttggcttcttatgcatgctatactgtttttggcttggggtctatacacccccgcttcctcatgttataggtgatggtatagcttagcctataggtgtgggttattgaccattattgaccactcccctattggtgacgatactttccattactaatccataacatggctctttgccacaactctctttattggctatatgccaatacactgtccttcagagactgacacggactctgtatttttacaggatggggtctcatttattatttacaaattcacatatacaacaccaccgtccccagtgcccgcagtttttattaaacataacgtgggatctccacgcgaatctcgggtacgtgttccggacatgggctcttctccggtagcggcggagcttctacatccgagccctgctcccatgcctccagcgactcatggtcgctcggcagctccttgctcctaacagtggaggccagacttaggcacagcacgatgcccaccaccaccagtgtgccgcacaaggccgtggcggtagggtatgtgtctgaaaatgagctcggggagcgggcttgcaccgctgacgcatttggaagacttaaggcagcggcagaagaagatgcaggcagctgagttgttgtgttctgataagagtcagaggtaactcccgttgcggtgctgttaacggtggagggcagtgtagtctgagcagtactcgttgctgccgcgcgcgccaccagacataatagctgacagactaacagactgttcctttccatgggtcttttctgca

SEQ ID NO: 51 - DNA, 673 bp, Artificial Sequence
  Promoter
cctttcactcattagatgcatgtcgttacataacttacggtaaatggcccgcctggctgaccgcccaacgacccccgcccattgacgtcaataatgacgtatgttcccatagtaacgccaatagggactttccattgacgtcaatgggtggagtatttacggtaaactgcccacttggcagtacatcaagtgtatcatatgccaagtacgccccctattgacgtcaatgacggtaaatggcccgcctggcattatgcccagtacatgaccttatgggactttcctacttggcagtacatctacgtattagtcatcgctattaccatggtgatgcggttttggcagtacatcaatgggcgtggatagcggtttgactcacggggatttccaagtctccaccccattgacgtcaatgggagtttgttttggaaccaaaatcaacgggactttccaaaatgtcgtaacaactccgccccattgacgcaaatgggcggtaggcgtgtacggtgggaggtctatataagcagagctctccctatcagtgatagagatctccctatcagtgatagagatcgtcgacgagctcgtttagtgaaccgtcagatcgcctggagacgccatccacgctgttttgacctccatagaagacaccgggaccgatccagcctccggt

SEQ ID NO: 52 - protein, 119 aa, Hepatitis B virus
MGGWSSKPRQGMGTNLSVPNPLGFFPDHQLDPAFGANSNNPDWDFNPNKDHWPEANQVGAGAFGPGFTPPHGGLLGWSPQAQGILTTVPAAPPPASTNRQSGRQPTPISPPLRDSHPQA

SEQ ID NO: 53 - protein, 55 aa, Hepatitis B virus
MQWNSTTFHQALLDPRVRGLYFPAGGSSSGTVNPVPTTASPISSIFSRTGDPAPN

SEQ ID NO: 54 - protein, 25 aa, Hepatitis B virus
FLGPLLVLQAGFFLLTRILTIPQSL

SEQ ID NO: 55 - protein, 19 aa, Hepatitis B virus
FIIFLFILLLCLIFLLVLL

SEQ ID NO: 56 - protein, 25 aa, Hepatitis B virus
RFLWEWASVRFSWLSLLVPFVQWFV

SEQ ID NO: 57 - protein, 22 aa, Hepatitis B virus
TVWLSVIWMMWYWGPSLYNILS

SEQ ID NO: 58 - DNA, 7239 bp, Artificial Sequence
  Vaccine construct
gtaatctattcgatataccgttgctaacagtatactggcccaataactgtggatggaaaatctataataatacattaatatcatccgatggtgctagggttatttggatggatgcgtataaattttcttgcggtttatctttacaagactattgttatcattggggtagcaaaccagagagccgaccattcgatttaataaaaaaatcagatgctaaacgcaattctaaatcgttggtcaaagaatctatggcatccttgaaatccttgtacgaggcattcgagacacaatcaggagcgttagaagttttaatgagtccatgtaggatgttttcgttttctagaatagaagacatgttcttaactagtgtcattaatagagtatccgagaatactggaatggggatgtattatcctaccaacgatataccttctctatttatcgaatcatctatctgtctagattatattatagtaaataatcaggaatccaacaaatatcgtatcaaatctgttctcgatatcatttcttcaaaacaataccctgcaggacgtcccaactacgttaaaaatggtacaaaaggaaagttatatatcgcgttgtgtaaagttaccgtacctactaacgaccatattccagtagtttatcacgatgatgacaatactaccacctttattacagtattgacgtccgtcgatattgaaactgctatcagagcaggatattcgatagtcgaattaggggctttacaatgggataataatattccagaacttaaaaacggtttactggatagtatcaagatgatttatgacttgaacgcagttacaacaaataatttattggaacagctcatagaaaatattaactttaacaactctagtataatttcgttgttttatacatttgccattagttattgccgagcattcatttactcaattatggaaaccatagatccggtgtatatatctcagttcagttataaagaattatacgttagtagctcttataaagatattaatgaatccatgagtcagatggtaaaattataaaaagtgaaaaacaatattatttttatcgttggttgttacactatgtcacttctttggggcggagttacagttcttgctgctatgcttattgctggacaagttgcttctgttgtgtttcttgtttctaaatctggacctccttctggaaaatctaattctaacaatcctgattgggatttcaatcctaacaaagatcattggcctgaagctaatcaagttggagctggtgcttttggacctggttttacacctcctcatggtggattgcttggatggtcacctcaagctcagggaattcttacaacagttccagctgctcctcctcctgcttctacaaatagacaatctggtagacaacctacacctatttctccacctcttagagattctcatcctcaagctatgcaatggaattctactacatttcatcaagctttgcttgatcctagagttagaggactttattttcctgctggtggaagttcttctggaacagttaatcctgttcctacaacagcttctccaatttcttctatattttctagaacaggcgatcctgctcctaatggatcaaaatctggatcaaaaatgcctctgtcttatcaacactttagaaaattgctgcttcttgatgatgaagctggacctcttgaagaagaattgcctagacttgctgatgaaggacttaatagaagagttgctgaagatcttaatctgggaaatcttaatgtttctattccttggacacacaaagttggaaatttcacaggacttgcatcttctacagtgcctgtttttaatcctgaatggcaaacaccttcttttccacatattcatctgcaagaggatatcatcaatagatgtcaacaatatgttggaccactgacagttaatgagaagagaaggcttaaacttattatgcctgctagattctatcctaatcttacaaagtatttgcctctggataagggaatcaaaccttattatcctgaacatgctgtgaatcactactttaaaacaagacattatctgcatacactgtggaaagctggtattctttacaaaagagaaacaacaagatctgcttcattttgtggatctccatattcttgggaacaagaacttcaacatggtagacttgtttttcaaacatctacaagacatggggatgaatcattttgttctcaaagttctggaattctttctagatctcctgttggaccttgtgttagatctcaacttaaacaatctagacttggacttcaacctcaacaaggatctcttgctagaggaaaaagtggaagatctggatctattagagctagagttcatcctacaactagaagatcttttggagttgaaccttctggatctggacatattgataattctgcctcttctacatcttcttgtctgcatcaatctgctgttagaaagacagcttattctcatttgtctacttctaagagacaatcatcttctggacatgctgttgaacttcataatattcctccaagtagtgctagaagtcaatctgaaggaccaatattttcagcttggtggcttcaattcagaaattctaaacctgcttctgattatgctctgacacatatagttaatttgcttgaagattggggacctgctacagaacatggcgaacacaatattagaatacctagaactcctgctagagttacaggcggagtctttttggttgataagaatcctcataataccacagaatcaagacttgttgttgatttttcacagttttctagaggatctacacatgtttcttggcctaaatttgctgttccaaatcttcaatctcttacaaatttgctttcatctaatctttcttggctgtctcttgatgtttctgctgccttttatcatattcctcttcatcctgctgcaatgcctcatttgcttgttggatcatctggacttccaagatatgttgctagacttagctctacatctagaaatatcaattatcagcatggaacaatgcaggatcttcacgattcttgtagtaggaatctgtatgtttctttgcttctgctgtataagacatttggaagaaaacttcatctgtattctcaccctattattctgggttttagaaagattcctatgggagttggactttctccttttttgcttgctcaattcacatctgctatttgttctgttgttagaagggcttttcctcattgtcttgcattttcttatatggatgatgttgttcttggagctaaatctgttcaacatcttgaaagtctgtttacctctattactaattttctgctttctctgggaattcatctgaatccaaacaaaacaaagagatggggatattctcttaatttcatgggatatgttattggatcttggggaacacttcctcaagaacatatcgttttgaaaatcaagcaatgtttcagaaaactgcctgtgaatagacctattgattggaaagtttgtcaaagaattgtgggacttcttggatttgctgctccttttacacaatgtggatatcctgctcttatgccactttatgcttgtattcaatctaaacaggcttttacattttctccaacatacaaagcttttctgtgtaaacagtatctgaatctttatcctgtggctagacaaagatctggtctttgtcaagtttttgctgatgctacaccaacaggatggggacttgctattggacatagagctatgagaggaacatttgttgctccattgcctattcatacagctgaattgcttgctgcttgttttgctagatctagaagcggagcaaaacttattggtacagataatagtgttgtcctgagtagaaagtacacatcttttccatggttgttgggatgtgctgctaattggattcttagaggaacttcttttgtttatgttccttctgctcttaatcctgcagctgatccatctgctggtagattgggactgtatagaccacttcttcatttgccttttagaccaacaactggaagaacatctctttatgctgtttctccttctgttccatctcatttgcctgatagagttcattttgcttctccacttcatgttgcttggaggccaccatctaaatctccaggttctggaccacctatgcaactttttcatttgtgtttgatcattagctgttcttgtcctacagttcaagcttctaaactttgtcttggatggctttggggaatggatattgatccatacaaagaatttggagctagtgttgaattgctgtcatttcttccatctgattttttcccttctattcgtgatcttcttgatacagcatctgctctgtatagagaagctcttgaatctcctgaacactgttctccacatcatacagcacttagacaagctattctttgttggggagaacttatgaatcttgctacatgggttggatctaatttggaagatccagcttctagagaattggtggtttcttatgttaatgtgaatatgggactgaaaattagacaactgctttggtttcatatctcttgtcttacatttggtagagaaacagttttggaatatttggtttcttttggcgtttggattagaacacctccagcttatagacctcctaatgctcctattttgtctacacttcctgaaacaacagtcgttagaagaagaggaagatctccaagaagaagaacaccaagtcctagaagaagaagatctcaatcaccaagaagaagaagaagtcaatctagagaatctcaatgttgatttttgttcgacattaaaaattgaaaataaatacaaaggttcttgagggttgtgttaaattgaaagcgagaaataatcataaatatgattcaggtgacggatccatggatgctatgaagcgaggactttgttgtgttttgcttctttgtggtgctgtgtttgtttctccatctcaagaaattcatgccagattcagaagaatgggaggctggtcatctaaacctagacaaggcatgggaacaaatctttctgttcctaatcctttgggattctttcctgatcatcaattggatccagcatttggagcaaatagtaacaatccagattgggactttaacccaaacaaagatcattggccagaagctaatcaagttggagcatctaaaggtggaaaaagtggaatggaaaacactacatctggatttcttggacctttgcttgttcttcaagctggatttttcctgttgacaagaatacttacaattcctcaatcactggattcttggtggacaagtcttaattttcttggaggtgctcctacatgtcctggacaaaattctcaatctccaacttctaatcattctcctacatcttgtcctccaatttgtcctggatatagatggatgtgtcttagaagattcattatctttcttttcatactgctgctgtgtctgattttccttcttgttttgttggattatcagggaatgcttcctgtttgtcctttgcttcctggaacttctacaacaagtacaggaccttgtaaaacatgtacaattccagcacagggaacatctatgtttccaagttgttgttgtacaaaaccttctgatggaaattgcacatgtattcctattccaagttcttgggcatttgctagatttctttgggaatgggcttctgttagattcagttggttgtctcttttggttccatttgttcagtggtttgttggattgtctcctacagtttggctttctgttatttggatgatgtggtattggggaccttctctttacaatattttgagtccttttctccctttgctgccaattttcttttgtctttgggtttacatttgattaaccgagtttctgcattattgtaattcgtatgctggcaccatcaaagaatcacttctaaaagatatcaatatcacacatacaaatattactaccctattgaatgagacagccaaggttatcaagttagtaaaatctctggtagataaagaagatactgatattgtgaataatttcattaccaaagaaattaaaaacagagacaaaatagttaatagtttgtctctatcaaacctggactttcgtttgtaaattggggctttttgtacaataaatgggtgttgccaatgattcatcccctgaatatcaatggatgtctccccatagattatcagatactgttatattaggagactgtttgtattttaacaatataatgtcccaattagatttacaccaaaattgggctccatcagttagattgttaaattattttaagaattttaataaggaaacactactaaagatagaagagaatgattacattaattcatcctttttccaacaaaaggataaacgattttatcctataaacgacgatttttatcacatatctacaggaggatatggtatagtctttaagatagataactatgtagtaaaatttgtattcgaggccacaaaattatatagtcccatggaaactacggcggagttcacagtacccaaatttctatacaacaatctaaagggagatgaaaaaaaattaatcgtgtgtgcgtgggccatgggattaaactataaattaacatttttacatactctgtataaacgtgttcttcatatgttgctattattgatacaaactatggatggtcaggaactatcattgagatattcttctaaagtttttttaaaggcgtttaacgagagaaaggacagtatcaaattcgtgaaattactatcccacttttatccggcagttattaacagtaatattaatgttataaactattttaaccgcatgtttcactttttcgaacatgaaaagagaactaactacgaatacgaaagaggaaatattataatttttcccctagcactgtattcggcagataaagtagataccgagctagctatcaaattaggatttaaatctttggtacaatacataaagtttatctttttacagatggctctgttatacattaaaatttacgaactaccatgctgcgacaactttttacacgcagatcttaaacccgataatatcttactttttgattccaatgaaccaataataattcatctaaaggataaaaagtttgtttttaatgaacgtattaaatcggcattaaacgactttgacttttcccaag

SEQ ID NO: 59 - DNA, 3741 bp, Artificial Sequence
  Vaccine construct
atgtcacttctttggggcggagttacagttcttgctgctatgcttattgctggacaagttgcttctgttgtgtttcttgtttctaaatctggacctccttctggaaaatctaattctaacaatcctgattgggatttcaatcctaacaaagatcattggcctgaagctaatcaagttggagctggtgcttttggacctggttttacacctcctcatggtggattgcttggatggtcacctcaagctcagggaattcttacaacagttccagctgctcctcctcctgcttctacaaatagacaatctggtagacaacctacacctatttctccacctcttagagattctcatcctcaagctatgcaatggaattctactacatttcatcaagctttgcttgatcctagagttagaggactttattttcctgctggtggaagttcttctggaacagttaatcctgttcctacaacagcttctccaatttcttctatattttctagaacaggcgatcctgctcctaatggatcaaaatctggatcaaaaatgcctctgtcttatcaacactttagaaaattgctgcttcttgatgatgaagctggacctcttgaagaagaattgcctagacttgctgatgaaggacttaatagaagagttgctgaagatcttaatctgggaaatcttaatgtttctattccttggacacacaaagttggaaatttcacaggacttgcatcttctacagtgcctgtttttaatcctgaatggcaaacaccttcttttccacatattcatctgcaagaggatatcatcaatagatgtcaacaatatgttggaccactgacagttaatgagaagagaaggcttaaacttattatgcctgctagattctatcctaatcttacaaagtatttgcctctggataagggaatcaaaccttattatcctgaacatgctgtgaatcactactttaaaacaagacattatctgcatacactgtggaaagctggtattctttacaaaagagaaacaacaagatctgcttcattttgtggatctccatattcttgggaacaagaacttcaacatggtagacttgtttttcaaacatctacaagacatggggatgaatcattttgttctcaaagttctggaattctttctagatctcctgttggaccttgtgttagatctcaacttaaacaatctagacttggacttcaacctcaacaaggatctcttgctagaggaaaaagtggaagatctggatctattagagctagagttcatcctacaactagaagatcttttggagttgaaccttctggatctggacatattgataattctgcctcttctacatcttcttgtctgcatcaatctgctgttagaaagacagcttattctcatttgtctacttctaagagacaatcatcttctggacatgctgttgaacttcataatattcctccaagtagtgctagaagtcaatctgaaggaccaatattttcagcttggtggcttcaattcagaaattctaaacctgcttctgattatgctctgacacatatagttaatttgcttgaagattggggacctgctacagaacatggcgaacacaatattagaatacctagaactcctgctagagttacaggcggagtctttttggttgataagaatcctcataataccacagaatcaagacttgttgttgatttttcacagttttctagaggatctacacatgtttcttggcctaaatttgctgttccaaatcttcaatctcttacaaatttgctttcatctaatctttcttggctgtctcttgatgtttctgctgccttttatcatattcctcttcatcctgctgcaatgcctcatttgcttgttggatcatctggacttccaagatatgttgctagacttagctctacatctagaaatatcaattatcagcatggaacaatgcaggatcttcacgattcttgtagtaggaatctgtatgtttctttgcttctgctgtataagacatttggaagaaaacttcatctgtattctcaccctattattctgggttttagaaagattcctatgggagttggactttctccttttttgcttgctcaattcacatctgctatttgttctgttgttagaagggcttttcctcattgtcttgcattttcttatatggatgatgttgttcttggagctaaatctgttcaacatcttgaaagtctgtttacctctattactaattttctgctttctctgggaattcatctgaatccaaacaaaacaaagagatggggatattctcttaatttcatgggatatgttattggatcttggggaacacttcctcaagaacatatcgttttgaaaatcaagcaatgtttcagaaaactgcctgtgaatagacctattgattggaaagtttgtcaaagaattgtgggacttcttggatttgctgctccttttacacaatgtggatatcctgctcttatgccactttatgcttgtattcaatctaaacaggcttttacattttctccaacatacaaagcttttctgtgtaaacagtatctgaatctttatcctgtggctagacaaagatctggtctttgtcaagtttttgctgatgctacaccaacaggatggggacttgctattggacatagagctatgagaggaacatttgttgctccattgcctattcatacagctgaattgcttgctgcttgttttgctagatctagaagcggagcaaaacttattggtacagataatagtgttgtcctgagtagaaagtacacatcttttccatggttgttgggatgtgctgctaattggattcttagaggaacttcttttgtttatgttccttctgctcttaatcctgcagctgatccatctgctggtagattgggactgtatagaccacttcttcatttgccttttagaccaacaactggaagaacatctctttatgctgtttctccttctgttccatctcatttgcctgatagagttcattttgcttctccacttcatgttgcttggaggccaccatctaaatctccaggttctggaccacctatgcaactttttcatttgtgtttgatcattagctgttcttgtcctacagttcaagcttctaaactttgtcttggatggctttggggaatggatattgatccatacaaagaatttggagctagtgttgaattgctgtcatttcttccatctgattttttcccttctattcgtgatcttcttgatacagcatctgctctgtatagagaagctcttgaatctcctgaacactgttctccacatcatacagcacttagacaagctattctttgttggggagaacttatgaatcttgctacatgggttggatctaatttggaagatccagcttctagagaattggtggtttcttatgttaatgtgaatatgggactgaaaattagacaactgctttggtttcatatctcttgtcttacatttggtagagaaacagttttggaatatttggtttcttttggcgtttggattagaacacctccagcttatagacctcctaatgctcctattttgtctacacttcctgaaacaacagtcgttagaagaagaggaagatctccaagaagaagaacaccaagtcctagaagaagaagatctcaatcaccaagaagaagaagaagtcaatctagagaatctcaatgttga

SEQ ID NO: 60 - DNA, 96 bp, Artificial Sequence
  TPA encoded
atggatgctatgaagcgaggactttgttgtgttttgcttctttgtggtgctgtgtttgtttctccatctcaagaaattcatgccagattcagaaga

SEQ ID NO: 61 - DNA, 882 bp, Artificial Sequence
  Vaccine construct
atgggaggctggtcatctaaacctagacaaggcatgggaacaaatctttctgttcctaatcctttgggattctttcctgatcatcaattggatccagcatttggagcaaatagtaacaatccagattgggactttaacccaaacaaagatcattggccagaagctaatcaagttggagcatctaaaggtggaaaaagtggaatggaaaacactacatctggatttcttggacctttgcttgttcttcaagctggatttttcctgttgacaagaatacttacaattcctcaatcactggattcttggtggacaagtcttaattttcttggaggtgctcctacatgtcctggacaaaattctcaatctccaacttctaatcattctcctacatcttgtcctccaatttgtcctggatatagatggatgtgtcttagaagattcattatctttcttttcatactgctgctgtgtctgattttccttcttgttttgttggattatcagggaatgcttcctgtttgtcctttgcttcctggaacttctacaacaagtacaggaccttgtaaaacatgtacaattccagcacagggaacatctatgtttccaagttgttgttgtacaaaaccttctgatggaaattgcacatgtattcctattccaagttcttgggcatttgctagatttctttgggaatgggcttctgttagattcagttggttgtctcttttggttccatttgttcagtggtttgttggattgtctcctacagtttggctttctgttatttggatgatgtggtattggggaccttctctttacaatattttgagtccttttctccctttgctgccaattttcttttgtctttgggtttacatttga